European Patent Specification EP 4 074 831 B1, published January 21, 2026. Title: Novel Polypeptide and Antibiotics against Gram-Negative Bacteria Comprising the Polypeptide. Applicant: LyseNTech Hankuk University OF Foreign Studies Research ＆ Business Foundation. The sequence listing filed with the application follows.

SEQUENCE LISTING (16 sequences)

SEQ ID NO: 1 - protein, 259 aa, Artificial Sequence
  synthetic_Endolysin LNT101
MGTVLKRGDRGSAVEDLQMKLRVAGYAVSADGIFGGDTEKAVRDFQASKALVVDGKVGPATLAELAKSATVPAKWEAIPFPTANKSRSAAMPTLNAVGAMTGTDSRLLATFASIESAFDYTVKASTSSATGWFQFLDATWDDMIKAHGSKYGIPKDPTRALRKDPRANALMGAEFLKGNAAVLRPVINREPSDTDLYLAHFLGAGGAKKFLSADQKTLGEVLFPKPAKANPSIFSNKGVPRTLAEIYKLFEDKVSKHRA

SEQ ID NO: 2 - DNA, 780 bp, Artificial Sequence
  synthetic_Endolysin LNT101 coding gene
atgggtactgtactcaaacgtggcgaccgcggctctgctgtggaagatctacaaatgaaacttcgagtcgcaggatacgcagttagcgctgacggaatcttcggtggagatacagagaaagctgttcgtgatttccaagcttctaaagctttggtggttgacggaaaagttggacctgctactctagctgaactagccaaatccgctactgttcctgctaaatgggaagctatccctttcccaacagctaataaatctcggtcggctgcaatgcccactctgaatgcggttggagcaatgactggtaccgattctcggttactcgctacattcgcttccattgagtctgcttttgattacactgtcaaagcatccacatcttcggctactggttggttccagttccttgatgctacatgggatgacatgatcaaagcacatggttccaaatacgggatacctaaagatcccactagggcactccgtaaagacccacgtgcaaatgcattaatgggtgcagaattccttaaaggaaatgcagctgtattacgtccagtaatcaatcgcgaaccgagtgatacagacttgtatttggcacatttccttggtgctggcggcgctaagaaattcctatccgcagatcagaaaactctcggtgaagttctattcccgaaacctgctaaagcaaacccgtcgatctttagcaataaaggtgtaccacgtacccttgcagagatctacaagctgttcgaagataaagtttcgaaacatcgggcatag

SEQ ID NO: 3 - DNA, 32 bp, Artificial Sequence
  synthetic_Forward primer
aaggatccatgggtactgtactcaaacgtggc

SEQ ID NO: 4 - DNA, 35 bp, Artificial Sequence
  synthetic_Reverse primer
aactcgagtgcccgatgtttcgaaactttatcttc

SEQ ID NO: 5 - DNA, 304052 bp, Artificial Sequence
  synthetic_PBPA90 genome
aagggtcccccccacatataattactatttatataaaatttcttttaaagaaaaagcatttaataaggaaaatactctttattaaagatatctattctttaacaacaagttacttatgcacggccggccccgcgaaaaaaaaaaaataaagtggaataaccctctcccgaaggagagggctttatgccttaacgattactaagcttgatcatggagacaaacttaggatcccaagccagcctatccatatcaaagtaacggataggatgcatcatgaatccaactgcaactccatgatagatactttcgacatcatcaactgcgataacaacagaacgggtgtattcattcgcatcgtttttcattacgtgtacgaacgatttgacacccttgctaccagtcaaccattcaagccgtcgtttagctacctccgcaaaacgcagaacctctggacgaacccattgcggataatgtaagacattattgttttccagtttacgaatagaatcagtctcttcatcgagatcaccaaatacataggacgataccaaacccatgatctggaaattaaccggtttatcagaggcgtctgtaatcacctggtacacaccagtagtattagacaagaagccacggtcagagaactcatctactacatcacgatacgcacgttgaatacgttgttcgatccacccacatttttcaatgtaaacgtcacgcaacaaagacttaacatgggcaacgtacgattcctcattgaaagaagaattcaatccacgtacgttcaagtaagaacgatctcgtccttcgaacgtgacagttggtttactccaaccactgtggctttccacctgtacacggatgttgtacgcatccaaggcgccattacctgtaatatcgaaccagatggtgtctagatggtttttggtgagccctaattcttttgcgttaaaactaaaatcaatattgctcatcgtaactcctatttagtgattgaatatcattttagtaatatagatttaaaaacaaatacaacataaagcctccccgaagggaggcgtttatattactcgcgttcaacccatggacgaagatccattactgtgggagcagccttcttaatgtaagttaagatagaggctttgtcaactgtaggttctaaagcgataccgattacgatactatctttattacggatcagtagacgtggtttattgctctccagacgttgttcttcgaagagaatcttacttggatagggtaagtcatagggaagttgaaaaagcttatgtaggaccattggaacgatttctagaggggtacctagttcggcttttatttcttccaaggtaacttcaaattgtgttgtcatgttaaatccttagattgtgtaatattcgtgataacggcgaagtttgtcatcatccaacgcgatctcttgataactgatcgtaatcttcatgtggttccatggagatcggaatgcgcgtccagttaacgatacttcacggtaatcatttacgtgttcgtctttcacttcttcctcgaacacgaccccgagtttactaaaacgtttaatcagtagttcaatagatctaccaagctcaccggggacatccggaaattctgttgctgatgcaattctaggcatgatcacaggaccatcttcaacttcataatctaccttgaatacaacaacacccaaatctttttggattggtcggaaaatacgataaccatctttggtcctccgaagcttatatccatcatccggatgtgcttcttgtagggcctctaaatgatcctctagtgcgcgaacgataccacggttataccgtagctctctttcacgataatcgcgttcaaacgcttcctgcgggccttcttttgtaaattcttttacaacggtgtattcaatcgtttcaccagtcagatgatcggtgataacgaataagtacgtcatggcatcaaccaaagaatgttgaacgctataccgggtcatatcacatggaatggcaccagctcgttcttctttgagataatcaaacatgtctttgagatgggcccaaacatcacaatcgctacctagtccatccaggtcaatcgatgtatccgggatttctctctgagcacaacaactcatacgcacctcttcaattatatttggcgttcacatgataaaagaaaaaggcgacatatagcctctcccgaaggagaggccaatgccaggttaagatttcacctgttcatccagggaagcaagaaacttctcccaagcggggcgaaccccatggaggtagtagctattctgagtagtctttttcagggactctacggtacattcttcaggatcccattgattatcgccaccactgcccggactgagcccatagcagctgcaatgtgaaccgtggacctcgtagtatttaccatcgcgctcaaagagcacgaaagcactacccgagtaatcctcgtattcataccacgcaaaaagaatggtagcattatcaagttcaccattagtcagaccgaactcagaaattacatcttgctcattttcaaaattaccgaagtacatgatttcacctctatgttgtctttgcggaatgcaaaaaaacgtttgcaacgttcatgcaaaatagacaacagggaaatctaacctgtattaaatactggatctcagtatttattcgtcatcaaactcaatgactaaaccaattttcttataaagcgctatagctgcttcattctttttgtgtacaaaaactttcttggcttgaatgtatcgtactagctgttcaccataccccataccttgggctgactctgctatatacagacagtccaaatgcatctccggtgtatagagaatagcataaccacgcaaatcaccatcaaaccaaataccataggctttcctagtgcaagcgaaagctttactggttaacaacgttcgtatattaccctcgtaatcgagaagagattcaagatagtcagggaggacaacatgtgtcctctcgacctttatgaactcaccaattacttcatgtcgaatttcaccaatctctaacatgaactatccaaacactttaacgaatgcttctggccagagcattgttttgaaatcaaccccattaagttcaatgacaagaagacctttatccagcttcagacggatgatatcagtctcgtccatctcacgctcagctacatttgacatgtaagcaaacacagcctcgttcggaatcatgtatgtctcatccacatatgcctttacaacgaacagaacgttctggcattggatgtaatgagtttcagagagttcatcataactgaatcgagctcgaacagcagtcttctggtgaagactatttgcggtgatctcgatatccgtgatgacagccatcgctttagacaatgcaaaggtagacatgctaccagagcctaaccaaaggcgatgaatttccgtgggagttagatcaacagcggacatgggaatttcgatagtcgaactatcgtaaacttcaatgcagtcactggcatactcaccattaatcaagaaacggaatacattcccatcttgctcatacttccagcgggaaccaacattgcgcatcattccatccagatacagtgcgacaacgtcagacttacttggggatttgaaagttacttcttcattacgcagggttggttgagacatgataactccttagaaatcaatggtgatggttatttcgtctttgttatcgtcaaaggcacggagactaatgacagtctcgtaatgacgaatggacttagaaacagataccagtttagtggcaccgagggcatggagagtatccatgatttctttggcattaacactaggagactgatttccgtaactaactatcagttgttcaatacgctcctgagtaagaggttcaacgaatgccgtttgctggtcgattgcagggtaatgaccaaaatgacaaattgtgtacttacgtttaagaatgccaccaacctgactaacgacatccacacgccgatgcgaataactgtagttttcaagaacatacagattgtcagggtacaggggagccaacttatcaacgaaaccatttgcggcttcaccaatggtggaatcgagttgtaccattacatcgtcaccggtataatctatccgcacacgggcgtaaggcttcgcatcaatacagcggtctgcttgttgctcggagtgtaggtaattcagagcgtagcctttaccagttagttcacccgatactttagccagcagtgtcagtagttcactaccagctggactcttttcggcatactcgccataaagcattgacagctctttactcacagatactttcgtgaaatcgacatcacgtagaacaatggtgtcactgtaattacggtaagggtcgtggtaaccaccctcttcaccaaagccatagaaaccaccatcgtatttacgtacgattccaatagtgccaatcatcttacgggtattgagatcgaagatgtactggctcagcttcgggcattgatttacagaaacttgggattgttcataaccagcgttataccaatcgctgactagtagattaccatgaacaccaggttcgatcagatcaagaccaacatatttagctgaccagttttcccaggtgaatttgggttcttcgtgttttacagcttcttcttttacaacaacattggacatattgcaaaacctctttttaacggaatgtttagcttgcatgtaatatagatctaagatattttttagcgcaatgatctgattaatcaaagaggtataaccatggctctcactattcgtcaagttcttgacaagcatttcgaagatgtcaagtttgaccgagacctttgcaaacgaatcatcgactacaccgtccgttacatgaaccgtaatgaagatcactctgcattttttggtggagttcttctaggtgttcaagaagttcgcttctatgatactgaccgtgagatttggtttgatgacgtgctacgtgtagatgacgatctactccgtcacgatttcgttaaagctgaaggtatcgatcctacacacattgtggcatctgatccattcaaccatattccaggttatcttacgatccaactgaataaacgtaatgacattccgttgaatatcaaacaagaagcaattacatgcgctttcatggtgctacattttaaatatctaacatctctattggttagacgatttaaatatccggctaggcgtgaagtggccgaagcgacatttgctgcccttaactacaagtttgatattaaagctattggtagctggggaaaattaattcgtgaacgttccgaggggatttcttcgaacgacacttcgaatatttattactcgtatcttcatgataagatcgaggataaagacggctatatgtcgaaacgtgttgtaactgacacgcagtcacgtattcgtgaattgatcaataaatactacgaagtttatatccgtactttacaatctggctctagattggttatgacctctgacattggtgtcaatactgatggagatcaaatactgagagataaagttaacggctattcgggttatcttcgttacatgcatggtgttgttaacaacgaacagaactttattagacctgagctattgggtgtgattgagaactcaatggcagctatgcctccaaagcttctagtggaatcgctacagtacatgtcgcgaaattatggtcaaccgagaatgggtcatctagagaaactagttgatgaatgtctgctctacgcgtttgactacatgcagtcgattaaaacctctgtacagcgtaataccgacctaaacggtattatcgtgaagatccgtgctaagctgatggcttcgcgttcagaagatccacgtgtactctttatgcgggacaccggtgaagcaatggtgaaagaagcaacgaagattaagaacccagctgttattgcagctacccgtactgggatcatgctttacattattcttcgagctatgaccaggaattattattccaggtaaagaaaaaaaaacataaatgccctctcccgaaggagagggcttatgtcgtgttacttgaataagtggtctgccaggattacaataaacaaagcgagtaatgtatttctcccgcctttgaatacgcgtatccaccacttagatcgtttcaatgtaactgagtcacacccagctagcttttcatgttcatattgctttgtcgaatagagatatccgatatttaaaatcattgcaataaagaacagactagccaaaccgaaagcgatcattagttattgtaatcaactacagatgcgagaagatcagcggcagtccgatcatcagcattccatagtttatcacaccactccttatcttccggattggtgattttgtgaagttccatgtgactatggaaagcttgaccccaacgtagattcttgtcgaggttcttaaaggaagccagtcgggtgtagggaattgttatggccataactcaccgtatgcatttaagggtacgtttagtttgcacactcagaggaccagtgcagtcaccagtcttcagtgctaccagggtttgataaaactcagttaacagtggtcgatatttgtcgatttcatgttcactgtatttgcctttaggaaaagcgattgtgtaaccatcaggtggcggcatgtcaaactcggtgaacaagtcaccattatcgacataattacagatacctttgttacagtagatcagatcagaactatctaccatttcagcgtagagttgggcatcgtattccaccggattgaacggatcagcgacagcgacttgtaatgcaatagtggataccacagcgatgaacagtttacgcatttcgatgttccttacttagcggttttgaaatggttggttacagcgttgatcaacatctcttcgatatcgaccttacggtattctggttctgagttctcgtcttctaccatatcccagtagatagtggcacgcagcagcgctggtgcaatgaaacgaatgatcttgccagtagcatcgaactccacgctgaacatggcatattgttcagaggtaccagctttgtagaagatgaacgatccggcgaaggtacgaatctccagttcaccgaaggtactgatacggacttgtttatcgaagtactcacctttggtgcgcatattgtcttcgataacagtgaacagttctttgagaagttctttattgaggtacatttgtagatccctattgtggtgttgaattcacatttgtaatataggtttttaatatatttaaatacaagccgacataaagcccagccgaagctgggccatatatcaagcgtactgtgcgtttgcttctacgggtaaaccacgagcgatgttatctgcatcggtagctacagaagcagctactcgattaatacgatgccaaagaccattatcttcagcagcgacatcagcagagatcaaatcgttgtacctttcaacggaacccccttgagcgggagtttgcgtcgaagcatcatctagcttaaggggattagccattagtcagcaccatcgtaggttacacggttagtagcggatttctccagctgatcacgcagaccaatgttggcagcacgtacgtcagcagagatggattcaatccaaccacgttgttcgttcgggttcatccctttaatgttcagtgtacggaacagttgacgagcatacatggtaacaccttcagatacgtcagtcatcgccgagaactcaatactgaggtcaaggttctggccgatctgagcggcatctttacggctctcccattgaccagtcgacagcgggaacatgttggtgcagagatatgcgctaacaacgtcttggaaagtcgggtctggttcaacgaatagaatcgtggcaccgtagaaggtagcatcgtatttctccggcggaacgttaccttctgcaacgatacgcgggatcttggtattctcgtcaccgataccgtaggtgatccaccacttcaggtaacgctggatagcacgaccttgcagttcccagcaacccaacgacggagtcgaacgagcacgggtaacgttggtggcagcctggatggcttcaccagaaccaccccaaggagcttctgcggtatcaacagttacagtctgctgtagaccatcgatagtacgaacatggttctctaccagggctttaagcgaacgaactagttgccggctattgctagcgtattggaagaagcgtggagcttccagaaggaacgggacgaggttccggctaacgtaaggagtgttactcgcaaggttagccagatcaggacgaaagacatccgtaccagcctgagccaggttgatggtgttcttggaaccacctgcaccgtagccggactgaggagccatcgggtcattataacgtttcatttcgattcctcaaaaatgagtagttaccgagcttattgctgctcggtaacgttctcgcggcgaacggtttccagttggaagttcagagtggtgcgcgggttattagccgcaacagtcacagtgcaagtccagctggtgccattgttctcatcaataccggtgatctcggtacgcgggatcacgtctacacgaccaccaaacagatcacgagtacgatcaaggatctcttggtcgcaacgttcaacaagctgttctttagtcaggaaagcgttacccgagaacttagcgtggatcttgtggatcaaccgcatgattacgcagcagatattcacagtgatcgggctaagcagtaccgatgtgtcgtccagatataccgaacgtagacacgggtagtaattcgaacgatggtcgtacgaagtagagtaagttgcaccattggcccagaggttagccgatgtacgagcattgaagaacggtacgttaagcttcttaaccatggttacacggttattcggatcaacgtccatttcagcgcctgcacgtaggataccggtgccagcaccagcataacgcgaccacatcatggcaacgtcgagcaactgcggaacaaacttattgtaaccgccgccaacaagcttaccagattgcattacaatcatcgcacggcacacaggggtaccatacagggtagcttccgggaaagccttcagacgagtcatcagagcctgtacacgggatacttcttcagatgccgtcggaagacgggtctcaccttcaacaaaggtagtgaagaagtactgtacgtcacgacgagcagacaatacttgcattgctttatatttcgaggccatcggcagaccggtgtcgtacaggataccgaattgatagagcgcaacgttttcgtactgatcaccaagcttaccaaagttggtattctcgatgtcaacaagcttgacgtattcatccagggtagtggtaccgtctttaccgccttgggcgtagacagtagcgttcttacctagaagcacaccaccttcaatcggaccttccagtttgatggattgatacgggtcaccatcttcaccaagcatagtgaggaagtcaatctgaccaggtgcatcgatatgtgcattgattgccgggtttacacgggtctctgcatcgtagataatctcgcgaacgagttctacgttgtcacgatatacatagcactgcgagaacgggctataaagcggggacatacccgactcaataccgtcgtcgttatactgatcgataagaacttcatcgatggttagatcacgatcatactgttccgaccaaacaccttcgtcgaacgatacgttgacgtagtcttcatcggtcttggtcttgatgatgatcggagtgcttgtcccgtccatgagttcaacgaattgaacacgatacagacgagtcttgaagcgctggccggtgaattcatcgtagccatccggatcgagctgagtcggtgcccagatacgcatgcccaggttattaccgggctgaccgaagaacgaagcgggtagttcgaacagcggatatacagtggactgactaccgtccataccggagaccatggtacccggcaggcgccgttgagtacccacttcggattggttatcagcaatcagaacgatgcgtgcacgataaccttcaacagtatcggtaccagaagcaatcggaccgttaccagtgtcagttacagcatcaggatagttaaagccactgagacgggtcacagaagcaggaatcatgtcttggaccatttccagggccacagtgattcgagcagggttaccagcgtcttcgggtttcaggcgtttaacatagaaaccgttaccttgaccaagcaggttcagcgccagcagcgattgctggttaaaatacttgctgcgtggatcaagagagctttgaccaaagatagacgcgaagccatcttcggaatcacctacataagtggtttcagttgggccagtctcagtgaagagacgaagcagaggagtgtgttgggcgaaagtaatctcgggacgaatgaacgcccgacggctacgatctcgaatcccgttaaacacaaccttaggaacagcgttgtagtacgtggacatctttatgtttctcccagatgtggagctttaaactcgatgttatgagtgttaactaacagtcaatcataaatattgttcatagttggctgtgatagttatttttccctacccatgaaaggagtaaaacggtaatgttttcgctaccgtatcaaacaacagtctgtgggatctatcctaaatatcaacaggtgatcgcagcagcccgtcgggcagaaattgatttgccattccccctggtagaaacacccggtggaaatcagttaatgaactctgcgttcgtaacacctcgtgaagaacacgaagcaattccgaacttcactcagattatcaatgtgggcgaacccaataaaccacggcttcttattgatagccgccaatacatgaagtttgacgctcgatctcagaagtattctttgatcgctcaaaacgactggcagttccaatgcgttcgtctagctttgaacaatcgcctgctttctggcgacgaagctttctttaatcgcttatcggacctacctgcaaaagtattccatcgttgggttagcggtgtattggttacacgctacaatctaccgatcgaatcgcagatggcactctttgtcattacggcttattactattacgccatgtccacccctgaacttcgtcaaccgggtgaagagcgtgagaaatttgcaccgattatttctcgctgcacttcggtgccgccagaatttgtactcgatgttgccgcaacgatgggtaagctggagaatgcctctgacctcattcatgagatgtcagttaactcccgtcaacagcgtaccggtgaattgaagtttggggatctttttgcattgatctcgacttcttggttcggtgtaaactcccgtgaaaacgtgggtgtagccctcgaacatttaccgactttcattgcattgctttacatggcaattgcagaacgctcataccgtaaaacagtaattactcaacgagtagaatcgttagctcgtggaaacgagcttaaagtctttactgacctcgttttcaaagcggtttccgagcaattcacacgtcttcatcagtaatgggtgattaatgaacgactatctattgcgctacgcaattgagaacgtttggtgtaaccctactcaggatcgacagttcgtatataagctccgtcaattaactccccgctacggtgtacggggtagttacgttgtggagcacgaacgttataaacttccacaaatctctactcgtgacttctggcatatctaccaaatcggtcaggttattcctcgccatcttggtattccaaagctgttgaataactggatcagccttgagcaactgggtaaagaggtacatactctcgcggaagtttatgtcagtaatggaattcagttcccacgttctgaaacatatatcctggtaacccaaacgcaaaacttgcttgtagctattcgacgaaatgatcgcttccctgatttggacgaagctgagaataatccatatctccatgtttatcacaacgcgtatttcaactctgatcgtagcgatatagcagcagcccgttatatcgatgtgatgactttgacacctaactctaacgaagaacttcgtcaattccaaattcaaattatggacttgattgaaactaaaggtggttacccccagtacttcgttaacggtaggttcgtacaagagatatcgttagtaacagccggtccgggtgattactgtgaattcatccttgatccaagtattaaacgtgtagtcgatttagatctacgtgatcttaaaacattcaattctacgctcgataaagaaaggaaatatatccttcactacgacgataagaatgtcaacacgattgagtacttcgacgatctagatgtttatctttgcaaaaggggttcatcgcctggtcggttcagtggtgtgatgtatcaccacaatgaaggtaattggcttcgaatgttgacgcataaagactattcggctcctgttgatcgaattcagtctttcatcacaagtcaccctgaagacccacgccatgcaaatgatccatcgcgctggccttctgacaaatggacaggtattgaagataagttccttcgcctttacattcgtcattctggatacgaacgacctctggtagccgatgttggtcgcattcaagaactctatcgtttatcctcggataatatccttagggccatgactggagcagacgctacttgcccattatggagagcagagaatcttgaacaatcggcttacgttcaattcatgtccgctgatccagatgtaatttaccctatcgctttccaagatcctgatgagatatctcagggtaagatcgatgcccagaattttgccggtgatgtattcggttaccataaagccgcagatattcaggcacataatccaaccaaggtccatgttgaccaaggtacagtatatgcaagtcttccatacaactattgggaaaatgctactgttttcgaatatgattcgaaagggattttgttgggttattaccatcatgtcgcagggcgccgataccgcgtggtaaatcaaaccgaatgtaagatggtagaatgtattactggtaaaggtgataccaatcttcatggtgtatttggtaatggaacagtcgatctttcggaaggttataacttccgtctttacgtctgtaaagtctgggctggtgtaccaaccaacgaatggattgatatcactgacctacctaatcgaaatgattggggtttccatgatacaactgatattgaacatcctaaatggacatggactgctttaccaaatgaatggtacggttatgttcgtatggataactacttctacctgaaggaaatgcggtttactaaagatcagggtattattcgatttggaatcgataactgggaagagcataacggtgaactaatcaacaagctcatggagatcccattcggacaactagatatcttcttaaataatcgaccgatcataaatggtctcgattactttgataaaggtattatgactgtactgaataaccatgagtatttggttgatggtattaataccgttcttgtacgaggtaccggttactgtactcctgatcttcagcgttataaacctggtgaagttggttgggtagagtataatgttctttccaataatggtatttatgatatccatacgcacaaaatgcaaaggatcattgtagatggacattaccgcgcccgtgaagatttggtgtttgaggaggataataattctcttctgattaccgatgaacgaaatggagcacccttccaaatccaaacaccgcaatccactttccgtgatgtttacgatactgatcagcacgcacgtatcgcagatgacgaacgtgataaacaagtttccgattacatgacagcgtatttccctaagagaacacgcgatcaagttgactcggttacacgtcgttatgtggtatattcggcattctctaacaaagttctccatgacattgttaagggtacgctgaagccaccgctggttaatggtcgttacaacgagatggatattgctcgggttatggcatcctacgagtggttggttccgtttgatatcctaaacacagattacaacaccaaccatgtggtagtttatccacattggcatagtgatcctattgggttagatactgatcagtatgacttctacattcgtgtactgaagttgtatttacagcgccctatggacatcgcgccattcgtatacctaacgaggacttaacatgcttcctgtaccatacgggaattccgactacatggaccctaataggggttggtgggtttggaaccgcaaagatatcgtccagcaagctggacaagtaaataagtgggtccccaatattggggacctcgtttgggaccgcgagaatggctggttcacagttgaggatgtcgaagagggtactcacgtagctactcttaaagaatggtatcctccaaccaaagttgaccccgatggcgaagaaaacgtactggtgggcgtaggtccaggctatagttccgaaagctaccgtctattccttgataccagcgttattccccatactctcgcacccgataaacgtctgcatttttatggctcgatggttgctagttacaaagtctttaagggtagtgatatctctgaagaatttggtaatatcatctctgctttcttcactccctctggtgattacacgggtccacttattccagttgagacagtaaccgtcggtaatggctctcagaacgtcattaaggcccctatggttggttttacagccgaggagatggatgacggtgagcgttgcaccttggtggcctacgatgaccttggtggggttgtgtctatagcacagttgctcgtacaaaacacgaaagcaattcgacagtctgataattcgaagaagtacattgccggtatcgagatcgagagtccgttcctgtctgctgccgatcctaaggttattgaattcccgctgaacgtaaacgttgaatctcttccgatggttggtatgattaactatcgtggtggttctaaagtacggcgcggtatcgataactcgacaatgttcttgtttggcatggaaaactatatcgctactgagattggacaggagttcccgcttactcttgcttaccagttagcagaagatgaaatttcctatgcgttgacaccaacagcaaatcgccggattacagaaaactacattgcccgtacaactgctgccgatggagcttacgaatgtcgtctattcgtttatccagtatggcaaaacgttactgctggttaccgtctggaattctggctttacaacttggatcgccaacgtttctacaacgttacttctttggttgaacttggtgttaactcagcgccattcaatccgaagggttatggtaatctacaaacgcttacctacgctgttaacctgaacaaggtcgatggtcgtttcgcaccacatcgattcgttactacattccaagttgcactcctgacatctggtgaaaaccgtgatgctaactgggaaatctacactcgtcctgatgtagacgcagcttatggacgtggtctgaaagccgatctggaatacatccaaaccaacgcttgggatctacgtctccagaacggagctaataccaaagaagcatggctgcggaagatgtatgaagcagccgagcctcttgtaaatccggactctgaaattgtggcacctacaccaactcactttgtattgcatttcttgcataacaaatacgagttcagtgttgaacaatggaaagataagttgcgtgttaataacgatcttgccgatggagaacttctctacatccaatggattcgtcgtgaatacgacactgatcttcaattggcgatgaccggtattccagtactgaaacgcgcttaaggcatagtgccgtctcattagagacggctttatgtcgttttagtatgtaacaaataggagctggaccatgattgaaattttattgtcggtcaactctaaaagagctaaaccaagtgttttacctaccgaactaatagccggtgattcaagtctaggttattacggtatagtaacggctgccgattttattggcgctgaacaaatgaacgatgtacatggtttttctggtaatccatatggaacacgaataccggatcaaacagatgtagattggttaatgttctctttaaatgacagacgactcttggtctctacaaagactatccgtcattcaatgtcctttaatcaattagttttggctgttaataacttcaatactaattcatctaaagtaaaagatattgactgtaagatagcttatctgtcaggcggcgccagtggatctccagctaactcggagtggggtcagttgatgtaccgtatatcggaaaatgatccaactggaacattctgggaaaatttaagtaatgaggatcttggatttgtacatccaagtaacctcggtatttggacatggacacccactaatggtaacactgggtctcctaggttcaaagtcttacgtggtggacctaatggcgtaacagggtgggggcagaacgcaccatctcaacctaacgtaggttatggttggcgcccagtactagagttaatctagatacagaagctttcccttcgggggaagctttatgtcgtaaattaaccctaaaggtatgaaccttttgtttctttaaggaaacggtcatggaacttattttattccgcgatgattgggagaagttcccaacagcaatagcggatacaaaaacgtcaaataaaacattcttaaaattagcagctctttatagagatgagcttaaaatagcaaactggaaattcattttagcattactccagcctgatcttcagggagtagatccctatgatccagatctagatgatgctacaaaaatgaagattgccttggaatgtaaatacaatccttggtattacttccgtgaagttgcccgtgtcccagcgacatctggtaacgtcccaaaccctttccgcgctaaccgtggtaacattgcacttttctggtgtttctttaaccacttagactttggtctgttacaaccacgacagactggtaaatcggtttcaactgacatcttgatgacgggtatgatgtatatctggggtgagaacaccacgatcaacctgatcactaaagataataaacttcgaacagcgaacattgaacgtctaaaggtaatgcgagatctattacctgattacattcactgggctaatccaaatgacgtagacaataacgagctgatgacgtgtattcgtttaggtaaccgttataagaccgcagttggtcgtaacgataagattgctgccgacaaacttggtcgtggtcttacagtacctatcatgcagttcgacgaatttgcgtacattaacttgattgagatctctcttcctgtagccctggcctctggttcagccgcccgtgccgaagccaagcgtcaaggtcaaccatacggaaacatctttacaacaactgctggcaacattaccactcgcgatggtgcatttgcttacaagttcatgacaggtggacatacctggtctgaaacaatgttcgatctagtgaaccaacgtatggcagtgttggtaatggagaaaggatccaaggctgatcagaaacctatcatctacggagcttttaaccataggcagttaggtcgtacagatgaatggttgttccaggaacttaaagagtctagttcttttggtgagatcgctgaccgagacttcttcaatatctggactgttggtggtgaaggttctccattatcacccgaacataagaagcaactaaaatcatctgaacgtgaaccaatttggaccgagatcacgccagatggttacaccattcgctggtatatccctaaacatgaagttgaccagagaatggctgaaggtcgctttatgatgggcatggacccaagtgaacttctaggatcaggtaatgacgccactggtatggttatattcgatgtggagacacacgaagtagtagcagctggttgttataatgaaacctctgttcctgttattgctgcattcgtcggtaatctattaattcgttatccgacgattacatgggtacctgaacgtaaatcgatgggcactgctctcattgacttcgttgtaatgcaactgcataaagctgggatagatccgttccgccgaatctttaatagaatcgtagatgaacacacggtactagaatctgagttccgtgatattcagactccgttgtctcaacgacctgcttcgttctatgatcgattcaaacgttactttggtttcaacacctcaggttccggtcggtattctcgtaacagcctgttccttgaagcattaccgagttcaatggattacggtagccggagaatggcggataagacgctgattacagaactacttgctttgacaattaagaatgggcgaattgaccacactcgtgataatcacgacgacatggtaatttccatgctgttggcgcactgggtatgtattcgtggacagaacctttcttattacggtattaatccagcaacaattttctcccgtgctgttactcgtgacgtagagttaactgctctggaaaaatatcgtgaagataaagagaagcaaaacaaaggtgagttcgaggacttgattgctcagctaaaaggtgagacaaatccattcgtaattaccaagcttgagatgcgccttcgtaatctttcgaagagtattaacatggaagaaacaaccggtgttggtatcgacgccatgttgaaacaagtacgtgatgatcgtgttagacgtgtccgtacttctcgtttccaacaagaacgtagtttcaattcacttggattctatggacggtaagtgacaacataaaagccttcccgttggggaaggctttatgccgttaagctctttgacctaaagaacattgttgttcaagtcgacgtttctctttcttaacattcggtttagagggacgtgtaacaattcggtagctatccacacctgcacgaatcaaaccacggataattggattaaccttagatacttttagcgcctcatagaagatatggtctatctcttttcgagttaccttaacttctgtctctttcccatctaccatctggaagatagtgtatgtctcacaaagcttatcatgcaacgctgctgcctgaccatgcttacctaatcgagggatcaaccaacgtactggccgtggaatagatgcaccatctgttaggaaacatttattaacaactgcgtatttaccagagccttcacttccaatgtcatattgaaaggtctccataatccgccagtagtcatcacccagaataacagatgcatcatcgtcatactggatagacatcttggcattaaacttagtatagctactcatttacaatctccgttaaccacagaggattgggttaacgtcttgcccagtattgcaaactatatccaagacctggattacggggagcgttagttacacctttctgacaggaaatgaatcgccatttaattggatcaatatattcctcgaacttagcaacgtcagttacgtcatcggaagaacaatcaatgtccatatcaacaatcgtgcgatagaactcactacaacgagtgataccatctttaaatagtctttcaccaccaatgataaaaaccttcttttcattttgggataattctagtacttcgtctaaagacttaacatggatatatccctctcccttcaagttatcactatctgaagaaaggacatagttagtccgacctggaagaggtttatttcctaacgattcccaagtcttccgccccattacaacagcatgccctaaagtcttttctttaaaccatttaaagtcttcaggaatatgccatggaatactcccattgattccaataatgccattcgtggatacagcaaagatcattgctagggtgggcatgattaactcacttactcggagaatttaacgttaaaggcaaagggcgtccaatggaaagtatattccacatcgaaagtgccacggaacccagcacactcctcgtgtagattagcgatgcaatgactcaaagcaatctgttgtagaatactgaattgattaagagagaactcaaactcttttttactaatcgtggaagacggatcaaagtcaggatgtccatcaactgtcgatttatgtgccagcgtaccacggaaaatagctttattaccagtgggaaggacatcgataaaatattcggtaattacaaatcctttctctccaacttccttaagatcctctagcagatattgcgtgataaggaatagttgtggcgggagttcgagtgaagggtgcttaccagtgatggtatcaatgaggctagtgatttgactgaaatgaagtgaatgaacaacaccgtcattatcaagaatagagagttcatgcgaaatcatcgtttcgctctcaccctcggcttgatgttcaaaaataagaccttttgtgatcttatcaaatttatccatggtatctacaaacgggtaattaacagcggtcatttcttaactccattggtaacaactttttcaaagatcgcttcaaattcttttttatgatgaagcctgtaactcagaatacgtttcttgtcatcccgaataaactcaatatagtcacctggacaaacaacagcgggactatcgtcagttcgaactttaaggatcccatgaagggccatcttacagttacagtcaggacagatcattccaccttgtatactaccatggctaatatgccgtccaacgatagccccttcgttaattccattaacggtgcggtccatgggatggtcgccatttttaaaccattggtgagcttctacgagtggtagaatagcttgataataaggcatttgtattctccagattgaaataaatagcatatccttttccatctgagtagttcttctttttaggtgttgtatggtatgctgttagaagattttaacttatttaaaactaaatgatcgtaaaaatacttgcgtggttttagttatgttagaattcatcaacttacgttttacgcaataaacaactggaaaaatagagatgattgaaactattatcaaactggatggcactgaacaacccttcgataacgagaaagcaaatggctggggcgagtgggcagcggcacgtctgggcaacaaagttgactggggtagtatcgtactaggtgctgtaagcggtaagcccaaaaaggttacatctcaggagttccagggttggctgatcgaagaatgtcttaatcgtaagacctggtcgtattacctaatggctggtcgtctgtacgcagtatttctgcgtaagaaaatctatggactgggcggtattccgacagtaaaacaacttcatgccaaaatgcatgaagatggagtaatgatcaaactggattataatgatgatgaatatcaggctatccaggagatgattgatcatgatcttgatttcaattcccctcatttcgctctccaccatatccgtggtaagtattcccttcgtaatcgcgtgtctgggaaagagtatgaaactcagcagtttacatacatgcggatggcaatggctctttctgagaaagaacctaaagctgagcggctggaacatgtgaagaactattatgaattgttctctcaaaaacaattgtcggcgccgactcctaactacgttaaccttggtactgtactgcggggctttgcttcttgctgcctcttcgcttctggcgacaacggtacttcgttggctatcggagactacatcgcgaacatcatgacccagtcctctgctggtattggcgttaacatcatgtctcgttctgttggagatcctgtacgtaacggtctcattgttcaccaaggtaagaaaccttacatcgacgtaatgggtaaggctgttcgagctaacctgcaaaatggtcgtggtggcgccgtaactagcttctacagtctctttgatccagaagctgatatgatttcccaactccgtaaccctcgctctaccgaagaccgtaagaatcgtgatcttcactatgcagcaatgggtaacgttcttttcgcagctaaagcagctaagaatgaaaaggtgttcgtatttaacccgtatactgctcctgacctgttcgaagccttctacggtaaagaccaagctaagttcaaagagctctatgaaaagtatgaagctgatccgaactttgctaagacctacatcgatgcacgggatcttctaaaaacggttcttaacgaagcctatgaaaccggtgttgcgtatactgctcaaatcgatgaaatgaatcgccataccccgttcaaagaaccgattcatagttcgaacctctgtatggaaattgctgaaccgacaaaaccttactatgacatgcgtgacctctattctgaggaagaccatggtcgaggtgagattgctacctgttcgctggcggctattgttgttgacaatatcccagatgcagcaacttatcgtaaagctgcttattatgcgctgaagatgattgactactgtattctcaatgcagaatacgccttccctcacctgggtttcactgctaagcagcgtatgagcgctggtgtcggtatcatgggtcttgctacccatatggcccgtgcaggtctagcatattcttccgaagctggtaagcgtgaaatgcactttgttgcagaacggcatatgtatcacctgatcgaggcttccctgcgtatctctaaagaacgtggtcttgctccatggatgcataagactctgtggcctgaaggttggctgcctcttgatacctacaagcgaaatgtagatgaaatcgtacctggtgggtttgagaacatttataactgggagaaactccgtaaggaaattattgctaacggtggtatcggtcactcggtgctcgttgcatatatgcctggtgaagcatcctctaaagcagtaggcggtgctaactcgatctatccggttcgtcgtcttgttattaacaagtcggacaataacaacctgattaactgggctgcaccgtttggtgatgataaagcgtacaagtatgaacttgcttacgatattccaactaaggatatgatcgaagcttacgctatcttccagaagtggactgaccaaggtatttctgctgacctgtatcgtcggattatcggcgacgagaagattagctctaacgaaatgcttcgcgactacttcttgcaggttaagcttggtatgaagactcgatactacatgaacaccgagacttccgctaatctgtcgcttgctgcattagaatccgcgtttgaaaataacgatggttccaaaggttgcgctggtggagcttgtactctgtaacgacatatcgccctctcctaaaggggagggctttatgataacaaacattaacatcactttaataattagaagaattactaacgttctatatcaagtgtaagtaatcttgatattaacaaggaaacgaaaatgactgacaagctccccaagaaaatttttaacgtagaaaagactgactatgacgtacccgaaattatccttggtcaagaacctggactcctagattctattcatacccacttccctgtaccatggtctctctacaaacgtctacgtaagcttgactgggacgaattggaattcgatttccaacaatgtcttatcgaatttgaaacatgtaataaatcgacttacgacatgatgatcaagacccttgcatggcaatgggaagctgactctgtagctagtcgagcgattgtgaatattcttggtccggtgatgaccgactctaggatctggacaggttacgttcgaatcaacgataacgaagacgttcatgctcttacttattctgagattgtgaggggttcgtttaagaatcctcgcgttatcctcgatgagatcctgcgtgttgaagaagcacaagaacgtatggttgctgttgcccgtgtaatgggtgaagcacatgacacgtctcatgcctatgcattgaagcaagtaccgaataaccaggagacttacaataagatcttcatgttcttcattgcactttatatgctggaacgtattcagttcatggcatcgtttgcagtgactttcgctatttgtaaaactggcctgttccaacagattggtgaagcggttaagaagatagcccaggatgaattcgagatccatgcacaatatggccaagaagtaattaaggcactgttgaagaccgaacgtggtatgactgcgtatgagcagtgcaaacctcagatcatcgaactgttctgggaaatcatccgtactgaagttacctgggttaaatacctgttctctgaaggtcgtagccttgctggtgttaacgcacagaaacttttccagtgggtactgtttaacggtaatgctgctggtactttcctgaacatcattcctgataccctagagaaacattcggcagaatatctggagctgactggtgttcctctggaattcccggaagataaccctctgccattcatggttgaatatctcgatatctctgcaacccaagcctccccacaagaagccgagaaaggtgactacatggttaaccttcttgacacacgtggcgagaaagatgagtttgatgtggacttcctgtaatgaaaaagatcgctctcgctgtaactctgatgttccctcttactacgatcgcagcgggggagatcaagtcttctacaactggtatcgtaaagcaatctgaatgtcaactgattgctaaagataatagcatcgttggcgcgactgtcggcggcacagctggcgcagttggtggtgcaatgctcggtcgtgctatctttggtaaatctggtggttggatcggtggtctcgttggaggtgctgctggcggcgccgttggaaacgaaatgggtgccatagagacattccaatgcaagatgattatcgaatctgatggtaagcaacatctaatgcaaactatcgttaacaagaaaccagaggttggtaaaacgatcactgttcttgaaatggtagatggtacccgtgaagtcatgtaatcatactgccctccttcgggagggctttatgttatgtcaattctaaaggtaacaaccatgcctaacattaaccttttgttgcgatatgcgatatctctcgaagcggaaatggatgatctaatcaatcagttatttgatgaggtcaataacccgcgtgccgatcgcccttacgatgtatgggtcgagccagattctgataacggtatacagccacccaccataaccgagcttattaataatacggacgatatgtggacatattacaatcgttcaggtagatctaatgtaaagagctacaaatatggtcctgattggatgcttgttgaattcggtggagaagtgttttatctttatacactaaagagcatcactgagatacaactacaggacatgaaatactttgcagatggtggcgctggtctgaatagctatattagcaaggttattcgtggcgggtatgtagctaaaaacattaataatgaaattattctaaccccaggctttgaaatgtataagtctgaaggaccaataattttcattcatgtaagaaacaaaaaagaggaaaagaacatgtcttctctcactaccttaactggttataaagctgccatcgaacaagctggcattgatggtcttagtcaacctgcacgcaaactaatgcaaatcggtctatctcagatagataccgaacatggttttactagcgtatctactgaaaactttgaagaaagtatcacagtagaaaatattgaagagcgtattgccttcattagcaatgaagaataacttacccactatgtaatgatatgtagagacgtcactcctcgtttttacatagaccacagctcgccggagccagcaacccttccagctggcttctaggaagtaagactccctgttgtggtcccctcctttcagttggtaagttgtatctttctccttgttgtgttgatgagcataatgcctcccatcgggaggctttatgttgaaaaatactgaagagcctctatttatagagaagaaatgcccggttggtgaaattggtagtacacaagagacttaaaatctctcggcgaaagccgtgtcggttcgagtccgacaccgggtaccaaatttacggagtgtagcgcagttggtagcgcgcctgctttgggagcaggatgtcgggagttcgagtctctccactccgaccatttaaatatagagcccctctgtcatagaggggttttatattgtatcgagataatagacatgaatatcgcaacaatgtttgttttagcgattcacgtggggttgtttggaattacatccacagaagaatcgactatccagtttgaaaataaagcacagtgtatttcgcgtctagatattttagaaaacaagtaccgtggatacgagatactacgaacagagaatacgttgaaagttactaatcctgacgagtattctatttttattttcaaatgtctttaagagaaactatggaacatcaagaacaaaaagcgctactaaaagaaccattgcagaaactctacaatcttacgtttagtccccgcttacgtaatggagcgaaagctcccgattggattcgccttactgatgaagtaaccctattcccaaacggattagatattacaatcaacgctattacacgttgtatcaaatgggaacttatcgaggagagtataagtaatattacttatgttgaaaccatgttctttaataaaggtcttaaagcagttgaaacctatctcaaacatacggagtaaatatgaatcatctaaccccaacacagaacgctgtatatttcacatttgttagtcctgagtttatgaaactgactcttgttgaatcttttgtagctatccacaagaaacatccagaagtaaaacattgcgttaagaaaaagattagtgataatgaaactcagtttatctttatcttcaaagatggaactgacaatctaatcatcacacgtaagactgaaccctgtcctgaactggatagtccagtaggcgatagaattaagttgtctggcgaagaacttaaaaatattcttaccaaacatggccgtcctaatgatggtaactatttcaagcactggactgaccgtccatgatgtcataagagccctatgtatactaatatgtagataatgaattagggtctatagctcagttggttagagcaggcgactcataatcgcttggtcgcaggttcaagtcctgctggacccaccaaattaataaagcataatgcctcccctatttaagggaggtattatgctgtctattataataaaataaatatctgagccgcaaaggttatcctatgatctaaaatgatttacttgagagcacactcatgtttgaattactattatcatcaggtttaggcgatgaaacacccttggttggatttagtgaaattataaaattaggtgacctaccagtagcattggcaggtacgatgtcgtacgtagatggaaatacgttatatgttggatccggacatcatacggaaggacaatcagcagcaactgttttcagacggttcactataaacccatttgcagagataagcgcaacagcatctggtacatttttaccgggtgtatcacttggatttggtacattacataaaaataactttattgtttatggtggtattactggatggaacgcagcaggtgatgggggtacaggtacttctaactttatacaacattttgatataagcacaggtagtcgcgttgagcgttatagtggtcctggtacattatggggaactgcgtcagcgtctgatggcaatgatcttattatgtgtgttaatccagttggtacaaacgccatgcgattaaaaccatcgactaagaactggctcggcggtcaagactatagcggtggacctaggtcaggtcaacaattattttattataatggttatttctaccattttggtggctgggataatactaagaacataccaaacttagaagtctatagatacaatgttactacacttatatgggaactaacaccatggctaataatacctgctgacaaagcaacaatatggcaaggtaatggttatgtagatggggaatattttaattaccttaatgcagttgatgtcggcggtgtaactaaaatgtttgcacagcgttttaatattaggcgccggaaatgggctgaaccatttgaactaggtattggattccttaatatttcatctatagccaaaggtccagataatagcatgatcattgcaggtggatctaaaatgccagttggtggtggagcatatatgttaaaaagccaattgttatcgggtatctatcaggtaaaactagcaccattagccattgattaaaataataatatttataataaggttaactacacgttatttacataatgtcataaaaaataaataatactcagattgtaataatatgtagtgaaatactgtaattcagttacttgtgatttttctacaagaaagaagttgttagtaattcttccgcgatagctcagtcggtagagcaagcgactggatagttttcttggtaagtacccgagcggtagcagggggcggactgttaatccgttggcgaaagcccatcgtaggttcgaatcctaccttaccagccaatttcaaagagtagctccggctactctttattccgtcacatagatcgaactagcgatctatttatatatcctaggttcgatatgaaagagaaaataattaacggctatagggcattatatttacccgaacatcgtcaagccatagctaaccctaaaatgtttggatgggtttacgaacatcgagtggttggagaagacacattaggtagaccactttacgatgacgaggaagttcatcatctggatgagaataagcttaacaaccatccagagaacttattgattctccctcagtcacaacacatgaagttacatggttggatgaaacggctcggtattgatcctaggaactatccaactaagctttgtgctggctgtggtattgtcattagtcaccgactgataacattctgtagccccgagtgttcagccaaaggtcgtcgtaaggtggatcgaccatccaaagaacaacttgccctcgatgttacattgctatcacttgtaaaaataggagagaagtatggtgtatccgataacgctattcgtaaatggtgccgagcatacaagatcaatattccggctaggtttattagggtcggtgctaatgggggtattagcaccttggtccccacacaataaaaaaaaaatatactgggtccctggttcgagtccaggtcgcggagccaaattcaattgagtagccattggctactcttttatgccgttagtggttatcttatgaatcattaatactaactgagagcacgcacatgttcgagatattactcagttctggtgcaatggagagagctccatatgtacccttttatatgcgaaccaagaaggtagctgaccttccagtgggtattgcaggtccaatcgttgcaatggataacgataacttatatgtagttggcggtcaagattctactggggctatccgctctgcaactgaaatatttaaactatctgatatgtcgatgactgttggtggaaaccacgctagaactatttccatcaatggagcaactatttataataatagaatgctaataccaggcggccaattttctactaatttagctggtcttttatcaacgacaggtgcattgaatttacctgggttaactagtgcagttgagttaacgggacgtttaccacagacgtcgtatgggaatgctgtatgtcagcatagaggggacatatatgttttacccagttataaagccggattctataaattaaatccacttactggcgcgactcttgaaaattatccaggattaccaagttttgatgatgtcggtggtgggatattagcaggtatgtcaatttttggacatggagattatatctattgtttgggtggatgggcaaataatcagaacctaagaatacatcgatttaatctgatttccaaacaatgggaattatggcagacaatggaccctgcgtatcaccatgtatggcatggtggttttattgatgaggaaggttactataactataccggctggggtaacctcggtcaaggtaacaaaatatacctccatcgttataatccagtcaaaaaatcttgggcgcgctcgtcggataccggattatcatatcgaaacatgtcgggtgttattggactaaaagatgatatttatattgtcggtggtacatctgaaccattctctactaattggactagcacaacaaataaaataaaagaaatctacaaggtatctcgtgctcccgaaaactgggaacctgtcccagagaaaacatgggtaagaaaagcagacatgcctggcggtagggtgcaagcagccgtagcaagtacttattcagaactgttcgttatgtttggtagtgatggtgcagtaaagaatacaaacttgatttacgatgtatttactgatacgtggaaagaaggaccagttaaaccatccgcacgttatcaatcggcagccacaactgtcgccgaccagattcttattttctctggtagtaactattctccagacctgtattcttataaccatctagaagacaagtggagtgacagtatatctgaaccaaacgcacccacatggcggacaaaccactgcatgacatcttttggtagatatgcctatctttttggtgatgatggacgtaccgatagagctatttatcgttatagtttagatgctgcggctggaagcaaatggtataaattacctcaacttgctccagaaggattggctagagcggcaatggttattgtgaataataaactttacattgcctgtggttggattagttccaacaccatgactaaaaccattcgtgttcttgatttggtcgctggtacatggtctaccatatctaacgtacccgccagctttgttgctcgtgtaggttgtctattagctgcgattgataataaactttacataggtggtggcgctagtccaagcactggattgaatgatttctgggaatatgatacagtcagtggtgcgtggacaagactccccgacattcctataaacggtgatgctgctatgatggctgcatgtgctgataccttatatatcgctggcggtaataggccaaacggtgtgaaaggtaatgagctctacgcatataggccataaaagaaataccggtatggtaatactatgtaagactatatcggatttcggagagataggaaaattggtaaccccagctgactgtaaatcagccgtccgtatcgggcattactggttcgagtccagtcctctccaccaatgcgtcatagtgctctcccttcggggagagctttatgtcaactattacaaaaggaaatagcatgtcagcattaagtttgattaaacgttggtcgcccgcagtacctaagattctattgagtccacaggacacggtcaatgagactaagatggtcttagataacgagagtggagaatatataaagtttaatgacttcttgatcctccttcaaaacggcgtgtacctagaagccaccaaagagatgcacgagactttgttagatggtaaagcacagcaaagtctcattgctcgactcagtcgcatgggttatgaagactttgatcaagtaatgaaagtcttagaagaacagcgtgattctgtacttaagaagaaagaatatgaaatttggcaagaaggacatcgcgctactggtgaatctagtatagccagctttgtaggtaaagctgaaggttattctttcttagatgctgtagacaactacatgaagacagctagtgcggaagttaagaaatgtttccgtgctgaactagatgcagcttatatttggggctgtcgtttgtttgacaatgaagccgacgcacgtaaatctttcgggtgacttatggttcctaatctttctataaaagcaattcatgctcgtcaaactccagaacaacttgctggcaaccgagagaaaactcttgaggccctggctaagttcaaccaggctcaacgtaaacttgaagagcattgcaaacgcaatggacttgaagtaccaattatggtttgttaataatgactgatgacaaaaaagaaaaacagcataaagggcgacaagccctcaatgtagttggtgaaatcattggcgctgtgttcgaagctatttggtgggtcttgacctgcccgttccgtttaatcggtgtactctgtacgcttgattaaaataatacctagttgattacaatatgtaacgaacaaagttacttcatcgaaagctacctgtagaaacatctcacattaggtccagcagactgtagtatttcgatgtgaccatttatagcacccggaaaccaaaggctaatagtggcaagccgatgattgagggaagtcgaatgggccgcccataccgaaaggtgtctcttcagttccactaactgtcacctcacgatggacattacgatcaaaaagagactggttttaatgtccgatatacgactctccgataaggagagttttatgtcgttttatactgggctatataacagtatgtcaaaggatgtaaagaggtaatcatgacagctttcatgccatgtcatactgaggctgatatagacctagcttcaagaaataaaatgttgtcagagctacttatagaagaattcccaaatacagaagggatgtcaacaaaagcagcagaagactatctacggtctaaggtcatagataaattcaatattaaccatcctgaatatcaagcacatgtaagctacgattgtattacacgtggagatttcattacagcttgggtaacccaccggctagcccttgtaaaacttgctataactacagaggaacaaaaatgtacgaaaccgctccgttccaagacgatggacttggcgcactcattacggaaatttttagtcgggacctgaataagaaattccaggaatggtatcgaccaattatggatgacccgaatattgaaaaagtaccagtttgtcgaaatggtcaaattgtaaaagagcctgtcaatttcgttgctcttcttaaagaatggttagctaatcaagattaaaaacataaagcctcccttcggggaggttatatgttatgattttgacgaaaggtaatcgttatgtttgaagcattgttaggaattggggaatataaaagtaagcaaggttgggttcagctacagggacccgacgtcggaagaaaccagtcaacctctgttgtcgtaggagacaaactttatatcttcggtggtagacgtgctaccactaacgcgttcaatactgtatccgtctatgatttcttaacagacgaatggaaagaactaccggcaggagcaaacgttaatttacgtgcagctggtggtttagttgataacaagttttatgtattcggtggatacactggttctgctgatacaaacacgatgattgagtttacgattgatggtgagacaattacacctgtaacacgctctaatggtggattggccgtacgtaacagtcattgcatgtcagctattgataataaggtgtacctatttggtggtaacggtgcacaaggtattatgtatgaatttaagagctataataccgataacttcacagtagctaacttgacaccaccttatcaaattcgttatgcgaccttaacaagtcatggtcgacgcctctacacgttaggtggctatgaaacagctaatacgtcagttacgtcattcagaagttataatgtcgacaacaacacatggactgcccacaagaatggtcttgtaaataggaacagacattcagccgtagctcttaataataagatctatgtattcggtgggcaatctggtacaagttctactcctaacactattaataacgatcatattttcagtgtttacgatattgaaactgacacatggtcaaatataattcttcctcctggtaagatgccgcctactcggttctacgccaatatggaagtttataacggtaagatttatttatctggcggttatacaaatggtgtctatcataatgacctgtgggtttacgatccagaaaacccgtgaaaagaaatactggtatagtgattatatgtaagaattagcgttaagcgctattttacatgggagcataggcgaattggtatagccagctggtttaggtccagccgtcgtaaggcactgtgggttcgagtccctctgctcctaccattttaataaggcctgccgaaaggcgggctttatgttgcaaattgtatgatttagtcttttggtaagtacctataatggggaggccttagacggaaagggagtaggaacgtgaagttctatacagccacccctctgtaaacagtcacttttcaatggataaaattatgttcgaatcattattgtctgcactcattaaggctacaggaaataaactaccgggtccatctacctttgaacaaggtgattcgacacttggtctgtatggtgagttgacaagcgacaagtttataacttaccctcagttaagaacacttgttgagcttgactccattggtactataaatacagatgctggttggattaaagtatctagaaataatgttattctttattattcgaagacagctattctccattccattagtccaaaccaacttgacgaggctggtttaatagatggtagtaaagttattgtaatcgatgggaatatgtttaaagttcgtctaatgaatgctggagtaaatccttattcggatatcactactcaaggtaatgaaggttctgaattgtgggatatttttggcaatgttacaactaaaggaagttgggcaaagtacacagatgaacaacttataggcgccggaaacggaagttataactgggcggctaatagaaataccaatagtaattacctacagttttcaccatcgacaactcatcctcaggcaaagaatggcctttatatttacgatggtcatccgccaacagaagctactagttatcgtggatggcgaccggtacttgaatatattccgccaaaggaacttaaaggtattacctctgtattgtcgactgtaaatccaccgccgcaacatgggatgccagtactcgcgtatgatttggataacaacgatatttacatggcctgtggatatacaacaggacctactactttcatgtccgacttacatcggttagaccgagatactaaaacatggaccaagttaccatctacagttccgttccaaggcgagacaactacaaccaatatggtttacaataatggtaagttgattttgcatggtaacccattgtctactggtccgactatttatatttacacgatagctacagacacatgggaaactaaaaagctagctgctattccaggtttagtcgatgcatattacatcgaacgtacagctagtatagttaaagacgatatactgtacattgttggtggtttctctgggcgcagtgataaaatccataagaacattataacagttaaccttacgacatatgaaatcggcatgattgctgatgttctaccaattgaattatggcatcataatttaggatttaacgataatggtgaattagttatcgttgcatctcaaggtagattaacaataggtgggacaaacatctcgccaacggactacgtaaagattagttctgattttagtacaactgaagtcattcctttgaatgcgcctgccaacaaatattcgacgtatagaggaatcatattcggtaataacatctatgtgacgaataactccggaacacgattagctttggtgcaacttaataaagagccagaactaatcggagatactttcccagctatttcttcgtatgaagagatgttagttgtatccgatggagtctatcgatttggtggtgatgtatccaaaacaacacccgtagtcgaatacgaaataaaataatacttcgtgtctaatagtatacgagagtattcagtgatgtagattccagtactcaattcaaatttcgccgttatagctcagcaggtagagcaactgacttgtaatcagtaggtccggggttcgattcctcgtggcggcaccagtttaaaaattaggctccatagttcagttggttagaacatccgcctgtcacgcggaaggtcgccggttcgagtccggctggagtcgccattcgaaaggacaagtctatgaaacattaaatagacttaggtctattccaattggaggtatagtctccagaggaactaaacctctcatctatccctcctcctaaatgtgctctggtaaatgtactgtttaagtacacctagctaaaagagtgagcacagatacagccgtaaaggtagccgaaaggctacctttattccgtcaactacaaatgtaatttactcaagggcttcactatgaatgacaatatcgttaacgcacacattaactacatcaatatgttaatcgaggattctcgtcagattaatgcaatcgcaattaatcgtggactacttcgtattaaacaagatgcggtaatgatccgtgaacatcaaaccgtaggattccacacgggtcctttgttgaaccctgatcaattcattattgattggtacgtagctaatgcagactcaacattggtgattccgtatagttccgaagatggagctaaaatcactttggaagtagcgcgacgtatgccagaagtaaacccacaaaggaacttcgatcatatccgttcgctctcggttcgacctgccgatactatcgagttctctagtaaacaagaacacatcaaatacgtgatcttgcagaatgctagcaacgtgtttacttacggtaccatcaagaagaaatcattttacaactgggttgctaaatggtttgctaaagatgtttatgtaattctcgttaactaaaggaaaatacaatgttgaataaaaaaaagaaacacgtaacgtatttctcgctattactaatgttaaggtaatgagattgctcgtgtagggattgggtgtcataacttcaatcccttctcctgtgttgattatggtgacaaaacagtaaactggggaaacaaatatgagtaaaactctagttcgtgcaaaacttatcacagaagctgatacctggatgtcttctgattgggggagtggatttatagctagtcggttcgttaagacgggtggtgataccattacccctaatgaattcgagtctctgatcactgactttgaagttggcaatatgctcgttgtatggcctaacggattgagaacttcttataaaacagaaagctttgataagaactttacacacgtgaaggacgagtattatcaaactgatttgcgtccattgttctatacagggagtaaacagtaatggctttcgcatgttgtaatgccgtctatatgaactacatcaatcgtgatggtagttttaacatcgatgtattaagaaagatatttggcgttgtagacgatatcgttcagaaagaacgtacagatgagttagctgtatggcatgctaagaaacatgacgtacctgtagctaaggctacgtttgtaatcataggtggaattgagcaagaactctgtacctgtgattgtcataagcatgacggtttgaacgttttacattgaggtgattatgagtacactggtacataaatacgttgcgttcacgcgaacttttaaactcactgaaatcaagatggataagggtgatcgtatggttcgtgttggtggtggtttcaataaaggtaaagggttttttagagtagacttaggtgcacttggctaccgtataactcgccgaaatagataacataaaagccttccccactgatgaaggctttgtttcgtcattagagatcgttagaactcccactgcactgaacaaccccgattacgctcgtcttgctcgtggtgttatgacaaagacagttgctaccgatacaacaaatagagtgttgtggccactgtttaaatatagagggcgagtttaatgaagattacgttttatgggactggagttgcttgtaaggaatatcgtgtttatgcatcagccgaaatcactgatcttaatacactaacgccaattgcaaccattccagctactccgccttaccgtaactatcatgaagttgatttcaatgccataaagaacgttcagtactatgttgttattaggcaggtattagaagaaggtttattcttagataccggtcatactacctgtatagaacgtaatactggtgccttgtctaataatgcggatatgggcgtagataggctacaaaggggtgattctacattgggctatttcggtacagtccctatggaagacttacctggactaacagaactcgtagcagcatatagctctctcaggagtgatgacctcaagggtactactaaacctccttatggaaagtttatggttaacaatgaggtatatttcattccatccagcgtacataactggttgtatccaaatgaaatatatgcagctgggtttgcagctatcgagggaacacttgacggcacttatataactccgcagatcaaaagtgacagtcgatttaaatgtctagttgaacaaggacgcgatattatctatcaaggacatacctaccgtccattcattatggatcaatggatgtttgataatctgttcactccgatgaacaataataaacagttgcggacagcatctaacttacaagttaaatatgatacaataagtaagaaggatgcttatacagcagttgcgctttctaataacaaggcatctaaatacgttaggcaaaatacagtcggggcaactattctttggtacgaccactggctattgtctaatattgatatctgctggaagctgatggaataaaaaaaaaataaggcataagccctctccttcgggagagggctatatgtcgtcttataccaactcgactacatcgtaatcgtgatgtttacctttaccggtccaccaggcaaatttaccgtccttgttgatccgataaccatctctttcggtcagaggattcacagccagataggtagcgaattggggatggtcgttatagactggaaaacgatcgataaggagtttggaaaatgggagaatgtcgcgcatcgacttatacagcggtgcggtgatagcgcggttatattctgtcaggatgcgattgacctcaatgaatacaggatctttttcatcgatcaaccatggcgtttcaccttcattcagaaggagctgctcaccatagatcggtatagcaacttcataatcctttacgaatgcgagaccacctttattaccggttacttcggtgtgaatgatattaccgttatcatcacgcatttgtacacgccaggtcataccgagcagttttgcagcgtgaaccatcctttcaacaaaggttttgaaagtgaagagttcttttgcaatagcgatttcatgttgagacattttaatttccttttaaaaaagttggataacagaaatgatgacaacgacactgatgaacgaccacatcaatccacgttgtagcttatctttacgcatatcacgttgacgacgtttaagccgttcttcagggaggttgcgcattatatttacctatttacgatattaactgggcgtggtttagagttaaccgaaatctttttcactgctcgactagcaacccaatgacgtgcacgatcactaaggtcgttgtcacgtgtgagtatattagattcagcattccagtggtcaaaccgcctacccaaaacgggataatgtgcttgcgctagaaccatacattccaacggactcagtttgttctcagccgaggtgaatacattattcagcagttcaaccgctacagcgcatccaaagatgattggtttccgtgcaggcgtggaataataattgctcctaaacatgtcatgggttgattcgaacacatgaagaacattatcctcatcgatgaggatgtattcggcattaggcgtaagcaggtgttggaaattctttgcggtctctgctagactatgtacatcatctcctgtctccaagaaattcagccagcaatgacgatgttccgtatctccaaccattgtaaatgcttttatagctcgaccccagactttagcttcccatttgttctcagaagcaagatagatcttggacttgtcaagttccacgtagtatggttgtggtgtaccatcctctccagtgatatcgctctgggtgatcgtagtaactcgatcgaccaaaagatccttaccatcccatatgacaatagtcattctttatattctcctgtttacaagctgagacggaataaaacccgctccgttgaggagcgggctattcgttagattaccttaccagaaagctggccagctaaggcaccgattacgggtcggcacccatctggttaggtaacgccactcggggatacccctctcaactggaggtagtaaccgtcgtaacttcagatataaagacggccaagtcaatatacctgcttcggcttgatcctttggcatggatcgctgttagtctctccgatcttatgcggagagagcccacttacaccgaaagctagtgggaataaggtgaggtcactgcggcaccctaatatggcgacggggagccttaggggagatgatccgggtgacctctgttctgttgggacattagtcctcgtatatcattacaactcaagtattcttttacgagagtttaacttctacgtcaactgactcaagaccagccccgtttcttttattagatccatgtgctagcaggtaacgagaccaggtctccgcttgtactcggtcaaacttaaagtagatatgctgcatgatcatcttactcaggtcagcgatttctttcgacaccatatcaaagaacaggtctttgtccattacatcagcatcataacgagccagctcaacgttgcaatactgtgctttcacttcatcatagaactcaacaacaggttcttgatgaaagtaatggactttgttatctttgatttcgataccatggagagtaatctcgatgtggttgctatgatagaaatgttcacgcatagctttattaaactcttccaccatcttatccagatggatacctctaataacctctttggcagtgaatagataattaccatttggatcaacgtattgttcgcgcgcccaaagacagcacagaccaataggaatgatctcagtggggatacgtagatcactgagctgcatcgagttgctccttctttgcatggatggatttggttatgatagtacgtcgttcgcttgctgcattggacattattgtaatttgttcttgcatttgagtaaacagcaaaagttccaacatggtgagcagcatatgctcaatccagagacgtacacacaccttgttcataggggcagtgtaattgagaggctggacgaccttagtaagtgcgccagtcagcgggcaggtaaagcagatatgtagattctcgctatcgctatcttctgcccagtgaacatcttctccctcgccatgtaccatattcgttacatggacaaccggctgatgctcaaatgcttcgggatgaggagtcgtgcctttctccgcgcattgatcaagatagatatcgcgaatgacagccgtaagctcagctggctcaagagacggcataaaagggaatttaagagttactgccatttgaaggttcctattgacgagagacaaaataaacccctcccccgatcaaggggagggagctcaaggttggttgtgacactagtcacagggatcagccgatggaagacccctaaaggtgatgggactctaacccattgtgtcgatcgctggatttcagcccagcttaaccaaattgtaaaagagctatcgtaaaggatcaggaaacgcatatgatagtgcgtaacctttaactaaacgattacctccctaggtggaggttcgacctttgtccaatctaaagttagaggagtagctatctcttccttcattttgaactcaacgatagtacgttgtccaaagtgcttaacacctaacatgtacccatcgatggcaacttcgtattgtctacataatttacggatgtataactcagtgtcagtttcaacacgaggatcttccgctgtagaacgatgttgatgatcccagaaaatacagaactctagtttctgccagttactgaattctgggttataggagaattgatgtagatgggtcgcctcatgttcctctccaacatagaacattagactatcagtgggctctctagtcaactcactgaagtcgactttttgcccacctttagtgagatcgacaacaatgagttgagaagccattatgcgctccgtcggctatcggtcagagaacggatggttctactgtccgcctcattacgatttttattccgcgtgcgttcaactacacggaatacatttacatgttgttcatcaacttcataattctcaaacagttcaccaaagttgttggtcaacgaatctacgatcagtcgtttggcatctacctcattgatgtagtgatagagaataacgccacgatgatacaggaacagaggatagtcctgaccattgattcgaacttcagctgcaaagcctccgtaagacatggtgtctgaattgatgtcttcgcgatatacatccaactgcacgttattgatcgtgtgcatttggatcatgtcgtttccatgaccaccaaagaaggtgggacgcttacgaccagttacaacatcttggatagattccatcagtcgtgatacgtctgtaacgatctcgattacatcgcacagtttgttgattgcttcgaggaaacgagctttcatttcatcgacctcgaaactggaccatgcccgagtttcgtggttgagaatgttaacgccaaaccaggcataaccgttgttatgttttacctttacgcacagatgcggtacatcatccaaaccagactgatgattcaacgtataatcactgatgcgtttcaggaccagttgtacgaagggaagattgatgatctttgtcgacatggagctattcctattaattcttaaaagagattagaggctacataagcactcactagattatgtagcctcagtacattttaatgacgagtgaagctttgattcaagcatcgacccataggggaatcgatggtgaagttttccatgatctcgattgcttcatcaatcgacttgaactcagctacctcggtgatagtgaaaccccgacatttcaggatatcttcagcttgttcagtaacgaagctctgaagaagcttgttcgaacggaaatggtgagagtgttcgatcttaccaatgtagtacatgaacttggtcagtacttcatattccgtggtattattattacgggttttagtcaggaaataatccgccgacttatcatggcggatgacgaacacccgaccattggaagatttacgtggcgcagttcgttgcagaagttgatccctttgatccaactcttctcgcagttgttccacattgatctccggtttagtacagaaccaaagatccagtttttggccagcctttactgcttcatcaatagcaaccggcatgtttgccatacttccagaacggaagcgttgcattacagcagaaaatgacggagactccgcaagccatacgtccccagtatcgcgggtgaccaaagcataccaaccctttttaactttaggtggggttgaggtattggtgaagtcagccatgtatttcatgatcaggcggcgagtattctcgtacgctgcggtcttggaatcattagtgtacatcaggtactcctcttagaatttgtattttctatttaattgagaaaagcggtgggttttccccaccgcaatatatcgtcaaacgatatctttcgggatagactcgatgaaggctttaacgtcattgcggttttctgcaaacagagcttgcagatcacaaccggcaattgaacggaacacaatacctttatctacttgagtagacgggaacatcagctcgatataatcacgaacttctgcatcctccagcagaccgatctcccattgatgatcaacacggcccttacgaaccaatgctggatcaaggtgctctggatggttggtagttagaagaatcagcgatccatccaacggaacaacaccatcaagggcattcaacaggccagagagtgttaggccacccatgcgagtatcttcttcacctccattagcacgacggttatgaagttcccatatgcgaagcataattgggtcatcggcaatgtatttagaaaggggttcttccggcaccggtgcatcaaagctgtttccaatgacatctcggtattggcgagattcagttgggttatgttgctgatacccaacactgaaatcttcaccgggtatatcccatatacacatgggtccgccgccattatctatcactcgatagttagtcaaccccatctgagtgataaggctatccaactcatcttcctcgccagctgtcagtttcttaagcgaacgattctggactgccttattggtatcgaagtcctcgatcatcagaacactaccagaaggcatagacgtaaccgctttacgaagcagttcatcggagatactggctaaagacaaccaataaatattcttattaaaagccgaagcgattgccttaccgatagatgtcttaccagtgccagggggacctgaaagcatagcgcacattttgtacggcatgccacgggactcataccactcccgtccagagaagaactcttcaatcttaccaatgatctccgctttttgtttgcggttcatgataactgtgttcagcgcgcgtttagtaatcgggatagaatcaccccaacgcaagccttcccatggaatgacgcagacttctttatcatctcccttaacacggaattcctctacaagatctaacagtagttgagtgttcctagtcaagccgtggatctcaatctggaatttttccatatgagtaccagagctatccagcttagagcgattgaaccagaagaagcgccctttgtagaagaagaaatgggtaccaaaaccagcgccgatatcggtgctaggagagggactaccattccacatagagttcaacgatagcttccgactgaacctggcgataggttgttgtttgaaccacttcatgaaggcgatacattgttcttcattagggccatgtccaccattgttcattatcagagatgtgacaacctgattccgaattgcgttgaacattttcttaggtaaacttcgcgccatcataagcacccatccacccaaaccaacaccgactaaagatgcgaatgtcggattgatcgacatgatctctttgtaccaggacataaactcctgaatcatttcttttccctcacatagctgaagtttccacgcgtgtaggtattttggatcggatgcttctcgataatctcatggttggccatcgaaagcatgttttcagtgagtgcgggaatatattccccaccgatcatgtaaccgaggttcttcctttcttcatcgccaatgtgacgttgatacaaaggttgctcataggtcacaatgaatagaccagtataacacttgaagatgataaagcattgtccgcggaggaacttataacgccattgctgctttttaattttctcaatagggaaccggtattctttaccaccttcacgggaaatacgacgaagctcacctgcacatttctgtgcccaggatccttcaccgacgacatagatttcttcgatcaaatcgtcgtaaccgggacggaactcagcctttctccctcgggcattcttgtaaattttgtacgactgaacttcaggaccgaaccagaatccttcagtgaagtttacgacgtgtggtggacgatacacattacgtgcgatttttacatccaccttaacgtcgccattaagggtgaaatcttcgatatatgccagacgacgcatcagttgatgatacgggtaaagcttttgcgtttgttctcccggcaaatgaaaacgaagaagatgtggttccacgttatcggaaatacgcatccgatggttcttggtgagttcactcagattgaatgacttaatttcctcacgcgcagctcgcgctacatatttcgcatatttattttcacggtcatcaacgtaaatgttcatgacagctgtgacactttcattgaagttcattgcattttccttttggttaagcttaacggcataaaagtaatatagacctctaaacggttagaatagaggtctactttttctagaacttcagttcatgttccctggctttgaataccagaggacgtgcacgatcctgaacactgaccacaaattgatcagtcccaggaatctgaccgagcagagttaggggttcatccttttctgcacagagataagaagtccgccctttcaaggctgaagcttcaattcgttcactagcacgaacagtaacacgataagtcatttcattcactcaaagtcaattacacgccaacgatcatacccgcacgcagcgagcaaaccgacacgctccattgcaggcacatagcccgacagtttgacggtcttcaattctccggtttccatcccatgatacaacgatttcgcaatagcagtgtccagataccactgcgtcaacggaatcgaagtattataggtataaccgcagaacacatcataaacgtgatgatgttcattaatgaacaggcagttaccttgagcgccgttatcgtgatgggtttcttggatcaacgcgcggatctcactcagatggccggaagtaaagctatcgtaaaaccggccaacatcatcatcccaaagcagatcacgaatacgacgaaccagagtatcttcaccaccaatgatgatacacttgattttctgtttgcgttcttcctgcgggggatggtaagtgttgtcgttattttcatggaagcgaacgacatgggtattgaaaccgcaatccttacgaccgaagaaaacaacctgatcggcaaaaactgcctgggcgaaatgcatttgtcctttcatattcactcctccaaaatatggatggcttcaccgcgttccaagaacggcagataagtctcgtagttgttgatgacccactgacaggattcgtgcttcggggtatcctgaatgaatacacgcataaaggtcagaaggtagatcagagaagcacggttgaaactcagaccagcctgttcccattcttccttgtattggcgggccttatcgatgtgataatccaaaccttccaatgcagcgatgttaacaccatcgacagcgttagccaaatcctcgatcatgtacgggaaaaccagatcgacgtactcatcatgttcaacagcgtttacttgttcgatagcgttcatacttcatttccttgtttgtaataaaccgatttacgagaatgtggaagacacgacatatcacggacggggaagatcccgtccgcgtatgctgttatcacctgtggtcttgcccgagtgggcatctcagcttcagctttcatggttacaggcagtacgcctttactgagaatatcatcaacgagttgattccaggcgatagagtacattattcggtaccttgttccgggaggaattggttaatagcatcacgatagtctcgatcagccagagccaacagagaccatttagttgctaccggaagttcacggcatttactggtaacctgatagagcgtgtagccagccacacgctcagcaatcggatccagatgccattgagtatcgcggatttgtttgatcgctttcggagaaaccagatcgtagacaacaccatggctggtaataccgatgatggtaaccttaccagcagctcgacgagaaatctcctccatatccgattctttcaggagccggctccggcgaacgatgtgctgcaaatagcggcgagcatttcgcagtgcgttatgttcacccatgaagtagaactcacgaatgaacaggtgttcgttgttgtcggtacggatttgaacaggacgagcgaacccatcaccaatacccagtgaacaggtttcttcacgggacattccgaagaagtctacatggctcttacaaagcagatacagatcaccacgtggtccaaggtataccttagtggcgctggaatcttctacgtcgacttcattgtgttcgcaatagataccgaggccattcagaatcagtttagcctgatgaagctgctcttccatataacgactgatgttaccaccagtgtaagcgactacaccagtcagcaagttctctccattacagggaatgatttccagatcgtcaagttcagttagcttgaaaacctgtttgaccttctccatatcgaaacggtcgtagataccaatgaatttagccatgtcgcattttcctcttttggttaaagtaattacatacaacgggggtggggagtgtattcttactcggtacagctactcttgaggtagctgctatccgaggaactattatgctggattgtattgggagtttaatactcatttcggatgtacctaaaggtagtgtatattaaaagaagaataaagaggggtaatctccccctcattagatcaaggtgatccagtataaaattccttatcttttttagataaggttattgctccaggtgaaaccatcaggagcattcttactaaagaattcattaccccaaccaaaagaaatcttaaagtctttaactacacctgaatcggagttaataactttatattcactgacctcatcgctattctgcaatacaatcaacagagcgataagatcttcaggattgccaatacagagctcatgacgcttgtcatgtctcttaaagataactgtcagcatatcaaacctcatgacggaataaagagagctccgaagagctctcagaatttatacatcaatacgtctttcggatatcgacgcagaagaaccttgaaatcggtatccatgggtgcagtggtcgaagtaacaactttacccttcataacttcacgaaggtctacctcttcaactgtgacattgtggatagtcttccgagtggtccattccgtatcaatgttgttatacggattattattcttctgccatccatctgaatcgcggaagggaatagtgtaaacataaatcgtcaacttgaggaattcttcaagtgtgattaatcgatcggagaagatccatatatcaccattgatctcaacgaagcgatcagagttaaactctttttctacagcactacctattccaagtagttcagcttctcgtttgacagaggtagcataaagatttaggttagactcaaccccatcccacactgttaacttaccggaccttttaaagccaggcatgagttccttctgtttgtagagagagccatgatacaacagctctggtttgtccatgatgcgtttctcttgataaactcatacgatggatgccttttacaacatccatcgtctatgagccttacacggccttgtagctatcatccatatcgataggacttccataataaatctggaacctattgaacagactgtccatgtctacacgtagagcacggatattcatgcggttatcactcggccgcccttcggactcccaaatggcatgtgcgatcgaaggagctacgttattcaggtagtcttcaacctcatgctcttcgagtaacagagtatcctggaaaccgatacgggagataatagcatagtcacgctgatcgtgttttttagaaccttcacgtaccaggtaactcgtgccagatccattcctacaaccattaccatgaatctctacaacgaacttaccgtgccatttgtagtccatgcgaagtactcctttatttgatccgcttcattacaagagggacagacaaagtaatcccattcgacagtttttccaggatgcggtttacagcagcagcctcttgggcgttctcacaagggagcataatagcatccccgtagtaatgactgtgatccagacgatcaccccagacactgtttacgaaaccatattccatgccgtcgtttgtagttacaatcgcaacgacatggtcaggaccaatcataccagtttcgaggtcaccaacaagatccagcttctgtacaacgccccgctggcagatccatacttcatgataacgataaggagtaaggtcaccaccagtgctcggatcgacctcgctaacgaaatacagagtaccccagttcatgctttgaaactgaacggtctgcttgtaagcttcccatttgtcttcaagacagtttacatgtttgtcgatccacaaaccctcgttattgaggctatcgacgataccgtcccggacacgtacgacatgaagagtcttagtcattttcaatctccttttaatagtttctgaatcgatcgtaagtgactttttctttaagccgatcgataatgtaattacgaccttgagtgaactgaagtttttgatgactgtccaactcgctccattcggtcaagcgaggaagatctgaaacctgatcatatttcgccttattgagcttcctgatcatgtcccagatatagtcaccttcaatgaaccagcggagaccagtgaacgtatccacgtcagttagcttgaccccatagaggctaagatcaactcctgcttcttctgccatcttacaggtctttttataggcatcgaataccgcacgaaggcgatggtcgaaaccatcaccctcgcacatttcgatagctacgatcaacatcggaaacgtatcactgtagaacttgatcagcttccgggtcgctgcttccagcgctttctgcttttgcgtttttgccatttttaatatccctaaattcacgaaggaattctttgtgttcatcgtaatgtttaaaagccagtgcaagcacattaagtgccttcccgaaagcgcgtcgttcactgacgggatattctgaccagattttaaacttgttctttggtagttgaaagttcagatgtacgatcgtgtcccaataggaatacgaaaacaaccagctcgcatgttcatagacagtgtggttagcagggtctacacccatcacatccatgtagatgccgttttctttcgccacgcacagaagattcctgtgacaatggagaaggtcagtcatcacatctacgtctggtatgcctttaccagaataagaatggaacttacgaaccattaccatccaggcctcgaatgctcttttaaatgcagcagtctgccgacgcgtcttcgttgatttcttagtctccatcatgatgctccactcgaccagaaaggttatattcaaccttgaactgcattcttaccggagcgtaagtttgcggatattctggaatacttttgtattcaccttcaaaacaggtgaacaacatttcacccgtattgactttgtagatacttggcatgtagtgtacgtaccacagcttgtcatcttttagaacataatgaccaaaactgttttcacgacgagcatcttttatgacctggatattcttaccaagtacgtctccgatgaaaccgaggtgatcatccagatccataccctcggaatcaccattcatgactaaagcttcaggagacaaatacatctttcgaatggtggcattaaccggttcgagataacctttctctacacccgacatccatttgttgaaagaaccaatccgcttgggatcgtctgtacctaccaggatagtggtatcgtcataaacgatattaatcaaatcgtagccagctgcacgattacgttgaatgatccaaccatgatagttgacccgcagaaaagccattgcatgtagtttgcctcggagggcttccagagtaagctttttcattttagttccttagtaaacgccattgatgatggcctcgcggaaacgagcccactcagtttgaccaactaccagctctctttcttttggacgccagaggtggtcgccgcaatcaagacctaggtaaagcatattagctttccattggttccgatggttacgcagtgtagccgacagactgaactcacgcataacttcattaacatccaaatgaaccagagtttcactggtcattccgctcatgctgataccaagaacctcacgaacacgaatcagatcatccgtcatcgaacgccaggcttggatatgtgcgtaatactcatctggagtcatgctgtttttatagttcgatgctccgggcgtcatggacatccaactcggaaattggatagacatgtagtaaagccagtcgctatcgtatcgcagttcgttcagtttttcctggataatggggttggtggttgctttagccattagactactacctcgcgtagataagcaatgagttcctcctggaactcagcccagacagatttcatatcaaccccttcaggttgacgtgcacgccatacatcggagtctgccggtagttccagcgctttacagatatcacgccattggtgaacatacttacggacaccagccggagtggaaagaaccaccagagaatcgatggtagccaatttaacgaaaggttcgtcttcaatcggcataccaccccaactgacatcaatctcacgaacgatgtcattcagttcagccaggcgatgatggaactcgacaacaccttcacgaccaggtttgtagttcagaccagacggcatggtacgcatcatggccgggaacagctcggtcagcacagcgtagtaacgctcgtccttggccagatcacggagtttgttttcgagcatggaattaactttaggcatttctatttcctcagggcttgatggaattaagcagttgtaactttaggttggacgggtttgataatttcgttataggacattcagttgtaggtggtgaagaacttcggatgacttactttcaaccatttaacgaacttattcagttcttcttcccgaacgaaaccattaccgtaaagatcacggcggcacggatcaccctcgggcatttcagcgcagtgggcatcatgcatttgtcggatcaactccaacaaattttctttacgtccaatcaggaacgtaaatacatgcagcggatcccaacttgtcatggtggtccacatggatttgttggcagtcagatttttgagcttgagctctttcaccttatccatcaccaatttgcattggaccaacatcccttcaagttgttcctccggatctccgtcaataatccagtgagaaccgccaggcatataaccgcagaaggtgtaaaggttatcacgcagatacgcatgacgaccacgttccaatgcttctgctttcttttgttccttagatttagccatcttagtaaccctcgtcagatttgaatgtgcgttcaggactgaacacgtatttgatatcgtcaatcacagctgtgatatagacctgatattcttttgaaatagattccatcaactctaccgatacgtactccgcagtttgaatacggttgtaagcatcgtcaagcatgtcatcatcatgaccgaacaacaaaccgagatcagtagaattgattaccgggtaatgtacccagttacggatatacggtttaccaagatgaattacttgaataacttcatcatgttcctgtttctttttcttgtttacgtatttgacgtgacgttcgatgaaagcatagataccggaaccattggtgttaccgtatgcagccagttcgaagccgtatttatggtcgatgttattggtgtcacgacgccattgaggaatgaaagcactcatttgaattcgtaccatccgttaatgatcagatcaagatccttccagaacaactgagagaattcatcgaaggtatctgcgttctccagtccatcgagatcaacgtcaggagacttaacgaaactcataccagtttcgggatagatatctgtgatgaccctagtactgttgtcagagtaatcacgggtgaatgtggttaccgaatggtcagtaaaaagagcgacacagatatcacctttatgattccccagttcatcggtaagagcatcgatgatatcgacatcgatgatatttccaccaaagtcaagaatttttagacgattacggacaagttcatttgctgcccaatcgccagactggataaccaaaagcttcgcggtttcaccgcgataggttacaagatcttcttcgccttctcgccgcataccccagtcgaaacggatgtccgtatcttcattggctttatcacgtgcgatgattacaccctgcttaccataaactacgatatgtttcatttgtatattccttttggttaattgaaacggctatattcaacccaccactcttcgtcacgaatgtgaagagtagtacacaggtcgatgattgcatcgaaaagcagaacagtcgttggattgcgtccaatgaactgacgttggaaagaagtgaagatagcgatgatgttatcgccatcttctgtgtcaaacaagatctgatcatgaacaagagacatgtcatagaaatcaatcttagacaatgcctctagaagaacttccatgcgagtgagggcggtattcagttcgaatacaatcagcggactgcaaccacgctccttatggtgatgcatgcgatgtttggagatacgttcgacgataagccggggaagaccttgtacatctacgagtttacgtttcatttttgattttcctctttacgaaatagaagccctcccgaaggagggcaattatgttgttacaggttgataacggttacgaactcgaatacacgacagagttcttcgtcacgataagcttgacggaaaggtttaccttctttaccacaatacgggaagaacagtttacgatgctccgtatcgccaaaccagaaggtagtggtattggaatcgatgatcccgtgtgtagccacatcccggatgttctggaatacatggaccactttgtcggcgataacgcgaagttccacaccatgctcggtcatcatggccagaatgtcttcacgactgtagtcggtccgttcgttgttggtcatgatctcgtgaaccagagaacgcttctctttgtcaccgaagcagatgcataccagatgaacagaagcaccttcgatcttcatgccattgataggtttaaacagaacaatgttctcgtatttgaaatcgttggtgacgatcaataccgaactatcacgtacagcgatacccaggctataggccatgacttattcctctttagcgattgaaatagttgtacttgccgcaatctcatgatcgcggagatacacaagtttaactttgtaattacccggagtttcacccattgccaggatcaacttaggtaggtcaggttgagtggttacatgtgccagcataagctgagctgttttgaagtctttccaccggaccaactcctcattaacataagaagtgacccattcagcgatcttctcaccgcgctttcgaacgaaccacaaaagatcccgaccatcttcggtcgagaccttcatgtagtacggcgattgaacggggagcatcaggttacgaatattattcgctcccgatgtatcccagttaaataccatgcttacctcacagacttggtagagggaacgccggatttacacggatatcagtttcagtgacatacacgtaattgatggtggtttcatctcgacgaataccatacatcaatggagcttttgccggatcgactaccatgattcgacccggttgatctgcttccatatagatctcacctttggcattctttacctgattattggtgagaatgaacgtaccacatttgaatttcttttccatgtttacctcaattcaaccaacggttatcggtatcagcgaaacgtgcagatgcacgatgcgggtaaccgtaagggatttgcgggaggataggttgatcgatgagattagaaggataaccttcttcatcagggaaatacccatccagggagtaaatcaattgcactacacgtacacggtcggagttcggtccataaaaacggccgcagttcaaaccaactccatgcatgaactgttcggagtcaataggaatgaaccgatagtagtagcgaagatttttggtcgacaacagcttttcgttcagatagtctgcccagtctccagcgttgtacagatcccgttcctcaatatcaacagtatctgcggctacagcagctgcacggaaaatgtcacgcacgtagtctttttcagtaagacccatggtaacaaattcaggtaacccggttcgaccaagaccaatggtgaaacgtgcttgcggcagttcgtcagcacgacgcgtataaataacgtagtcattaccttcgaattgattaacaatcgccttctggatatctgctactttttgttcgagtacatgcgacatctcgaatacagggttgttcggttgaatggccataccagatacagttcctgcaacatcaactacattagacatgttcgctcctaagggaataaagaggacccgaaggtcctcaattgagtaacagatagctatactgcgtttcttttagggcgatccgaatgcgaccttcgatttgtttggcttctgcttgacttgcaggaaactccaacaattccagatcgctgttttctggatcaccttccatcaatcgattcatcttaggccaagggctagcttgtcctttaatgcgtacgatcaattggtctacatctttagagactgttttacttcgccccatgacgaacttaccggtcccaagatggacaatgcagtacaacccattcgttacaacatctttacgtttccccctaccccagatagtcgaagaccatttgttgtattgggtttcaccatggaatgcctgttgcatttcaaaatccttgctaaatgactattacatttagcagcccagtattacttgtggtattctgggaagagcagacgggattcttctcgatatgtaacaacaagcgattccagcttactgagaatctcagccatgttgagatacgcatctcggctagctttatgttgctcatacataggatcgaatacaccaatagattccatttcggagtcgagttgaatggctttgtccaatgcctcgtcagaaatcataaagatctgacgaccttccatcgccaccttcaattgcatttcgaggatacggttgtaacctttgcggaagaactcggggctaccatcatatcctcgtgcaacagcacggcggaaaagttcaggatcgactgggatatcagtggctaccccattatgaggtccgaccacgaatcgacgtccgcagctatctacaccgataaacagtgtagtgccttccatttctttttcgagggtaagtacccagccaggatgataggttacattcggattatcctgcgtgcgcagtgtggtggttgtatagaactgatcacctactttcattttcgaatcctctattaatgaatgacaatctgactacgggaggcatagaacgatacagcttcaggatcactcgatagaacaacctcgtaagtgtccccgcttaccttacgaatgatcttgagttcatcacctttatttgccattattaaaccaggcccactatcactaacgttggcagtgatgttttccagagcagtagctttaacactcatggtttattcctcttgatcgagataactatgtttatttaccatagtcgttgaatgtatcttccatctcactaaatgggatggtttcaatctgattgaaattatcatggttgattacccggaaaccaccagctggattatctacatcctcacaaatgatttcaaggtcatcaccttcattggcatactttgtttcggtataacctttttctctatcagtacgggtaataaagatatccctggccgcctgcaataccatgcctttaacgacatcgttctttgccaggttagcactaagtttcattgtatcactaatgagagtactgaagttcatttctttttacctttcgctttatctgtcactacatctttacgctctctccatttttggtcgagtatcgtgttgatgatatatttttgtttacttgttgtaacttgttgcattttacaccgttgaagcaattacagcgacagagattagttcacgttggaaacgatttgcatcgggccaattcagagtgtgatttgcatgtgcattgatctcacccgtggaacgatcaacccaaacagtgaggtaacggcgatcccgtccctcgaagatacagtttacaacaaacagacgttcatcgtttgcgttatccctcagttcagctttgaagtcgaaacgattgttgaaagcatcaacgatagcattcgttgcagcttcggtcgttacaccagccttatgttgttgatcgtaataaatacgcatgacgctagttacagccgcattacgtgattcacggatcagtatatccttcattacatgttccccggttgaccaagcttgtaatataggcttttaaaacaattgaatgtaacgacataatgctctccccgaagggagagctctatgttaagccaccagagagaacttaactccgataatcggagattcccgatcgatcttgatcacagcacgaccagtaacaccatcgacttcgaaggtagttccccaccgcagtccatccatcttggataccataccaaaacggaaaagaccatcgcgacgaatttcgataggatcgtgttcggtgactttgtggaatagaatattatcacccgaatcaacgtaggcgacttcttcaatcttcagtttacgaatgtcttcatcaccaccgcagagtgcaaagatattgaacgtggaatccaccttcacataactagacagtaccgaaccaacaccttctatatcaacccgataaacaggcatacgtaaatgttgtgcgaagtgtttatcgctcttacccatttggtaaagcggtacacggatagaactagagactttctcagtcatcagtattctccaaatttgaaattgaagctaatgggtttatcagatcgcgttctaatgactcgaacaaattcattcaatgaagtttcaatgacataatagaacgaggactgatatatcaaatcttccctatagcgttgatctagtataaccatgtcattagaaagatagacataaaatgtcgaatctaagctatcgaccacaacaggattcgaacagaccggagtcgtttttataccgtcatgtgagtatcctactacttctatattcacgcgcttattattcactacaagaggacgatgaataataatcattacccaagctagtagtaatgcagtcatgaataatagaaaagataactcaatgagagttttatccatacggaatctccgtgttagattgtcctccaatcaataacgttattgttacccttcaaatcgaattcctcgaatttataagcaccaccgcctcttaaccagacttggtgatatttgaagtacagggtatcagcatcgttggagattaaatctatctccagattggtaaggtttttgtggtaggtcacttcaccatttctaactacaacatagaactggttcctaccatcacgcagcccatagcaattacctttatttttaattggtattttgcgactcactgcacctcggacatgtagtacatttacgacaaaatgtttcctgatcctaaatacaaaacgaacgattgtataagcaagtgcaattacagcaactatgatgcataagttaaccagtgtttcaataaacattgataacctcattgaatattaagttggcgtgcaagaccatggttagatgggatttcaaccacatcaagatcaatgttgtctttcacccgataaacccgttctagaacaccactcatattgcattcgaaacgaagacccgagtcaggatgaattcctagtgacacccaactggtatcatcatccagcgaaaacgtaaacttgttctgagtttccattttctgtaccagccattcgccttcgttttttaccagtttgatgttagaattcatgtctattctccgggtaattttacgaccttataaacagactgaccattgtcatgtgtctcattagtcgtatgttcatctaaatagagataagctatctgcacagctttgctaatggtatcggcccagatgcacaaggttttagttcgatatgtttgtttttcccacgagtactttttaggttctttgtaggtaagctcgatgctaagcgatacgaattgcttcgtagccttagcggattcaaacatagtcttctggtcttcatcagacaccaagagtttattggcatcgatgaaggatccataatagcaactacggccacatagcatttgtgtcagagtggcctttccattataatggcgaggctctatctctacacgccaactccagtccaatagcttctttatcttttcgtcgagttcagtcattatggcatctcaaattgaatggtgaccatagatttttcagggttgtattcgatgtaagggttgacataacccaaacggaaaagccattgccggagttcttgatagtctgccatgttccacggcatactgcccatactgacgcgatagaccagacctttagtgtggtcatcgagtttccagttctccggttccaatacaccagaccgaataataatgcgcgtttgatcaacgacattgaacatttctggattagcttcgcgtaccttacggaatgcttcagaagccttactcgtgttgtcgaagagagacaacgactcggggagtgaaccccaaccttgtttaacttgcattttcaagaccctaaagaaaaatgtatagaaaggggacccgaaggtcccctgtcattagttcagagaagtgcgatgagcgtactcgaaggtatcgacaccatcaaccatgttgaacacagcgatgatcgcgctcatgggtttcttgcccatgttgaagtgcacgatgaagctgtctttgtaacactcgatggaacgaatgccataaacgacattgatgcgatcgatttggttacgaataaccagcgcttcctcatcggtcatattttcgatgtagttctcgatcagctggaacacccgctcatcgcccaggatcagatttttacgttcgacttccaccggagcgaaggtcagtaggtgaggcatgaattccggaagagcctccacgttgaacaacagcttgtcgtccatcagaggagttgcacgatacagatccgacaggacgatattaccacccacgatctcgattttgttttcttgagccagagtggaagcgaggcggcgatcagcagtattattagaaccgaacattacattttcctttttagttaatcagtagattgggattccgggttagacttcccaggtgtctttccagcgagttacaggaagttggaacatctcacagagtttagttactgcacgatgttccaggttattttctggatggaatgtgatggggcttatcgaataaccccagtcaacacgacagccagtttctttatggatttcactgagagcggtataagaaccactgccatcatcgtaacccattttgtacgggttaacgcagatctgggtattacgcttcatcagaaccttatcaacttcaatcgacaagagtcggacgaattcgttggttttctcgatgtcatcaacccagaattccagaaggatccattttccacgtgggtcattatgaccgccttggaagaatacactgaaaccttgttttgcttgatagaacggagaggacatcaggttacatgtaacaacccgatgaacagcttcccatacacgctcggtgacatagtcaccatagagttcaatgcatggaccacgaccagggaaactttccttttcagcgaatttgagttcgaacatgttattctcccgagcgatagcggttgtaacgaacccagtttccatcacccggccgctggaattcaatggtatccatcatgtggtaaccgaagtgttcgatgatccacagagctacttgcttggaacgcttcatgcccatttcacaatggacaacgatattttcgccattacaggctttcacccattcgacgagctctgcattacggctattgatgggattatcgaatccatcaatctcgaagacattgacaccgtcagcgataccgtaattatcagcacggttgtattcgatactgatcagattggtaccgggattaacggcacacccaacaccacgaggaacatggataacgcctttacgcttacgagtaacctttacagatacgatgctcatttggaatcaacctctcgcagtgcttgaatcagtttttctttggcttctacgctggaaccccagcattcgatcacgtcgtagccgcgcccatctttcttcatgaaagcacgtgcatcatgtccgagtttaccagccacatgcatgttgtaagcctggaagcgctcgggagtcatggtaaccggatccagatggatgatggtaaccatatcgttcaggatgttgtaagtcagcattttgaattttccttttaaatattagtggtgtagtggcgaacgacactatgtgtacgctctgcggtttttcggagaacactgaagttaacgacatcatgatcgttgaaaactccagttttgatgatttcggttacggacgccatctcgcatgcgagtccaaggcgagcgataatcatgtcagcatgtccaagattattgaagttacatgccttgctgatatccgatgtgaagtgaagagaattgggatcatctccaacagtgagaaacacaaatttgttcccagccgagatctcgatgataagttcatcatcaccgtttttgtcttccagtagctcataaagctcatggtatttgatgcacccttgtacccgcccgagttcgatctcggtgttaccataccaggtagctttagcgagttgcatgaaattcatcgcggaatagaaatccacgaacacagcaccgtaacgacgaacatcgtctacatcgaaatctttagctagttgattatggacgatgaacacaggtacgttaaaaatgaaatcaacgtacaggtgaagctcacatgcagacggaataccgtcgatggtattgctcagaatttcttttcgcaattgtttcattgtactatcctttttacatggtggaatatcacatttgtaatatagggatttaaaaggtttaaatataaccttctattatcacagttgtaatataggcttttaatgcgtttaaatataaaagaaaaaaaaggacataacgcctctcccgaaggagaggcaattatgtttactcaccaacgtcgggttcggtttcgccgccagtctccggaggagtaccgccagtgccaccattctcaccttcgttatcgccgccttcacccggttcaggttctaccggagcttccggttgttcttcaacatagaagctaacgaacatctcatttccattcttgatttcaacggaaacggatttccaaccggcatcttcaatcgctttctttagagcagcaacggaagtttcagcaatggtgacattacggaaatgacggtgaacgaaatggacagcttgttccggatcgttaaggaaatcaacagtcccaggaagagacagatattcgttgatagcatcttcgtactgagcaatctcagcatcggacatagccttgccggcttcgtccagggaataaatcgccattgggtgattctccatagtcatgaacagcggtattgctgtacataacatcggtcacttcatagcgataataccaaagccaagttcagtccgtacaccggtttgcccctcggtaacctgctctactttaacactccattcaggatcgccaaccaaagtaacttctagaatagaatgcgtatcttcccctgccattcggtatgccgattcaagagattggtatacttcaattgttctatcctgacagcaaagaaacacagtgccctgggtatctggaaagtctagatacattcgacggaagtctgaataagcaataaggttactaccgacgtagtgtgtcatactaccgataataacacgacgcttttctttcttttttggcttttctttcttttttgattctgttggtagtgttaaccaaattaaaccggccagaattaaaagaataatagccgatgtcggaatagtaaatggcatactttccacctaaaaattaaacggtaaaaaagctgtccccgtggggacagccttatgtcagatcagttgttgacagtggcccagtaggatgccgccagatcaatctccagagtattcggagcgacttcaaccgtctgagattcaccactctcattaacaatgaacttcggtaccagatggaaatcattctggataccggccatggtaccagcgatagcacgatcgataaatgccgaatgtactttgactgcttcggcttcaacatcaagacctttaagaagatcgcttttgagatcttcgcagtatttcagtacagaagcaccagcgttggtcagagccgaatgttgttcaattacgttttctacatgttccattttcgtatccttaattagagagaaggtataactgcgtctcctaagagacgcagattaaattacttgctgaatacacgattgctcatgccagtgctgttcagtgcttcatatggaacaaagatggacgagccggagttacccagactgttagccattttttcttgaacttccagagcacgatattgcagaagcttctcgctaatacccgctgcaacaatttggttctgatcacgcagggtacgtgctttagtcagctcaacctcacgatcagcttcggccagtttcaaggcgttagtgcgtttggtcatttcaatcgcttgctggttattctcggtctgaatagcaagttcacgctcagcttgtttctcaatagcttcagtaataacactcggatacttcagactgccgagagtaacgttagatacttcaagcggagaatttttcattgcttcttggagtttggccagaagatcagcggtgatcttatcgaagtttgcaggaacttcttcgactttatatttgccaagtacagaacgagaaaccgagctaactacatctcgaccatagatactgtaaacttgatccagggtaacgatattgtccacaacggtgatcgagttgaacatggcgttgataacttgttcgttaccagcaacgcgagtccggaagctaacggtaaaagtcagatcgagtttatctgccatttttacagtcagttgttcgtttttggtctgtaccgaaccatccaacaggataagttggtctcgtccataaacggtgagtttaccaggttcaagaacttccggagagtagccattcacagtgagtagcttacctttatgtgccggaggaataacctcgaacgaacagccggtaacagcgagagcgatcagaattgcaaaaacaaattggacgtactttttcattgcgcgttttcctgtttagatttcttgagttgttcgtcaaaagagagttgggctttcgacacattatcttgaggtttggtaactttttccgggatcgatgtttgatcaacaataggtgcatcgaatcgagttaccgctgattgtttcaccggagtggtaatttgaagcagcgacaattggaagaagattacgatgaccaaagcgatgaggaagcgttttgcaaaaccaagttgttttacccagttctttttagagaacagaatccatcccgccagaccaatcgaaatcagtgtgaggattccatagaggaatggactaccaataataacgatgtttagattatgcatacttacctcattgattaacgtgtttgaaatattgatctgctaaggtattgttattatcagaaataagtctaacaccaacagcgcgatcagttacagatttactccgcttgagcttagagtcataatccctggagcaacgatagttacctgaactcaggaaccgaagggccagaaggataccttctttaattccttcatcgaacgcgtcttgttgtgcagcgtccgtgtaacggagcacattttctcggctgaacgtttcatgagtttctgaaaactcttggaggaataagtcatttgctcttaaccactcttttgtaggtttaaagggacaatcatctttcgtatcagtcacgtgttaactccctcaaaaagagattgcgtgagatcaggataccacggcgtactagtgaggcggattttaccctcttcatcgtacacatcactaccgacgatcatgatttgaccatgagtctgaatagcatcgatagtagccaaagcagcttttcttgcagtatcagtgaagagtttagacatcattcgtccttcgccgttatatgaaatatcagcgaaaccttcattgatgatgccatctacccgttcgcgaatttcatcttgtaggaattttgttttcccgctctgaaattcgttatcatggtaggggtattctactttcgcttcttccatacattcacctcggttatggaactacgcttcattcgccgccttagcgatgatgctgctttctctgttgtctcggtccaaccaccaccgaagatgatgtgatcgtcgttgatctgtgtatgtagttcatgtgtagccattacgccactaagaccacgagatgcgtaatactcgataagagcgttagccggatcactcatgtgttaaccctgtcgtagtgataggagtagatggaacccacaacgtgactagcagctgaagtatccagagaatggttctccaccattttcacagcggagaggttaatatcaccgagcttgtaagcaaagtcagtgagccattcacggacaggtccttcagctatacccgtcttgtcaaccacgtcaaccgttgctttatccagaagatcatttaacattgcaacaccgacattgataatggatttctcaaggtcgataacaacggcagaaaactccccactcactcggagcaaggagtcaaggtctggatcgttccaatctaacgaaggaaccttcatcaggtattcacggactcgaagtaggtttccgagagcccggagacacaagtgagattcacaccagggtcttcatcgtggtcggtagacccagtgatgatatcctcgtaatggttttcaacagcgtcgagaacaccacccaccgcatagtcaatagcggcagcagctgccccgcaaagaacatcattgccgtcgttggtgtcatctttactgagttcacgaactttgttcttgaacagttcaattgcctcagtacgtacttctacagcagcgccaatcagttgagtagccattaagcttctcctacaagttgtttggttttaagacgtagtttgtgttgccggtatttcagaatggatgatgctttaacttcacccctcagaatgcgtttagtttcttcagtcgtgaagtcagcatcgacttggtagatgtaatgcttctcgtagaaatgttggtatccatggaaaccataataaccacgtagaagttttgaaccagtcaatcgtcgtagttctttcaccatacctgaaccgacgccttttcgccggaattcgggtttaacgtagaacatacagagattacgacggccagtattgtgcaagatataaccaaccagtgcaccatcagtatcatcgatcgccattaccacacggtaacgtctcacggtaccatttttcagaatggttttgatataacgacagagtgaaccggattgttcgtaaagtttgttctctatgatcgaacgtagggacatcttcacaagaatgggagcttcgatgatactgtagttcattagctgtttaccaatttgaaataatcaactaccccatcggaaatatcgattgcttccacatcttcagatgcgactggaatccagtttccacctgcttcaatagcttcggctttttcttcttcacccaccttaggaatgagtgaaaaaccgggacagtcgggatggttaccttcaatcacaccgagtacaccagagacaatatcatccgccatggcagcattcggattgacatatgcctcatacttaccttgttcagcttcagcgagaatttcatctcgtttactatttaccgcgtctataaacagatcacgtacttcactgaacgtggctgcgcgcggttcaccagtgccttcgaaatatacggtcatggtttttcgatcgctttgttgagttcttgttctagttgcacgagttcttcatcggtgagatcccttgaagcacacatgcaacgccctggtcgtttgtaccacgtgatacagacatcacgccaaatcaaagcaccctcatcttcacctggaatcctgaatgtttcaagttcatcggtgttaagagtgggaccacccggataagggttaactcgatcgtggtctattttactaaacttcatcaggaggtcgtaaagaggaccggtagatacgagtttccaatgcgaagcaagtttgatgtcttcactcggtatagtcgcccagtattctttttcattttcatcaaggtcttctggctcaggcagaccaccgattaaacaataggcatgtttagccacttctactaaacgggtgtttttcatagcttgatcctgatctttgtaataccgcaactatgttcgcagaactctaccttcgtccatcctgcttctttcaaccgcgctttaacaactttctttacagacaaagcaatgtcgtctttatgttcgacaacaatctcatagtttctgacataatggaagttattgaaaccaggtagatcttcaaggatctttttacggatgcttgcacagacttcattagcctggcgttctaccagcatcgcaataacttcactttttgtcggaatagaacaattgtcggtttccatccggagagttttgattgcatcttccagaagcgattttgaaataccaagggtcatcggacaagctctccatgagtgagatagattttaatacgggtcacaattgactcacctgtttcattagtagggctagcctcatcaatgatttcaattgaccaaccatgcttacccattgcttctcttagagagagttttaactcttttgtgagtatgtgggatacatgtatttcgaaccaggctgctccagacgaatcatattttacgttcgcgtaatttccaccataatcatccaattccatttcagaacggatatcccgaagaatttgagttgtcatgtagcgaacatatttgtcatagaactcttctttagaatctatgacaatggttctatctcgaagcataaaagataactcttttttatttagtgacgtgacatttgagtcattcaccgaagcggacttgcttgagaagttccaaggtagccaattccaacagctcatcttcttcaacctcgatgtctctcagtaagtacattccatcccattcaaaacaccggtctttaagagcggcattaatattacttgggatcatcaggtaaacatcatactcttcaccttcatcgtccaactggccgagattatgcatggtgatactacctgttttaggaacaggtgtcattcgatgaatacctggtttatttgttaccttgataaaagtttcaatgtcatgcgtaaatgacattgagttattaatagccttatcgagaacagtatcatcagtcagattaatcagactgaattgaccaccagggatataacgagtacaatttgaattgcaatacgtctgaacaagcggaacgacagcgagttcccagccggtctcattatctggatcaggcatccatgtaccgtggattattgcgatcttgttagccaattacaccacccctcaaaggttctggatctcggaatgtaatttttacagtgggaagtaattcaccagaacgttcttcccaacctatctcaagactggtgatacgttttgcgatatctgggtttgtagcgataaccgatttaccaccatttacaagtacttgaagacgatcagcggaacggctggacatgtgtaactacctcttgacaagaaaggggatattttttacattgctcaacttgacgttcagcgtgtttcttcgtgtagatacaggcaataatgacaaagacgactagtccaattatcattaaccagatagactgtttcctcttatacgtcatttgtaaagtccttatggattcagcaaatacgtaatatagatctgaaaaaaaatttagtacatacagccctctcccgaaggagagggcatatgcatttatttcttatcggctgggttaggtaccgtaaaaggtttaggatcgaaactcttactcatccgacatgcagaaaacaatctttcagccgcacgatcggtcgcagtcatcccattaaaaccatttggaccaaactgtttcctgtatcgcgtaatgtcaacatggaagttaacgatcttgtctttgatataccacagagccgtaaggtttgcagtgatttcgtactccatggatttcggcatgtctttcactttattccatagagtccaatacgcattctgaacagcaatcgaagcttgatcagaattagcgttcttctcctcaatctgattaccgacaacgatgctggtttgataaaccaacgcacatacatcatcgttcaacacgagatgattattcgcattgactgcaaaggacaagacgagaagaaatagagctactacatgtttcatgaaatatcctcagtttaaagggcgcgacctacaataggacgaaggtattcgaacttagtgccgattgcttttttgcaatcgaggtaagctgcaccgccaataaaatcagggtattggctgagattacctttcagattaagccagctaagccggtaggttttactgtagaggttaccgtgcaacgttggcgaatagaccgaaatgaaatggaatgttgcccaactggttgggtctttactctcgttattaagaagagcagtaactacttgctgagaaagatcccgtgcacccacagaactctgcatgttatcgatggcaagagcagtcgcgataatctcgactttttcacagagctcagtgtcaaccatccggatatcccgcatgaaacctttaggtaccggcgctgcattggccacgctcattaccgctatcattacaaaacctacaataagacgaacgaacatattcatttactccctgcgaatttgtaacccatgttagcttcacaactttcgattacggcctgaataatatctttatcaggaaaacgtttagttatgttgcgtttaatatctattacaagaacttgtgcatagatggcaccagtacgaatgtcatcgttatcagtgtcgcccatgcgcttattcaaataggacattgcttggaactggtcaccgccattccgaaagatcttgataacatcgcgggacatagatacagcgatcttacaggatttttcggttatctgttgatcacgttcagcgaacgatggttggcaaccagtaaacatcatgatcagaaaagcgattatatagcgtttcatctccttaacctcttttgagtatatgtcaagtttgttatgtagtgattcaaatgttttaaatgtaatatccatccaacataaagtcctccccgaagggaggactatgtttagatagcatacgactctacaattggaccgaccagatagccaatccatatagcgaatacgcatggcatcaaaaagttatgtccaattacccaacgtttataccacacgggtgaccatttgaaaatatctttccaaataccacgtgcttccagttgtatataaaggtagaaccagatggatgtacctatgaacataactatcgctacactctcatgataagcagaaatataggcggttactataccaactataaaagcaaggtagtatgacattaagcctccagtttagcaaatgcctcgtctaagaaaatcttgaatacatctcttactaccggatgagctttagtcattcgattatagaggtccaatttctctttgaggaagacgggcgcaaacttaggagcatcatcaacgatgacatacacgttggtgagagattcaataagtttgcacgtctgtgtaacgtcacaacattcttctaattgccgatgatacgcatcgattcgaactttccgaggagcatcaaaattcggctgcgttaaaccttgtacaagtttggtgatatacggcgtgaaatgagttagaacgtcatcgagagtccagctactatcttcgacgatgtcatgtaaccacaaggcagcctgttcgccaggaccaagtccaaacattttaccgatggatgctgcattgtgcaaatgtgtccataccggtagcccagaacctttacgtcgttcaccagaaccgatcgtataacctacaccaatagctgctgctaactctactgtgtgatgccctttccatagcggaagcacgttcgccgggatgcgagtatccaagatagctttaacttgctgatatgcttctgctacaatatccatcatttactccacgttaagcgttagtactattgaggaaaaaggatcttctcgttaggatcaacaaagaatccacaattaacgagaattacgtccatccaagttttagtttggagaatacccgtttcatatgcatcttcaagatcgattagatcaagcggatcgaatgaaccataatagatcggaccatcttcaatctgcaattgatagaatcgaagtttggacatatcctcttcgtctagggtatcatcgaggtcttcgtcgtcatcatcctcatcgtccacaccgctcattaaatcaagcacgtgttcacgataaaggaattgttgaccactttcaactgtgaaccaatgtttcttatctttaattggaatccggcgcttaaattgaggctcggcaaagaatgccctatattcctcttcaagctcgtccgctctaccgcatgccatggtagaagaacggatggctgtaagtacaaccgcctccaaaataggatgtagttctatcatggacacctcctagtaatgagttcatgatcatctacatgatgtagatctgagataatctttaacggtaaagaaaaagatagagtaccctctccttcgggagagggctttatgcaccttaagcttttaatgcaccgcagttctgggctacgtagcgaagcacttcatgaagaagacttctcatccaaccctcggagcgacttccttgacgatatttcttaaagatcgtcaaatggttcatacagtctatgtcgaattcatattcgatccaagatgtctctttgtcacgagttgccgtgatatggacgatgaaacgttctggtgcttcagatttccaatcaatcctcacatcaaccgagtggttatctggaccagtgatgttgttgaggatatatggaagcttctctggtgtaactttatcgagaatgaacctgaacaatgccattgagattgcatcgtgttcaaggatataaagttcattacgacgaaggcgatggaattcttgatccattactttttccttatcgagttacatactcggcccatttcacaagaacctgcgcacagtcacggtatagctcagcagattcgatacaaccgcgactagcgtagtcattaattattacgccaccgtcatgaacggtcacatcgaagtgaaggataccaggaccggtacctacggcgattgtccaggtttttacttccggatcaaaactggtatcaccgattatcacctgtgtcccatcgcagaaatgtacatgctctttatccaagcaacttggatgcgacatgaccgtatcggtgacaaccatgactattgttttcttccacagctcttgataacgcttatcggtatccataaattaaatccttgcaatgagggttagaagaaacagttagactttagttttaaccgtgataggtttaccgtattgatcgaagttagaggaacagtatgcaactgcctctgtaaacaaactgttcacttcttccatatccgaaatgatgtcatcagaaactgtacctccaactagttggaagtcaatgccaccagggacgccatagctatattcctgtacgacgttccacagacgatcagatacctttacctcagcaacgacatagctcaggcgacgatcaacggagcgatgatggaaggtaacagtagcgtcaccaacctcaacagtggggagggcattagcagcttcacgacggaaagcgttattatagtaaacgaatacagcttctgcaatgcgttgcagaatggtgatatgtacgctggtttggatttcggtgttcatggaacattcctctatggactatcgatgatcttctttacgtatttgaatgatatctttacgaatatcaaattggtaatgtaggtttttaatgtatttaaatgcaaaaaaaagaaaagaacaaaggggagccgaagctccccgtgattcagatggagcgacgcagaatcggatcgagactctgggtagattccaggaacaccgaacgcagatcgataccccaacgactaatggcttcagccgcagcaggccaatgctctgtaccaagaggacactcgatggcgaaacgaggaccatcgatatcacgtagagtgaacttgttagcatcaaccagtttcaggtgttctaccagaatgtggtaaatggcgctacacagaattgatttaccacgatgagtaccaccaagaacagcaatgcggagttctttactccaaagtgggttaattgcattattcaccggtggagacactttggttccacatggatgaatagcatgttcactgacagtgagatgatacttgtcttctttgaacttacccaagattacagcgggatcgagattatcatagtcttcacgaccggtgtgcattacttcgtggttaagaccaagagatgtcaacccattagaaagcacattgcgaatagccaggctggtagcagggtcatcggtcataacgaggatttgattacggatactgttagattgcattttattttccttcaagttctttttcgatggcgatgtagatttctttgatttctgagaagggaggataaacaatttctgcccttctattccaaacccatctgtaataagattcgatatggaatagatctgttcggtaaacatactcatctacaccgactccattccaattaggagagtcgatccaaatacgacaaatatcgaacagccaatcgagttcggtttgaatttctttttgaatagcttctttatcttcttcaaccattactctgtaaagttgaacgagataatgactattgttccagatgagaggagctctggttacgtttttataaaaatagcgtacctttctgacaaactcttttttgaattgctcgaattcagtacgtggaagttttatcgcctgattcaaataaatgaagcggagatacacttcgtatagatctatgttgattttattttttgctgacatcggaataccctaatcgatataaagcccagctaacgccgggcttatatgacgttaagagaagatgtagtcttcccaagaatcagaaaccttcataatcgtctctcatagagctttcctaatgcgaatagaaagagtactaccatcgtcacctttgaacttaaacagagctgtaccaggttgaagaatcgaaggtacaacggtgactgtccatgtacgcgctttcttacgactgcgtacataatcattgatagcttcactcaactgttcagtccagtgatacttttcgaaatgtgcaattacctggagaatatactccttatctccaacaaaagtagctcgatcttttagatagttggggaaaccaacagtggcgatagcatgcagtcgttgacaagcagaaaggagcagactcataatgacctcgttaagtaagcgctaatgatttcgataccaatccaacatccagagagaaaggcgatgcagaaccatgtccacggcgatataccgtcaaacagattgaatcgttctctgggtacaaacttgacaccagatttcttctcattccaatctatgtctatcgtcgaatagactggatcgacactcactggaattggttctttcaatggaggtgggacaggaactaacgattcgatgtcgcgataaatatcacggacgtccgtagcattcattcgcggcttcgatggtttccttgtagtagtcggggtttcccatgatcgccttatatggttccttgacgtacgcggcgtagtattcttcctcataagctatcctcgtattaatatcgccattaagaagacgataaggttgcgcaccgatcttctctgcaaaggctctaacccgagcgacagttattgggtaagcatctagacgctttttatcaagagtatacaggacactgatatcgtaattgaagaagctgttatttagactaaccccttgttcaattgctttatcataagctgtctcaagatagtccagcttattgtttacaacacgcatccattgatcaatacggaaatcagattctgcaatgagccgaggggttctttcgatgctccccttcgactcaaatgtgatagaatgactttccaaccatttctttgcatcgggaagacgatctgaaataacttgtggaccgagagcagaggtcgtacaaaattcagaaatgaattcgtcaagcagacctttttgtgtcagttgttcaagaattttcatttaaaccgttccaggaaagtccaacgttcatacgcgctatacacacgaagaccaggattagtaaccagttccagttgtccaccttctacataggggcgcatcgcaatttcgaaattctcttcgccaccacagttaagatctacgtcagattcgaacttaaagtcttctttaacaatggcaatgaccatgttatttttaagatcgctaccactataaacagggcgagggaaaagaacaatcatttcaccggctttatagtcaatcttaccagcagtcatggtttcaaacagaacttcagttcgatccttcagatcttccagcgtagtcggcagatttttaccacgaaggaatttcaatccgagatcatgacggtagacagtaactacgtcaggattaaaatcgagttcttctggagtggcatcttcatagcagagacgtttaaagtcttcagtaagaccacacttacggacgatgtcaaaaacgtcagtcggttgtaggggagtctctttacgaggttccagcggagatacagtcaaatcgatttcttgagacattttcgtttcctgtttatagttaataacacattatcagttaactcggtattttctaattccgagaaaaaagttcacgccagcttcgtttccatttgtagttaggtgagtatatactacagaaaccttcatctgccatgaagattggattaactcgttcaacgatttttacaattgcgtgagggctatcagaattagctagaatacattctctagcctctttcgtgtaagtaccccaatcatcaatgtaaccttccttcagctgatcaactcgaccaatccaacaccgaggtataaacagacaacggaaccaacccacgaatagaatatggatcaaccacattgacagaaggagagaacagaaatataacgctgtaaagaacgtgtgtccatcagatgcattagctgtggtgagttcttgccaaccacgtttaatccaactaatgggattccaccaaacaatttctgttttaggttgactagcgtaacggtaaaatattgacatgtttatccctctacgtcaagaatagtttcccaggttttatccgtctgaagctggatctttatttgattgacatacatctgatccgagtattggcggaatatcgtcatccggattttctgccatagtggcatataacgacgatagctgatggtgaagcgctgatttgggtcatacgcttcaatagctttcctgattgtctcagcaaagaaagcaaacgaatatacattgttgttatacagcaatgcagttatggttttcttagagccgacgaggtttaccttcatggaagatgtccattacgtcaatggtagtactatactcgacacgagcatatccaggttcttcaaagataacaatattgaatccatcgtcacgccagataaacttaaagtagttgcgaacaacactgatgagatcttcttggaactctggaagattatgttcggcccggataagtcgacaaagtttccaaatggcgttatcgaacttatagtagacgcgtcgcccttcttcacccatttcttcagataggataccaactgtctgaagaataggagagagaaccttatcggtcttccagttcaatatcaggtatagttcttcactatccaaattacgagtcaggaattttagagcttgtgacatatattcaccttcttgacaaaaataaaaaagggagctagagctccctttatgtcgttatacagcgtcttctttagcagctgctttctcttcttcttttgctttcttgagaagatatgcgttactgatagccttccaagatagtacacgttggttggacttaaataccagaccttcccggtatccacgcttgttcttaaatgcagatggaccttcagccatagcgagaacatctttaacagacatttccttagaaggtttccagcacgggtcaagcacgggaacataattcagaccaaggtcttttacaacagctcgtgcttcggccggcaggagttcacgattaccatcctcatacacgttgaagatgtaataatcgtaatcagccacttcttcaaagttatcttgaatagatggtccaatcagttccccttgtacagaaatgaagcgaccggtgttcttgtggaacttgagaagacgttcgatgatctgttgttggttagttacacgtacgaagttattgtcttcgatagcggtacctttcgtccaaaggggcagaataataccattacgaagtttaccttctggagtaacccaggtcttcttacggaacagattacggttacggataaggaagttaccaacccaataccgaagctgctggatgaatccccacttctcaccgcccattccgagttcgtagttccgcgaacaaacgccagtacgaatacctttgtcatcgacacagaatacggtcatggagctaccatccagcttataggtaacttccatgtcatcaccgtcttctttcaggttataaaacgcaacggtcttattctgaatgcggtcttgatcggacttagttagcatctcaggccacggtttcagagcgccacccagattaccaatcagcttggcaccaagtttaacgatccacggagcgttacgtgccgcatgagccttcgataccatcggaggagcagactcgtacttaaggatacccagcttcagggtcaggttagtatcaacgggttcatctttgaactcatcgggaatcggaaccagtagtccttgagagagctctttacgaagcttgatagttttcaaacgatgatagtttttaccgtctacacgtcgattgtcggaccgacggctctcaagaaaaccgaagagcttaacgttatccagaggaagaagagaatcaatctcgcagtaaatagcgcgatcacctttcttatattcgcccatctttacacaaagttgccaaccaccaacaatagccaattccagagcatcggcattagggtgtttcacaacatcatcgatctcaacaatgcgtgcaagcttacgagtttcttctactacaccaaaaccttcgcggatcggtttcaattcatccatttcaatcgtcattttatttacctttatcagtgatggttgtgcgaacgtcattacggaaccgccgcactatttcgagtatttctttttgatctacataacgaatgtctgtcagttcaatttcacgacaagccaatgaaatttcagcttcaatctgatctgacaacgttcgacgtaaaccatctatcgttactttacccggtggcggcggcgctgcgatcatgtattcacaccccagttataatcatagaaggtttcaacgaaagacttaccaggtagttcttgtacgacctgctctgtgctatttaccaaggttacagcttgctcaaatgggacaggatgcccacttaccggcgagatgatcttgtaaccattctcgcgtaggtgatcaacgaagttcaccataccagtttcaagaccgacattataaatatcgttctcctggttggtagtgatttcataggtctttccagcagggatatcgacaatgggagtacggtcgtcactggtacgtgctacgtcgcccattgtacgacttacagcccagcagaactcattgagaactgggttcgattcttgccattctttcttttcatctaaacggtctttattcgacattgcagttacctcgttgtggatacaagagagtaatatagatttgaaatcttttttatgacataaaggggagccgaagctccccatgtctattacagagaggtcgcaatccgttcccggatcttagccatcgtgtcgtgcttgtagaactcaccattcttgaagaacagtttaagttcacccgattcggtttccaaagcagcccagctaaggtcagcttcttgttccagaacgaacttaccatcttcggttttcaccacacgcaggaaacctttagccgacttcttggaagaagcagctttaggatctttgtacagttcaacgaactcgtcttcgatctgaacagcagtagctttgacagccatgccgaaagtatcgcgagtgttgtactgataggtgaagctaccgataccaagaactacgttgctagaagcgaagcctttacgttccaggcgagacatgatctgctcggtacggtctacagtgatcgagtcaccatagatcaggccaacgtattcgttcaggcacttgaagcctttactgttctcagtgccgccgaaggagtcccacaggacttcaattgcaccacgtacttccacctcagggatttcagtctcagagaggaagtcagacagactgacagcgaggtcgttgatctcgtagtacttaccacctacgctaacaacttcgtaaccagcgtactcaatggaaccgtattcggcaatgtgtttctcgaaatcaacacgatcagcgaatttaatcggataagccatgtagccagtgatgactttaaccggatcaccagagtcaggacgtacaacaactttcgccagacccagctcgttcttcagacgactttcgatttctgcacggatgctcgggagaacatcagagataacaccccagaaatcgaaggaatcacagaccagcgaaataatgccttccgggactttctgaagaatgatctccaggatatagtcacgttcagcttccagtcgcagttggtcatgcagctccggagtgatcacagtaccttcctcttggaggaagttgatcttcatttgcagacggtacaggatgttggttgtggcgacagcgtgttcagttgcagtaactgatgcacccaacaattcagtatcactgttagcaccgtaatacatctcagcgtaatcgagagccgggatggtatcggtaccagcgaagctagtcaggtgagctgtaccagaacgcattgcatcttcaggaccactcataccacggaagctgaagtcgtgtgcctggaacttgacgtgctcacggttatcgcaggtgcgatcagcgtagtggttcagtacacgctgatactcagctgcaatagttgcgttgcagatcatcttccagttgtaggcactgacgatggtttccaggtagttcaccagccagtagtgatcatcgtcacccaggctgttgtaaaccacaaaggtaggtacgccaacatctacacgttcgccttcgtcaatagccagcacagtcagaggcaggtaacccagagcatgcagcttgtacagacactcgtgtttgataacgcctttaccgcacatgttgtcgaaacgacgtgcagcgcgtttaacagcgatttcacgaggcagattgaagaaggtacgatcccacagttctaccagttcgtgccaggtaccttgcagaccgaagttaacgactttgttgtcgtagaacgcagagcaagacttcgaccgcaggaactgcttagcagaacgtggggtgaagtttgcatacttacgttcggtaccttgcgggtacagagcgccatggccgggcttgtagcagtcagttgcggttactgcatagagagcattagacatatttttgatcctcggattagaaaacagaatgagagaagaatttcgggtcacgtacaccatcatgccgataatcatttacagcgttaggatgataggtgttagtggtctggatataatcgtagtattcgttcagttcatcgaaacccttggagaaaataccatgggttacaaacagacccaattgatctacgatgcactgctcgtggataaccttagcaagttcaatgaacgtgcggccaccatcacagatgtcatcgataaccaacagctttgtcaatcgaggaacgtcatgggcattcaacaaagacgtatgagtgatcttaccagttgacagttcacggttcttacaagcgtacagtacgccagcagcaccgatctctttcgcaatggcttcggtctttttacgtgcaccttcatcaggggcaaccaaccaccagtcactcggattttccagaagttgtccttcgacacacacccagcttttgatgatatctgcttgggtaatctcgcggcaattgttgatgagtggcagcgacacattactgtgcggatcgtacaggtatacagacgtagcgtccaatgcattgatcaaaccagtcatcacactaatcgacagaggttcaccttcatcgcaaacacgatcttgtcgtgcgtacggcagataaccaataaccaagtgtatttcaggacgaatacgctggcgacgaatagcgtcgaataccaggaacagttccatgatatcgtcactattacgaagccaagcattgattatgaatcgttcgcctttctttctgagatctttcagagggatcttgataccgatctcaccgccagggaatttaaagggttgacaatcgtagtgatctgccaagccgttaccgtgaagctgagtaattcgaatcatttatttttcctttagggaagaagttggggaccgaagtccccgttcgggttagcccttgacgcaaacaatctgacgcagggtgtggacgatctcaatgaggtcatcctgagcagccattacgtcttcaatgttcttataagcctttggagtctcgtcgatcacgtcaatgtctttccggcattctacaccggcagtatcacgagcgtggtcagcaagagtgaaagtcttagcggcttgggttcgggacatgacacgtcctgctccgtgcgaacacgaacagaaggactcgcggttccctttacctttcacgatgaagctcttcgcgcccatcgatccaggaataacgcccagcataccctcatctgcacgcactgcgcctttacgagttacggatactttcgcaccgaagtggttctcgaaggagacgtagttatggtgacattgcacagctgataagctggtattgattggtcgacccatgtaatctgcaactgcctcgatagtggcgcgcatcatgatcgtacggttgagcgtggcataacgctgagcccaatgtacagcttcgatgtagtcgctgtagtacttggtaccttccggtagataagcgaggtcctgatcaggcaggttgatgtggtagagccgcatctcctcttttgctttctcaatgaagtaccgaccgattgcgttaccgatcccacgcgaacccgaatggagcatgatccaaactcgatcttgttcatccagacagatctctacgaagtggttaccagtgccgagggtaccagcatggttgaatgcacggttagcagccttacccagtttcgggtgtttagccacgatgagcttcagttcctcttcaagcttcttaacctgagcttggagctccggttcgagtttcttgtaaacgaggttgaagtcactccatgcaccacggtcattcgggccaccattgtcagtacgaccatgggggatacgggattcgattttataacgaagatgttgcagaccatgagtcatgtcgttagctgtcagatcagtaagctggcatgcaatcccgcacccaatatcgacccctaccgcagacggaatgattgcaccccgcgtagcgattacggaaccgatggttgcaccggtaccaaggtggacatcaggcattacagccaaatgcttgtaaatgaacgggagtcccgcgatgttcttcagctgacgttttgcatcagcttcaacagggacgcctttaacccaagctttaattgggaattcattttgttcgttcagcataacgtatttttgagtagtcattgtagacgctccgagagttttaaggtttaggaattcaacgatttaacgttgtgccaaggtcgggatcgcagaattccaaggataggtagagtaatgtcatgcctatccgtattagataagacttttgagtaaattgtcatcagtccgattcaacggccatggataactctttatgtttccttcgtctttcaatattagcaaaccatggtcttacacttaaccatattgcaggccaactgagaatagccgctacagccatccacactgcactgagtagcacccatgcgtcgttaccatcgtcaacatctcgtggagctatgtcgagttgatagtcagttccaacggggacatggtgataagtgtaatcacctagcttagtttcgtatacgaaggggacacctttcatcttcccttcccaacgacccattagctctgtgtagatcccatgtttgtatttgtgggtctcttcccatttccaggtcaatacaacctgggtcttacgtttggttacgtagtcagagaagaatgagttgtagactgcaccacccataaatgctaagcagattaggtagagcaccacacaacgcagtttaacccacttggagattggtacatacggctcttgtttcatagtcatcgtacagccgattgcgtttgcataacccaagggattccttgatgccattgcatttattgcggctgcctccagagttatactcatttaggattctcatggataagctggaatgtgtcgaacttgtattgatcaacgaagtgccacgcgagttcactcagcttaaagatatccggacgttcgtatttaccgaagtcgggtttctctttagccaaatggaaatcgatgaaacggtccaatacagggcaacgatcgatcaagtcttgttcagtggaacctaccttacagttgaccagttcctgaatacgtttgtacaaggtgggatcagacagaatcggtaggagttcatggaataccatcggtggatgttcacgactagtctcaacccacaatgctgctaacagtggacggagagcatagaagtatttcttcatgcggactttctcatccgacagccaacgcatcttggtttgcttggccatggagatatagtgcatgaagctcgattcgggaatgaagtgcttgatagcgtaatcacgaatcagtttgtaatcccattcgttcttacggtaaacgatcggggagttcaaccactccaacagagtcgggttagacttgtaagccagttgaagtgtcttggtgatactccaaccagccagatcgagttccttggaaaccatctcttcgatggtgtcacgaccttcgttatcaacccggacataatgactcggatggttaacgtagatgaagcgaacatcgtagtcactattagtagaagcgaaaccccaaccacgactaccggactcacaggcgtaaatgatctttacaccatacttctgttcgatacgagttaactcggtgtctataactgcacgcatctcatcactaacagggtgacgtggatccatcattcacctaccttttcaagtttgagtttctcttctttacccgtgtccaaatacatgaacatcgaatttcccagtaggttgtaatacatccaaccttccttaaccacttgatcgccatacgtcagaggaatgttcaattcgtaaatggcgtcataagggatgactacaggatctttgtcaggcttgttgaggacgagtgcatcgtcagtaagctcaagccattgcttacgactgatgaccccaagaccgatactgaattcgctacctgggtctttcccattgaagataccacagcgaacagcaggatcaactcgatcaccagcaataccgatcttaagagggtcagggtctacgcccatcaattcaacaaccagttccagttgacgcttgagttcaatcttgttcacagtgtaaattccttcgtgttgtattgacgtgcagagtcggtccaccatgtaggtgtctgtgcgtagtagtattcaccaaagatacaagtggctaaggttttatccaaagcttcctgataagacatctcgccatctttagtagcgaagtgaaccatgttgttgaagcaggtaatgatgtcagcgttttcttttgtggagaaaacaacggtacctttggctcccacttcggaatggatcatcgagctccacggacgaacaccacgatcagtgaccagatagatatcttgtacagccgatatggagaagaacgtacgaagaaggttaccgtaatcgggtaggtcttgctcgaacagaatatcgaggatcttacagaccttatcgatcttcttcattttctcggtgtaacgcgcaccaccatcattctcagtgcaaccgatattgaagatgatactgtaaatggattccacaagcttacagcatttgtagacgtacggagttccctttactttaggagtccatacgaaaagattgctctttcctggattaggttgcttgaactgatggatgcggtacggaatacctttttcaaacagcatgaagtccattattttctccaaaggaaataaagcctccacgaagggaggcgtttatgttaaacagcaactttaccagcaatgtgcggatggaactgataatccagaatctcgtaatcttcccgagtgatatcaaggaaaggtttacctttggcctcaggcttgaagcggatggtaggagtaggataagtattccgcgaacgttgcagagtaacctgttcctcatggttactgtagatgtgacagtcaccaccagtccagatgaactcttctgctaccatgttaaactggttcgccaactgatgagtcatcagcgaatagaacatgatgttaaagggcacgcccaaaaattcgtccgccgatctttgatagagttgacaactgatagctcgtttcggagcaccatgttgatccaaccattctaccactgcttcatcggtagccttttcataaccacgacagatacgcagaagtgctttaacctgctcagcaccaccgaatggaggttgaccacgagtagtctcaccactaatctgatcatggtaagcatcagcttcgaaatgcgtttggtctagagcttgcactcgttcatctacggtaagttcacgggtccagaactgaataaatgcatggcatggcgggagtgcctgatcttcgaccaaacgtggatcccaggcacagataatcagtcgacgactatctggattgttttccagttggtaaagcagttcttgaacctgatccacacgccggcgaataacacactcatctttcgtgtaatcaacaccaggtacgtcaactacgaacttaaagccgcgtttctcgtaattagcccagtctactttaggaacgatacgaacatcgtcgatatcacgccaggttttaccatagaccggaccaagatcaccaccaaccaaacggaaggcagccaacagaccatcgttgtctttaatcacgatcttcgcatcgccaatgacaatacgatatacgcgtagagccatgccatagtagtcgaatgcatcgggaccaggaccgaaacgacttacatcagcccaggctttcaggttgatcaacagtagtgccgatttgtcctgttcaggatcaatccacctccaatcgacatcaccgatctcattgctgaaatgcatctcaaacggaatgttcttgaacttcttctgaacagctgtagtcagccaatcatcagaaaccttttcgaatacttcagtacccggcttaacccactcgttccagatggtgacgttcttgctcaggagatactcaaggcgagtgtcaccagacttcatccagttgagttcttcttcaaccgacggaagatgaatcttcttggtggtcactacagggaggttaccgttacgaagatcatagcggaactgtctaccgaacaaagaggtagtacccgtaccagtacggtcacctttaaatacaccgtacttctgggtatcttcaagtagttgtagatactgatgcattaaacacctccatcgttagaagctacggtcaacttgctaggaagacctagagttttatgggtagtttcttcaatagctttcagaagagcttccatattaccagtaggatgacccagatgaggatcattttgataactgatttcgaaggtcatggggacatccacgacatgactgaaatcgacatcaccaacattcaccggataacccagactgatacctttaataaccttacggtcatgaccgatagcaatgaagtccatggtagcacggttatggacgactgcccaagcaccagtggattgcagtaggttacgacttacgatttcagagattgtcatcttcaactacctttaggaactttgcagttacttggagaatgataccagattcggcacgggcgtcatcaccatcagattcataatggatactaccgccatcaacccacacgcgagcaccgttcggaacaagttcatcagttgccatgtattgaacttcggtgtaatcgcctgaactattgctagtgcgagagatacccatcaggtgatcgcaactgggtacgatgatacccatgttacctgggttaatgtaagcagtgacttcagtcaacccgatgaagtagtgaccacgagacggcggtacagtcagtttataattgttgaacggagtcaacaaaaatttgacttcattagtagttggaagaggtaaagcgtttacggttggattgttcatttttcacctttgaatttcaccgagtgaggaccgaatatgaattcataattctcagtgtgtttacgttcggtaagaagacgaatactgttattgaattcatcatatttgacaacagctacgactaggttattacgtttatcgtaatactgataagtgttatcatcagtgttgatttcacccagttcgaaaacttcatcattttgcttaatggcaatcagtttacggggagttggaatagtaccgaagtcgactttgtatttaaccagcgaatcttcagtggtgctttcagcaacgtaactaatcatttcttttcctcagggtcgtaggatttcgggataccagctacttcgtagaaatgatcccaatatggactttcgtcacggcggtgcatattgaaattctgataatccgtacagatgactttaaacccatctgcaactgattccacgaccggcatattaccagtgtgactgttgtcgataacgaagtggatgttattattgtgtttgtacttcagatcgaattctcgtttgcgttcaacaggggtatagctaattaaggatgccatgtttattcctcaagacgaagtttccagaacctgccctcttctttccaggtttcacgaatagcgttgtcagtacgttgaccgtccttaaacagcttctctacattggacgggtaagtatagttgtacaacgcaattgcaaattgggttacagctactcgggctggaataacaccagtgccggttcccatcaggcaaccgaggacacggaaagaatctttcttttgtttaccgtaccattcacatccagcaatgccatcgagggctgccttagaggctagatacggaacatccgaacctttgggtagcctgcgaggaacacgcatcgtaggggtgtacaggagtgttgcagtgataccattaagtttggtgaattgaacgcaagcacaggaacctacgtttaactcaccgttgtggaaacgattgatatcgtgaaccacatttttctgcatgttaacaaaacgggcagctagggcaccatcatatccaccggtcatatgcccgtatgagttacccgcggtcatgtagtagtcaaactcgtccgcgtggtctccgagtgcatcaagcgtaccatgaaacactttaaggtcatgtccaagttgcttgacaaaatcagagatagctacgagttcttgaaactcttcataactgggggtgcaaaatacgaactccagtggtttgcgtccgatatctacagtaccaagagaaagaccatcagcgatctctttatggatacgggacattacgaatggagatgtcatttctatacctcacgacaaaaagaaaatagatggagctcccgaaggagccccggtgcgctgacctttacgatcaactacataatattacattgaaacgcatgacatttcgcgacgaatgtttttattatcgaattcgtattccagaaccacaccggcctgagtacgaacgactttaactttagttccattcgctgctgttgtatcttgaatagcacctacagctttccaacaggagtcaatgctttccatcttagtggtggtttcagaagaaccaccagcataaataccagagacaatagtagtgctaatgagaatagctcctgcaagagacattactttttacctcctttaattacggtaagcttcggcttgcctttataacgggatggagcaacattaactggtgcaccgggaagatcgccaaaatcgagaagaggtttatcaacaaccttcagttcgggggatttcttgatcggactaacctccacaccaggttgattagcaatgaaatcttcagcttcttccagttcttttagtttccgagtatttgcacgttcggaaacataggacaagaactgagagaacaaatcgtcatcgttgctaaccatgtgctgtacatgttcaagcgctttctctacgggaacatcggtgattcccttctctgccagccatgccattacatctacgatatcaatgctgacggtaccaggcgcaccattggcaatatcgcggaagggatgaacatacgtcggattctcggcatcaaacaaaatccgatcgacattagggaacggagagaacacacttgcattctcagagatctgcacattcacaccaatgaaagaatgccatggcagatgcaaacgagtaggcatacccgagaaagcaatttcaccatagaagcaatcacccgaataatcaatgtggcggcacgcatttaccgacagattgagaacgatggtaccattagtggcattgaaatctttcgaacgcatcatgattttacgaagcggttctgccagataacctacatcgataacacagtcgaagcgatacatgttgttatcggcattccagttgtagtatgcttcaaccagtttttgattcagtgcggaagtgagtttgatcattttgagtctccagattaaaggaatcgttcagtgatagaagtgatcagtttcttttctttattgagagaagacatgtgatcacggtatttcttgaagtaacctacatcttcaggaccatttgccattttgggattggccgtgagtatgtgatggatctgggtacccgtatagacactaatgttccatgtcttggattccgagattattttctttacagctgcattagactcatcgctatcttcaatgagataagcatcgatggattgactaaccgatcggctgaattcatcgagagcactaagatcacctttgggaaggttagcatgtacttctttgagttcttttaaagtacgcggtgctacacccggaacccaacgattggtaataacatcaccatcaagttcatgacgtggttgcagctcattgggtttctggaatggatacatgattacctcaacggaacatgttctttatgaaattccatggcttaagataccatggagttgtcgatgcatagactacaccaggttcgttcgaaagtaagtttagattgccattgccatcacagatataaattttcccttcaccaataacaacatcgtcttttactggagtttctccattaggacgaatagtaacacctcgtgaagaacttttgtagtaatcgttgatagcttccgcttcaagctgtacgaagacattgttcatgatcacacatatttctttgtccagttcttccagtcgatgatcgaatgaatcctcgtcaccaccactgacaacgaagacatctggaatgacaaatagatctttgaataaaataccatcaatatgcaacctgggtctacctattacatcgccaaagaacaaaattgctcggtggcgacacagttgtaaatgtttgcgatgctgttttctcaattccttatagaacttccaattagtgaaagattccgcagatataaaagacattgattttcctcgttgggtgtgtagggggatcaaacacatgatgtagatctgagatattttttagcgtaagtaaataaaaaaacgacatatagccctccccgaagggagggccaaatgtaccattacctaatcacgaccattttgccgtaatcttcagacatgcatgaatcaaacgatgccatgtatgcgtctcgcggactatccttagcgtcgtatataccacggacgtcttgaatagctttgggcaggattttgtaaagaacgttatctttgtccttcacaccgtatccctttagggcaaggaggttctgtttccattttgcaatgggttcagaacggccgcgggcttctgctgtagcatgagcagctagtgctagtgcttcacaataaacctcatcgacacgcacctctgtagcttcagcttgcagtggaaccattaagattccagctacaaccattagccgcattacgtgtgtaaaacattgcatcacgttggtacctttggttgttaggtcagaatataatacactacagcgtatcttattctttctttggggtagcctcattaacgtcgatgaagacaatggaatacatcttagttccattgggtgtcccatctgtaataagttcaataaatgtattctcgtctccaaatatgacattagagttgttactctcgaaatattctttaacgttctcaaccattgaatttatagcatgttcagtcagaagacccctaccatttattccatagagctgacttgttgtttcgtaaacaatggatctagggtcatcataaccagaaacatcggcggataccataaaacgaattagttctggatccgactttgcagttgatggaatccactcgcagttattattgaaccactcaataaactgcgtatatagacttgaccctttctcgatggagagtgaattagattctgtatgctgttgtatgaatgtcacgagtttgtgatactgaataacagcagtgcagaacgacaggccgtgcgagaattgatgaatgtttacggacatatgctctcctaggacttgcgattaactttacgttgcaaactagccaatgctgtctgctggcgttcgatgatccgtcttgattcacttagcatttttactatagattcaaactggatcgccatatcgtctaaacgctgctctagtagagctatacgttcactcttatcacccattaaagtttacctttatagtgaatgtcgccatgatgggtattgttccgatacagcagagctggatcaggttctcgatttgcgataattaaattaaattccatcgtgaaacggtttttcatatatcgctcagaaacttcaacaacataagtatctgcaatggtgtcgatttttacagtagctacaagtttaggcgtactattacgaagcttatcccaaacctcgaacgtaagattgttttcgtatcgagcagttgtaggtattgtcttgaattcgaaaacgtttaatccatctggagtgaagacagctactggtactagccaaaacacttcagttaattttaaattaccatcacgtgaatagaagaactgcttcaagtccccttttaccccgtggtacattggtataataacacgttgtgccgacattataattgctccgatcccgaccaattacgtttagatgtatcctgtactatcttaagacgtagcttaaaattaggcatgttccaacgcgtaataggtttcttccaatatatacgtttcttatcgagttcaacatgcagctcgactaagacacggtttctttgtttttcgaagatggtgaaacagacatgtcttggtttttctaaccaagtttctttataaaactttagtgtgtctgcatctttttgtgtatcaccgttgataatactttcaatatctacgtctgtgaattccaatgcttcaataccattcttacgaagtgatttaaagcgctcagaataggttccacggaaatagtattcaagatcaacaaacacggagtttaatcgagtactcatatatcctcagattgtaataatctacaggattggttaggaaaataaaaaaaggcataaagcctccccttagggaagcgatatgccagatggtgttttgatatgaataaaacgttttcttaacccggcaatgaagaatggatcgccagcaaaacgacctgttgctgagttgtatctaaaccaataccgtttgaactttaggaagcgacggcagttcggtttagcctgaattgtaactaaccattcatcatcgaacaagtcatccaactcgactgtaatggaataggtattgtcaaccctacctttacggtctagtatcgatatacagtctgttagatcaccatatttaaaaataacatgctcgaagttattgtctaaactaagcggtatagttagttccattatcaacctccaaatcgaatgttacggaaataaaccgtgttcgataacttggacttacaaaggtttcaaaatggtttgaaccatactgaagttcgatataagcaacgacaataccttgttgatcacgcggaacaataaagatagtgtcaaccaaaccatctatattttttgaccgactgatagaccaattaaactcgtctgtaactttattatcggagaggatctctactcgtgttattgcctgttgtagagtgagatccaattcttctgtaaacagggagttcaacttccctctgtaaaccgtaaataaatcgatgtgtgtttgcatagctgagtcctcgatagttcattatagtacccagctcaagctgggattatttttgtatgggggtgtctttaaaaaccatggaaccaattagagtaagtgctgaggcgcgccctggattacctgattcgacaataagaatgtctctcacagtgtgtcacccatcgctacaccgacgtaatgattcattaacggcgccttaaagtacatgttgttggcactcttcattttgtttttgaattggtcaatgattacacgttcatcttcgccatttgcttcgaccagatacatcctgagatcatagatccatttaaggatgtcattttggtcttgttcctttttatgacgtttcttcccaattcgtttctttaggaagatactgcttcgacgtggctttagtttacgagagaaaggaatagttttgattaccccgttctcatcaatgaccttcatcccttctgcaatgacatccatgtaatagtcattgtgcagagctatctgttgatgcatattgtccatagcttctttatgatcgtacattcctatttcctttaaatagcatagacaacatattaccccatcctatccggaaggagtaatatgccatttcggtttgagggtgttgcttacaaatttgcttcccagggtgacggttctggtctacccttatcgagttcatgcaattgtttcctaactgcaaaacgtactcgactataccataggtacacattttccggcataaaagacgagagttctttagctaagagtattgcatatctttgagctgcggcattttcttgcgtataggctaacgagaaaatcttcgccaatacatcggtattacgatgccattcgcggagctctcttgcaataatgtcgcagttacgattatctccaattgactcgattaggaaacatgtgaattcatcacctagtccaatactaacattagtcaagaagtcaatcagagcaatagactctttcattttattagggttgaacaacttccgcttaggatcaagtctttgtagtctaaaccacatcgcttgtgtaccttcacgatgtagtgaatgcacttgacggaaaccccgccacatcttaaataatccaatcatcaggacctcacggaatatagcctgtcccgatggacaggctatttttatttaactgcacgtgcaaggttgtagtcagcatggaaattagcgtctgcaagtttccattccaacgaactatctacagggttactatagaatcctgctcgtcgagcttttgctttaacgatggggtcaactatctggactcgggtaatgaaagccaatacccagagtacccgtttagctattactttaaccaatcgcagctttttcattattgagacctcgaccgaccctaatggaaggggaacttacagcgctttcaacgcttgctgatgttcccatacgatggtcttatattcaacctcaagttctacacgggcgtcattagaaatgctgatatctttagcattcccaactacacgacctttacgtacagtcagaccccatttatcgatcttgtcaaggaaagccttaacatctttacggtgtttttcttccagcttggcaatccgaatagaacgaacatggttacggaaccattctttgatagacgcgaacattgtaatctcctaggataattaaggaagttggaacatttcaagtttggatgggtcgccggaaagtataccatcagcatcataggtaacatacgggacatctaattcaatagctgtctttctcttgtgctctgtgaatttagtcccaaggacacaaaagtacgtattacctgttacagacgatgttactttcgctcctagatctttatagtactgagttatttctttcctcgacatcttaccaaattgtgaccccgtaatcattactgatttacccacaagtggaccttctggtttcttgggagaaatgatatttaccccttccagatgtttcttataggaggactgcggtcgtgagttatcctcgtcgaagaactcgaatatactcattgcagttataggaccgatatcatcaatctgttcaagctcctctgtagtggctttactcagtgcttcaagagaaccgaagtgctgtgctaacctaagagccgtgcctttggcaacattactaataccaaacgccatgatgattcgttctaactgaatacctgctctaactttgttaacttcatcaatgatcttatcggctattttctccgatacattcagttgaagaagaatatcttttgtcagacacagtagaccgaacataccttgaggatccaccatcccccacctatataagtctttgatcatctcaataccaataccttgaatattgagaacttctctgcttacacaataggcataatggttaataacgcgatcagtacatatggggtttgtgcaatataattcagtacatccagatgaaccattaataacggtatcaacttgattcttacagcatgggcacactttcggaatttcaacttctttcagttcacccatccgcatctcagttaacgcgccagttattttcgggataacgtctccggcacgctttacaacaatcttatcacctatcattaagccaaggcgacgaatttcatcgatgttgtgaagagtgacattcgagatggttgtaccatggatatacactggttcaatgcgagcaacaggggttaacttaccagtacgacctacttgaaattcgacatcatgtaaagtactcactccttctgaagctggaaacttataagcaattgcccatcgcggaaaacgacttgttgtacccaactctatccgcttacccatgtcgttgactttgaatacaataccatcaatatcgtagccataggtatttcttttttctagctcctcttccagaatttcttcccagtaaccgtattcgagcgctccgggtatagcaccatcgtcgacagataccgacgaaaaacccatttgtcgtaataggctagcaccttctgtccaagtcgcgtagtggagatccgacgagtcaagcgaatacgcaatgaactcgacacccctagctcttgtttcaattggatctttgtttcggagtgcaccggaggcgtagttcctcgggttcgcaaatttgtcttttccagctgcttcgagttcagcattgactttttcatagtgctcatgacttacaataacttcaccacgaacaacaacacgttctaacggtttactaatatcgagtttagacggtacccctttaatctcaagtgcattcaaagttacatcttcaccaaccaatccatcaccacgggtgattgcttgatgtagagaacctttaacgtaaataagatcgagggaagcaccatccagtttaagatcgcgtgttacttgacaacgaggaggtagggtctttaaccaaccaaccaattcctctacactaaatacgttatcaagactcaacatgggaaaatcatgtttagccttggtgaaatgtttagcggccatgtaaccaactgtttgtgttggagaactagctgtaatcagttcggggtatttctcttcgagatcgattagctgtttacggagttcatcataaaccgcatcagttataggagatccgttttcctgataatacttcttatcgtaatcacggattactttacagagtttggcatgttcctgtttatagttactcaactttattcctcgctcgcggatacaggtcgtcgatgtatacaccggtttcaccaaaaaggttaagtttatccatagacttgatccagtcaatcaaatctttatcgaacggacacgaacttacagatcgtaccatgacagcagcttctgttgcattacttgtaatacatgcattctcacggaaggaccaacccataacagcttgtccattagcatagtggtctttaccattctgtgcgtacgtaagaataccacgatcggtcaggatgtaaatcttgccgtggtcgttttgtagatccattatgttcttaagaacggcttcactttgtttatcaccctggggtacatgttcggtaagctgttctagatatttcccaagaacatcaatctttttgtctagatccttacgttgcacgatcgctcgtacattaaaataatttccattgtagaatgctttccaaggtttctcaaatggatgaactttaagttcattattactcgcttggataatgaccgcttcattacgacgaacgaacaaataaccaaccatgaacaaatctccgatagttatacattttgataatgtagatctgagaaaaaataaaaagaaagcaaatgctcctacccgaaggtaggagcactatgttttaaacctttacacggaacttagaatcatagagatcttggaactctttgatcattgcccgttgagtcggtgtctcagttgcatcattaaagaactcatcagcgaattctttcttcttgcgaacttcacaaccaaacagttcaagaccgagacaatcaagtttatttttaaagtgacccagttcagacaaaccagattggtccggcttggagacctctttctgcccctcgggtttaacgcggaaatccgttacttgggcgtagcgaatttccttttcaggtgcaggacgatgtaccggatctttcttcttgttcttcactcgcttaggtactgtaggcatcggaagaacagttttaggtacagctacaggctctgccttcttcttttctttcttgggtgccggtacagttgcaataggaccttgagcagcaataaggtctttaagcgagttgaatttaacgcgtgccatgcttgtattctcctattggtggtttgtagttcacatttgtaatatagcctttaaaaaggcttaaatgtaaaccaaaccaccttaataaattatacccgaggcagaataaccttatctgcctgtttcatgtatttaccaccacgatctgcataggaagtttcacaatcttgatcgagatcatggaacaccagttgcaaaacaccttcatgtgcatagaacacgttagggcgattagtagtgttctggaactcgaacgtgatatgtccttcccaacctggttcgatcggagtacacagacagttccaaccagctcgcgcgatggtagatttaccaatacacattgcgattacattccgaggcattcgaacatactctttcgaatgagtcagaaggaaaccacctgggggaactacaactttatcaccgtagactgtatcaaacagatcagcgctgatgttcttgtaatccagtacagggtgttcaagttctttacctgttacccaggctttgaaacgttgccaaagagtgaacttaggtagagacttgaatactttaaactcagtaccagctcgaagatcataacccccagaggacagaccataggaagcgatacgctttccatgactatcttctttcactgacgaaccgtgaaatggttctatcattggaccatgtgcaccgaccattgtgccttcgcagtattcacgaattgttttatcagagagaactgtcattttttaatttacctgttggagacgtacactattaacatggtcagtaaatcaacactctaccagagtctcttcgtcagatttatcagtcagagttgcgacatattgcttcagagcagctgcacgatcttgctcttgtttacgcaggtcatacggaccattctcttttaccatgtattcacggaactgcatgacgccttgaacataaccttccgggagaacagtagtcagactatcggcagttactttacgggtgcgaatagccttaccagtttcaagaacatggtggatacggatgagctgacggttggtgtcaatacgctccgatacacacgggaagtaaacgggatcatcgccctgcttactattgcccatgtccacttcagcgtataatgtcttaccatgattagcttcaaagaaagctcgtgcttccctaatacgtttcgtgcgaataatctccgcttctctaaccgctttctgatgtgctggttgcaggaaaggattcatctttcgaacatgtcgtcgaatcagtttggtgctataacgcggcgaggtatcggccatagcaacaagattgttgtatgcttcgatggacatgataatttgttgcggatcattattgcgctgcatgggaatctccgttagtggtaaagtaatgcttcttgaggtgatccggattaaactctgctttacggaattcatatttctcagcgagttcaatgattggattttcatctcctttcattgacagtttgagtttccgacgaacccaatcctcagatgctttaattgtcacggcttttctccaattgataggtgggagctctttttccgaagataacgtttctacaagagaagcatccacaaacagtgctcttcggttccgacccatcgagcgaaatagcttgttgcagcaaacattcatacataccctctacatcgttacctagtaagatttcttcaattatagtcaattcaatattagccaaaatcatctgttcatccaatggacgttgatgaacatgatgccattgaactgacgcattagctgaatccagtgtacctttgattttttccagtttgtatgtttcccctgtgttccgtttgagttgtttgccgaactcaatcggatcaataggggaattcttgaatatgacgccttttatttgtttattcaaaatcaagtatcctcgggtcttgtggatgatggatagctgtccagtcaatcggctcgtatggataatcaagctcgtatttatctaggaacttgatgacccattttaagtcatcatcgtagtacaggttcttacggataggaacaccagcattaacacttaagcgaactgctgtgttagtaccgccgtctaccacttcattctcacgcttccccttagggacggcataatagaagataccagtgaccaactcatcgagagtatgaccatggatctggaagacgttccgagtatggagagctttaccgtaatcgttcaacccaccaaaactaccacgagcacaagcagccatactttcagctgtagcccatgtatcggtaaactgggatgcatccataaagaaagcattatcacgaatacgatagaagcttctacctgtaccactagcgagatatatcctagcacctacctcaccatacttacgcgactgctttgcaccataccaaccagcccgatcagaatcataggcgtcgccagagctaatagcccaaccgtagtccgtgagcgtacgaccaagacggatcattacttcaaggatccattcaggtacgttacgagaacctacgattgccatgtatcccctagccacgataacgactcttcgatgaatcccattgaagccgagcaagttccatcggcgtccatgtacctgccggtttggtgatagtcaattggttcagatcaaccaattgctcacgaccattgaaaccatgttctttgacacgaatcttaactcggttaggaagataaacagaaagtaccttaaccgggataacgacgaactcgtcataacgcatgtaaacagtagtgccgccatgagcaccaacgaactgcttgacctgttgtttcaggttagcatagttgcgacgagcctcttgagtatcttgcatgtgtttatcacgtaaccaagtgttgcgtttacgtgcgtgcttgtgcagagagtttgctttctcagggcaaccagcttcttcacagccaatcctcgcatacgccatcagttcttcgaatgcattcgtactaagtacaataatggattcgtctttgttcttgtctgtcatttcaatgcctcgggattttgtagtaatctgggccagccatgttaaagacataatggttgtgatctttatccatcggacctgggtatctatccactggaaacttatgtggaatcagtgctctacgtgctgtagcgaatacagtttccttatgtcgaattttgtaatcgctaagaacacgagtcatggttacacacggcttacatttgccacaatgtttttcatcattaggcgtctcacatatccaaatgtcgttcagtactctcttatctagatcatgaagaatatcgaccttcgtcatgccgagtaaagggaactcaattggaataggatcattaacacaagataccttttgtagattataccaagcgtcttcgatgtaccgtatatgtgatccgaagtaggcaccatcatcactgacataccctatcatcaacttgctatgtcgagccgagtcagctatagccagcgccccaaataaccacggtgcaacttgtgaccatttggtattatcaccttgtaactgggtacttttcagacgttcatattgcgcttgtactttgtaagggtagaactcagaaaacttttcgaggattacttgacgttgcctgagttctaacttcatcttttcttcgtcttgaccagcattgatgtacatgacatccgctgaaccttcctgaagatactgctggagcatgtaagtggaatctaaaccacccgagaataatatcaatgggttcattgctatttccaaaaagaaataaaaaggggagccgaagctccccgttttagttacagcttgtctacttctttcctaaccagatcacgggcttgtgctcgttcgatccgatggcatttcactttagcccatttacaggaagtgaaataacgcattggacggcgactccagaactctttggaccactggtgtttggaatgattgctacgcgacatgagagtgcctcctttggctctacgttaataaagccaggaaacacttggttgtagataggcatgttaagacctcattgctttttaattacgatcgattgaatacagcgagattcatcaaagaaattcccgctccagttcatacggtattcgaatccgtctggcagctgatcaatatgcaagaacttaggtgccccagcagaaacgattttagccgcttttgaaatagcgaaaccataaccctgtccagctggattaatagcttccaggaaaaggaagtcaccaccacgtttgaattcaattgtgagttcatcacccatttcattcaatacggggctatcagtgtgaatgattgaccagcgatcgttacgttcttccagatggacaaacatgtcacttttaccacgacctatgtttttgagctctacatctttaagctcaatacccaagccattgagggtgacagtaacgagttgacgttgtttctttttcgacattagtagccccttctagtgtggaacggaagtgttccttcaatgtagcgacgttggtacgaactgcctctaactgtaattccgttttccctctgtacagacaaatggaaaggtcgatgtctgtatgtagtacgcttagcaatgtatttacgaacccaaggagcctctctctttgactgacatctaagtcgagttctaaggctagaggtttcatagagtagatcacgcagtactcctacgattgcatcgcgcaattcaacggttttcttattagaagactttacgatttctataagatcgatagtttcaacgaacattagtacaaaccttccgaaaaaagctcatctcgtgtgcaatgttcagggtaacgcaactggccagttttcttcacgtgttccagtgcatcacttctagaccagaagacaccgtattgatcaatgaagccttgttcatagtcatctgctgcataagccctgagtgcgtccataccaataagatcgatttgcgcattcatggaaacacagtaatgacgagaacccgttacaatgtaatctttgtaacggttagctgcacagacgatgtagcgggtattattatacttatcccaacgccatccagtgaaaccatcttcatcatcttcgatccagcagcgctcacggagagtttctttatgtttgcgtacagctgcttcaatgatctttattcgatgttcgatagggacagcacctaccgctgctttcacttgatcccaagcgtcttcaaacgcttctgaatgtgccattctttttccttagaaaccaatacggtttgctttacggggagaactagctgcatcagtgttcaatgcttcagccagagtgaagttattaccaacgaaatccacaggttcaagaccgttagcaatacgagcatcgttcgcttgttcagccgtaagggtcttaaaggtgaggatatcgaaagcacgtccaggacgaaccagagcctcgtcaacatcacgaagagttgggaggttagtagagatgatgatcttggttttggtagacacaagaccagcagtagcattcaacagaccggccatattactgttaccatcctcgcgcttggcaaccatcttatcagagtcttcagtaatgatcagcgagttatcctcaacaccacgaataaagctggtgagatcaccatgactcagtacggagtcttggtcagccagatagacgttgcgatcttcataaccacgagcacggaccatctcgttgatgaagttcgacttaccagtaccaggcggaccaatcaacagaagtacgttggcctcagatgctgcaaactcagcccaggtttcagccggagaacgatccaggaacggatacatatccatcagcttctcgttgtaatcacgagtagcgattacttcactccatgcatagagttcgtctttctggcgattcaaccggatacgcttgatgcttggcggtttggtctgatcgaataccgattcgaacatctctttaaacttggtagagaagtcttcagtagagtagatagagaaaccatggcaggtcgcttcctccataccctcgataaggaaaccgagaataccttcgtcgtccaacaacgcccaaccaccactgataccaaatgcatggagattgaacttggcgatgactttgtccttaatctcccgtatgcgttctttgatgtacacttcacgatctacaccgaacgtgtaatagatgcgaagtttctcactggctgattccagaccttgttcgttaagagtgaaatggtaagcgctgtaacggttacctgcctggattgccttcatgcacagatgagtataacgctcaatccaatattgctggttaggattaagtttagggccacgataagacatttgattttccttttaatgagagatggcataaagctccccgaagggagcagtatgttagtcaggtttcttagcgactactagacgagaccactttgtagaggaattaccttcaccttcaacattgaagattcggtcctggctattaggtggcatgcgaccagtaatactactgaggtctttaataatgaaaccagcttcacccagatctttaataagtttggtgattacgtcggaatcagtaatgtgaccaaggacgtggaactgaaaagtactagttccattgaccaggcgatgaccagctttaactttatcagcatctgccatgtcggcttctaatgcagctacgactgctgcggagtcaacatcatcagctttgataatatcgacaagttcatcaaatgttgggaatgccatgttacaccttcttttgaatagacatatcgttaagcttcatttttggaacggctataatgtacagtacgaagcataccgtagactcgaccattagccatgtctaatttaccattacaaaaacgatctttcttgatttcccagccaatgccctgaagaaacttagccacagctgcactacgtgatacgccagcctcgcagtgaacgattaacgtttcgccatccggaatcttatcgatgaatgtaagaatcttatcagcatgcacgtaatcgaacatctgatagcggttatcgacgtaatcttcgacatcatcgaaaacaagaaccaatacagctttgtgttcgcgtacaaattttacgtcttgttcgggacagcgaatagaaataatgtagctttcgtcagtcaatgcctgtgcagctaaccgtgaatagaattttactctcctcatacagctacctttcgatgtaacatgagacgagtccaagaaccagaggccataccagatacagcagtagacgcaccagtccaaccttgttctttcagaacgctgtatagttcattcaagatatcaatatggataactccgttgataccgaattcgtaaatcaacatatctttcttttgtcgaactgcatgttggccagcacatttaaccttatcagcattctgccatttgaaagtacgcagcaaggttaagatatcttggacagacagaatatcgaatccatcaaagaaatctggagtcacacgagcattaagctgttctacaacgacggaatccatggattccttatcatgaacgattataggtttctcttccgtcacatgaacgggtgggaaaacataaccggcttgaacatctccctctttactaacggtgaaacctaaacggagcgaattatcatattcgaccatacagggagctagctctatgtcccaatcaccaacccaggctgggtaatccatattggctgacttaataagactctgatgtgtacgagtcgttactaaacagtatccaaggttaatgaagagactaatatcatcttttaccgggttaaatagagttgctttccgatggtctcggtcgagcctcgctcctgccagatcatcacaaagatagaaatgttggcactctccatcaactcgttggttgaactgaatgagataaaatttgttattgtctagttccttaataagctcatttactttttcagcaatattcatcggtattctcctttctttgaaaagatgttctcttaggtaatatagatgtaagataatttttattaggcaatcctatagttcttccttaacagcaaaggtgctaatatgtttgaagtgctgttatcattgagtcaaaagaagcaagctatagagtatccattttctggaccaggaagtaaattcctaataaagggtaatgagacacttgggtatttcggtctagtcgattcgaaagatatttattttcgtgaacggtttatcgaacaggcagatatagccgactataccaactctattgtaggttcattcgctaatcaacaatgggttaaatatttctggatgggtaaggtttgttttgcacctttatctatctacatgaccaacgtctcatggaaggttctttacgacaaaggccttgtatttggagacaacacgattggtcaaaatattccaagtggatataataccgttcaagataagttctatcattttactgacgatgaagggagctggcagtttagaatccgtatgggtcatctaactgagaacccattcactccaactaataatgaagacccaacaagtgaacttggtcaggtatttacacgagtgactaatgggtcttgggacaatagacccacaagtgttatcggtcttggtaacggtacatggacaaaggcattgaatacagcccagcgcccaatgtatcagttttacaacacaagtatcacgtctgtaaataataatgccccaacgaataatggtatttggcgtccggtattagagctgattcctaaagatgaatatcacctagtaccaatagaaacgactattaatgcttacagtaatttagccgaagctagtattataactaatacagaaatcagctctggtggaattcaacctattattcagcttacttcactaccaactcctgtaagtattgcttatattagcaatgccccacaagatgaaacgcttatcgacttgaacagtatatcgcgaaagatagataaaacagctgaagttagaattaatagctttagtttcacatgaggatgatttaacatggcatttacaatcaatctacgttgggtaaacccaaacgacgcgtccgtaagtattaaaatttatcgatcagcaacaatgattgatagaaacaaccctggtacaccaatagcagaagtcaatggtgacgttgatggttatgctgacgaagggcttacatatggacttatttactactacatgtttgaatcatcgaaagatggggatgtagctaaatctcgtgtattccagttccatgcggtacctttcactggacctggtccacagcgcttggttgcaggtaacatcaattatggttactacggttctcttcccactgttgaatttatttcggacagtgaactaatcgctcgttgtggtttgtcctggaacgcagctaataatgctggtcaacgttggcataaattcgcatggaaaggacggactttctatgtacctgaatattccatcgcaactggtactctgtactggatggacctctataatgcgggtctagtatacagtaagaacgcagtaccatccgctgtccccggtgttactactcctgttcctcagggcaagcgaatcaattttgctctatctgaatttgaagtatctttgccttccgttctagttgatcacgatgatcctaattctgttagtgatctatcgtcatccgcagcgactgcattaggtaattctgacccatctctcagtaatggtaccgtcgagttatttttagccggtatgactagtcagttctatgctaataaaacattggaacgagttaacgtaaccggtgataatgaggctacacgtgttaatagtaaagctattctaacacgagatactccaaccactccagcttctgcatatatttcgcgaaatacgagtgcaacgaaagcttcggcttttgtacctcaacatacaggtagaacctcaagttcaaacatttggttccctgtactggaacttatccctggtaacttcgttgactttgaggtgtaatcatgggtattaaagtacaatggggtttgaccaatgatcgagaagcagtcacatttgatatttttcgatctgaaacaaaattcgatgaatcgacattacctagtgtattagttaatgtgcaaggaaacatcaaagaatacgatgatacaacagctattagaaataaagtctactattactgcatcggttctaattttgaaaatggtgatgtaacctattccaaagtggttgcacttgctaacatgccttacactggtttcggaccaaatacccttcgttctggagactatgaattaggttattttggtgaggttccagattttgtattacctggtgaaataacagatctttgtggactcagtcttttgactgatattagaattccacctgtaacggatttcatttggcataagttcgttgtagatgggcgcattttcatgctgccaattcgctacgtggcttataacctacgttgggccgatgtctataatgcgggttgtgcttggtcaacgtccggagaccattgggatgatcttcctgctcctgttaagactgtagttggtacgccaaccgaacaaggtaagactgtcattattaagaatcatagttacagagttggcctgcctacatttgctggtgaacgatcactcgcaagtatagctgctggacaggctgtctatgatcagtttaatgatctacttggcctcacatgggatcgtctaattgcatatgcatcgaacatcaataagcctaaccttaaaacacgcgttaactcgacttcaacgaacgttgtaatgacgggcggcgcacctggttcgggtatcttcatgacgcgtacattcgtaggtgaaacccagtctatattggtcagaggtgcagcgcttataaacgtttccagtactctggtaaatagcgcggctgcattcatgccaattctagaactagagctataggtgattcgatgattaaagtaggcttttcggttacaggtgatattgttgacttaaaagcttatcgttctacagaaccatttgatgtgaataatcttccagctgtttttaagcagctggatgttactgatcgagaatttgtagacgatactgctttgaaagatacaccttatttctatcttgttattggtatggacaatacaggttctttcgtattgagtgatgtaaaagctatttgcattattgattacactaataaaggacctggtcccgaaactcccgtattcggtgactggtggattggctacttcggaacatgtccaatcgaagatgtctttgaggtggctgattttaaaacaaatttggctttaccatctaacttcacgaatactgttgatcaaccaacagaggcatggaaaatacagttcaaaggtgtaacgtattacatcccgaacagagttccatattctggaatgtcattcatggatgtttataggacaggtgttctccttgatacggtagaagacggtgttggtactttgccatcatctctcactaatccagctgtaatgcagggtaggatctattctaggaatggtaatagttttgctgttggatgtatcccacatggtgataaggtagtatacaccaatgctactgatgcgatggtaagtctccatgtgatgaatgatctagctttagataccttcgaacgtctattcaatacagcagtaaacccaactggacagttgtattctggttatcaacgcagtcgttatggtaatcagttaccatcgtctatagctccaggtaatggcttgaatattttctataaagctgttactgaagataaccgttgtatccaacgtggatttagcacatctatcgctcaccagcttgacaatgcttttacagcttatggtagtagctgtggattcaatccagctttacgtttgattcgatgagacaacataaagcccggcattgagccgggcgatatgtctgtttagattagagagtccaaacatagtcgtcaaggcaccgtagttagatactcgtctttgctcccgcaaatactttaacgtatcaagttaaagaatcggctggatcacccccttaaagtgcagcgctatgcgcgactgccttgactatatcattactgttttagtaatctttttctaaatcttacacgtaggccaattctatgaatttaccccttaaggataaacccacatgttagactcattccgttcgatatttggcggcttgacagtcaaagaaactgaaacggagattatcatctctggtattcgtggcttcgacatagtccgagatatcagtaagcattggaagacttccaagattacaaccaacttgttcaacaacattggtcggaactcattaagcttctataagttctttgcacctgaagtaatgtacatgttggaaaacattgtctattaccgttctcgatacacctctgtaaaaatgatcgctgctattaaagatgcgcttttacagaatacttggcttgcctctactaaagccattgatgagaaatcagtacaagggcgacttaatctagctaatctgtctcgattaaaatttgatccaaaaccgtatcaattagaatatttcaagaactatacctatcggctagatcaatacaatctaaatggtgacttaattgccgcggccgccggtacgggtaaggcacaaccactaaacgccatggttaaaattcctggtggctggaaacgtatgggtgatattcaagttggtgacatggtcactgcttgggacggtaccccgactaaggtcaccggcgtttacccacaagggaagaaacaaacttttacggttacattcaaagacggtcgcacgaccgaagcatgtgatgagcacctatggcgagtctattgctataattggacgagggacggtagtgatggttggcgagtaatcaacaccaccaccctgttcggttacatgtctatgaaatcataccggaatcgactttacgtgcaactctgtaagtccgaagaaggtatggatgtcgatctaccgatcgatccgtataacctcggggttattcttggcgatggcgggatcagttcgagttgtgtgaccattaccagtggtgaccctcaactattcgatacgttcagtaaagctctcccggataacctcaatcttatcgcccgtgacgccattaccatgggggtcatcaacaagaaaggtgagcgtaacccgtatatcagtgctcttcgagatatgaatttgctaggaacgaattccctttctaaattcattccgcaagaatacctattcggttctactgcccagcgattggctcttgtacaaggtcttatggacacggatggtacagttgacgagaatagcaacctaagtttcaccagttgcagctacatgttagccaagcagttccagtacctagttcgttccctgggtggaattgccaaactggcgttcaaagagcctacattcacgtacaacggcgtcaagaagtacggtaacatgtcttatcgggtagctgtccggtttgatacccccagtgcacttttccgccttgatcgcaaaatagctcgatgcaacgacaataaccaatacgcggataatcttcgtttacaggtgaaacatgttaacctgtcggatcgagtggagtgtcaatgtattcaggttgaacatcccgatcacctttacgtgaccgatgatttcgtcgtgacacataacacatatcttacttcagctattgccgagatgcttgatgctgaactcattgttgtaatgtgccctaagaatgctttggatctagtctggttagattccctgaaagagatgttccataaaccgcaaacagtttggcatacgttcgaacctaatatgccctacaaaggacagcgttggatcgtctgtcattacgatgcaatggataaggtagtagaacttcttagaaaccgtaatatagttggtagcaaacgtactgtgacgattctagatgaatcgcacaacatgaatgaccctaactctacacggactaaactttatcaactcattgtaaagatggtcggttctcgtaataatcttttagcttcgggtacgcctgtaaaagcattgggtgttgaactgattaacttactgcgaatagtagatcctctattcactccgcaggtagaagaacgcttcaagaagatgtatggtaaagaagcctctaaaggactcgatattatcagacatcgattaggtcttgtatcctacaaggtagagaaacaagaactcgatctagagcccccgatcatgcgtccttatccaattaaaattccgaatggtgatgacttcacccttccggctattagaaaggtaatggaagcatttattcaagaacgctgggcttactacaagaagcggagacctgaagatgatagacgctgggcagagttctgtggactccatcgaaaaaccctcaaaacagctgcacaagaaagagccttcaaagagtacttggatctggtcaagtatgttcaacagatccctgatccacgctttgcaggagaggaaatcaaagcaacgaaccaatatgaaaaattagtatttggtccttcccttccaaagcagttcatccatgagttcagggatattaaatcggttatcaaatatactaacctcaagattcaaggtgaatgtcttggtcgtgtgttaggtggtaaacgtattgaatgtcatgtggcaatggtcccgtatgttgactgggtcggtattacagaatccactcacaagaagacgattatgtttactagctttgttgaagcagtagaagctgcggatacacattgcgttaagctaggtatgaaaccactggccgtttatgggaagactactaatgaactggctgaaatcgttaaacgtttcgattcgagtaaggaactaaatccactcaatgctacatatgcttctctatcgacagctgttcgcctgacaatggcagatactctgattctattgaatagtccattcagagcttatattctagaacaggctatatctcgtgcttatcgtttaggtcaagattctcaagttgtcgtttaccagtgttctctcgatactggagatatcccaaatatctctacccgatcggctgatattcttaaatggagtcaagatcaggtagaagcgattatgggtatcaaatctccatttgaaattggagaagcaatggaagatcatggtgatgaaacagagttcgatgagaacaaagtaatacacaacgttcttcagaaagcattcgaaaaattcgacatcgagattccggcagttgatttcgagataccccttaaacccaaatctaatgttcccgcatatttgcggtgattggagtctacaatgagtgatacaaataaaggtatgattgcggccatcaaccgttatctacttaagatcgaagaactaatcgctggcggcggttctggtggaggtggtgcagcagccatcatctacgagagtacaacggtaccggcaggcggaactaagacgtatgatcttgttcctttgattccagctggttcagaggtaccccgtgcagcttctgtagaagtaaagattagagatactgtaagtggttctctcaccgaaggttgttacattgacgcttctgctgtattaacctggggtattaaagacgatggtacgttagttattgctaacccgtcgtctgccactgttgcatacattgtcattgtcagagcaccccataaaaaaatcgtaccttaataggagcctgaaatggcatatgctaaccctgacaaacaacctggggcctatcctagtacccaggttgtaaaatggacatttgattctaatgtcgctactaatggtgtcgcgtattctgttaatggtttaccgccagtcgtttctgagtatatcgcttacgattctttaagcccgcctactccattcattgccgttacccaagatggtaacggtaacgttgtttacgatggtggttttccgaagttcatgaatccacaggcagcaaacatttccatgactcagggtgttctagatttctcagctagactacaacctgatgcaaacggtctagacctttgctactatgaagtaattaacaataagacttacattgttaaaagtggagatgttcttgtttatgaccactatgtgttcgatgatgcatattttggtttagactgtaccgtttatgatgaaactggtaataaccctgttagatttagggactacagtcctgtaatcaaagacaatggtaaccccgctactgcaacacatccagttatgtgcagagacaggccagaatggaaaaacaaatgggtaacacgtacagtcccattagaagccattgttggtaagagattatcgacttggactgtagcattcgagaacgatgcagatcctatccttgcaagagagtatcgtggtcagctgagaaatgcacgggtccttaacggaacaactgttgcttttgatgtcatgacagataatcttgtagttaatccaacaacaccgcaagattggataggtagttggactgttacccgtaaacgttatcttggtccaggtaaaaacctaaactctagtcagatctattttaagaactgtcttgactttattgctaaccctgcaaaagttgctagtggtaataaaaacattcttgtcctaggtgatgcaactactggtagctatgcactgaagaccgcgttcaatgaatacattactaaggttgcaggggccggcggttttacatgtacattgaaggatcagaccgattatgatggaacccatttaaatccaaccttaacggaattaaacaattacgcagggttggtatttgttggttctttaagtgatccggatcaatcggttaacggtaagttcacgaaaactgcggttcaggatattcttacatatcggaaagccggtaatggtattttcatattcactgatcatggtccagctattaacagtattgaagaagcatatccggttccaactgcaactaactgcttctttgttactgctaaccaacttgctgtaaacttcaacgcatacttcaatggctccgttgacagatcaaatgtgaatgttggatttatacgatcgacttatggggatcatgtcctttataatgatctaaccgatggcgattttatcgtagccggcggcagtgaatcgagtgtagtcgttaaagaagttgttttccaaaagaaggatccagtaacactgaccctcaaccctggaaaacatactgttaacttcttgctgaagcttactaacggcgacgtcgttccaatgacgtttgtctacttgatcggagcaggtaagtacgttatattccgagataacaagggagttgaaattacacaactactcaatgacatttctgatatcgctgatatcgtagttgaattggatggcacaagtgttggctccatgatagcggatatattccgtgtagacataactaaagtagatccatttagagatattaaagtgggtactgctgtttacgatccggcaaccggaagtcatcaaactatctatcctgttgatggtatctacgttaacaacgcggatctcattaaggtacgtatcactcaaccattcacttatgaagcaactcttcctgtgactcggtatcaacctccgatcgctggtaaatatggtcgtgccgagaatacacttccgttaatgccgcgatataagacgggtggtactaccactgagccaatctactcgatctctcatatccaagttccacggagaattattgaagagatccaagttgttcgacctgtgtacaaccttactgcgataacgcagagtgtagctgatcacttcaaaaatatcattagttactttgctggtgagcttcctcgtaacgaagggcaagcatttgcctataaaaccgctgctgacacaagtgcagctctagctcgactatctccaccgacacctaagcaaatcttcgatacatgggatcgtttctatgctgatgaatattttgctaaaggtcaaggtatcccaccgttcctttccgatgggactacccctcatccagcgggccgttggtattgggacgatacgatcaaagctgctgtaatgcctgacaatacaagttccattactggtttcctttcagatgaagaaccagaacaatacacacttgaagttacatgtcaatctaacaatggtgacgacgacttcttgggtgtggttctggcgtttgttaaagagggcgatcaaagccatcatttgacactcgcattgtctcgtagtaactcgaatggaaatggacgaggtaatgaagcacagaacatcatctacgatttgagtatgggtaccagacagaatatcatttctgttaatactggcgattactctaatcaaggttggaacggtgctttcaaacgagttaaggttattaggactggtgatatatttaacatcagtatctccaaatggggaacgaccgaatatgatccaactctgtccatgacggttgacctgaacagtgatccactattggctaagtttaaaggtcctaagaaatacggttacatggccttctcgcaaccgcaatcgtatttcaaagacatcgtttatactggacttccacgcaacattgtttgcgatatgggttccaataaagtttattcttggaatggtaccggttgggtactaatgcagaatacaacacctaaaacgatttacggtgcaccacgggtaatcagaagttttgaggacccaacgcaagcttggagaattccagttaatggaactccggtacctgtgcaataacggcataatagcctcccttcggggaggctttatgttgtcagcccttgctaacgccccagacgcgcttacgttgatccagaagcagaaaggcattctgtgtaaggactaggtggaaacggcgcttacagagcgaagcagtgattgtttctactacaccttcaaagtcaaggttagtatcgatagcagtttgctcagctttcgatttacgacggtcagattcacgataacgacatttccatgtagtcgttgcaatctcagtaccgcgtttaaccttaacttgagaacggtagaaaacttctaggagtttaactgctagttgttcaacatcttcgatgcgatcatctgcattagatagagtcacacaagagcttgccatgtgttcatgcgtatcaacactgtcattcagtgcccgcattgttggatcgaaatcaagacgtttaacaatgatgttaatgacatcgccatctcgtctaatttcaatacagcggatgaagtcgaacatatcaaattctttttcgatatttcgcattagtactgcaagtttttcaagcgactcttcgtcatctgttccagagtgcttagtaaaagcaaatgttagatccgacagaattgtctgtggataactcgtggagatcagaagacgtaaaagagattcgcctcggcatttacgaccgggtttacctgtcatctgttcaagtacggttgtcatttctatttatccaaaatggtttcatgtatagccattctttttaaaccagtcctcgcgtgtcgccctggcatcgaatagcgcattatgcaaaagtttagatcctttaccactgagacgatcatcgatatcaaaagtcaatggttgaatcataatccacttccccttctcccctaatagggctttgttaaaataaataacatcgttggggtggttaacgattatattcatgccagcaaattgtgatacaaatttctcaaggcggatctggaattcttcaaacgaaataggatctttctgaagaataggaatgacgttagcctttacccagtcgtcttgaatatgcttatgttcgagtacttcatagaactctctgttaccatcttcggaaacaatagcaagagaaattaaactatcagttggtacatcaaattcagcgtcacaaaagaatctcatagggagtgaacctttacgataaggaagtcataagaataagggactacacgaaataaaaggagcccgaaggctccagttattttgatagaccacggatattacgaagaatctgacaactagcaattatcttaccacgagataccctggaataatatccttgtgcctctagatatttctttggattatcatcggataaagcttgctctagaataaatgtatcaattccgtagttagttagtacaaactgtgccacctcatgatcccaacgttttgcaacggtagaactagctttaagataaacatgagctgtttgctcagagtaacctaaagctactaaccacgctattcgaccagcagcataaataagtcgagtgcgtgtattcgatggaaccgccacaatataccctgttccgggtgacctctgttcctctactgttctgatattccagtcaccgatcatacgagggatctgagatagatcatctcctttaccgaaatacccaatagataaacctttggcaacttgagagtcaatctcagtagcagtattctgactaataaccatcttcccctcctataggggccacggtctcttccacaacacgaaaatatatatccttatactttcatcagataaggcataaagcccgccctaaggcgagctatgcgtttatacagggagttgttgcaggaagtcaaactgatatgctagtagaattacccaaagtaccttacacccaatatgaatccattggtcagtatggaatccaattttaccatcacatttcagataatctgtgatgcaatggataattgtttcagccgcccctagaacaaaactacccgttactacgtatacccaacctccatggataagaccatgtgctggaagaacgtagggccaataggtcttacctagttcagtagtatggttctttgcagcggccataaaatcattctgtagcgcgtaatcgcaaacagcatgaccgacgagtaatacgaagagaagttcgataagggagaatatttccatggtgatgttccgggcggtgggtatgaggctttgtagtctttgctacatatggttacaacttaagtatttaactgcgacgaacattaaaaccagagatattctgacgtctcccttgtcgacgtacttccagattacgcaatgtttgtataccagaaatagttggagtaggtgccattaagtcatgtaccaaacgaccgagcacttccttctgttctggaataaattcaaaatgttcatctggtggaagaccttgacgagaaccctcttgccaagctttatcaatcggatggataattccatttaagctaccgaattctaagaatggtacatcggatgcagtagcattatgttcagctgctaatctacaagcgcgaccgtgtgctacgtatagtttaacatcagcttcccatgcgtacatttcactaacatcgcggacaataacttcacaaccgagatccttcaggaaagaagtaacctcagcgtaatacttttcagatagttcaattttcccaaatttgggactacctttgatgactactactttaaccatgatcgtatctcgaatgctggattataggattgagagcaaaaaaaaagaaagaaggtattggagtccccaaggggactccatttatattgttatttgatgccatcgtaaatatcacgtcgcgcggggttgataccagctacttgagatttacggttatcgatgtaacaaagatactcgtcacatgttgcagtcttaacaaagggaaccaattgagccagctctagtagagtccactctttcccaagatagttacaacgctccatctctacattacaatacacattgtaaagtgcttcagtaaaacgtaaatctagagtttcaccatctgctttcttatcgttgtatttagaaggcagaagatcacgaattgggaactcatgtttcaatgacccattaccaaatttaatagcggtgaatgagttattaaccatggttaagtaataaccacgaggaagttcccaataggtagtacccgaatgtccacgtactacaccaacgagttgtccgtatgcatcccgacaatattcatcaatgcatactacttctacattaccattagttacatagctgtagacctcagtaggtttagagcgacgcgtaacggctactgtgatctcatctggccatgtcttccatccacacaccccatggcgtgagtcattgttaaagaaacaaggtgcaacttttggagtgaaggtagaaaagaataaaggtgtttgtgcgtatatcagcgggtctttcacttcttggccaaacacagtgcatgcaaatgacattagaaagagggcgataatcttggtaaagcgcatttgaagtttcctcttgataacataaagaggctcccgaaggagcctcctgtgtttacaacttaaggagcaagttggtagtacttaccaaactctgcacgaggtagggagaaaccatcctgacggtcacccatgcgtttcagatagatcttgttggttttaactttatccaacgtgacagcggtggtaataccgttgcgcttaacgatgaatgtacgaccgatatagtcggacagagtatcgtcgatttccgatgcttggatgtaacgtttcacagagagagtctcagacatcatgtttccttttattctgctacagcggtttcaggttcaaccggctcgtctttgttgatcagatctttccagtcttgcagacgttcatggaagtggaacagagaatggatttcgcggttcaactcaccaacacgcgctggatggaagatagtctcgtcattggtcttttcgaagatcttacgtacaatcttcttggccaggtctttgtaatacggcaggagttcttctcgacccaaaatcacctctttgataatttgggtttcagcgtattgctccagtgccacttccagatcaaagacagccggttcaacaggttcttcgtcaacagaagattgttgtacaacatcaccgctttcatcgtgttcttcaccagggatggtttccggaggaagatggccgctgttctcggttttctcttcaagctcatctttagctcgcagagcttcgtgggcttgaacagtttcaatgatgaattgaacttgttcatcaatgggagccgtgccgtcaattaccttagtcgaaggactaaacttaatctgagcgtatgcgttgttaacacgagtttggtaaacttcgtcatcttcataacgatccagagaacgaccactgttaaccatacgttctttccgtacttcctcaggagtttccagatagaagcacagcggttcaggaacaccatcaccgataacatgcggcattacacccatgaacagatctgccagattcggattggtgtccagataaggagctacgttcaagcaccaagtagagaaaacaaagcgatcagatacaacccatttaccttcattcagagatggcttgacgatattctggatattctgtcggcgatatgccatatgcaggaaaatatctgaaactgggtcaatcttttcttcacgatgtttcaatagaacagtgcgaatctcttcagccatttccgttccacccggttcacgaagagccacgtggtcgataccatcagctttgagtcgttcaataagagcacgatgcagcgtcgatttaccggagaactcggggccttccagtacgatgaaattacggctagcagatttggtcatcttgtttcctgtatttacataaaaattaattagatggaaaggggctccgtagagccccattcgatcaggtatttacttcttcgaacagctggttgatgtgagcgcaaacacgcttcatctcagccgagttagtcttggtcgatacggtaacaacactatggtctttaccatcacgactaaagataccagctacctgagagttggtggtacccatattgtagttaaagccgatctcagaaagatccggattttctttcatgcgagctgcggcttgttcaccagcaacaagagtaacaccggccagaagttcaccttccagtcgttctttcttcttcagttgctcaaggctgataccggcgccacccagaaccaccgattcatagagatcgttcgggatgtcgaaggtattggcttcaccgagaatcaccttctcgcggagtttgtgttcttcgatgaatgcaaagctcttcagatctttagacatgtgagtatttccttgtgaaagtttgatgtgttaattatgattttgaggtgcggttcggaacaacctactctgctgtaagttccttacgatcatgagaggctgtaagagaagccatcgtattacgctcatcgaagatacgcctggacattgcaaccagttctccaagtcgaggtagaggcatcatacgcatgtccgattcatcgaacttagctccaccagcacgacaaggagtttcccaacagcaggagcaatcagagagagccataacgattccttaggtcatacgcgccggaataccgaaacgagtaatcaacttgaccggttgattttctttttccattatctccacatctacaccaacgtaaccgtcgtattgcagacgttcgtaaacactctgggtaatcaacggccagaatttcttatcggctccaaatagagtctcgatatggaaaaccagtcgaccattgttaccagtttcccagttatcgggctcagcaagggccttaccgattttggacatgatgccttcaagcatcttgtagaaacctggaatagttgcacgaaggagacgagtagactcggacgaatgaggcatattgcggatgccttcctcgatatgttctaccttggctttaccacccgtaccgacagcatagtcgatctgttctttcagggtgctacccatggtagtatgtacacgcgtattgccttcagtatcactgaccacgtaagtataaggtttattgtggtcgatgttctgttctttcattttttattaccttctgttaaaggaattaacttgttgttcatggtatcgttttcacaaatgaataatctgttagctgttacatggtaataccctcaagatgttaatctctaatgcatacctgtgatatagatttgaaattatttttaatggaacataaagcctccccgaagggaggcgtttatatcagttaccttcgtaggtaccttcagtgccttgtgcttgacggcgctccaatcgagcacgaatcagttcacgagcagcgttcatatggaacagtgctttggcattttcttcacaggcaaacttacccgattggaaaccttcgaatacaatgatcgaagcagtcagcagatcttcaacagttaccccgttaataccaacttcagggattactccgttttgaagcaggataaccagttcgagtttattatcactcggttcagcagctttgtttgtagatgcatcgaaaccagagatcacaatacgttttggtgcgccagacatttcatcgacaccataggcatcaatagtcttaccaccggaactaccggatacctgaccatcttctagttgttcaacggagatatctaccgtagtactagccttaacatcgtccggttgggattcagcattagcattatccacatccagattaccttggtcgagatctttaacctcagtttcagattcgacattactagcatctaccggttgggcgacaccatcttggctctctacactaagagcccagtccagacctttcatcagttcaccttaagagtagcggactttaacaatttgcagaagcagttctacagcgtagttaccatcagccttagcgatacccggcatctgtgcacgaatagcgaccatggcagcagccttacgcttcagaatattacgttctttgctgttctctacttcggctacaccaccgatcagtgcattgactgcgatgttctcaatggaagaattgatacgagcaccagcagtatatttgcgaacaagtttacgaagctcagcttccaggttctgaccacggtactgttcagcttccagataaccagaagccagttcggcgaagttacgaacaccggacttaccaaccagcagattggtcagagtatctaccggaagagtcgacgcgagttgagccaggtcattacctttgatctcagagcgagccagttccagtacggattcaacaccaaggagtttcagagcgattttgcgaacgatagacattattgcgtttcctatattaaaagcgatcagaagtttgagcgaaggcagagaccgtacgggcgacctcaccatcgagaacccaagacattaggttcgaaggactacgccaagacttgaagctttgaactgcacgagtcaggttaagattcaaacgtttaccagcgtaatagaaatctgcccaggattgtgacgttagagtcgacacgtaatcttggaacagactttgttcatcccacaccgctccatcagtaagagctagcgcagtagcaataccaccatcacctgcaacggcttcaccggctgtagccgaaatagcacgaccagcagtacccaaccaactcggactagcaaagccagccttcagtgggatatgcattagcttagatagatctttaacactgaaggttacttcacaaccaagcatttcgtgttcagcgttccaaccaacgttaccgacaccgcgacggatctgaatgctatccacgatccccagttgtctctgtactcgacctttatggaaaatttgacagatgaacggagaggtgtaagcacttcgaccagctgaccttggtaatcccattgggagaatcatggctagtggtacgtatatgttcatgaacctggatattttatttccataaggggagatcaattgaacagtatacgaagcagatggtaaagaagccatcgctgattcccagtactctggtgcatctacgaaagccgcgcctgctaatgtctcaagtccagataagttaacagagtctagtgctccggaaataaatcctttaagcatgtctgtaaccgcaccaacgccttccgtgatgttaccacccatgaagtcaaacgatgcagctcgaccttcccctaccttcgtattaagtgtttgtacaacacctacatctcgtgtagtgttagtaaaggattcagatacttcaccattatagtcaacacggaatgtaacgaactgagaaccgtcgcgctgtgcgcctacaacgaagtcatatacgttcttcaattcaccccaactgctaaaactctcggtatcaataacaccattcttttcggatggtttcttatcagcttccagatacttcaagaaatagtcacgtgcgtcagcgcctggtttagggtctgttacagctttggccatttcagattcaataccagcccgaagttcggcaagggtacgcgccttctctgccattgcacgcattgatttttgagcttggtcagacatacgttgcgtacgtccagccaaagacattacatcgacgccgccatctgggcggaagaaacctgggaagatttcgtgcatacgtttaacatcatctaatcctactcgatggcctgggtcttctagaggacgttgagaatcatcgagaatacgcgggaccatgcccatagcgatagcgaactcgttagctagcgtattcacagacgaccagtatgcatgcatagtcggtttaaaatagaaccacttcgatggttgtgatttagtcaagaaactaataacacgagatacgccagttaccccaagaataaatggttgtagcggtagagtgatgaaataaccagtcacgttacctaagttataccaaaggtcagatgtaacaccagtattagctaggcccgccgccgaacgatcatagaagttcgtaaagaacgaggtccagcttgaataacgtggaacaccaaacgacatatggacttcttgtttagtatcgtcgtgtgcttctgaatagtaacgacccatacctaagaaacgatcttcgtaggtgcggcctcggccaggctggcgaatatcagcatagcgtgtgtattgtgggagagggttgatagcaaaactaccacccagcgacgtatttgtaaatttgaaagcagccgagttagcataacgccgtttggtctgagaaccatacgagttcttattgtcattaataggcaataagaaagcttggcgcaaccaaataggcttaacatctgttgccattttgatttcccttcttaacggaaaataaagcctccccgaagggaggctccattgattaagttagcgagagcggcgacggtcgattttgagccgaggtcgatctcattaacgtggaggtcatactattatttcctccggcttgggttttcgaagcttctttggtaccactgtccttttgttcgttcaattgtaccaaacgcttgagatgatcacgcatctcaattaacgtcttaagctgctcagcttggatatcatcgatctgttgagccttctcgttattacgacgtacttcagcttgacgagtcgagttctgttgctgtgctgcttgaagagctgcttcttgttgggcttggataacattaccgccactatcagcagatggattagttccgctagtagttgttccacccacggggttcattggagtaataccaggaagtaccggtgtttgggcagccgtaccagtggcactgtatgcttcttcacgagcaaccgctgcattaccagcattgttactatcatcagtattccaaagttcggcagcagacgccttagcattagccttggcttgttcttctgtcgcctcttccggagtcatggttttacccgcttcctgtgtagctacagaactaccttcagctccaccacgatgctttgcaatcttctcttcgaacatttgatagatttccccgagagtacgaggttgtccacctttcttgtagaagatcggtcggttagcagatgctgcttcagggaagaccgatgcgccgatggtatcctgattacgagtcaagaacttacgtgcaccacctggtcccatgaagtgagcgatgtaaagatctacgtctgttggatcgcgtcctaatgcatctttaaggtaggtgtagttatctttaaggaagcatgcacccattaaggcgttgatcctcggatcaacacgtaaactacgttgggcgtcgtctggaggaataccgaacttggagccatgtttcgccaacattgcgtcccatgtactattaataaactggaaccatccggttgcagacgatgtcttagctttgacggtgtaatcaaaaccagactcaagcgatgcgaagatgaacagaagttctactggaataccgaccatcgctgcaactgcttggaatgtttcagcagctgcttgacgagacttattggctttcggatatggaatctgttcccaagctccaccgttaccctttgtcagggttccgtatgtacgacctgttgcagatacctcgccagccataccaagtttgtactgtgtgttcgccgcagcgtcggatacataatccattgctttagcgccagctgccttggtattactccatgcgttacttactgtttctttagcagactcccaagtattcgagatagaagccattgccctctcggcaaagctaccaccagcggctgcgttttgtgttccagctgcttggtcacccgcagattgagtcggcgtagacatgatgtctttgcttgcatctttcttcaattgttccaaatcagcttcagccattttcttgagatcgtctttgctacccttaatcgggaagatagaatcaacctgccatacactagagccgtcccaattagtgacgcccaatacggcattacccacaataacagcatcactgggtttgagtttagattccatgttcgcaatggttgttccttgagtcgaattacgcattgcaccgtagtaagcacgagcaacaggcatgaaacgaccaacgaaccaatcgtaataggtagaacgatcctcatcgttaccaacgatatctttaccaaataacggtgctgtttcctgcatgatcgattctaggtcaccacggaattcaggaacaccgccctgaatagatagaccatcgaataccattgcttcagcattgagaagaggatagacgttgtagaaactcagtacttccaaaccgtaggcacgcatccggatggattggagtgcagttagcttagtagtagctgccgaagtcgcaacgattggagcacctgttgaaccacccagaccagggaaagccttcttagcagcagccaagggcattgctgacttagtaggatccattggactcggtgcggttttaccagttgctgtatctgccgctttcttggcgatatcctgagctttggtagctacttcggtattagccgctgtagcaggtaccgtatcatctttcttctcgcccgctttataacgaacgtatagagctttccaaagttgatcagctgctgggatagtgtcttccaattcgccttcttcggagaatgggtcaacacgatactgcattggtgtatcacccgatacagaaatcttaacagctttaactaatggtcctttcaattcttgagggaacttactatcaatgtcaacgagtttgacttcattctttttgagtttagctagtgctttaacccaagtcaagaagaccggacggaaacgcatttccaaccagcgggacatacgcattacttgaacttcattcttaacatcgatgccaagaatatcaagaatagccttaccaccaactccactgatattaaagtcgggttcttctgtccgttcggttacgcgatcaaaagcatcttcaagtgcagaaactttctgttgttgatcgtgatcggtaataccgtactgtagcattctgagtcggcggaactctgctctttgatcgttcatctgaccaaagataggtttcaggatatagcgagcagttaattgtccaagtggattaagactcattgcagtcagaatacctgtctgctttgcatccattccatctttgctataaccataagccatagcacctgtacccactgcggcagctgtaccaccaagtatccaaggaactgcgcgtttagcaaggcccattaaacgacctttagcgccacctttcataccaccgcccatcagcacgtcgaacgcaccagagccttcttcaccttctgtaccggtaagtttactgaagatacctttaagtccatctgacaatcccttcaggactttattttcagctttaccggtatcgccatctcccttacccttcaatttatccatcaagccagcagcgccttctttggccttttctgctttatcctgccaactaccagcccggagcttttctggaacttgtgcttgaagagtttcaagaatgcgacccaatagtacttgatcagttgtttcgaagtcttcgtatggtacgcgttcaaagatacgtccaagaacgttaccacccgctttagcgaaaccacctaacactttcttagctgcacctccatagaacttacccgtcttcttcaatgcccaacccatgtacttcatggaagcatcgatatacttcgaacgagcagcgcgaataccacgccatacagtcttacggatgatacctttattcttagctaagatatgtttggtaccgtcgtagttcttaaggtctttatacagagatggttctattacaggttcgcctctctcgttaaagatcgtgccatacacatcaccaaagttttcaattacgcgacctttatcgtcgaagtacttaccagcgttaaccagtcttcgttcgagtacaggtacatcgtcaccaggtaaataagcattctgagtttcaatcgtgaaattgaatagggccgaacccataccgatcgcagtcttagcaccaaacttcagtgcggaccacgctaaggtagatgtattcgttgccatgaacttggcgccccagcccgctacatttgctagacgccgacctgtcttagtaagacgccaacgtttacgagtagcacgcgaccatagaccagaagctagttccttagcagttgcaatgatagatccattcttatcaagtacatcacctttgatgtcttgcatcgaattaatctggtcaccatctgcgttgaagtattcgccgttctttagaccacgagcagagatagtaggttcttgctcaccatccaaataccagtcatgcttatcatcttcagctgcttgtttttgctgtgcgttttcaccttcagcaaactgttgagccggaggagtttgtccacccattagagcaccgcggattttgtccgctgcattgctcatgaaggcaggtaattcaagacgcattcctttcttatcaaacagaccttgggcaacttcagatgctgttagaaccgtcatgccagttgtagaaacaaccttaccggtaatgtcgtgtacagattcgatgatctttttggtattaaagtcaacaaagttaccttgaacaaaatcaatacctttaataatgggttcatttggattaaacttcgtgaacacatcgatgatcttatctttctgaccgattgcatattgggttggatcattctggaactgatccatgtgttctccaaacttagcacgtgtcttagaatagagatcttgacccattacattcgcatcattccaagctccttgcagaccagcaacgtaaggaccaaattggccattacgcatgttgttagcaaagtcatggataccggcgccgtgcttattgttcaggtactggaatttcccctgtgcaatacggctgtagcgagatagttctttcttgattcgatcttcttgtggtgcatgtttatttcggaaacgacgcattgcattaagcgcattggctttagctgcacctgggtaagcaggaccaaagaagttcttatcattcatatcaccagaagcttcaggttgatagtcaccattaacccatgggttggtatcagtaacgccagagcgcatgatctcccaaatacggttatagtttatcctatcttgtccttgttcagtaatgatgataccgagcatccgtaaaggttcagtttgaccagcattaataagacgatgtacttctttaactgggtcacgacttacagaacgaatgtcaaggaaggcacgagagtattcatcccgtagacgatggttttcagcattatctgccattttacctttatcgtcatactggaacttactcttaaagaacctttgaatttcatccgtggttgtggcatccaagccatccatataaccgccggatttaaggtaagcttctggatcaaatctacggtttgtagatgcatcgcgaagcatacgttcaccaagtgccttacgtgcagctggagaaagtttaccctcttcatccatcaagttcaatgtgtcattaatggcaccactcgcacttcgaattgctgctgctggaataatcttcttctgaagacgatcatccgacagcgattgaacttcgaatcgaccagttgtaatatcgaatacttcacgctcgatatcatcgcgaccagtgcgaatcattcgcaattcttgaagctggcgagacaggtaacctgggatgacttcaacgatactacgctgcgtcaattggttaaaggccgcgccttgatcaattgtttgatagtttccgttttccaaacgatcgttcatgtggtactgaggaacgaatggcataatagcatcacgaataacgccacggaaaccataagtgttttggtagttattaacgaactcttgtagatatgctggaacgttgtctagggcataccctacctgatgatggcgtccaccaaaacggttggatagtttttccatagtcggacgaactttacgacctgcccatggaacaatagacgatttaaggatatcggcaccgtattcaccggcgatttgaccagcgaacttatagcgattatcccaaacggatgaacctgccatatcgcccatgcgtagaccggctacgatctccgatagacgtccgcccaggccgctggcaacacgttcgtttactttgttaccataactacccaagaagccatgaaggccctgtgcagctccgccagctaggcgtccgagcatgttgccccggccgcgacctgaaccaaaactggttagatcgccaacattgcctttcttgtagtctggtaagccggtattacgaactaatgcttcataagccttattctgcaattcaagattagcttcttgtactttaacaagatccctaatacccatgtaggtacggaactgaagttcaaggcctttacgttgaattccataattaacttgttcgttatatcctacaagacgagttagactatctacagccatccccatcgaacgggacataaagtcaaagcgtccagcacttactttatcacgaattccacgttctgctctttcaacggcagcgcgtgcaactgcaccctgttcactacgttggaagttttctctgcttaccagcgtattctgatcgagagcagctttaattacatttgcatcatcattttcttgccggcggcgacgaatagcgatttggtccctttgggaatccacttcgtactgatattgttcaacctttctggtgagcgtatcagagatattttcgtataaggcatttggaatgcgatcttttaactggggtagataatcctgtgctttacgaccaaggtaatctaggtcggatgcattgactctttcgaccgtatctttgatatcggttaccgaagccattacatcatcataggcaccaaaaagacgcgcgaaaccatcaggcgctgcgcttcgtaagaaattccttacgatgtctttggttttcaatccaccgaggaagccctctttcagaccagatttgaaatcggttactggatcaccaggtttggtggtttcaccgacatcatcaaacaggtcgtccagctcattaaggtcaagtacaccaattctgttctgggcattcatcccagcaggttttggcagcttggtcttttttgtagccatggtcaactccatcgatataaacaatcatatcgtttagctttttgtaacccctaagaggaaatttgaaatgaagaaggcactagtcccattcaacattgatcttttgattccgacccaagcacagctttcgatgttgggacaagtaactagccacgagatcttcgaaggtaccggtggtaactttcatgagaaaggtttattctccgtagagattttcggacgagtaggctctactgaacgtgaaggtcgattcggttatatcaacatgggtcttgagattatccaccctgtgatctatcgtaaccttattaaactaaaggctttctacgaagagatcattcttggtaaatcattcgctgtatttgatccagttgctaaagacttcgtacgttccaatgagcttgaaggtaaaaccggttacgcctttttctttgataactggaagaagatcgatttcggtgaaactaaatcatctattcgtcgagtacgggtagagttgatgaagaagtacatgaaaaactgtacattcaaaaacatgctcgttattccagctgcatatcgtgaggccgagattgatgttgatggccgtgtatcgatggacgaagttaacgaacactatcgatatctgcttaaccagtcttatggtgtccctgaatatttcggacctaatgacgatctgagtatttatgatcgtaagcgtacttcgatgcagttgactgctcttgcgatttataaccattacgaaaacctattatctggcaagggtggttatattcaacagaaatgggcatctcgtcgagtatttaatggtactcgtaacgttattagttcgcttgataccaatgctgctgatcttgatcagccaaaccgtcctaagttcaaagatgccgtaattggtatttatcaagcagctgtatccgttaaaccaaagactatttaccatttacgcaatggtgttgtcggtcaagtcttcgatagtctctctactcgtgttgagcttatcaataagaagacattgaaactggaatgggttaatattagtaacgaagagatggacctatggggaactcccgaaggtcttgaacgcgttattggtgaactaaaggtcatcgaaaagcgttctcgtgcaattgagatcgctgggcattatttggcattggtctatcttgatgacaagcaaaacttcaagatctttagggatattgaagaaatgccgaagaagctcgacaagaagttcgtgcgtcctatttcctatgctgaattgatttacctaagcggattacctatgtggaaaagaaactccgcattcgttactcgttaccctgttgagaactataacagttctattcctgtaaagatgtacgtgaagacaactgttaaaggtgagatgcgctacccacttggttgggactgggaacgagatactaatgctgagatcgcattagaatatccaatcatcactattaacgaaccggcgcaatggcatgactccacgtctatttccccgtctattcttgctcctcttggtgcggacttcgacggtgacactgtgtcattcaacgccgtgtattctaaagaggctattgaagaatccgatcgattctttaaatctcgtttagcttatatcaaggctggtggtggtcttgcattcagtgtcaacatccacacgcttaatctaactctccggtatatgaccggggaaccgaaaagtaggatttaaccatgcgtttgaaaattcatcagtttctgaagaattacagtcttcgaaactcaggcgaactactgcgtcctcgtctgttcccgttgacgaagctagagctaccccaagaggtagtgtatcagttccttgatgacaacgctgctgtaaagggtccgagtcaatcggaccccctctttgctaagttgcagggaaaggtgttcattgaacacattacacagctagaaacactcgatggtaacgctcggcgtacttctcttattccgactacccttgaagctgatttccgtcgccaacaccgtttcttcaaaccactgcgtaaagatgcggctgtaaaactcaatattcaaaacgttgctgtgtttaactacagcatgctaaacccactctggaagtaccaagctaatttcaaatctaactggtatcgctggagtaacaacaccgctaccttctggaaaggtgttgtcgatgtacataaacgctttggttggaatcagttcatcgaactccatattccagaatccatgccaacgtttaatgaatttaagatgttagagcgcggtaccactcaggcactacttgagaaattccgtactaacgctgtattaaacgttttcgatctttatcgtttccttggtgataatcgatcttcgtcttatatgtcgatcgtacctaaagaagcttacgaaaagattaacttcctgattcgtgtccagaataacttctttgttattaaccttggacaacttgaagcatggcgtgatgctccagaagtaatagcggaacaagagacagtagctactgaaagttttgtggatgaactcggtcttgaagttttctataaaccggatgtaatgcaacgtcgagttatcagcctgttgactactttggttgagttcaataatggtaacgacactctaatggaagtcgaacctgaaactccaaagatcactgacctgatcgaacccgaagataaggttgacacagacgacgaagaagtcgaagaagttacagaacgtgctgaagaaactgaagaagctaacgacattgatgcgatcgatgattccaatgcaactggatctaatgttagcacattactcgatctcgggatgctcgaagttgtttatgatccaccgcctgaatctgagcttgagaaaactactctcgtcatcgagaaagatccgctcgaaacggcgccgatcaataaaacaccaactctcaaagtagagacagccccggtaactaaatcggtcgtacctgcttttagcagcggtgacgctttagtagaccctgttggacaaaaagcatttgaactgtatcaagttggcatgatctctggtcgttcgtttgaacaagccgttgatgatgcttctatgtacaagtctattcctgatccatttggatctggtaaaactatcgctgaggcgatggtttatgaagaagaagactttaaagtaccagtcgaacagttcgctgataaatccacgattactgataaatcgatgttgggttctattcacaaatcgatgatgcgtaagtacacgaagactcttctacctaaagacatcatgcaatctatcttgtctgttcaagcgcaaggtgttgcagtaactgatgttcgtatggaagaagtacgtgacgcgatgaaccattatcagtcgttcactgtaacagtcaagcctattcgtggccgaccctctcaactgcgcttccgtattccagttatcgatcgcgatggacgtttccgttctaatggtgtaacttatcgtcagcgtctgcaacgtgcggatattccaattcgtaaagtaaacccacttaaagttgctctgacaagttattacaataagacattcgttacacgttctgaacgagcagaaaacaactacgatacttggttgattcgacagattggtgttagggcaagagataataacgatgtctctgtaactgaggtgcgttatgcagaactagaccagtctatgttcgttctaccgcgagtgtactctgcattgggtagagcttatcgttctttcaagaacggagcaaatgagttctattttaagttcgatgaccatgccgaatatttccaaaagacttacggtatttcggtagaagcattagagaaagatgggatggttgtagtaggcgcccataataggttacctattctagttgacagctcgtctcagttctatgttaaagaaggtaatgaacttgaacccatgggcaccatggtagatatcctaggtcttaatcaggttaaagctcctcttgaagctattctagtttcagttgctaacaaagagcttccacttggtttcattcttggttatcgccaaggcctgtccactctacttgatacacttggagttcaataccagagccatccgcgtggcactcgcattagtgttagtcctgatgattatacactggcattctctgacgagatccttgtattcagtcgtcaagattatcgtgcgacattggtgttgtccgggctgaaacgttaccatcaatctttgaagaagttctctcgatgggactttgaccggcgtgatgtttacttccgtctattagaagaagctggtatgtctgcccgatacactcgtgaaatcgatggcttgtttacttctttcgttgacccgatcacaaaaggtcttctggaagaaatgaaagaacctactgatttccaagggctactgtatcgttccgtagagctgctaactaatgactggtcaccagcagaagtagatggtgcatatatgcgctatcgtggttatgaacgcatggcaggaactatctacggtagtctgaaccgcgctgttcgtatctacaacaaccgtgaaggttctgcggatcaacagatcgtgatggaccaacacgaagtttggcgtaagattgcatctgacccaactgtagctactattgaagattctaacccaatcgctaacttgcgtgagcaagaagccatgacttatcgtggtgatggtggtcgtgggtcgacttcaatggttgcccgtacacgtatctaccatgaatctgacgtgggtgtagtttctgaatccactgtagactctggtgatgtgggtgtaatcgcttatctatctcctgatgctaacttcaacagcatgcgtggtacaactcggttgtttgagaaaggtaaggatggcgccgctaagatgctatctaccggtgctctcaccggggttgctacaacaaacgatgacccgaaacggattaacttcgttagtattcagcaacagcaaggtatctatgcagatggctatgaggtaactcctcttcgcactggttatgagcagattatcgctcaacgtaccagttcgatctttgcgtctgccgccgaacaagatggagaggtgattgcagtagacggtcatggcattacagttaaatatgctgacggtgagatctttagttctcagcttggaaccgtccatggtactgctgcgggtgtaaactatccgcatactctcgttaccacacttaagaagggtgataagttcaaacgcggtgatacgcttactttcaatagtaagtattttaccgaagatcgttatacccctggacaagttctttggaaagctggtgtcatggttcgtgttgcattctgcgataaccttgatacacttgaagacggatctgttattagtaaagacgtggctattaagcttaatactcagacaactgacatcaagaacattactgttcgatttgatcagtcgattgagaatttggtcaaagttggagaacacgtagacttggattcaattctatgtactattcaagaccccgaaatggccgagaactctctgtttggtgccgctgctattgaaacactgaagaaactttcggctaatgcaccccgtgctaaagtcgtagggaccatctctaaaatcgaatgttactatcatggtgacattgaagacatgtccagtaatcttcagaagatagccagagcatctgataaagagagagccgatagggccaagtcgttgaacgaaccagaattcacaggtgaagtcgacgcatccttccgtgttaaaggtcaaatgcttgaacctgacaacatggttatccgaatctacatcgaccatgatatcccttgtggtactggtgacaaaggtgtagtagcgaaccagatgaaaactgtattctctcgggtaatggatggccgtaacgaatgtgaagacggtactccgattggtctgatcttcggcaacacttcggttgaagaacggatggtcatgtcccctaaactgattgcgaccactacaatcttgcagcaagctctttccaagcacgtagctgctctctatcgaggaaccacaaatgcaaaatcaaagtaacaacgtagtactcagtcagaacatcgctgttctgactgctgctgccgaacttggagccgaagctttgcttcgctccatcggcggtgacacctcggcagctactctagaaggtgagtatctgaccaaagaagatattcaggcagctatcgttgcccgtatgtgcaaattcctcggttaattaggagtcaacatgtttaatcccgaaactctggacgctgttcgcgatgcagctcaagcattcactgaacaggaacgtgttctgacaattccgaaccccgagttccctctagctgtatatgctgacggtttcaactgtgaaaccgaaggtaataaagttgcaatgtccgatgaactggctgcttccgttgaagctcatttcgtcgaaagtaacgttgaagcacccgagaacgttaatgaagaacgtgaagcgatcatcagcaatatgcatactgctattgccaagattcaattcaatactcaaaacgttatcattccggctattaaagcaatggccactgactatgcctcccgtcagaacgtaagttctcaagcggattgcgatgtcagcactttcaactacgacccgattcataacgatcctcgtctagttaaccacatccaaactcgctatgctaaagtgcgtcctctaccggaatatcgtacctttatgcttcgcccggttgatgctgctaccatcatcgagatggtatccatcaataacccacacctggatcaagagcaagttactgaatgggctcttaagattccggcacaacgggtagaaaacgtttggagtgaactatttggtactgcacgtggtttgactgtttctaacctgagctttatcaatcctaatgctttcccgtttaatcttgatgaactgactctagcttatttcatctgtggtcattacatcgagaacccacaagaagtacctggtgaatccgtaacatcggaagaatgggaacaaacggttcgtctactccacgagatgcttggtttctacatcatccgtgcgtatgaaaatcgtcttgaaatgcgagagtctaatactcttgtacttcgttatgaagctcatcgcccagttgaaaaccgtcgtgtacttgttactcttaacggtgacgttgctgagagctggctcgttaaaggtggttctgttgaagctctgcttggtgcagctatcgacggtggtaatgtcgtacatgcacaaggcattgacgcacgtgctgatcattacatcaaacgctggaccgctacatatccgctaatcaaacaagcagcactcgactacgctgagagccgtcgtcggcaggacgttattgataccttcctcgcacactgtggtgaaggtcctttacgtgaaatgaatatcggtaacgtacgtgaactactggctaccgccatgcgtttcgttcggcgcgaagatctggataatccatactgcgtattcagtaatcttatctgccgtacttactacaccgaaccgatgtataagctgtatctcgatactatcgatgaatatggccaaaatttccccggtgcagaactacgtgaattgaatactcaagctctgatttcgctgattgctattttccaagcacagcagatcaaagtagaaacattcaatcctgatgttgatccgaatgcaactcttcctgaaccagaagaagtgccagaggaaatcactgaaccaactagtgaagaagttgccgatgctgtcggtgatgcagtagaaggtgaaggtcccctggctgaaactccggaagtagaagacgaagaagatccttacgctgatgaaactcctactgaatctgagactgaagaagtcgaagaagagcaggaagaagccagtgaagaagaaactgagtccgaaactgaagaagaagaacaagcataattgataacctccggtatccttcggggtaccggagtgtgtcaactttcctttttctaagaagagacttatatgaacgttaggcaattaacacgtgatgctgcacgcgtaaatgcaaatctgattgaattggaagatggtggtattgctacaaaccttccctgtaagattcaaattccagaacgttttgctgctaagaacttggctgtattaggtagtgaagtattcatatttggattctttcctatcatcatgaatgaagagttttacgcggttaataatacaatcgcgatgatgcgcattcttccaaactctactgagcgtgttgttgtagagagtgaaccttattacgaatttagtttcgagaaaggtgataaagttttctattcgacacatcttgtggtcaacgacacactaacatattacatgtacgacgagttcgtatccaaagggaacatcccttggtatatgaactattatgacatggcgaaaatgttcgaaactgcaaaagaacatgcagatacatttattggtggtcgttcgattatcgagcttatcatttcaaccatcgctcgtgatccggatgatatgacaagactataccgccacattctgtcgcggcatgatgatgttaaaaataaacctccagtaaccgtacctttccgatcggttatttggaacacctcagataccacctcaaaacttaatggtgcttacttcagcgacgctatcaactctgcactagtgaaccctagtgagaaagtagaagtgattgaagagctattgaggacataacacggagttgcagaaatgcatcctttggcacaatcttcttttggtgtccaaaattctccgcagaatcaggtacgtattggctgcactatgttagctggtacggacaaaaaaggaattcttgcgccgaatgcggacggttattatactgtagttctgggtgcctatggtacacataactctgctggtatgttctatgacgaagccagtggcgttgcgatgtttgatccgaactcttccctgatgcgtcgccttaagaaaggtgttctcttcatggagttcaaacaccctgaaccgtttacagacctgatgattgatggtcgtgttgttcgtcaaccgatggatgatcgtcaatacctgcaacgtattcgtatgatcgacgataaccgggtttgtgcacatatccgtgcattgactattgttcccggtaagaatgaaaatggtaagactgttaaaatggtcgtcggtgaggttaaaccttacggtccgtttggtcacatttttaaagagtctttggataacccaagtatcaatacctattgttccgttcgttctatcacacaggacgacgtaatgcgtggtattaagtatacacgggaaatctccacctgggacttcgtcggtgagggtggtatctatattgctaacaaatatacctcccctgctttggaaagtttctccgataccgaagttatcatcacacctgctaccctttggaagatgcaggatgaagcacagaagcgtgctaatatcggtatggaatctgatcctaatctagacgttactgatctaattcaacaactaggttggtcgcgtaagaagccgattcgtgtacctgcttacatgcgataaaaaaaatggaacataaagccctctcccgaaggagagggcgatatacctttatgctacgaagccataagcttcttcattaacaggtggccaacggactaactgtggtttatcattgatctgttcttctgttacatcttgaccgtccaggtagactgatctcccgaacacaccttgggttataagttcacgagctttatttaaagcaagtttatacttatctaccgaattatatgcgatagtattactcacatcatccagtgctaaaccttcaggtgtaaggtaatattcccgcccttcatctaccgagaagattcttactaatcttcggaagttctcgttaatgaaaggccattttttcataggtttctatcccatgtgaagaaagtctgagtttaaccgaatcagacgtatcgcaaactgggtgagatgttcgagcatctcacccaattcacgtttgtaatatagttctcaattaagttagattaagacggcatattaccctcccttttggggagggctttatgtcgctattgaatagcagcatcaggatagaacgacttgatcagctctattgggttttccatcttgtagaacggagctgtcaacattgcttcacgatgagtttcactactaagaatcaatgtggtcgcatcttcagaagcgtgacttaggaagtaaagattccacacgggttgaccctggcgccgagtagtgaaccaatctggtttgagttgattaaggatgcgtactaaagtagccatttggtcggcgtagttaggacgttcctgtgcaccagttggatctgggatctcaggtccggttggattattcgggtcaggaatcattttagggaaaggaccaccaggtacacattcttcagggaacacgtaattctgtagtaactgcgcaggaaaatttgggttctcagcgatcagtgctgaaacaccgccatgcagcattaacctttcgattgtggcaagatcagtactagggctaatactagcagaagctcgcttaacaacagagaatctgaaatcatcatcatagtcgtattcatacttgttatccgtccacttggctccaaaggtttcatcaactagatcgggtataccccaagctgtaacctcttcgataatccctttcatcagtgctgcttcagcaccaagatcgaatacacggagcaatgagttattagtcaggtcacccatgaacccaataatactattaactccgctaaagttcccatctttaaaataataatccttttggttgagaaccattttaacgccatcgatcatatccgttgctttacgaacataacctgtaccggtatcttctccggttaactcttccataatcgatcgttcaacgtccgtagctagacttacaatggaactacgtgacccttttagggcatccgcaattcgtgttctagccatgttgagatcaataccgttgttaaggatcttgttaccgatacctttaacaacaccaagtgatttttgaatgagttcgtctgcacctacaccaaatgctgttaccttagaggctagctgattttttaattcagcgctttgttctgtataggcatcaacctctttgacagccgcatctggtaaaccagtaaatgaagggatcgctaattgtaccattgaatttcaccaaaaaaaaaataagagtcatacaatgattgccattaggctctccccgaagggagaacccaaggcagtcactttacatacttgaagcaacacgtttaacgatattaacccattcttcttcagctggggtaataccgtgagcacgccacacaatctgtgtgtttttattaagtttaagttttaggagggggtacttggcaatgcacacacgaagagtttcctccatcttttcgtacagatctggaacgaacttgtatctactttccaccccagcttcttcaaggttgataccatctagatatttgggatgaacctttcctgtaataagatacaaacggaaaccgttccagctgtaaaaagctgttccggtaaccgtatgtttcaacacggatgaatggaactgaaggacatcagggcaaaggggagagctcaggtcaatacagttatccattctcttactccacaactacagggtcagttatagtgatcttgtgaacagagtccggaagtgattcacggacaactggatcatcggaccaacggagggtcagaatatattcttccttaactgcgcgtagcaaatggatgccacgacggaagttattcaaagataccctcggatcaagcagagcacgtcgtaacgtgtttacattttggttcacttctttctgagtcaatccaactacattaacgggattcttcgtgtaatcatcaaaaagcttctcccaccagagtttaatatctggtttatctttcccttccattgcaacaacgtgcctgaaaagatgcgccatcaatgtacctgcgggtttagcattctcgaatatcttacaatcctgccaagggaaactgttggtcgtcagaacatcttcccgttcttcgggatccatcgtgatgacatacgaactaacacgatcgtcacgccatgtcagtttaatctccagtgttgcgtggactgggttcaggaagtcaattgcttttctgaaagcggaccactgcatcgtgtctgacttaagagctttattcaggttacccttgtcttgattatttttattccaaggtttctcaaagaaagcttcttgccgccggttccatgtacgttggttaatcttacgccacaatagaacttcacgaaacagataacacgggatatcggatgctcgcaacgttcccttaaggggatcggaaagaaggtcttgtacagaatccatttttcatttacacctacggtgattaaagagaaggtttcgtttcgcaactctatttatttcatagtttcttccttcatggtatcaacaagcgtttgggtaagtacaaggatatcatgatacactcttcctaaaactcttctatagaagctcgcggtttgtgtttcaagaatcattgcatgtttatcaagatacgtcttaagcttttctaaagagtcgactatatctacagaataacctcttgcatcagcaaagtattcatctaagttaactctactgaattgagtgaattcattcttactaatttgttctaaagctgcttgatcgccggtggataccattgtgttaatgacattcatctgttcaatcagataagttacgttagtatgtcgcagctccatgtttactgccatcatgtctctaggtgaaatttcaccgaagtctttgacatcgattctattccataattctgcaagcatgatgggataattatcacgacgcacgccctcgtcttcaaactgatcaagcagtgctgaatacagttgttttttggatactggctggaacacccgtaaccagcggtgtagcgtattaatcatatagaaaactccctaatccgcattttatggcatattgttattccgttgagtatttctcaacagtgaggtagtaaaatggaaactccgatcccggaatttattccgacagaaccagaggttttgtactctgagctttcttatgaagaccagctaaaacttacacaaaacgttaagcatcggattcttcatggtgtaatgacctcccgtgtggatggtactattccaaccgacaaagaatctattgattcgatgttgaaagttatggactcgatggatcgcacgactatccagaatcgtcgtacacagattgaagcagaaggtaataagtctgcacgtgatctggttgaatcgatggcagagttcattaggcaagctaagaacaagaacccgttcgttgccgtacctggtgaagataaccgcggttcagaaccagatatcgataatgaagatcttggtgagtttgaacacgccgccggtgaaggtgaaattggtgtcattaacgagacatctgaagagttcaacgaacgcatgcgcgcggttgctgaaaagaaagcacgtgaggaagaagccgcacttggtctctcttaacgacatagagcccagcctatggaaggctgggctctatgttgtcttaatcaacaataacgtcttcaaatgtaccatactcatcgatatggatttcgacggtcggtggttcaaattcttgcattgtcttacggacggtttcttctgtggttttgaccagatcgtcttgtaacttttttgcaaagagtacactacctgcaacgagtgcaattccagcaatagagcctttattctgatatgctagttcaaccaacggatttatactttctttaaactgttcaaagaaacctttcttacggggtttctctttattgtaatctttcagcttaaaggtatcgaataccattggcatgtcagggacttgttcatatttctggagaattgctccaatatcaacaataccttgtgcaaaccaaccaaatacaaatcgattagtttttactttcagaacgatgttatcgcctgctttatagttatcacggatccaatcaatgatagcatcatcaactagatcatcttgtcctttaacttctaacaatacatcgaggtctactagagtaccatcgatgatagtatcgtttacactgtcaacttcttcatgaagacgaagtacggtgttgattaattcggattcggttaaaccggttgtttttacagtccagtagaaagggatgttgctcatgagtatttacctaggtctatttaaaagaactgtaggataaaagaatataaagagtcccctccttattcttagtcctacatatccttacctatcaggtaaatattcccatgaacaaacatcactcaaactacttattccacatccgatagatgtggcaacttgttacagtaaacattgttcccatgaacaatgctgccatcaattcactagcactctcctcttctactttcttttcattttgtttcaagtaatcataatactccttttgttcttcttttacttcagtagtatcatctaactcaatgccagcaagtatacgccattcgtgatcgagtaccttaaattcagaaaggattgtttcagtgagttgctctttaacccactccccattacgtcctctatgaagacaccaatactcgcctttctctttacagatatgtctttcagtaccacggtaatagaaacggaaatgttcaatctgttctcttaccgaatctatgtacaacagatccgttaaatgatcgacagcaaagtggctcctaaggacctctatgctgcggtaagtcattctacgttgattggagttgcatctgcctcatcgacagtagtttcatcattctgattagtcgcgaatagatctcctccgaatacgatggtagcaccaatgaatacgccgatgctaatagcggtcaaagttttccagttcatgttagtcacctctttaaacgaacggtatccttagatacggctcaattaggtaatatagatctgaaaaaaattttattgacataaagccctctcccgaaggagagggcatatgcctatttacaacttacttgaagataccagctttgtaaccttcgacgaccgccttcgcttccgatacggacagttcggggatattgcgacgaagcgccaccaccgctttgatggtgtgttcggtatcggcaacctcacgccagtcgcccttaccgttggccagctctacgtcttggacgtacagagcagccttgagaagagccatgttacgttcaatcgtcttcatgtccatctccacgagctgttgcaggtgagacagagacatatcggacgcttcacgaacatcatccatgaacgaacggttgtcggcgttgttcaggatatcgcgagtgagggtagccagattaccagccgtcgcggtcaggttaacgaggtggccagcgtatttctgagcaagagtagtcattgtatattcctttcgttggggttgaatttatgttgattagaaaagtgccgtacctttccactcgttatcccgcgggggagtacagaagtgttgagtgtacagatcgatgaaaacaatacggtagacgtcaccgtattcaccagtgcgaagcaagcgttcaatgaaagaggagcgccacatggcgtctatgacgttttgggtctcagagacctgacgatgcagctctttcactatcgtgcgatatacagcctttttggcggcttcctcggcctctttacgacgacgttcctctgagacagcaaaggcttcaccgtaagtagctttaccgaaaagaatatcgcatgcttcggaagccgacatggaattgaataggcccgatacagctgcccatacgccagtcggtggagtggacttcaggatcttattataagcatccagaggaattacgaactcacggaatttttcatccgtaaggtccatcattttccaggtctcttcattggtatcacgttcatgatatttccaaccagtggagttggaagccgatcgaaccaggttcatcggaaccctacggtggaacataggtacgtgcgcgatatcgataagagactggtttgaaccttcagaagaaatcatatccagcgaattcttgacgccataaacctggcaaaggaaatcgatggagtacgttacaccaattgctacgtcacgcgagagatctttgttaaacatgaaatgtatccttaaaaagatgtttgttagcaagtacaatgtaattgcattctgtatgcagtgcgatagtacgatctattgtgtggagaaggtctccaacttcgtcgtcagtcagcgtacatgtccattgagtcaattggatgtacccaccaacatcctctttataatgaccgtaaacagtagcatctggtcggccattacgcattacaaagatgaaagcgtcaccactgatatcaagatcatagtaatgcccatgctctgatctcagtgtaacaaacatccgagcgggacaccctttaataaggcgtatacgcttagctaaccgattgatactgtctacgttaaacatgactagtccttgacgttaaacgtcagcgagaagctcttcgtagcacttacctacattcatgtcatgataatcttgttcagtgagatcctgaccagaatcatatttcatgaacgcgtgcaagtatgcagttgaaacagagcgagtgttaaagaacttggcatataccaagaacttatcgaggtcttctttaggatcgatactacttactgcaaaataagaaaggtctcgtcctggaagagtctgctcgaagcgatagattgctatcgatttgtttttgtcaccatcacggtaaccacactcaaggagtacattggtttgaatattcatggtaatttccttttacataggtagttttatcacatttgtaatatagggtttaaaatgctttaaatgtaagacaacataaagcctcccagaagggaggcgtttatattaacacgatgctcttaggacatacgatgaactaccaactatagccttcaacagggagcgccagagttgtccatttaaaccttctaggagctccaccttaacaccttcttcccattctactacaaggacacgtgtttcattgatcgccaccgtaaagagcgttttagacctaatatgaggtacttctatacgtagatcccccaacaacaatctcgcttgctctttaaacacatattcaaaccgactagtgatggctgaaagatcatgtcggtaatgtggtataagtaggtaatagaagttatcgaagataatctccagcaactctactctctctttttcggtcatttgatagactccaaacagattaccttgtactcacttgataactacgttcttgttataagcttcaggtacggtgatattagttgggttaataacaactacttctgcattattgaaagcaccatgagtagactggaagtggctgataaagaacacttgtttaaattgaccgttctcgataagacgagagataaacggaattaagtttgcgcggtgttgttcatcaaacgtacgaccaaattcatcaagatacaatggcatgtcttcaagaccgaggaacttcagaatagccatcttgaatgcaaagttaacgatttccaattgactatcggaaccatacgaaatgtcaggtgccattacttgaccacctgctactttgagagggaagttgtagtctaactcctccttttcaactttagaaggtagtacttccattgggtatgtccacacctcgtcaatgaatgcattgacaatgtaagtaacaccctgcaagaagccaagcatatatcgacccaacaatccaccgtttggagataacgacttaattagaataccaagatcgctatgtacttcagtagcatttgttacttcgttttcaagcgtacgtatggtcgtttcacgttgttccatctgtgtgagctgtcgcgttgtttcagcgagttttacctggatggttcctatctcttcagtataggctctatcaagcaaatactccgaatgacgctctactttatctttccacatttcataacggtccaggacatcatggatacgtttattgttacgtagaatagattgttcaccagaccgtagatcttgcatgtactgattgatatctgaagctttaacatacatgatgttaatttcagtttccaattcttcggcgcggcgtttcatataaccgattgcatcttggtctatctcagcgataactttaagacgtttctcgatattagtagcaagctctagttcagtacgggatttgacataactccgcatggctgtatgccattgcaaagcatcagtcttatgcaatgcaggagtccgatacattgtcatgttagttgcacagtaatcccacagttcattaaactctgggtagtcttttgtcaaagacatgtactggaaaacataacttgaatagtcctggaatttctcaagatattcttcgttctctttttgttctgcttcgatacgatcaatagcttcgtggagtttaactttagaagcttcaagcatatccgtttcagatggatctacgccaggtttaaattcatgggtacaagatggacataccacagattcacaacctttcaaacgcgacaacctggaattagcctgctcgattttatctgagacttgtgcgtaaatattcctaagctctttctgacggttctgtcgtttggttgcttcttcccgattcatccaaccgtcaccgttatcagggaaactagttaacagatcaaaccatcggtcgaacattccatccaacttacaaataggatcagcaccggctgtattaaacttaataattggaaattgaccagtataagttttcatcgagttaatacacgattcaacattcgccagattcgcagcatgctgttgtttcaatgcattaacatcatcttccgatatttcaatcgccgatggagagttagtacgaagcttttctagttcttctgcaagacgattaatcactgcattgatcgaagagtattgctccgatacccgattgaattctgcctggaattctccatggttagctacacgaatagcggccggtaacattggataatcacgtaggcaagcgcgtgcatcattcagaatagattcgagttcgttttcagcttgttgcacattctggaaagcaggtcgaacatcattttgcttttcttggaagagtttattcaaacgcttagtaagacgagaggtctcttcgcgcatcagtgtcatttcactatcactaaagatatcgtgattttcagtgactaggcgttttgtgattagatcgatgacacctttctgactgcgatgttcctgtttaatgtctctgtatacatctaacgcataagtcaaatcaacagttgacatccgcgtaagaatctcgcggcgctttgctgtagacatagcggtaaatttaactcgaccagttgcaatctcatggatttcacgcgtaagtccaaactcttgtagacagagttcttcttggattttatatgtaccgccgctattcaactcttcattatcccgtttgaaagagtgacgaccagtaccatgaccatataccgaatgaagtacataaaggcttccattatggtagcaatggaattctttaaaaccatctttatcaaagtttgtatgtcgagatggcaatggagttagttcatccataactgacgatttacccgaaccattagaaccgagtataatcatcatgttcttagtgggggtccattcgaagaattggatatttgccgtcataagtcgtttgaattttttcaaacgcagtagagtgatttgcattggtaagcccttaaaatcgtacgttaccctatagaactaaggttaccagtaattattcagaggaacatatggaagcttcaattttcaaattagtaagtattggtagagtagctgcaaacaaagaacgttcttcaaggcatgtggacgttttacctgtagagcttgccactggtactgatggtgaagtaacgtttgacccattgcaggaaacactacaaggtttcgatgccgagggtaatcagtataatgttaaagctactacaactagaacgactaactgtgaatggctaccgaacgaagacaaccgtgttactccaccagatgtacgtcgtaacgagatcgtagagatttggcgaatgggagacaccgatcagtactattggcggtgtatgggtcttcgtaacaatcttcgtacattagaatccgttgtatttgcatggaatgcttcgcccaaacctggtggtggtggtatcgattttagcacgtgttatttcatggctatatcagcacatgacaaacactggacaatcggtacatctaaagcaaatggagaacctttcgcatacacattccaaatcaatactgattatggcgcagtctatattaaagacgatgttggtcagcttatagaacttgattcaactgaacgacgtgtacaattaataaactcggacaactcttttgttaaggtagaacggcaatggatcgaaatgtctgcggatgatcatatcaaaatgaccgtgggcggaacaactcttgagctgcgaccagattcgattaacagtaatacgtctaatactacactaacgagtagtgggacacatacaactgtggcgggtcacattatcgaacaaactggaagatgggatattgtctaatgcctggtatagctgtttgtaatatagattctgctggtggaacaataagaccaagtggtaattcaactggcttctataaaggtaatccaattgctgtattaggtgatcccgtagatggtcatgggcgatccccacataacagcgcaaacatggtacaagcttcaacgaaagcttttattaaaggcgtgccaattgttctgcaaggaatgtccgctagctgtggtcatactgcaaccggtagacccgatgcgactagtagcggttgacaacataaagcccctaccattcggtaggggctttatgccgttatacgccttcagcttcgtaatgcttgatgcaatgactaatgaaagtcaaatacacattaagcgatacagccagccagtgagtatagaaacccattggttcagctaacttcttcgaaatctcgccgataatagagagaacagaattataggatttacctgcctcttcacccgcttcagcgatctgtcgaatagcgtcgtctacaactactttgaccgtggagaagtcccgctgacccgtttcagctttctctgctagagaaaggatgctggagatcaactgagtgatctcactaagagtacggacagaaggtacatcaatctcacgttcagaacggtcagctacatttagctgtagctcagcgaactgcattgtaaacgaacgtcttacaacatcctcattagcgactttactattattcaacatctgactgataacgtcaggtggtgtatagatgaacgctacgttgccaggtaggacaaccgaacgatggacacctttttccgcagtagtcagttctctctgttggagaggggcatgaccaggcggaggggtaaaatcacgttggaggatatttgcaaatgcttctacaacctcaccagctacttcattagagctagcatccttagatttatccaagatattcaggaactgtcgagaactgttccgtgcaatctttgcaaccgatttaggataatggttgagaatgtagttggttagatctttgatgtcgttcaagtggttaaggtctaaccccacgaagttaccatcaatagatagacgttgtacaccagctacagacattttctggtaagtagttgccgagcctagtttacctaagcgtcgactaatgctttcttgtgtgcgacgaacacgacgaatgctaccggtgaatttgacgtagaaagagttaagcaattcccagatgtagcggacaatatcgcgggtggctttcgccgccgcgataatgccttctttgattgctctcagagtaattttagaaccttctttgatatcaaagtcagggtcaatactctcaagggctaccgagataacatcagcagtagcccctgttacaacgtcacgtccagctagcagatcgcggtagcgctctagagaagaaccaagacgctgaatcttactcaggtcttcagatacttcattccattgtgccagataggacatgctttcacccttaggctttctcgccttcgataacatcaccatgttcagctttcagcatggcttcaataacagcgatttcagctttaaccaggttcaggcaataacctgtaaacagatggttagcattagcagtttgacgagccagagtaatggcaagcagactggaaatagccgagttctcatcaccggtcatcagtgcaccaaacaggaagctagatcctttctggttaacccgttgggcgagttcattcagcttgctacgaccttcaacagctgcttcaactttattgatcagttgctcggtagcgcgaataacagaaactgcttcaccagcagacatcgttttgatggtatcggcaccaccatagctatcgccacccggaataaccgagaagttgatattaatagcgttgttgaagttgaaagtcttatcggctgcgtaatcggtgttcacaccaacgaacattgcacggttacccggaagaacttcggacatatgaaccgaggtgctattcaacataccactcggaactttatctttctcgttggaattaacgttcttgaatccacggaaggagttagacagaatgtcatcgatcgcatcgagcatttcaggagcgagaccgctttgaacgccgaagtagtaagtagatttatcatcaaacttcttcagaatttcagcaagtttgctcggccagttgatgagaacgatatcagcggtattctcaacacgcttaatagcttcaggactatcgccaacgaattctttaccaatggacagacgttgcagaccaccaatcttaatctgcttaccaccatcaagagtacctactttactacggagagtacgcagacgttctttcagtttggtagcatcttgagtaaaggagcgccagaagtccatcaatgcgttgaagatacgcatcagaacattacgggctgcttccagcaaagacttcatcttagcagtgagtttgctttcagtagcatcgcgagcagaagtatgcttatcgctgtcgtcaagttcttcaacggataccacggtatcagagaagaaatcaggatcaatcatttccagaccgacacgcatcgactcagccagctcgttagtaacttcatagccgttttcacgcatgccacgcaggataccaagataacgctcaacggaagctttggcgttttcaatgtcgcccatatccgaagcaatctcgtttacaacggcacctttggcatcagtagcggatgtaaggccatcggcagtaagagcttcaacagcttcatcgatgtcctgcaccatgtcgtcagcttcgccaacggattcagtttcaccagattcgatggtatcgagaccatcagtgtgttcttctacagaagtagtggtagcgacgttatcatcgtcagccgatacttcgtcatgtgcagaaccaacatccccaagaccagtttggtcaacggcggttacgtgattctcaacggtgtccgaagtatgaacattggtcacatctacagtttcggcagtaccatcgccaccaccttcagtgggacctggttcactagtctgtgtgttagtgaccgaagcatcaacatcatcagcatcaggcttttcgccctcatcactcttcagttgaggttcgagatctttcttgccttccagatccacgttctgatcggaggcttcagtgacagtaccagcagctttgttctctacttcttcagtaatggattcgttagagatgctacggcacagatcgaaaaggttagcgcgggccatttatatactccacaattgcgggggatttcgtgagtttaaactacataaggttgttaaggcagcaggttgttatccttgatgattttctcaagaataaggttctgttgctttaaaatagagttggcattttccagttcaagtagacgagcataatccgtcgtacgattcttgatcttaccttgtcgtgctgcctcacgtgtttcgtggacggctggtgttacagcatctgacaacggcataatgccaaagtggacttctggattaacaccgatcgtatcactaactgcattcgcagcagcattagcggctgtatctagaattacgtcatctggcaatgcaccaagcgacagagtcatgatgacttggttgtatggcttagagctaagatcaggataagatttgatgtagctcgatggtacataaacaggtgggaatttaggtgacagcaacgttacgattacatgaccttgctgtcgatctgtcgcgacgcgtgactcgtcgattttccaaggcttgtaataaaggtcataaactgaacgaccattattttctacatcctcgaagtagcggatagcaccgcattcgtaaagttcagctgcttccaatactttatcaaacggaggtagaagaacatatagtccctttgtaccaattggagggaccattaaattgttagtggccatgtatcatactcactattgaattgtcatgtaattggtaatgaaagtaaagagtggctcggttaaccgagccacattcttagtattgacgctctatcagttctgataattgccagtaatatttgttagtccacttatcaataaacaatgtcactctgatggcttcacctgattcaaaataataggtgccatctggagtgagacttggataattagaacgtagacgatgataatcaccattactgtcttcgtagagtacacaacctccacttatgatacctgtcggaaagacgatatcacatgcagtaccagaaacataatcgctatcgtattttaaaacaataccgatgtcatattccctaccttcatctgagggattaccaagtataagaatagtatcgacgtatttagaaacatcgatcttgttaacggccattgtgtaaccgtcataactaaactgctcagggtaatcagtgatcagaagctggtttggtgattcaacaaagttccagcaattaattggattaatgtccatataacacctacatgttgttgaattcgtaatgtggtccacgcatgatccatcgaataatcggtgtatcttcatcaatccagactacacgtagaatctcaactccgttaccaggttggataactagttgaataccattccgtttaccaagccatctctctgggacgttgaatatgatcgaacgttcgctatggttgaaaactttaaatcggacacgctggtcagcaggcatatctggagtatccaggtagaagataaacgcgtcattataatttccattagctttatctttaccatcgaaagtaccaccggttaaaatcagtgtactactcaaaatatcctttctattgcttacagtctctccacctgcgccggcaccagaaagatccatggtgatgatctctggccaactaacacacatcgtagccatcattcctccttaaacaagagtttcataagtacgaccttgaccattgttgtatagccacgcgatctcttctttctctagcggtcgccagcataatccaacttcatctacagcaccatcaaacttggaatcactaaagatttctccgaactgtagaccatcataagaaccactacttggtaatggaatttctttacgtatcggattaccattgtcaacatagatctcaaggaatcgatcttttacttgaagaacgatgaattgccattctcctttacccatgtgttgaccgccagtagatacagtagtctctgtgttagcagcattgcgagagaatcctctccagccgttggaacctctgtacgataagccgtacttacagccatagtactcgccaaacttaccaagagtcaatacatattcctgacttacggttgggttatttactttaaaccaaccaaacattgccgtaccgctattatagctaccgaagttaccttcagcaccggaagcttttataccacttagtgcttgaccaactttaccaggtatcgtactttcagagttaaatccgaagttatgaccgccgtgtgagtctgtagcaatcccttccatggcataccaactaatcaagtcatccatgatagaactacctacagttttaccttgaacaatatccccagaaattgcccaaatccattgattggtattattatcccaaccgatggcagtaccacgaatagtcccaccctgtttaactgcgattacattccacgcaggcaagaggaatttattatgactaagtccctctggatcaaatgtgatctcatgtccggagttattgataataatccattcatgtccaggtacaagtgtagctggatcattttcatggtaggtaggccagttcagtgtaggtaccttctcaccctcaggaattggttcgagtacataaacacggttaccattctgttgtacactaagagatacatagtaacctgggttaccaaatgtaccagtaatgtaattagagatcgaaccttcgaagatatgttcatagaacccatctgtaggttcaggctctggaccaggaccatctccacctgaatgtaaccaaagaactagttcgccggtaaaatacagtgagttgtaaatagactttaataaccagttaggtccgacttgtccaccggtataatcgatagaagtatcgttaacccaaatatctgattttgttaaattcaaagtcgatttacgagccacttcaccaaggacttcagtagagttctccatctgttggagttcttcaacttcagaagccgtccagtatggattctcaataaaatcgtttaggttaaatcgatcgtaataaaaatcgtaaatagtgtcataagaagttcccttctgaataaacactactgtctggttgggtctttctttagttgctgctggttgtactctaataacccgagagtttgcttgggtcagacctaggctggaatatttagcgttaatcgctttataaagtccaactaatggactagcaccgatagggttatcggcaagtgaaatagaaatttgacgcatgtgtatcccctaataaaaggagagggtttcccctctcccttatgtttttaggataattcttctacgctagctttagctacaaccatgtagttaacgttcttaaagtatgcgcttgcataaatcacattatcacgaatcatgcgagacaccccttgtggaacagagctatagcgagtcatcccttcggctgctttcagtagcttcgagaacaacatcatccattcaattgtttcaggcgacgatttattgatatccccagtatcgttagttactaactgataatctttaaatttctgcgagaactgtgtaataccattcctgttttgagggttacccaatacggagaaggcaatggatttgtatgtgttcgaagacagctcgaatttattgtctacgtaggtttgagtataacctggcccacgtgctgttcgacgaatcaaaggaagtcgtttacgatggtctacagtaggactgtaggtaccagctcgataatcggcttgttcgatagaatactggttccagaatggagtaaagatgaactcagttgtcatgaacaggtctggaagaataacttcccaatctgtccgtggatgtgcagagtcagccagtagttcttctacaatcttgtctttgatgaggtcagggttgttgccagcctcgccatagacgattgcaatccaataggcggggaaacgcatagaatcatcacggggattatggtattcaaacatgaatgcccgttgatgtgtatatggatattgtgcccgcttagcctgaacttcttcgatcttctcaacgagatcataatcgtccagtagctgcttaacaataagcggatctttaaagaaatcgtcatacggaattatcggatgtacgatctcgatgatgtattcatcgtactgagctgcaaaggattcatctgcaagccagatattcatctggttagcttcagaaccaactaatacgaattcaacccattctggcatccaaatgctaccgttagaaatcatttgaccactacggaaactttggataaccccattaaactctgccatcaccagttgacgaagtacgttaggatcggaaccgatcgtaccagaaatcgactgttgataaatatattcacctagcttaagaacttgatctttgttgttaccagcaacatcaacaacgtttccatcctttacgctatgaaaagaaataaaaacaacgtttggtgcggacgtaccggtgtggaaagtcttgtcctttgcataggttgcgctgttcgacgaaagttcgccgagcttcgctacagtttcaggtgcattcgaaatgagtgcagggaagctgtaaaagcctttcaaattgtacatgtgctatcctcatgagcgagagatcgatggtcttccatctataaaatcagtcactccgcttgtgcttatttaaaacgtcgggtatactaatgcttttaaacggttagtatattgtctttaatgtctattgatctcagccatccacggcttttatgggtaggcgcaatgtctaactgaacagaggaaatcatgctcagtttaactgcaaaagccttgctcctgttgtggcccttcctgaaacgggcgatcttcggtgatcgtactgtccgtgaagtgatgctggaaaacaagcacgttacgtttatgtttgcgatggtactggtcttggccatgtcgctcatgttaactatcggcgagttgaatgatgttaagtcagagaactggaagttgaaacaacgtccggaatgtgtatgcgatgtagactctgtcgaatcgcttcaagccaggcgaaagcttctgggtgaaattctgaaataacctttaatgggctgtaggtgaaccacatgtctaaaaaatatttactagtactttgtttgactctttctggttgcgttatttatgcaccgaggtacaccacacagactgtggttcagcaagagacaacttccagctgggaatttagccagccgcaaattaaaacaataacggaagtgaaagaacgagttatacaaacacctgtcacagaacaaaagcgtccgttagcaagctgtgaaccgtttgtactcccacgtgctgctttactccccgagaaaccgaacgaagaagaattagcgagtgcgcagtcttcagaagaaatcgatcggaaactctcggagtatgtagccgaacttcgtgcgtacaatgttgccgaacgatccaagatagagcaagcccaccaaaagtggttggatcactgtcaaagaaaactcgactgatttatactttagttaagagtctgttgacagaggtaaaaaacaatgtgcgacggtatagtgctatacacagatggatcattccgtcaaggtctagctggttggggagtccatggttacacttacaccaatacaccgatgaagtctaaagctgctacaaaacagcagccaactgcatcgggttatcaggatgtcggtgccgaggatacttgtacggttattgaatatatcgactccttcggtaaggtagtcgataatccgacgaacaacaccgctgagcttagtgcggcgattaacggctttaagattgcagatgcctctaaggctactaaactaaccatgcttatggatagtgagtatgtcagaaaaggtctcgaatcttatctcccaaaatggataaaaaacaattgggttaaggtagatggtaatcctgtagccaacaaagatctatggattgctctgaaccagcaaaagatggattggcttaagaacgaccgcaaactggaactcaaatgggttaaaggccattcgggagatataggcaacgagaaggctgacgtcaatgcgctacgcggaggcggtgcttcggttacacctaaaacagttaaggttgaaggcgatgccatcaacaagctgaaaaaagttcagatgaatccactgatcctggagtcccgtctgctctttggaattaatagtgggaaaccctcggatgggacctactacatgtacaacctcggaagtatgcataatgcgggccatcgtcctagggatactgccaaagataaattggccaaagcagatttgctacttgggagaaggatttccgaagcaacctttggagtctataaatctcgggaacctgacgagtatttagagaatctaattgagctacatacgaaagcatttgggactgacctcccagaactcggtattctcaatctgggtaatgcttgtggagcaaagcaacgccagcaaatcgaatcacttgggcttgatgctcttgtacgttttgatgacatctttgttcttgcaactccagatatgggtctcattagtaggactctcaacccaccacgtatggctaacgatgcggtaagcatgtttaacgtgctggaacgtcgtttggcggaatacacggcgggaacgataggagagtcggtttataaaatcgacattaccgatcacctgtatgaaactgtacagagcggtaagaagacggtaacccaacttaagaagtctatcactcaaaatacaccatatctcgatattcctatcgattataaaggacagaaggtatcactccgattggcattgacaatcgatattccttctcgtaaccaactcgctcgaatcagctgcgagggtgttaaagtggaagtactgattgtagctacgggtccgttagcctattcatactcgactgtgtttgtaactgatgatggttctgccatctatgaagcaccgtacacacagttcattttgaaaaaatagtgggtaactcatgagccttattagcagattcttgaggctggatgaaaatccattcaggacattctgggttttcatctggaatcacctggataacggcttcaaacggatgtgcgtaatggcgtcattgcatgccgcactggtgcagtgtcgcgatcacgaatgcgagcggatatcttcgcttaattcagtgatgcgtctcgtgagggatgaaagcgccttacgcttaccaacgttatttggaccttacgtttggaaaggtatcctccctatcgagaaggttgatcttgaatctgacaagtacttcgaaaggatcgctcgaaagactccctgctggcttctatatacagacaaggaaactttcgttaaagaacttaagcaattagtacaccattgcatgaaggaacgtcaggcgacagcttaacggcataaagccccaccattaggtggggcaatatgttgtcttacagagaacgaagatgtttctctgtttcagctaagacattattggtttcaataattcgtgtcatttgaatggagaaccactctacccacttagctacttgggttagttcctcagacatcatcttagcgaactcgctggatgttttgatatcgccttctttaccgatccgttccatcaaagcagttacggtttgacttaatgcttctactgcactcttaacggtagaggtttcaccacctttaagaatggtattaatctcgaacatatgttgttcagattcatagaagtcattcatcgaactgtaaatcttaccaaatgcaacagttgactggcggttattagcaaagaactgagcgtcttctttaataagctggtcaatcgatttatcaatatcgataccgtattggaagtctcgacgttctgcacgatcttctggagtagtcagataatgaccaaaacgagatgtcgcgggtcgaataaccttctctactacttgcgccattacctgtgcacgcgataccagaccagcggtatatggaagcatttcgcctttaaagccagctggttgcggaacaatttctttctcaacttcgaaataatccagagtagccacaaagcctttcatggatagaggattaagaggtagaagcggatcatagttccacgtagtcagataacggaaaccgtctttaatatgaactcccatattggatactttacgggcaaaccaattagaaacattaccaatgaaaccagcttcagtggaaattgtacccagagcatcgaatagtttgtctgtaggagtttgatctacaggaagaacttctgtttcaggggtttgctctgctgcttgaggatcaccctcagtgaagaacttattctgagaactatcaaagataacgtcatcagtctggacgttttcattggagaccttctcagtgtatttattaagaacatttttaatcatggttgttttcctatggcacaagagttgcgaattctctaaacataaaattactctcaatatcaataaagtgattggctaatcactaaaaggtaatatcaatgttcgctaaacacttccaacgtccggccttccgcccggcggttaatatcggctgcctgatggatgtatccactggtaaatatgaacaaggtaaacacggcgagatgatctgtaacggtggtctcggtccgatgaccggtatcgcatctcgacctaacaactttaaaactgcactcgctgtgtatatgctagcgatggttcgtcgagctatgccgggttcccatggcatgatctatgataccgagggtaccttgaacccggttgcacgtttcagtagtcttgcagctcaattcagtgatctgcaaaagatcgattgggaacatgatgaacaattcatgttcactgacctttctcgatataccggcgatgagttctttaaactcttccgtacagcacttggtgagaaagagaaagcagaaaaagaatatcagcgcactactccgttccttgatgttgaaggtaacaacaagaaatgcatgtacccgacaactggcctgatcgatagtttctcgaagtttatcgttactgccgtatcggatatgtacgagaagaatgctatcggtgcatctggtaacaacaccgatgccatgactaatggtaaggctaagaaccagctgttcaaccaattgcctcaggtatgtgctaagaccggtacttatatcgtactgactgcgcacactggtgacatcatccaaatggagatgtacccgactgataaacgtaatctttcccacatgaagaaggatacggttcttaaaggcgttagttctggcttctattcgctgcctaacaacgtattctctatcgagtctaacaaacctcttgttaacaaagagaagatgcctctgtatccgatcgataactcgaccgcaatggaaggggataccgatcttaagattctggaggtaatgaaccttcgtggtaaaggtggtattactggccttcctttccatatcgtagtttctcagactgaaggtgtacttccttcgctcactgagttccattactgcaaagaaaatggttggggtattggtggtaaccttctgaactactacattgaactttgcccagatatcaagcttagtcgtaccactgtacgtaagaagcttatggaaaacgaatcccttcgtcgggctgttgaaattcaatctgagatgcttcagttgatccagttccagcgttggacggctgaagatgtatgtgatccaaagacactgtacgaagatctgaaagcgatgggttatgattgggatatgatcctgaatacgactcgtggctattggatgtgtgaagaagacgaagctctcaccgataagaaattcctttcgacctacgatcttcttcgtatgcgtaccggtgactataaaccttactggatgactgatgatgaacgtgctaagattattccgttggatctggccaaagcgaaagctgcctaaagaaggagttgtgatcgttgaacctatccctgccgagcgcggggatttgggtaaatgcgaacagatctctttggcacgcgaagccgttgaaatgggcagtgaaaaatatagatccactttatctgacccagcaaaagaatggtacgagcactatagagcaaacgaatcaaaacaggttcaacctttaaggatcccagaaggccgtggttacgcttctggtagaggagccgaggatatggacctgtccaacacaatcttcgctgtaggagctgctgtggccctttctagcgatactaccgatagtggttcaagtagcgatagcagttgttgtgattaatatcatagacgggagcattagctccctctatgtcaagtaggtattccaatgaacgtctatacttatcaaatcgctaaatggcgaaaggttagacagaaacatatctttcctttggatacaactataaaaagtggtgaggaattacttgcccctacctggaatatggtaatgggacataaagccggtgccattacagatgagcaatatgaggatgcgtatatggacatcctctctgaacgatacgctgcattcccagattacttcgaatggctgactgagttggacaaggttgcactaggatgttactgtccagctggtaagttttgccatcgacacattctcgttaaatttttaaaagaaataactgaggtaaactacctaggcgaaatagagtagttacccgatcaggaaacaaattatgtctaataccatcgattatcgcgctgttatttttcagcgtacccgtgctcttgatgtagaggttgctgaagatctgtatagacgcatgcccgaaatcaaggatcttgcaactcttaatcaattcttccatctgttgttggctcaatacaaaatcaacaccctggaattacgttgtaccctaaatgaagtgaatgattttgaagcatggtggcgtaacttcgctgctaatttcattccgttgttccgtaaaaagcggttacctccatgtacagacgctgctgcacagccaatgtatcactgcgagtctaaatcaatctgagtaatcgtatgctcatttgatttgtagaggtaactatgaaacccgatcgtaaagtccttgaaaaagaaattctatacttcatcgacatgttccgaccaggaagcgagaacgttaaaatctatcaagaactttttgaccgttattctgacgaagagttttttgaatggatggaacgtctagaggcaggtgaagtgctggctctctacgctcctaacttagaagaaccaactctaagtatcgctcagaattataaagtagctgatgctcttggttttgaactattccaacaccttatcttaactgatccgggcactggtcaagtttataagactcagaataaacacctagttggtatggttccgcttcgtcggcaggttcagatgctagctaagaaagcttctatcccaggttctaatactgttgttgacgagcgttctggacaggcaactggtgatagtaaaggtgcacgtctatctgcccctgagattcaggttaacgcctctaaaggtcttaacaacatggttctcgaactgattaagtttcgtggtggtgatgaaaaggcatataacgctatgaatcgatccatcattgaaacaggtgaagcttctctcgattccattatggtcgagacgccttctcaagttaaatctaacaaaaccatgtccgtctatttgaaggccatgcatttacagaataacctagtggggtaatcatggctattaagaatgcggaagaaggtattagcgaagtattgcagaatgcattaggtgttgcaattagtgaattggtatctgttgatgatgatctcgttattgctcaaattctagagcatattaacgaacttagaaacaatatgatgatttctagttttaatgatagagttatcattaatcagatttggtcaggtatccgttctaagcaggatgtattgggtgctcttctgtctaccaccactacattcactttagaaattgaaaacattgatgtagcaattgagtatctcactagacgcttggttccattcacacctgattcagcaatggtcgatagggagttactgggtaaagcagctaatgtagatgaactctatggtacgctacagcaaaatcactggttgttcttccttgtatatgcatctacgcaacttcgccatgtaaataacattattgcacaggcgaaaatgaaatgatcaaacgtattctgatacctcttgatgtattacttgacacccgtcttggagtcatgtctacaattaacaaggaggcagcagaacggttggtttccactaaggaatattggcttcgtgaaaatgatgactggaccactctaacaggtggtcttgttacaacggagcaattcaaagaagcgtatgctaatagaggcggagataattccgctgatactatcaacgcttctatcctaacaggtatcagtccgttcttgatgcgaattctcgcggaagatcatgtaaacagaatggataacatgggtaatcctgaagacgagattggtcttacgatcaacatctggccttacacgttacctggtgaagttatcgatgatcttgaaaatatcatccaagaaatatacggcgaagaaatgcccgtggaagtagttagtcatccattagaagagctcacacctaaattcttggatgctctctatgcgatgtatatcacttacgatttccatgaatggatgcacactcattatcttgctttgtctaaagttcaaatgccatgcttcaattttattggacctaaactcttcgaacgtgacgttagtaaactcactatcgaggagaagaagtttgaactatttaagttcagggtcgagcggctgattcacatggactttgaatttatagatgctaaatatttctccatgattcgtcctggagataacggtatcgaagttgataaagacgacataaaagcccagggttaaccctgggctttatgccgctattattagtagccagcacctttagcgccgagccattcactaccatcccacagaagggtgatgacagtcttggttgcagcagcttcaggagccgtgttatcattccatttgaagttaccgctgaaggtcggaatgaccgtaccagttagaaccagtacagctgtaatcattcggccagacggaccatcacctagagtgatagtacgagcagcagtagatggaacagtatagcactgttggttagccggagtgatggtgaagttaccagcaggagcagcaccagatagcagggagtaggtatcaaattctttcttgatctctacccacgccgatgtaccagcagcagttgtctgacgaccccaaactttagtagcatcgatacctggttccggaatggttaccagttctttccactcaccgttagaacgagtgtagttcttggcatccggagcatccgatgcgataattgcagccggtacctctacccagctggacacgccagcaacagtagttttacgagcgtacagtttatcatcattggtagtttcaggtactaccgcagcccaagcaccatccttacgagcgtaagacttaccatcgctagccgcgtctttaaagacatcggtttcgacccagctagccttacccttcagaacgtaatgcttatcaacatcgttggcaatgacaataggtgcaccttgtttccactcaccgtccttacgaaccattgcaagagcaatgttgggagtaggaacgtctggtacagcatctacttcaagcggagcccattcggtggtgccatcagctttacccttacggatatactgttcaccttcttcaggggtttccacttcatcgaccagtagaggtgcccagccaagttgatagcgaaccatcttcttgttctgatcggcagtttctacttcggctacaggaacatccagaagttggatgaattctttccagccagttgcgtcacgataccaaactttaccagacttatcaaggcaccagtcatcttgagtaccaatagtgttattcgggatatcgacaccgttcggtagaattacccaacgagaacctttatcaccttttgcaccttgaataccgcgaggaccaacaataccttggtcacccttatcacctttttcgcctttggcgccaacggtgaagctacccaggttcagatacttctcagtatcatcagcaccatcgacagcccaaacaaacagttctttactgttttcaggaccaaccgaatatgcatcaccaatagcactagtcggatgagcagctgtaagagcagcttcagacggatagtcgccaacaattttgataccttggccgatttcaccgcgaggacctacttcaccctgcggaccatcgttaccttgcggaccctggatattgaacggaccatcgtaggtattcgtagagcggttagctacgtagattaccttaatggtgtcatcaccctggataacggtaacaatgtacgcctcgccatcagcgggatcagtttcaccggctaccagttcaggtagagcttcaacagaacctacttcaccaacgatgcgcatcgaggcgccacgatcaccctgatcacctttctggccaatgggaccaacagatacgaactgagtaccactaatgtttacataaacatcgccgcctttaacaacaacggctttacctttgttgtcggcagtggccggaggaacttcacctacagtgtcaacaacagcgatgatttcaaagttttcaccctgatcacctttgtcgcctttatcaccagtgtcacccttggcgccagtatcacccttatcgcccttgtcccctttatcgcctttggcgccagtatgagtaccaaggtcaacccatgttccatcaatgaacatgtagaggtggcggttatcggcagctacccaagcttcctgttcttgcggatcaggtacggcttgaatggcagcaaggtcaggaagaacaccggagacaaccaggttcttaccaccgtcaccggtgtcacccttatcaccttttgcaccggtatcccctttgtcacctttatcccctttgtcgcccttctcacctttgaattgacctaggttaatcaggtcgccttcagaggtaacaggagtagtagctacgtagaagagggtgttaacatcgcgaacagcgtaagctttcttgatgacaagagtagcacctgcggccagaagatctgccatggtcggatacgtaccgaggatttccaggttttcaccaggagcaccgtcttgaccatcgataccatcttgaccaggatcgcctttatcacccttatcgcctttgtcccctttcgggccgtcgccaccgatgataccgtcttgaccaggttcacctttcgggccctgccaagtaccgagatccatccagcggttttcatcgacggagaagacgaatagatggcgtacatcgtcaaccataaccgaatatgcttcttcaggcttggcatcgccagccagaggcagatcatcttcggaagctaagtcagctttaatagtgaacggagtagcgtccttaccaggtgcaccagtgtcacctttcagaccacggtcgcctttatcacctttggcaccagtatcacctttaggaccctcaggacccatcggcacgatctggatgtatgcatagttgtcagggaagatatcttcttcaccagctacaagcatgaaagtgtaaagagcatttttccaaccgtaggtatcgcctttggcagccaagggcggaagttcttggttatcaggccattgaccacgaataacgagaccagtaccttccggaccacgcatgtcaccggagtcgatccactggccagcatccggcgaaccggtttctggggcagaccatactttcagtacagtagcagtggaagaacgaacgaaccaagcatcaccaaattcccaactatcgatgggagcaatgttggtttcgaaatcgtcaagagttacggtacctttgatattggtaacgggacccggttcaccaggattaccttgcagaccagtatcacctttagcgccgtcttcgcctttcagcgattcgagccactcggcttcagtaccaataaagccagcttcgagtgccagctgataagcggatttaccatccgcgccatcctcacctttcattccctcgatttcggtcgggtctttgaaagttgtagccaggccagccccggtcgaaaccgggatcttgcctgcaactatctcaagaggattgtcttcggtggagatacgttttggtaactcaccgttaacgaaaacttcaaatgcggattcaccagccattatacaacttcctcaagttcgacgcgcatcagaccggatgtgttagatacagcgttagctgcgtcgcagttataccaactattgctattcttgatggtgtaagtatttacagcatcagcatcgtcagctttataggtgaagttaagagaaccgctagcacccttagacaggttagtgcagcgaagtttaccagtcataactacatctgtaccaatagcaccttcacgattcgggaaagcagcgatagacatggtacgaagaacgaagccaccaagggtatactcgccaccagctttaagggtattgactgtaacgccagccagacctttggctacaacatcggtaaagttgaagatacctttagcatcatcatcatgaacgagcagtgtgcgtgtccatactttcttagctgcatcacccacccaaccagcagaatcccagttaccgccaggagcagtcatcacaggggcttcagccagcgattgagtcgaagtgatagtgatggtgtgacgctgtacaacagtacctgcattaccaccagagcgcagacgagtggcaggagtggtaacagtcagttcaggggcaccgttagcaatcttaacgattgtcgatgcagtagacgaactaccgttagcagcacgttgcgcagtgattgtcaggttattagtcaggtcgttgtaattaccagtcaggtaagaaacagttttgtttgcttcaatctgagtcgggttagttacagtcagctgaccattagccgaggtgtaagtagcgctagtagcgttagttacagtgttagcaacggttgcatcttcaccagctttaatggcagtttgaccagccggataagttacagcaccgaatgtaatcgtcggtttcaggttgttcagcttgacaacgttgactttctcagtagtaccagctacgtcggacttataccacgcggagaaactaccggaggctttcttaacgcggatactgaacggttggttagtagcagtgttaccacggtcagcaataaccagaccagtcagactgtgagtcttaccagcagtcagtgtaccattgcgtgctacgaatgcaccttcatcacgaatctcataacctaccacatcttggtcagtggtgaaagtgatcgacattgtgtcgcctgctttcagctcggtttgagaaccaggatattcacctgtaaatgtagccgcagttacaaccggcgcggtatccatgattacatcagtagatgccttagcaccatcttcgtgaacagcttcgaccttaatgggatcactaccaaccggctcaggcagattaatagttacttcaccggtccacatcggggcatttgcaccagcgacgagagatacatctacgccgttaactttaacgacaggacgatagttagtatgaccggtaatagcagccactttaactttaacgtcacgagtagacgaagaacattgcaccagagagaaactatccgcggacttaaccttctcaccgacgttatcagcggcattaaccggagtgatatcagtgatgaatacgccaccatttacacctttcggttcggcaagcgacaggttaaattcttcttcagtaccaacgtatccaccatcaacagcggattcgtatgcggacttaccattagcgccttctaggctttccagccattgttcttcagtaccaacgaaaccattatcacgagcgatctgataagcagacttaccatcagctccgtgtaggctttcgagatattcttcttcagtaccaacgaaaccggctgctacggctagctcgtaagcagatttgccgtcagcgccatcgataccgtcatcacctttagtaccgtcgataccgtggagagattccaggtactcagcttcggttccagtgaaaccagcttcgacagctagatcgtaagcggacttaccttgatcaccctggtcgcctttgtcacccttatcacctttctcgccggcatcgcctttgtcaccttttagggactggatgaactcggcctcggtaccggtaaaaccagtatcaagagcggattgataggcagacttaccgacgagagttgcaaggaattcttgttcagtgccagtgaagccgttatctacggcaacttcatagatggatttacctacagcgccatctgcgccgtcttcacctttaagagaggcgaggaattcgtcttcagtacctacgaagccctgttgaagagccagctgataaataccttgaccttttagactttcgagccactcagtttcagtgcctacgaaaccattctttaccgcaacttcataagccgataggccttcattgttacggattttagaaaccatgagacggaagttcttataagaaccatctgcctcaagacggataacttctacaaactcttcacctgtgatggtgttaagaggctgcattccggagatcatacccggactggatttaatggccattacgtattcctttgttggagagagtcttcgcaactactcgtgcacgtcttaaaaggaaaataagactcatagagtagtgtattattttagcaacatataggagtcccaaaggggactccagtatgccttttcaggagagcatctatctggagttgcgactattttatttacgccacaacggctggatcgagtttccaagaaccattttcgtctttggtaaaaccaatggcgtccagaagtgcatgaatacctttagcagtagcaaagcctgtatcatcctcaccagcaatgacagcagcttcatcaaccttagtcggaatatccagttcaggaagctgttctattttcagtttaccgtcctcatcgagatctgctttcttagcaagagcatcaaccagtccagtaactttatcgatagcaatacctgcatcgatgatgacttgtacttcagcggcagttagaccaccgatctgagcaccaccgacagtaacgccatcgtgaacataaagcttcttattctcaagatctacaaagaacgttccttctttgcctgtccaagctgccgcttctagagcagagccgcgatgatgttgtagaagcagttcactgacttctgtggcacgcccttcatcgaacgatacttctttaccatcttcagaaacaactacaccgatttgttgtagagtggacataaccgcactcggtgcatctttgatgtaaagctttcgatcaagttctttcttctgctgacgagaaataggtttatcagcatctgctgtattatcgaccttatctaagtttgcaaacgaaaggtcaattactttccactctggaagacctagttcatttacagtgagtaccataccagcgttttctggaaggatctcaaatagaggattggttgcagaaacccattgttcttcagtgccttcataaccctgatcaactgcgatttgatacgcagattttccaacgagtgtttctaaccattcttcttcagtaccgacaaaaccagctttgacagcgccatcaaaagcagaagcgcctacacgtaatttatctgcgagtacacgatagttcttataagaaccttctgtatcgcgagcaacaacctctacgaattcctgtccggttagaccagacagaaaatcgagttcagaaacctttttcttttcttcagccatcatagatgtccttcaggattggctgcgttgcacatattcttttaacctgataataccaccttcaaacctggggaagtatcaggttaacaaaatccttttctaagtgttaccaccgttaaaagaacaggtggacgctatgcccgatgtttcgaaactttatcttcgaacagcttgtagatctctgcaagggtacgtggtacacctttattgctaaagatcgacgggtttgctttagcaggtttcgggaatagaacttcaccgagagttttctgatctgcggataggaatttcttagcgccgccagcaccaaggaaatgtgccaaatacaagtctgtatcactcggttcgcgattgattactggacgtaatacagctgcatttcctttaaggaattctgcacccattaatgcatttgcacgtgggtctttacggagtgccctagtgggatctttaggtatcccgtatttggaaccatgtgctttgatcatgtcatcccatgtagcatcaaggaactggaaccaaccagtagccgaagatgtggatgctttgacagtgtaatcaaaagcagactcaatggaagcgaatgtagcgagtaaccgagaatcggtaccagtcattgctccaaccgcattcagagtgggcattgcagccgaccgagatttattagctgttgggaaagggatagcttcccatttagcaggaacagtagcggatttggctagttcagctagagtagcaggtccaacttttccgtcaaccaccaaagctttagaagcttggaaatcacgaacagctttctctgtatctccaccgaagattccgtcagcgctaactgcgtatcctgcgactcgaagtttcatttgtagatcttccacagcagagccgcggtcgccacgtttgagtacagtacccatttgtctgtctccagtaattaatgttccagctcacgaatcaagccgtcttccattagacgataaccaccatcctcaagtagacgtgcatattggttaccttcaaccatttcgatcgtaacgatagtcgaaccgaagtaggcgtaactaccagtcattgcaacgagttcatattcgaatacgtcgtctttggtattaatgacagtggtagagaaggatagatcgtccggaccgaatgtcatcttacgggaacggttgatctcttctgcgatggccgcaggtgtagctacaccagatagtttaatagacggattaggtccaagacaatcagggtgagacaattccagacgacgataaacgaaccagtcttttagactagctttgttatcgatcatctcgatataagtacgccccggaacaccagaagtaggactgaagaacatatcttcgaagtttacaaactcgtcctgaatattcttgtgtttagacgtttcccgaatcaaacggcaaagtgccgcacgagacgggaggttataaggaaaacgatcgctcattgttaaaccctcaattgtggtttacaaaatttacttaacccacatagcattataaaagcccctccacttaaggaggggctaatattattgttactgagtagaaattaccatcttaatgatttcaataaggcccatacctaaagttttaaagatatcggctacttctgaagtcattggaccatcagtgttaataacactcatcactacaccagtggacagtatagctaacaaggcacttgcagttaaaatagaactgcggtaggtatcactagctcgaacaccagtgtattctttttcgagaagcttcgactgcttttcaagatcagaaagagaatagatctcagttaatacttcatcggcagttgtattcccattaacacgtgcactaccatctgcatgtaacataccgttcaagtatgctacgatttgacgatagttaggagctttcgacaaaggcttatcgccaaggtcacttaatattttttccagagtcatagcttctctccatctctgactgttttttatcccagtcacggagcttctcgatttgcaaattacacgaaccgagatagtcagtctgtaataaccagtgatctgtcatcaataggaaacgagcttcccatggatcagtgatcccagctactttataccgactaggtgcattgatgagatcgtcagctgacggtggaggagctacatagcaaagttgagtaaagctacttggtaccgcactgcgggtccagccgcttggctttgcagtagtgctcgtacatcctattagcaagggtgataagagcaacatcgtcagtaacactaccattatctttaatggcggcggtgggattcttccgaatagattcatcccgaattttttccacagggatattttctgtagtagaccacttgaccccagaattcccggataagttaatgtactcatcaatcactcctgctcgtgattgttccagctctctcagctcatcgactttttgagtggtatactgagtaacggtttcatcagtgatggcagctgacttaccctgcatttcgactttgacttctagttgaccatttttctcaactaaactgccattgtgtacaagctgatcagtatactggttatagaagaacaacagtccaagcccaccggtaataactataccgataaacacccaattaaaccacttgatgttttttaaccagttgaacatactacctcgcatctagaacaactgcgtaaggaaatagtaaccgattgctacagcatcgatggagtgttcatctagttgattatggtcaacatcaccccaaacaacatcgggtctacttaccaatgcacgtcgcacatcttctttgtctgtacccttaattttcttcatacccacgttggttttaactgttgtagggtcaaccatgtaaagcggtataaaagggtcatactcaaaaagagcacttcgtataacggcaacacattcaaccaatgcggcaaagcttgtggcaaatctacctagatagttagattcaacaataacagcatgtggtctatgtgtccttaagaagtctagtatcaaatctcgcatgatcattaatcggactacccgactaccatgcaattccccgaacattgaatagtccggatgagtatctctaagaacagaggtataggcggtcttcaccgccacaccttcattcttaaagccatgttccagcagcgcttgacccaagttagacgaacctgggtcgaacgaagcaacacggaatggttcatcgctttcaggcatctgcaacataaccaagtccttatacgaacttagctacgtttactgccttgtcgccaagagtaggctcaacgccaccaatatcgaaggtcagattaagaccattcgagttataaccgattggatggttagtagcgatatgcacgttaacttgacaagcgattacttcgagatattggaacgatccaccggtaccagctggtgcgtcaaccttacggtcaacaccagagcaaagaccaatctcggaaataatcggagagcgggtcgaggcagtacggattcgatgcgcattggtgatctcgataatatcttcagcagacaaacttaccttaacaattgcactagccgagatatttacgttagaaccgataactgtaccgttgttcgaaatagctggcggtactgggttaagatcatcaacagttggtgtgtacggtttcggtgttggaataccattaattacttcgatttccagaagctgtggttgtacacctgtaacgttaatgcgcattccataataggcaacgtagtttttaccattatgtttttccggaacacgtaagcagaaccgatcccgttgtgcggctggaagatcatcagttacttcacgcagtgcaaacggaatatggttataaagtgcagcatggttagaacggtgaatacggttttctacttcatcggagccatcagcggctttgattgtgtagtgacccatgttaccaattaccatataacgcacgttcggaatttcacccgctgctggagttacgccattttgtacaccgaacttctcattcagagttgtatgtgcaatcacacggaacggagatagaccgagatattttgtagtttgcagataagatgcatagcacgtacgtactacgttgataatctgctgatcgatagggttactagccattcttttaatccttgacttagaaagttcattgtaccattgtgtaagaatttttggcttgcctcccgttagggaggtttatgccgttaggtgtactgttggaagtcaccacgtatcattacacatgcccacaactgaccatggtcggatttaggaatcgcgtgaactgtactaaggttaaaggcgatctgttcacctttacgaagttcgatcaaacgtccattaagttgaatggcttgtctatcttttaatgcagttgcgacgatggtacctgcaccagttttattgacccacgttgtcatctgatcgaggaaaccacgaccagctggaatatctaggaaccaaccttgaacagctttattttggatatcttcactaaaaccaaccttgaagatatctcgttgtttagatgtccaatcaaaccacttagaatagttgtaaatactcagtgctttggttttgttcttaccgatacggcaacgagagccatacgagtctttatatttaaccttacgagagaggtctactaaagtagttacttcctcttcggtaagggggtcgtaatgtttatacatatctgtcctactcgtagagatagatgagaacgaagcgtaggtgttttacgggtggtacagaatgcggtggtgttttagctggaaagattactgctcttccaggaacatctgggatgaactcaccatttaggtcgagtccatctccattatcacacaatgcaatcaccatattaaatcgatacattgcaatgtcgatatgttccggcataccaaaaccaacctcgtacatattgacacatgcttctttgggttttatcccattgatagttggtgcaatttcaaacagataatcgctaagttcttttggcatctgaccattaccaaggaaccagtagtttgcttccactgtacccttggtagggatactatttatcttcttgcgattgtaccatcttgcacgaggtagcgcttttaagtactccaccagtctttcactaactggttgcgaaaacacgaccgccttcgatgtttcttgggccaatgagttcatggagaccgccttcgaaggtagcagctcgatcttcggcttcttgctcattggtaatgtattcgtagttgggatcattctgatagaactctttgtgatttcgactagtatctttacagagtttgatatagtctagcatctcactaagttcagtaagttcaagaccggtcttctctgcaagagccacgattgcacgcccaagcacgtttacttgttctacgacaggataacgttgagtgatcttgtaagccatctggttgtccagctgtgcttcatagatcagacgaggaccttcgttctctccaagaatagagtagttcttttcccaggttccatcgtcattgatggtgaggtcaccgacaactcggtcaccattaaacagatccatgttgtcttcaacatagatcacgtttgggttatctggatcgcattgatcgatagtcatcgaagtagcaacgatgaacttaccattcagacggttaaaacaaaggacaacaggtttacgacccttttcaggttctggtacattatgaaaatcgaacatgtgtaatttcctttagacgattcgagtgagactactaccgttacggcgcattacaaccattgttggcattttgcgaccattgttgaagtccagcaagtattgagcaaatccataaccaccatcagcaatctgcgagatatttgcctggagagcactgatagcagcttgagcgctagcataacgcccaccagcataatagtgcccgcgtgcattagcattataagtcgcaaatagatcacggaagtgaacgatttgtccattacccataatgcagtagtcagacgggatatttggacgaccttgaggatcagttccagtaggaggccatggagttgggaaagtcgtaacgaattgctttaattcaaagcgagtgatattccaaacgttactagcatctaggtcaactcgtgcagggaaatacaattgttcccaaccaaccccagccaaccgtttagatgtaaatgcgcgttgtgtacggtgaagccgttgtgcataaatagcatcgatttcagctttactgtacaagttcatgatcgccagtgttaacccatgagggttattttgattacgaatgtgatctgtaatctttggaatcaaaatggattggatcagattgaaaataccaccaatcggcatatacacattggttaggctagtatctgttgtctgagcttttgtagccattggccagttgttaatttgcccaagcttaatctttaccttatccgaagagtgcggattattttcatcggttatgtgagcgttcacacggttgatataattctgcacgtcgtctttcgcaagctgaacgtaatatttgtaataatccgtaccagccgctagaattgcagttcgacccactgcccatgcatcacctaaacggttaatattgacaaccgtggattcaagaccatacaactgccaatatttgtgcatgtgttctgatggagtatatgcagttggtttaccgatgatttcttcccaagtaaacttaagattagtctcatctatcttctccattagtgctttaagttcttttacagaaacactaaagaatccacctactgcatgatattccgcacgaacgactggtgtgacggaggcgttgatgataacaacgagacccatcacattttgaccagtcatttcagaaagcttttcgtagtgatacgttagaacatagtctttaccacgcacaagagctttaccagtagagtccctcagtacaaagccattcgtatagaaaccgccatgggtacaaacgaatacgcgatgcttcttaccaggaacttgaattagagtgtgttcctcacctttaatccagttatctggatcttcaccggtaaggtcaagctcaagaaaagtaatatcgttcatttataccttccaggaatttaacgatgtattaaatacagcgaaaccaacggagttaatatacgttgtgattgcaccgttaccagtaccgataccccagccaccaagataacggaaaatggccgttgtaccagcagggtggttcctacctagcacgttgttcaactgagcttcagcgtttgcaccgttaggatcaaatgaccctgccgcataaataacgctctttggtttatcgatccatgctgtttggatatcgatccaatgaagccagcttgctgcatcagcagaagcaggaacaaggaatgcgtagttgttagcaggtggaatagccccacttgcaaaagtttgcggtggcaacaaaccagtcttcagctgtccaaggatttcatcctgacgagtgaactcgtaaagctcttggaaagtcatgccattgttagtcgtattgttgttggcatctttaacgccaccaatacgttcggtactgttaacggtttcaccacggttgtaatagttcccagcaacttgctgatgttcttgaacggtatacgtaccaagtttagcagctgtctctttgtgtgggttattacggtcatcaacgtgcgcctgtagaatcggtaggaagttcttgtcgatactttgcttagctcgtaatggcgtagcgtaacgatccagaatatccccgttagctgcttcagcttgatctttcgtagcaatagcagcattcttcactttatccagctgaactttagcggcagtgagtttgtgcgggttattacgatcgttaatgtgggtagtaagacgttgctcaatggaagtaagttcatctccaactaaagcaagctcggctttatattggtcaaacaaagcatccatgtctttctttacgaacttttcaccggcggcagtaattcgcttaagcagtaatacttgaggcgtaaacccgtaaagttcccacaacgcatgtaggtgaccgttgggtttgtaatcatccggtttaccagtaatattgttccaatgaatcttccgagtattgttgatcaacccgagtgcttggttagcgattgctttaccaagattacagtaaacaccaccgaccatctgggcatcaaccctgatctcatggtgaacccgtgggttcttaatgacaataactgcaaaagctggaatgccagtcttcttagtaatctctggatgcatctgagtgcattggaaatcgtccttctcttttaacacatagccacgaccatcgatcatgtgcagattgttattgtagaagtaacctttatccagaacaatcacccgatatggcagaccagcttgatctgccaagttgtggtattctccacgcgtgcggttattgaaacaagtgcccgtcccatcgtagggaagagcgtgaagtaatgggttcatgttgattcctttagattggtacccaaccttgacctgggatattcatagaagcgtaaagaatgtcgtatacaccgttccatgcaccgttaccagaaccccatgccttagtctcgcgaatgtaatagaaaacaatactattcaaacgcatgttagagaacggcggtgttgtagcaaccattgcgttggcttgcgcctgagtgatattgacactgaaagatgcgaatgcaacatcaccactgccaccttgaggaagaagagatagcagggcatcaatgttagtccagttccgattgttatcgagaacagcacgattattcagaacaccacgacctaatcgaccaagaggaagcttaccttgatcatagttagtaaaagcatttgcaggaatatctttacgatacaactgtagaatttggttatacgtcatatcctggtttaaccaaaatccgaggttagagttttcaacaacttcatttctcagatacttggtattagccagagtatttacttcttgcttgctattggtattcaactgtgcattagtgacgccatgaacgttgccacgtgcatcgatgtgggcctgtagtggatctccaccgatcttatttacttccgcagccgaaagctgtggggtaagatagagttcgttcgatatacctgctgtagcctctgcaagactcgctacgcggtagttttctacaagacctaaacctacatgttcttttgtgtcgacgtgtgggttttctttatcttgaatgtgtagatcgaggcgattattgaaacgttgtaagaaacgatcatattcagcttttacatcaacacggaactctgcttctgtattaccaagttggccagtgattgcccgagagatattctcaatctcgttgttaaacggctgatatgtatccaaacgccagcgtagggcagctaactcgccaggaccataaatcggctcagtgccgttataatcaagccatttaggaatatagtcagaaggcttagttttccagaagtttacataatcgtcgatgactgtgaaactaaatgcaacatcgccgcctaccatctgcgccgacatgtaaatcttaccggtacgagtacgatccaagaaaacaataccactggcaatatcaaggccatagaactcgctggcttgcttatggtaatacgtgacgatataatctttatcacgaattaaaggaacgtaacgagagtcatatacacggaggctattaacatagaaaccaccgtgatacatggttaccattttaaaagggaaccccgagataggggtaagagttgcttcttcgctacctaccaggttattcggatcacgtccggtcttatctaacggtagttgtacgattacatcggacatttaaattctccaaattgaacaaaagacggaaccaccgtgcttttacacacagtgattccatccgttgccagggtaggttacaaacgatcgtaagcgtcgttaaacactttctctatcgctttgaagatattctcctcagcgtagttgtctacccgtttaggtgtcatgaacgaagagttattcgttccacctttagcttgtgcttgctgtgccggtagccagtcagggacattacctaaaccaatatctctaggctcaagtccatgaacgttacctttttcaaggatgtgtgcgttcatacgatcccgagcactacggagtaggttgagaatgatgttattaaactgaccgatattgcctttcagcttatcgagttcgacacgaaatactgtcatagccatcttaagtctccttagggtgcgacaatagtcgtcccatcattccagatgagagcattggtcggagaatcaccccagaattcggtataaccaagattgtttactgtaacagtgaaacctttaccagcagccgcactatagaaaggtgctgacccgtaaggaatttctaactgtccattctcgttggaaccgaacatagcgatgtctgtatccatattctcaaggctagatggatcacgtcgaatctgaacggcgtggtgtccatagttgccagagatagaactcacatcggttagggtgtttgctttgaccaaacgattatctttcgctgaccaaacatcgagagtagaagtgacttcagtcaatttaaatgtaggcgtatatgtaatctcatacacacggattcgactagcatttccattagtggtattaccaccttggaatactagatacttggaaccaatccggatatcggagatttcccagccgccagtcaattgagcagcgattacaggcgtagcagcagaaacccaatcactagcacctattgctgtataagtcgggtcaccagacggtggggacttttcaacaattgccatttgacgagaatccgcttcttcggttgctacccacatttcggttacattgtcagactcggcgtacagttgagttactgtacctccggcgatcttcatgatcttaccttcatctgcaccgtcacttggttttagttgaacatatagagcagttttagagccccacatagcaaccatcgcatttgcctggttgaagccagcaccagcagcccaaccagcaggaattgctagtttagcagaaccggctgaacggataccatcgccctgtgaccaagtaccggactggaagtcacgtatggctggaactagatgatagtctgcatcctgtaggcttaaccaagaccaagctgcaccacggattggagtgatcggatatgcatcggcacccgctggttcagagcgataaactgtatcacctgaaccgttgaataacgcatatgctgctgcaccggcgttaacaccttgaatcttactcagacgttctttatcttgctcgtctggaggagtcgggtcattgaaactgatatctgccgaagaagcaataccttctccgatcttctcagtcacttctgccatgatgccattaatatcgctgttgagcgggaacttagcttcccattcctcaggagtttccccaccaaaggtagtcgcatcaccaccacttccaccagccgcaatcttctgatcaatttcctgtttggtatatgtaccaattaaaccaggggtgatattgtgcgggttggtatcagtaaggtgtttattgaaatcaataattaattgatccagacgcgggtcaccttgaactgcttggataagcaaagacaccgtatatggagtcatcaaggtactattgttagtcgggtcaactgcctgttgtggtgttgcagccggatagttaggaacgttacctaaaccaatgtcacgtggtaccattccatgaacgttacccgtggcggcaatgtgtgcattaagaggcttgagtgcgttttcttggatggacaacagtacaccacgagggttcgtaaacatgtcgttacgattaccatctttgtgctgttggtctgttgccatagagaagttgggcacattaccaagctggatttgcaccttgttaacacggtgcgggttatcatagtttcttaagtgcgactcggttgtaccggaagcggtagcctccatgatatcaccaagacgttgaagagaagcattaatctcttcagaacccacaagactatcgatcggttgatcatgatcgagtggtgggaacgaggcagggagtacatcaatattaccccatgcacgaatcagcgggttgtactgtcgacgagacagttccgccagaatggcttggtcgctaaagccccactgcccaccgatggtccgataatcaagacgagcttgaccggcgatagagcgtttcatgaagcggatagaaccagcgatcggtcgaccaatagaatccattgcttcgatgaaacggtgaccgatcatgtagtcgacgccttctacaaacagagcaccggtctggttgttccgtacttttagagagtcgacaaagaaaggagccgctttcggaataatgaaataataatcggtagggccgggtacttgcagggtttggatttcccctgtgatgaggttagctgggttagtgccatgcaaatcctcgtcatatagaccggttgtactaacggtggacatcgcgccctcctttaaagcgctagcgcgcggttgttagcgtaatgatgtgaaattcacataagattgtccgatcttttctaacggagacatgacaatgtacgtgcttgtacgttctaggtatcgccctagtcgccgaggtggtcggtggcaggaagcggactttacaaatgagctagtaactacactagctgcgaagtatggggatatctatctctacatccaatatcctggccaaggtgagcctgtaacaagagcactgcactgggttaatgttactaattggctaaacgatgttggtccaacagttactgttcaagagtggctaacctctttaggtaataaagctctaccttttgatgcagaactacctaacgaaaaaattcgtttggtaaagtatgctcaagcatggcactgtggttataactttaccccagttgctcgtggaggccatcctttagatcaagggagtgatttccataaggaagatctccttatgactcatccaaaacatcagccttcaaagatcagagattattccatgatctctgttaatggttatttccatttatgtgactataccagtgctggtgtaaggattattgatggaaatacgacgttacgtaaatgtaacgataatcagattggtgtttacagtttcgaaactattggtaagcttacttttgttcctattgttgacagtatgattagcggacttaatcccactgctcctttgtgggatggtacttatctaaccatgcctgagaatgttgacatcgagaataaaactgtattgcttgttactggcggttatctaaacgttctatctagtgtttataatcgtgtaggcgaaagaacatggagagttcagtttggtaacatgatgtttttagatcgttatctagagtcataccacgcaatggatctctcttctctcggattaacattcgataaagagaacccgactctattcaatgtagatgaactcaaaaacaatgatgttatccgaaagtatttaactcttagtcagagtttctttgtaatcgttgattcccaatcattcttccaggaatacgaagctgtagaatatctcaatctacctggacgttacttcgataacaaatacgatagatcgcctctcgttggtgcgtatggtaggatgctagattatcacacaatcaaagaacctcaccatgaaggtataatccctcaacatgaaaatatgtatgtctactgcgctgtattaaaccgtaggaattcctatgatgctaatacgcgagcatggcctgagcaagagatcgttgatggtggacgttatccagctcatccgtttagagacgaaacagcatattatcgaattttaggggttgaaggttaaagcaacatattgcccggctcaaggccgggctttatgtcgttaacggaagtcagatgtatcttcttcgtcttccagttcatcctgttcagcggccgatattggatcttcaagaccctcaacttgcggctcatcttcgggattagtttcatcggtattttcactggacgattcatccatgtcagtgatatcactatcaccagctggagtatcacctgtaccaccatcaacaccaaggtcagtatcagaaccatctaaatcagagaaggagtcatctccagactcgtcattattgtcattgttccaactgtcaccaccacctacatcatcagctccatcgatagtagatttatacttagcctcaagacgcttcttagcttcttgttgatgcttagcatagctaaggatagcagagccaacagtttcctgttgtacgttcagccaatccagcaagctgaatgcaggtttatcaccatccatttctgtaagaacattaagttctggaaggatgttgtgtgttgccataaactgacgtttaaatacagctttcaactgaaccattatctggtcagacagaccaggtatggaagtaaactcatcagggaagagttcgctggtgatgtagttttccaagcccatagtcagaagtcgatcataggcatccatcgattctgcttgacgttcatgttgagtattatcgggtgccggtagagaaacctcaatggcagtgataaactcatcaactacttcttcaactgtcaactgtttaagttcaggcgatgtcaacatgtcaacgttgtcttgaatgattttgtacatttgattacgcaggatagaactgtgcgttacaaatacacgaatgaatttagacaagtgttgacagaacgctttctgtttctctttaacacgtcgagacattacaaggtcattctgtaccacagaagtagcgaagtctggagaagacatcgggtctactttctcaggtggtacacccatacccgagatgtgcatacggcgaaggcgatcttgtagatcaggattcccagcattaacgttggtattgtaatcgtcgtattgcacctttgtctctgcgtagtcagcaccattggtgttgatttcaaagtcaaagccagaacgaatcagatggtccatcgcttgcgtagggtcaggagcagccagagggaaactacggtgcgccgattccatgatattcgattggatattactgattgtttgttccggatctgtatcgtcgggatcaagagtaatacttacacgcttacgaccaacagcattacgcatacccccaatagcttctgccataagaagagtagaacgcatggttgcgataatcttcgagcgagacagaagagtttcaccaatgccattttcgttatagtcgaatgcaatataaactaaaagctctgccgggatgaataccagttgagtatgtttagctttccaagaacgatacaacatgatcctctgaatttcttcagttagaccgatctcaatttcttgatcatacatgccgttacgaagacggttgttaagatcattcacaataatcgcgttgtatgtttgctggatttcatccacttcgaaatcttgtttagaagtattagcacccatcgcttcccgagtaaggcgtagaacttcagaactgttgtcgttattcttaccacctttccaacctgattgaagctcaccataaaaatctcgggttgagtctttggagagcgggtaaccatgttggtcgaccaacaagaaatagccgatgtgttcatgtgggcgcccctgtacgaatacgggtacaatggattccattggaagagggagagtcaatggatgtccaaccgaaggccgattcatgtacttaggagctgtgattacctgagtatgttcagtgccgcctagtctattctgataaagctgttcgatttcagcgttaccgaatttatgaacagcgttttccatcgagatctgattaccgcgaagcttacgcgcaatattcatttcgcgtacacgttgtgacatcgatggaactttgagaatgttaaagttatccgttacagtgaggagcttatctccacgaatacggttagctgtagcattatcatgatatccctcaagagagatattgttcttatctgggtgaccaaggaaacccaagttttcattagttgtattctggacacgatctctaatagaggagaaagtttccatagatacctggcgacgcccattaataaggttatctagaacgttttcagggagaacagctaagatggaagcacccttacggaacaagcaatcccgaaggatcaggtccagacgctcgtcaatcttatagtctcgtttaaagtacgtttcaactggctcaagcaaaagctttgcaatctcgctatcaaagatagctggatcaatagcgaatgtgaggtccgtatccgaaagtgctttaggatcgatgatactaccgacgtatactgtttctaccaactctaggtctggtagcaactgcataatagagtcggagtcaacgatctcttgcgaagtatcacgcgaaaccttatctaatgtgaaacggtttacgttcacacgaggctttgctgcttcgctgccaattgcgttcgggtccttacgcaacaggttgaggagggcgttagtcggagttgctttcgatcctaaacggagcgtctgcaactttgggtacgctacctcattcgtttgtcgagccatttgaagctcctcgtttaacaagtgagtaaattaccatgagtagcatgtattttggagtttaccgtgacgatgtcatgagacttgcaagatctgtagtaatcaagttttctgaaatagctaatcagattaatgaacgcctaaaagaggtcggacatgaagctgatccagcaagaccggagacttggaaatattatcagaaccttgctggtgagtatcatgaaacagatgtcatgatgacagttcgttccgcggatactcttgaaatcatcgatttcacaaaagaaaatctggcgcttcaccgcgctactgcgcgagagtatattccgggtagcgttttatacaatagccttgtaagacagttcccagaacaagcaggtttgattactggaatcttatatccaattgacatccaaacggcaatagattcaaatgatggggatattttgtactttgatccgaagtatgtagaagataatgaatactctttcttccatcaacttcagtcgtgggttaatgtatttattactcgctggtataacccgcagtttaatttaactgacgatctataccttgcaaacttccttggtcatttatatacccgtttacctattgctattatgcttattcgtctgcggaatgcaaagactaacgaagcgcatagttatcacgttacggaatacctcgcatctcaccaagggttggatgagtttattccctatctttctcttgagcaacgtttatggttatatcgtaacattgcgtttctagaacgcaatgcgggtaagaaggaaatttggcaacgtcttgttaagaatattcttacacctcgtggcattccgttgatcagttttactattgaacaaaacagttctaaaatgcctgagcagcatcgaccaaccgtcgatatgataaaacacgacgttaacttccctgtcgtacaagaaggccaagaaacgacatctgtggcagacgttcttgaaagggaagatgaccttgcaagagagaaccctcttgttcgtttcgatgctgagcaagatatcaccgataagatgagttccgatcaatacagttggcttagaactaaagttcttgactctgaggtgattgaccggtctaatagttctgtacgttcattaatgagcgtattgctgaacgaatggttacatttggcctcaagtgataaatatagggcttatgttcaaatacctaatcctaagactggcgaattcatgaccatgacggttaaagatgccttcattgtgatgatgtatacctatgccaaggctcgtgatattccaaccgataacatccctagtcttgtagcatatgaagtactaagagataagttacctacctttggtgaacttcgaccagctgttgataaacgtattatccctgaccgtctaattactgctgtgcaagacatggttactccaatgggtaactatatctccactgagcagttctatctggactgtgtccgtttacacaaagaatatctcctgcaatgggaaatgtattctttccaggagcatcctgctggtcgtgcttattgtgagcaacttgtaaagttccattacatgcatcggatgtgtaaactggctccaccaaataccaagtttgaagattatttccgtagagcatctttcgatatcctcaatctaaataagactgaggcagaacagatgtgtatggattgcatcaatattgcaactggctccaacttggttcgtgttattacactaggtgaagtgcaacgtgaattgctacggttgatgggtcgtctatccagttatcctcttcaatatcttcgtaacgttagctttaccgatttccatattcttggtatggtaatgccgcgtgtgggggatattacagtagatgccgctggtaactatatctgcaacgtcgctgttcaaaatgtcaaagcatatagaacgtcggcagggcatacgtatcgtgttgttgatgattctacttctccattcgtcgactacgtttatagtcaacaggatatgttctggattaatccatttgtagaagtgagagaccttagttacgctgacgcccattattacattccagtaaatggtgttaacgtaagtaatgttgttatcgaaactaataattcgccgaatacaactggcgacttggatcaatatcagaattccactgaccctaactggccgaaacttaaggagtaatcatgtacattacgagagactatttacagtctactccttggacatctataatcgacatgatcaacgatgcttgttttacccaattgtttccgggtagtactaagcttgaacagttcgaatcactgggtggtaccaagactcgtattgttataagtgtaaatcgcagtaaggcttccggtaacttactaccggaagtcgaactcgatacttatacgtacgatcgattagatttgacgacattttttagacaaacccaagtgcttgatttatcgaatgtggatactccatattccagtttaaaggttgtcgaaaaattatccgagttaaataacattgtttttgatgtagatgatttcgaacataccgagtataatgtattcaaccaagaattcattctccatgcgaataaaaagtctcttcgttttgtaggttttcttcgggttcgtttgattaatacactacgaaaggaattatctactttcagtaaagttgaattccctgacgtaggtaaacctgacaatgttaaagctaatgatctttcactgatcaatggtacttattacatcactggatatgactttagtgaacatagagagtatcttcgtcatctaacaaaggctggtacccatccagatcctaagaagatggccgctattctcgctgaggtgacgaataaaccttggacagcatcaaagacaccagcttctcacaacatcgcttatactgaagaaataggggttctaaagtacaggatcatttataatggcattgtactacctcgatttagtgggcgtactgatatacaaaatgtacttgttatcgagttacataaaactttatgtcaggatgtcgttggcgaaattagaattcattataactaaggagtagagatgcacgttaaaaacatgaaatctaaactactccaacagtttagtattcagaacaagttggatccagctattcgtcctgaggatgttatttggactggtattgaaatatggttgcagaacggtaataactcaagagctactattcaggctgttgggacaagcaagtattttaaaggacagaaacaaatattctttaatcgatatcgaattgaagaagctctcaatggggttgttattccagggaagagaattgattattcaactatccatgatgttattaaagtactccgtgataaagtgactgtacccgtcgatactgatgaattcctagatggtcctctaactggtaatacggttattttaaaacccactactcgttctctagcctacattccaacttcacaagttgaattaagtttcgagaaataaaaaaaataaagcatatcgccctctcccgaaggagagggctttatgttgttactcatcgctgttcaatcgaccatactctatcgatctctttcatctcgatcattcgtagagtagccccaaatacaacgacaatacacaacagcattgtaattgaagtaagggacatcttaatgaaatcacgtttgccaatcttttcaaatggcacgtagatgagatacctaaaccgatgatttagataaagagcaaagaaagcagcgagaacagctatcaggaaccacatgtgaaattcctgagtccacgtcaatacataaccgaagacagacatttacaccagcgccacgaaagtgccatctttaaagccaactttacgtttagcttcatcgtaccatacatcaacacccatgcgagccaggccttctacgacatatttatcatagttacctttaccacgcatgatggacttcagttgacgagtcaggatggtgtggttagtggaaaggaacatacctggtacgtcaaggtctttaacacggagattacgcggtagcagcgactccatggaaatgttcagaagttccatgcgacggagatcttcacgcagagcccgaacattataaaccatggccagtctgatgtcaccacctttacggagatgttcctcggtcagatgtggcagagttgcggttggatcaacaatcactgctctttcaccaaaactttgcacgactggatcgaggtaagggttatgtacaacatattccccattaacccaacgatacaaatccaaagtagaagttactttgtaagttgcctcaggatcaccccgcaaaggaagatcatcgacagtaaggacatcaatagacatactctctcctttgcctttagggagttcagttggactataactgctagcgtccattatggtttcaaagaaatccatatcatgttctacatcacgaattgccttaccgaacacttcacgatgagacggaatgaacatggattttacagcgttgaaaacctgattcattttgcaatttccttttgatagagtgtatttatatcacctctgtgatataggcgttatttatctttaaatacaggattatcgaaatcatcttcatagaggatatcgatacctacaatatcaaccacctgctcattgtcattcagttgatatctaaacccaactgtaagaggaagcagattataaagggcattcagatcacgggccaagggacctgctgcggtaatatccaaaatcaatacaagtggtgtattgatggtgttactatattgaatggaccaactatcaatagtagcacatacacgatttgcatctactactagagaacgaagaataatattctcaagtgaagatacttttacttggggatgacctaattcgattcctgtcaacaggagttcattcttcttaacaaaagaagaattctcccacaggtgaagttgactcaaaccaaatgcattttcaacgattgcttctactcgttcttcaccgagtacggcaagatcccggcgaataccagcgaccatacgttggcgcatttcatcgaaggaaacggttacccgatatttggcattcggtagtttttcgaatttcattactctgctcctagagggacatatagcccctctaatgaggggctagttatcaatctgacaatatgtcgaatgtgataatttctttcaatacaccagccgcattcttgaggccgcgtacaccaagtcgcattggaatatcgttcttgatcatcgcatgcatccgatcatgattgggcccgaatggacggatgtatacgttgaagccaatgagtttagctttctcatgtacagggtcgataccgagtactaaagctgcaccattattgcagttgatggatgttgctcgtttgtagtctgtttcaatgttacctgtcatcttaggatgaccaaactcacaagcgatcacgccggaacgaatatcattgctaaacttactgacttcataattcacatgcatgtattttggaagtcgatctaaagcaatgaattctacgcctactccattttcaaatgataacatctcattttcctatgaaaaggtccctccgaagagggacacttatgtttacttcaggcgcttcaacagaaccgctttctcggtcagacgtccacgaataacttccatgtaaacgccatcaacggtgatcaaccgcatacggacattagcaaggccagatgccgtagcacgagtgatcatacctttcagcacttcacgaacagtcgggtgagttccttcagaaacaaggacggctttctcggtcagaacgttcagagtggccatctgttcaagagtccaacctacctggaagttaacgtactgatcggcaacaccacggatatcatcaacctcagccatcgttaccgaacgagcgataatttgagctgcacacgctttgatgatttgcagtacttgcacacctttcttgttactgatgtaatccagcagatcaccgatgtcatgtgcgaaatcactgatggtgatattttggatcgacaggctatctgccatgaagtcattgatggaatcggtcagacgatcattcaggaaacggaaatagcggatgctcagttgaccgcgatttaccatttctttcagttcggtagcaatcccgatcagatcggtatagttacgcagattactcagctgctcgaaggtttcatcgctaacatccatgtgatagatgctcatcgatttatattcgtgtgcaggcagagtgatcgactgcgattcttcgtcgtcaccaatgttcaggagttcccgaacagcagcacgtgcttcagattcgttttcgagatcgttagcacccatgaacatcttgttatcaagaatgatcggacgcattgccgccgcttcaccgagttcattatccttgacgaggctttctacttcttcaatacccattgcatctccaccgatagtagagatgggagtggtggaagcatataccacaccgttaggacgatattcacgacgacgcaggtcatcattcagttcgtgtttcaggtattccatttgcgggttccattcaatgaatttctcttttactacaccatcggggaacttgacgaagaaacggcaatagtgttccggatcaaccagaggactgtacggatcttcatcaccaacggtccgttcccaatcaaccagttgtgccggtttaatcagaattcccccagggttatgaatctcatcgtaaggacgagcgatgtttacacggaaaccagtaggttggtaatacatcggatcgatcatcacctgagatacgtcgatcggaacagggagatcagtatcttccacaacgggtgtattttgcacttgcggttgttgactgtacatcggttgttgctcctgttgatgggagtagccaccgtaaatatcagtactgatctcttccttcggcatcaggggagcagatgcagccggagtatcatcgtaatacgaactggtggtgctcgataccgtgtttggcgctgcgccataagtaccagcgggttgagagaaagtagcttgggtggttgttgcgaactgtcccatgttacctgggttaatgggaggcaaattacctgccatctggataccttgcggttgacccatcattcccatttgctgttgttggggacgatagttaccagatttgtacgcttgaatctcttggaggatctgctgatacatggcttgagcagtttgcagaccttggaacatatgttgcggaactgcacccatttgcacgagagcaggatacgatgcaacgcattgaccaaggaatgcttcatacatacgctgtgcagctttcggcggagcatccgtctgactgtagttcttgcagacacacaggaactcaacgaaatccaccaggtgctgacaccattgttggaagatctggttttggaaccagttcgacgacagcaggttgtacgcgaaaatatgaaggttgctttttccaaccgacgattgcgcaagcccacggaacagaccaatagccatgagcaccagctgttggttattcatcaggttctggctgagttggagttgaggtacccggtcattgccatgaggcagattaccattaaaggtactctgatcgacttgttggcaggataccgggagttgagcttgttggttgtacatctgacttttcctatttgagaagtttaagagacaaaacgttgttgagctttgtcaataagttcacgatcttcttcacgtcgttcaaccaatccgtcgtatctaactccgacgaagaggtttagtcggccacgaccatccgggttgtttttcggttggtttttgtattggcccacctccgcgatcgaagcgtggattagacgagagctatcaccgattagtgatttgttgtgtgctttagaagtcttcgcgcgatcctgcggtacaaggatcgaggttactttaataaccttgctatcaccaggagacgacagtgtgtcgagctcaccgtgttcactggtaagtttcttaatgcacgtattgagtttgaatgaacgtttcagggcatcgttgatttcctgtccagtccactctttatctttacgaccttggaacgtatacgcaaacatggagacagcatagttaaactctgccatcacatacctaagaatactcaggcgtttgtcgtacatactagtttcatcaatgtcagtggcatacagatggtgtgccatatctgtcatgatcgcatatagcagttcccagatggtattgactttcactccaactgaacgaagttcttcaatggtcatctcatccagagagttgttgaagctatccaggtgagattcaatgttctcagcaattttaccttgatgctcgaagtcaccaaagatcatcagaccgagaatgattcgccatagctgtttattatccatgtagctcggctcgtagaaccggcttgggaatgcatctacgacgtaccagaaccctgcaacgagtcgacggacaaagtctgtctccttgtctttgggtagaaccagaaccatatctccagttggatgacgacgtttcagaaccgcagattcataaacgttccattgatcacgcggatactgggactcaggaaagtctttcaaatatccaatttgaatatctactccagcccaacgcttgaacgtttcaacgacaccaaactcacagaagaagtaatgtgcaagacacgactcgatgtgctgccggttatccagatcacgtttagtgcgcttagacatttcgttgtgaatctgagaccagatcacatacatcacttcacgctgaccattacacatgtagtggtggtcaacttgcttaaacgtcagtttggcacgccggaatggaatgaagatactgccattcaataccgagaagccaacatcagtcaacaccggagagatcgaataggttgcaccattgagcgtacagataccaccatcacgaacatatggtaatagtacccttcgtgggaacatcatttcgcctttatagctagtgatcagctcgatcatgtacgtattactctcggcgatatttgctacacgcttagagccatactcacgggttatctcttcgaaatgaacttcgggtttacacagacggtttccatgatacttgaagtcagcagggaatagcgccgagttgatttcaaacaacttatcaacatatgcacgagttgcgttcatgcctgtttctgggttgatctccatcatgtgctttactgcaagcccattggctaaatctttatttagcttgggtatgacaccatcaatcctactgattacgtacgggtccatcacccctcctatcgctttcggaatatcttttcgagcaatgcatctgccttggctacttcagctaagaagtccacgacagttccaactgatatatccctaaacaggatgatatctctcacagccaaaggttcgagttcttcgtcgtatagatgtcgatggaacatatcaaaacaatccatacgtctctgagcatcttcctttgacattccttttgtactttcctttacagcttctctccattcacgtaaactggaatagatgccatacttcttaaagtctccaggtttgataacaatcgctttcgcattatcccgtcgtgctgcaaatgtcacattaccccttaggttaatatgaataccaacaggcatatctggcatgaagacaggctttacctcaagtagatcgctgccgaatggcataaatacactttcggttatacgctcatcgtctacgaaataggcaacagttgtagtagtagtccagatgatatcttcctgacggtagagttcatcgttcttcgagaagaaacaatcgcgcgggaagaatgtagtcttcttcgctcgatctgtggaaactacttgaacgttgagcgcttcgatccaaagcccataaggatcggtatcgatgtggtcaaggtcaacaatgaaatagaaatccagttcacatggcgtgttggttcctttgttcttaacagaacctaccagttgttccagatattcttgagtgagattaggccaatgtttaatcattgctccgatattaagttctacatcgccaccccatgtaaagttgatacaaataacaagtctattttcaatacggttagtacccggtagatccaggacaatacctgttccatcgataatacttatttcatgcgtcgactggtttaagtaacgtacacgtttatcgacgagaccttgaccgaagaaaatgttttggaaaacagatgtctgccatctgtccatgtacgatgtgtcaagaggacactccagtacgggatcgtcctcaatatgacccgcacgggaacggttgatctttaccatttaaaacaatcctatccaataccatttctactttacgtcctttgggcctactccgttcttgactaggttcatatcgactcgtttgggatgctttcgaatctctatgatttctgtctccacgtttcccatgcgcaacacgcgttttacctttacccttccgcgtgttgcgcgaacgttgtttttcttcaggggtacctcccgattcataacaacggccattggatatattaacatgtcttatttgcttctcgaagcgattagcaaaatgggacatattctcatcctgggtaggatgaatagtagtggtagtttgagaattggtttggttagacgtattattactaaccgtagtattttctttcatgacgacaatgtcgccaggattcatttgggaatcagtgagctcttgctcaacatgatgcccgtgtgtattccagaacattgtctgatcctctaattagggaatgattcttcaataccgtaatatagatttgaaatattttttaatgacgacataaagcctctacccgaaggtagaggctgttatgccagcagtcagcttaacacttccgctttaccgctctaggcggcgggccactccgtcttcaagataacgggtagtaccattttcaagcttacggaaggtaccctttccagttcaaccttttacggcttcaaccaggggcttgttccactgagactcacccatcacttcttcgaagccagtaacgtcgaattcgagagcgaacgggatgttgttaacgtgcaggttgaacggaatcgcagcgatttcgcgagtaacttgctggccaccacgggtgatcggcaggtcggcgattacggtcgatacgtagtagaattgaccgaagctgaggatgtcgttctcttgcggagtcttacgggtcggaatcactaccagcttaccgtcgaacagttcgttgttggtcgataccaggtcgtattccaggtaagcgcccagggtacgatcgtcgcccttggtcatcaggtagttagcgatctctttgtccgagcagaacaggaacatcggacgctcgtcttggttaccggagatcacgcggaaagctgcttcgatgttggattcacggtaagccgggaacagtacacctttaacagcgttcaggattgccgagcagacgtcttcccaacggtcttgcgacttcagggtgtcgatcatgtcaggcaggtgcagcttcttgtagcggtaggtcggacgcattactgcggacagagcaccttcaacagcaccgaactgcggacggtcgaaaccgttagcggttacttctttcagctgagccaggtagttcagcaggcgcttaacagcgttgttgctgttacggatgttggtgttgacagtcagagccttaacaacttcgcccggaccttcttcgtccatagtgctcagcggcagggtaaccggagcatgcatcggaatcgggtgacggaattgcagggcacgagtttgcagcaggtgaccacgctgacggcggttagtgttggtgaagcgggtatcgaggtcgaaaccaacgatttccatttcgccaatgctgtcggccagagctttaccatcgccagtttccaggtcgatgcgacgcttgtcttcgtccaggatgcgatcgatagttacttcaccgatggtgaaacggctatcgccacggctcaggctgatgtgaccactgaattgcatgctcagacgcagaacccacttacgttgttccagttctttcatgccagcagtttgtgcagcgtcagtagtgcgagttacggccgaaacagtcaggtcatccgaccagaagtcgatcttggcaccgcgggtatcaccaaccaggtccggctggaacactgcgcgcggcagacgttcagtttggaacttgatgactttaccttggaacttaacgtacagagccttcagacggcccgacggatcgatggtatccgaaatgtccagcatgcctttgttgatcagcaggttggcgttcgagttacccatcaggtccagtttaacgcccggcttcagcggagcagtttcgatggacatgttttgttcgttgataacggttaccggaggcagcagagccggatcagcgaagtacttcaggttagtgccagcaggatcgatagccgggatcagtgcagtgcactcgtcgtccaggatggacggatcacgataggcttcaaccatgttgacttcttggttgtcgagtttctgaccggaaacagcgtggtaaacgtctttcattaccgcgatgtacggaagaacctgaacaacaccaccttcaatcgggttgataacggtggtcggatagatacgctcagcgaactcatcctgacgggaagcagccaggttataaccaacggtcacaacgcggaaatcacgctgggatttctcgttgtagttttccagaccgacgccagcagcagcttcgaaagtttggatcgaaccagccgggccgtcgaaacgatgttcaaccgaaatgacgttcttgtcagtggaagcaattttcttaccaacttgtttcagagccttaacgtactcagtggagttggacattgccagggcagccatggtggcagcggacagttggttttcgcctacacggctgttagcgccttcgaaggattcgaagccacactgacgggcaactttttgcaggctagcgtacataccagcagcactttgagcatcttcgtcgctcagttggccgaagttttccagaccgatcttactaatcagtttgctaccagcggacaggatgctgtcgccgtagtctttttccaggtccagtttaccaaggaaggattccatggagaaacgagtcagggagcggtcgccgttcactttgaacagagatttaaggtctttcatgttttattcctacgcaggatgggttttggatgttacaaatatcttgtcatcaaagctggtattttccggattcagccttgtgactccagataataagtgaagagatttgttgccattacttgctcaaatgggcaagctctagtcagctcgctaatcatactatcaaagaaagtgtggttagccttaattgtgagccggtcaggatcgcttgaaccagtgtgcagactcttctgcaccgcaacccaaagatactcatctacaggataaaggctataaacactgatataatcagaatcatttgccttacgcagagccatattggcaatacgttcctctacacgattgtgcaattcttgcatcttgaattgattatcgtcgtcggaggttgcctttagggcgatcccaacaaccggactgtcagccttctcgatctgagttccctgacagaaccggaatgggaattcattaattgcagcgtcgatctccgcaaggtcatttaccgagcttacggaagctatatagttggggcagagtagcttagtaaactgcacaccatcagctttgtactgatcatagactgcttcggggattacaagtaacttgatcatcggggtattgacctattgtgggaccaaggctattaagtgtctacataggaatatatacttaaattggtgacaaattacttaagataaaaatgatacacggtacatcattttaattttactaaaaggatgcggttcaaatgtcctccccaaaacagcttcttgtcagttgcgttaccctgctttgcttggagcaccgcccagattctccggcctctccgtctactgaactaattgataaaattgttggttcacttgaaattaaagagactactgttgatcatgatcatggtcgacaaacttttcttgagcttcgtaaacttgttcaagatctcaataagaaagttaagcacgaatttccaagtatcgctgaagtactacaatctgtgcaagtgagctgccgtgaagagaactatctttacgaagctgtactaaatggtgttaatgaaaacttcccagatgggatggctatcatgcaccggattaactcttatcgtcgttcgcttaatgaatacatcaatgatgaaactattaaagcgatcatgaaagagtattccactaagcttctgtttaaccgtggtggcggtaatgatatcgctggtatgatcaacgagatgggagctaagctcgatccttatgtaaaggctcgtgctgaaagtcgacatcccgctgaaatgggttgccttgattttgacaacccggaaggtgtagaagaattcttcgaagctgtacaaactactttgtctgccgatggtgctttcaaactaggttggaaaggtttcaaccgtgtattgggtagcctaggtgctttccgtcgtggtgagtttattaccaccgcagctctacaacataactttaaatcgtatctggttatgttactgtttgtacatgtcgcattgtttaataagccatggatgcgtgataaatcgaagaagcctcttcttctatttgcaacccttgaaaacgaaatctctgataaccttctgactatttacaaatacatccgtgaaaacgaaacgggtgaagaagtcattgtcaaagatatcgataaacgtgaagctgctgcttatgtttgcgcgcgccttgaagagaatggctttaaagttaagatggttcggttcgaccccactgaatttacaattggtggtttcactaactatctagatggtcttcagggacagggatacgagattcaattcctggtagttgactatctgaacatgctacctaagacaggacttgatgctaaagtagcaggtgacgatattcgtcttctattccgtcgcatgcgtaactacactactcctcgtggtatcactttcatcagccctcatcagcttggttctgatgcactgcaactgatgcgtgaaaataccgaggacttcgttaaggtagtagcgaacaaaggttattacgatggttgtcgtcgtctgggtcaggaacctgaccttgagctgttccaccacatcatccgccataaaggaaaagcgtatctcgctattcaacgtggtaaacaccgtaacactgtaacggcagaagaagaccaatatgttcttctaccatttagtaatatcggtacgattccatgggacattgataaagaggaagattattctctgaaagttgttcctgggtctgtaattggcggcgatctcgattctgacgcatggtctatctaacgacataaatgccttcccttcggggaaggctttattcacaaattcacaagagtaaatatcatgagttgtattgacgcacttatcgataacctaaaaggttaccttcgtttcaatctacaacaacgtcacggtacttctgttctggtacatgtggcatcccaaaatctttataaggtccgctttgagatagcaaaactgtttatcaatgcattagaaggaatggatgtagacttcctcaccatgtcggccaacgagatcatggagaaaggagagaggtatagagcatctctgttctttagtcatcatctgcatatcgacattctccagaaagctgcaccttgcccagatggtgattttatatcagtagatgtatctaactactctaaatatttctttgatacagatccatgccaggaaggccaggcgatgttgactaactatctcgaagaacgtaagacctaacatactgctcccttcggggagctttatgccgtaaaaggctctacaacgcgtttatagagatattagagataaagcctacatggtgacacttaatattagaaatgtcgtgtagaggctcctgagaggcaaggcgactgtgttgtttttaaagcttaattcatttggtatggcgatgtttgggcatcgcctccgttagatccccttcgggtaaaagcaggaataaggattaaagaagtttataattagaataaggaaataccttcggtattgtttattactaaataaaacccccctcctccggaggtaccttttcctcgttctacagattcattaaacacccaagtaaaacttctaaatcaacaaaaaaaaaataaactaagtaaagccctctccacaaggaagagggcaattgaggttaagctgctctagtaaacaaaagattactggagttagacttgatatgatagttcgatgatccgttaatccatttagcatcggaaagcttgcttacaagctgaccattgccaatgtaaccaaggaacatcttaccatcgtatacagcaactttgatttgctcatttcgcccatagacgatcggcttaccattgaatgctgttacctctagaccagtcaagtacccgtggtggggatctggtctggaacttgtttcaaagacttccattaggagtctcctctgcaagtgggcccatttgggcaaaaagtcaagcttaaacttgacgacatatagccctcctggttgcacaggagggctaatcttttcagaacgtacggtgttgttataatactgctagcgaaaatgcccacgaggggtaagtagctaatccgcagttctcttggacgacacctgctgacagtgtagtcgcgaatgcactgtttggaaccccattggtttagcggccaatggggatttccttttatgccgcttcggacttctgtttaacaggtttcttgtacttccacttgtacagttggtgcaggatgaaactcggaagacccagtgccagtacaccagcgacggctgtaccgacaatctcttggggagtgattgcattgaactcggtgccgaaaacaacctgagtaatgataatgatcatcaaaccgatcagagtggtgatccacagacgtggatgcaaggaacgactcagacgaagccctggagcagaaacgcgttccatccgagtagaccaggtgtggttacggtagtacatcatgtcagtgaagtaatcactgtagatgtgcaacagttctccacgttgatcaccggtaccatgagccaagccatggtagtagtaaataccaccatcttctttgtgggtgtaaagttcagcgttgtctttggtatacatcgacatttttattactccggcattccagtgtgcacaagagaattgaaacgaacatcgaacgtatcgtacatatccgatgttagttcctcgaagactggactatccatgaaggcttccagtgcgcggcgagctgcaagacgcttatcaccttcaccattagctccgggataaaccgaattaccctcgccaggcttggcaaagccgtcaaagatatgcgactcgccttcacggtcagtcacagttgctttaacggaataacccatgtaacggagtcccattattcatcccatccttttacttcgtaccagagacaggcactattgtattcaacaatgtaaccgtctttacggaggatttccgcttgacgattattcatcttcccttcaactggcgtgttctcgttgctgtaatcgaagtttacctctgaatcaccagcgagcgcccgttgcttaattttagcatggattgattccataccagcttctttataaagaagttcacgcagctcttgtaatgtcatgtaactactcctacaataaagactcgactgatttcattgagataagcgagcactagaagaatacctgtccagatagcgatattcattgtagtacgcttctcttccaatccaggattagtggaattaactattcgatgacagaaagcaccgaataaaccaagacccatcaccacgaagatgatggtgaaccaaccaagatagatcattgctgttgcaccggggtaagttgtttgagggcattgatgatacggtgaacagtatcacgtgccaactcgcgattgtggaagttattggaaatctgatactgaagctctacttcgcccgtttccgagttccgatcgaaatcttttacagtgtaactgctatccaagatagcttccaccatttcgtcgttaagtttgaactcggcaatcgttggcgaaactaaacgcccctggagatttctgatgacctcgttacggaacgcgatggcgccttctgcaatctccagtcgttcttcaacagagatgaacgggttcttccagagttcggtttccattgtagggcgaacagaagctttctcccatgcgatgcaccaatagaaccaacgttcttgaatttcttcgttggctttatcgaatgcctctattgctttcttattgcggaaacagtccattgggcgagtatctttggggagccaggtgtcagttttctcgtaataaacgaaacgatctacacccggagtcactgcttggaattctttcagttttttgtccatgtgaaataatacctattggctgatagtatgtaaggagattacgcgttacttcttattcctactgctgggttagtgcccaaaacgcgcaatgcccgagacgaactctttggcgaaaagaaatgggatttagcccctaccggaaggtaggggctttatgccgtcaaccgacaataagaccttcgatcgatagggtctcggtatcggcggcgggttgggtaagacgagttacacgaatataatccgtgtagtcatccagatccaaacaacagctgcaaccacgtactttgatcttggttgcttcgatttcgaaatcatccagcttgatatcgctgccgaagtgatcgaccatacgttgaaacaacttaccgaacgagaacgtttcgtactcgcagtcgatatggaggacatcaacagtgtccaccggtgggttataactactgctcatttgccatctccttacgtttatttttagcccagttcttttcatagccagaacgaatgaatttacccgatccagcattgagccaatagcgctcacctttgagataacgttcccgtttagcacgggtcaggcgaagaggatcgaacatatcctgttcctggcacatgaggcgatcacgcaagaagcagttgtcgttcaggatacgaaccgaatacaattgccccagtcggcagttcgccagttgggctttctcagtgcgcaacttgtgttcatatgccttagcatcttcgtaacgattgcgaggatgtttctttccgagtttacgagacattgtttttcctattttgttaatttacgaaaaatcttatcatggaatgtcattgccaacacgacacctatggaaccacctagaccactagatataatagcgggaagacccactatcacaaatagaccaatggtggtcaactcaagggtactgataccccacgaggtgaagaaagcagcctttttataaccatgaaagatgtttctttgctgaaaggtttttacaaaagcgtagatgaatgatgtggctgtacttaatagtagtaatacccagataggtagatcgtgattaatgttaatcacttcccttgttcccactcggtaggttcacgtttagtacgctggatgttgtggatatcttccagcttataaccacgaccagtcgccatgtagatatgctctttgtcgacatgagtttggaatgcagtcagtgcttcaacaggagcttccagagggaagtattcggtgttgttgcaatcccaacagaattcccattcattatcacgaacttcgtagctgttctcgctgaggtaagtaatattgatcgtgtgcgctgtcgcattctttccatcgaagtggtaggaacctacgttggaacgaatatcgatgcgcccgccatcgatggtgtcttggtagtagaacccacgctcatagaaaaacttcagcatcgatacgaagtagctattcagcactgccttagcgttagcttcattcactacccatttcccatcgacgatgttgttcaggtaatcacggtcgtgattgatcccgaagtcatcaacgatatcggcgtacagcttgtgatatttagccacctcatagagacgttcgagagtagcccagaggaataccccattgggctgcaagccgagaatgattcgacctacggcccacatcccacttccattcaccttgtagtcttcatacagatgccctttgatattagaaccaggttgcagttcatccgccgggtaaccagtacgaagccgggcacgaataacattcagaacagcttcaccgttattgatgtccacaaggttaataccaaaggtagtccagctaccacggatacgtccctgatatgcaatacgaatggcatttccaaattcagagatgatccaacgatggtcatcgtcgatcacgaaacggcagccgttcttccacagtgcaaccaaattatctttggccgccaggatacgttttgtagcattatcctcggtagcggccgcatcgggtgaggtacgcagataagacaacagaagcagctcggcagcttcgttggtctgagtggaaaacatagcgcggttcagacttgcattaatgatcatggtaatttcctttttgcggtttatgggtttattactaaataaaaaattacgacataaaaaataaaaaaggggacccgaaggtcccctgttatcacgcagctacatgagcataggtcaatgcattgcatttcggtttggtcggagagacctcactgaagaacattactcgatcgttgatgtactcacgggcgtgttcttcactctcgaagaacatacccatggccagtttatctttcacgttttcctgagttaccggaatgccacgagcttcgatcaccaccgcccagacacgaccatcggtatccattacagttaccagatggaagaagatcttggtcggattgggcatggcagcagtagcgggtttggaccactctgctacagtacccatggactggacagtcatgtccgccgtattgcgctgatgcatccaaccttccacagtcggtacaccgtttttcaggatgatgatatcataccagtttgcattgttacgcatgacgcagcgttcgtatttgccaccggcattgacattacccatgatcagcacatcgtgaagcggaacttcgatgtgagtgatcttggaagtatagtcaggaatcagtcgatcttcgacctttacccagttagctgcacgggggtgagtcaatgcaacgcgaacaacgcctttgacggcttgttctttaagggcagccattaccagaactgcttgaacgacgtccataattactccttaatgcatgttttctattttgacaatatcccactgcgacaattcagtgtcacgatagaacttttgaagtgcctcttcgattcccatttgagagggagcctcccagacagtaccattgtaacacgtgattttccagagcatgcctattccttattgaaagttcttaggaacgaattatttgataacaaccgcttccgagagagtttccatactgctgataaccagtttggatttatcttcgtcgggttcttccattgcttcacgcaggagttcaccgatggttttgggttgaacgtcatcactgatttcacgagaacatgccgaatcttcatacatgtcagtcatctcgatgtcgtcatccaaaccagagtcgtagtacgagtcttccatggagtagcacgattcatcagaagaatccgaagactctccatacatttcatcgaagtcacgttccatttctttttcgtacatttcggacattgctttgttatcttcttcctgcgccttacgacgagaagtcttgtagaatggcagcaagcgttgcaggactttatggaacttcttcttgctgatcaaccagctaccgaaataacgagacagttttacttcagctgccttgatagtcggatcagcatacatcgctgctaccagtttctccagatcgtacagatgatccttcgaagggttggtatatgcaggatgctcttggagagcgaacatcacgaacgtacgcatgtcagtgatgaagtactggttgtggtgcttgttgatctcgacgtagaccggatcggtatgacgatggtagtcgaactcctcagcccaggtcaggttgcgaaccttagtagggcgaggaccttctacccaacgaacagtcggatgtttctcacgaatgttccaaccatgcgcacgatcgtactcagtcggttcttctttgaaccaggtgaagttaccttcgccacgttcgaggatctttttacaccagctaatgttgatgctgtacttgcgtccttcgatcaagttgcagggtttatccagaacagcgacatagctgtcatgaccattggccacgataccaagaacggtagcttcgaaggtttcataacgctgaccgggatacacgcgttcattttcgtccaggaaacggagagaacaggactcgaagattgcacgggtaccagcagggaaatgagcgcggccgaaggggctctcggctttacgttccttgcgacgttcgataacccattccagtttttctttggtcagacgggtggtgggttcgcgatattgtttcatggtaatttcctttttacatttgggtttagttgagtacatctcaatgcatcctttccaagacacattgagatggggtctccgaagagacccatctattattcttgggtcagttccccaagacgaccttcagctttcatacggcggatctccgaaatggacttaccgtattttgcagccagttcctttacggtgccttcaggggcaggtttactcatgttgcgaaagttttgcttggcgatgttgtagttttgagcctgaagagttctcagctcagaacgaaccaaagcattgccaatgcactgagaggtgaaagtgaccatgaaagacttcagcttatcacggtacgtattgacccatgcacaggattcatccacgtgcgtgcacatgtactcggcggctttggcatattccaacaagccgactgcatctggtccaacatcctggtaaaccattttgttgaaaaggcccagtgcgatatcagatgcacgttcagctgtaatgaaatcgattgcatcattaatgatcaacgtttccagatctttgaacttaaccgcatcgtttttgatcaacgccagcatagcgtcaacctttacggtcaacatcatgtcttcattacgacgattgaccagttcattggtctgctcttgggtgaacacatggtccacgttttggaagactttcgacagacgactatccatttatttatcctcatttacagtgaatgcaaacatagtacatttcggtttagccggatgttgacaccattccttcgaaaccttaccttcgggtttggtcagttcataatagaactcaccgcaagcagcagcgagtcccatcagaactgcaagaaaacctacacctattttggttttcacttagcgatgatccgttgtacgaaatgttggagatttgcaaccagccgatcgaactcttcctcggtcagctgatcacgatgagattccagaagtacttctacctccggaagaacgttcagagcgatgtccagctggatacgcgaaatgaactctgcgacatccagttcacgatcacgcctgagccgattcaccaacttgcgatgttgatcactattacggtaggccgagatcttatcgataagaatatcggagataccgctttcgatctgttccgctacagttcgcccttcttccttggtggttgcttttacggcgaggatagcagcaacggcggttgcactaaccgccaatgcaatgagaccgtatttaacgtaggtttccatcctattacccccaacccatttcggatttgaattcatcgatgcgtacatcgaatgcagctttgtactcaccgtcacgatcacgcatttcaatagccattttaatgcggagactcaacaggccctgagagaaacgcagacgagcagcggtatcattctcgatcgcagctttacgtgcttcttggatcagtacgtccaaccgcttactgaaatcagcgaaaagaatcttatcgttcagactcttagccacgatatcagtaccgatcatgacaccagcgacagccagggcaacgccaagaccaattgccatttctttgaggacttgattcatttgtatattcctattttcgaatttgaagtgagaatggattaacgcagttcagcttttggttttgcagtttcgtccttggtcttacgacgctcttccatccagttgttatggtaagcagcaacgccgacgaagccgacaacggctacggcgatgagacccaagctgagtgcattttctttaatgaagtccatgactattaccctttcagagtggcatccgaattgaagacgtcgggaccaaccgagagacttcccagaagatccggagcaaggtaaacagagttgagggtttcgtatacaccagcaacagtgtctactttaaccaggctagaactgcgcagggatacccattcaccgttacggaaggtttcaccgaccagtacacgaacatcatctacgtcagtgcgatttggccatagatccttaccttccactatttctacgttacgcgcatggtagaccagtttaccattcatgcgagcaacgatattcggacggcacatgttgtcgattactttaactgctacggacttttccatttttatctccttatttagttacgagcatttcttggccattgggaccgatacgatgaccgagaataacctcggattctttttcaactttcggagcttcataggaaccgccgtaaacaacagctgcaccgagaaccataccaaccagaaccattacgatagctttcatgttgagtttccttctctagataggggtattatcacatttgtaatatacgttttaaaaagacttaaatgtacattcgaatatgataaaaagaaagggctccgaagagcccttcttattacagtttacgcaggaacttgacaacctcctcacgcagttcgcgcagagttgccgtcagcagaatacgttcttctgcttcatggatcaggcgttctgccagatcggacagttcttctttacgtttatcgagatcgtaatccggcgggattcgatcattggcgtcacgcagtttctgcatgacttcttctgctgtgttctcgtcggtccatgtaatggcgatcatcgagattacaccgccgactacaacacaacccagaccttttacaaaattaccgaacatgttactttccttatttgcagatggggttattgagcagttgtttcttcagccggagcagaggtatcctgttcttgaacaggagattcagctgcggtatccgtggatgcatcatcgccagttggttcgacaacgttgtcgttcagagtttcatacagcttacatgcagctgtaccgagagcgataacggcagccagagcaccagtaacaaccagaatctttttcatgatggagttccctttttaaggtaggtctcgatagatgacctgtttgatataatgatcgacacgcggttcagcagtctttcggattggctcgtattcctgatctaggatctcacgaacctcttcccaacatgctttacgtagcatcgcgtagcgtctctctggatcaccaaagaggtactgactcctacggagcaagacatggtgatagctttcaacgaccttaccggccttagctacgactttattaaccatgtctatatgcctttgcattagataagctgcaccagcaaaaccggatacaattatacctaatgcaacggcaccaacaacatagcgggttttcatgcacccactacttcatcgtaaagagtaccagcaatattcattgccaggataccgacagttacgacaaatacagtttttacgagagtgttcatgtttattctccttgagcagcattgaatacttcatcaactgcccaacaggcagcattaacaacgatgatgcatgcagcgagttttacacagaagcgtgcgagtcccatgttgatctccttgatctgttgactaatatcacacttgtaatatagcctttaaattggtttgaatgtagtctttagactacggacttacgagcgatgcgctgaagcagattctgatcggtgatgaaatgaccgagaacacgatcaattacatcgtcggccacatgttcgttgtgattacttacttcattacacagaccactcacgagtccagcttgacgaagtttactttcggtattagcgatcgacttaatacgatattcgcgaataacttcaacaaactgacgttcaccggctacgaaactactcttcaaactagagtacctgagaatgttctccatcttaccgatcatgttatccatagttttcatgtgccagcgccagatatccgatttgatccctttagctagctcatgttgacggtgcatgtaaattgcataagccatgtaggccaggaaagcgattacacttacagctacaattgcgttgattgcgatattcatttttcaatttccttttgggtttggtttgacacgacataaagccctgatcgaagaccagggctttttaggtttgattaagcaagggccgccatccagggcggtactacgaccaccatctcgttagggatatgactactgaacttttctaatgtttgtttaacatcaggccatttcagcatgccgtttccgcaaccgagcggtggtactacgatcttccacttagggtcgatcccatcttctacatcaatattgtcgactatccattggaggccgtcattgatatagcttaactgtgaatcatcttgccaacgatctttcgttgggaacatcatgtaacgtttaccatcatcggcaagatagatggttgggttaccgatggtgatgattcgatacttgcaatcatgtttatatctttgatacagttcagggaacttctcacggaagctttccgctaaacctgtacccattacgccacgggtattaacagttattaggtaaagatccccaggctctttaaaaatgtctttacctatcacgaattcagccatagtcaatggctcctttgtcctacaaaatctaatggtcgcgaaaccacaactcatcagattgtgcaagattaggtgaactcattcactgccttttttaccgctatagtaagggtaattgcagcggttattaaagcaataccagcggttgcatattgcataagttcacgattgtgggcgtactcacgacgactcttttcgttttcttcgtgaggtttattatgatcatagaacatggtttatccttagaagccgttgaaaatgattgttgcaacaagagatataacgaacacgattacaacatgctctagtttaacccagctcggtgggacattgggatcactcttattggaacgcgggaacatttcttccttagcttgttcttgcataaagcacctaatataactggtttattcccaattgtgatatagggtttaaaatgctttgaatgcaaggtggacactcacgaagttctataatgaacgcctctatattcccttcgtcgttgcaatatgtctttatagtctcgatttcaccttttaagctattaaatgctaatcgatgaaagttatatagttctttgaaattaccttcaaagaaacttgtatcgattggatagcgttgtagttccataaggatgtattgataccctttattgaactctttagcgttgtggttataaataaagttgtgctgtagtttcacatactcagtggctaaagagtataagtggtttactacatctattgaaagatcgatgaatccttttatagatccaataaagttgtatgaccaaacgtggtcaatacgaaagaacacgttctgcatatggtcctacctaaataaaaacccaccccaattacggggtgggctctataccgtcttctgttacttcgaagcgattaatgaaaacgcccaatgtgactttaccgacgtggcgattgactgtggccccagcgtcagctgatctacgttgttcgtttacacctaataacacgccgtggtatgttttcactcggttatcagatattgtctgaaatttaacaggcatccccggatagagtaaatcaggattaccatgtgtccattccaatttgatctcttgtccttgctttctagccatatccgtatattgcttgaaagggttagatgtcaatctatcttttgcccagcgaacgttattgaatcctgtttccaaatccttcatcttgacttcgaataagttagtagccctatcaactaacattttgttgtctttgtcaattgcaaagtcttggaatactttacgagcatccccaaatcggaaagagttaccattctgaagttgctcggcgagtccttggtcaagtgaagtcgcatcgccagtggctaacactgtgatatggcgcatcgtgtttctaaacgtcttctcggcaccctggtaccgatcattaggaacgttgatcaagtttagcacttttgtattctttccataacgagttgtatcgtaaagaggatacaagaataaaacctgattttgtatataacgtccaatacccgtagaatagattcctccttctttatcttggaagaatcgatgaacgtctttcaaaggcattccatctgggatgataatctgattacgttcttcttgactatatccatctgcgatatcgatggcaagtaatctttggctatccgagcctcccactaattgcccaaattgcgtccacagtgatttaagagcattcattgtggtcgtaactcgatatgtagtgccacaagttaccatcatcagtttatacgtcagttcatccacaagttgcatctgtacgctgatcaatccgatctggttcatcgcttctctggatttaagattagagttctttcctgacaaggccgggttatcgtcaccactaacggaaataatccctcggtaacgtttggtaactgctttccgttcgacgttacgtgtagctactgcttccagtagaggtatctcagatacatcgacttgtaggttatcgcgataagggacgatatcatggacatagtcaccataaccaattaagaactgaacctctctgatatcaccaagttgaccactcccgtagtctctattcaaataaagaaaatcaagacgtacaggagtaatccactttttattagcaaggattttaatctcattgcggaagttagaatagctttcaccaatttcggtaacctgttcgacttcacgcattaaaagcgtactatcgacagacattattcagcctccacgatgtaacgttcaatctgatctacgatagaaacgtatggctttaatttaccttcgacttcactacgtgcctgcaaccacttattagtggatgccaagttacgacgacggttcattgccacaagcgagtcaaatatttgactacgtacgtcttcacgcggttccagctttttcgctagttcataaacctcaatagcaagtgcttcgaaaagacgaagatcttcaataggtgggaaaccagctggatgtgcatggaatagagtttgttctcgccagtcacccagatgtttctggatgtcagcatagatctgcacgcagtctttatagttaacgagacctacgctatacccctcacccatcatcattgcaataccagcggctgtttgttgaccacgggacatttgcgatacacgttcacggtcgactagtcgatctcccgttacgttgatatggttattacgtagatagttagtgctataagctgcaagatctggtgtaacaacttcataacgaagatggaacaaacgccatgccgcagtatatcgttcacagagttgcattggagattacctcgttgcgtatttaagtagtgctatcaggacagggtgataataaaatcgttccaaattgtcccacgaaaggcaacatttcgtcacttttcttaattggttcatgtccataggttgacgattgatcatttgccaagttaacatttccagtttagtctggagcttggcatcttccgtataaaaggcttcggtaaatacatagaagttatcacgaactacgggcgcgatgtcagccgggcgatcccacgcttcatcttgttttatgacatctggatcagcacgtttaaaccattcgctgtttcgttcttcttgcgtcttatacggtatttgaggacgacggggttgaccttcatggaacggaattccttctggtcgagcacggtcttcaccatcgtattgtgaatccacgtcagttggtccctcgatagggaacacgaacctagggataccggtataaccaattgcctgtagttctggccgccagcgggagattctagtagctacgagatgtgcacgttcagtagaaccgcaaagacgggtagcatcttgacgtaagatagcatcccaaatagttggttgcttcattacaggttcggacattacattcagtaacttaacattcatcatccgtcgatcagttttcatgtcaaccatcataaccatcgctttagttacaaaatggtcataggttttcattaactgatctggtaccaggaatgtactatgttcaacagagaagaaatcactaatgtatctccgaatgatctctttacgaagagcagcaaaatctttttgatcttgttgttcttgttcagtaacaaacggaccacaaccactagtaagagaacttgcagaataatagtaagtgattatagtcttacgttcaaggtcttctacttgttgttcattaagtttactcaccatcttccattcgatagcgtatgtggaatcacgcaagaatgtttcacgacgagccgccgtaatagtgaatagacctagtacaccatcaccaatgttaccaatgaacatatctccaacgttaggaacgaggaacggatatgtgtgtccggcaccagtaacagagaatgtacgaatacgttcatcttgggaaatatctaaagactggttaaccttaagatccattcctttaatgcaacggtattgttgatatggtggttgacgatggagagccaggggagttggttcttgagtttcgtcaagaatttgtgagaaatacgttacgttccagttagaaccatttatccatgcaagcatcgaactttttggtacgaactttgtatcaatggcaatgccccgataaacctcggggcgtgctttgacagtaacaggattaacttctggactctgaggagcaatttcttcctcatctacaaaaagagacatcgttaactcctaatgtcagaaataatgtgcgaaaataatacgttcaatggaccgactttgtgttgatctatataaccaccactggctccaacttctgcgatgatcttgtcttgctcttcacgagctttagcaatatcaccccatttcacgataccacgcttaaacgtattaggcaggtcagacgtgattggtgtagtaccttcacctggagcatcgggatcttctggacgaggaccacttagacccagtagttccattttctcgatcgggttacgaccaatactaacacggaacaaccggaacagactccagcaggtagttggataacgacgaatcatctcccagtacttatcatggataccatagaagttcttagagagactaatttgaatgtggtagtacttcaaaggatccagtgggatggttgttctcagaagagtagtcccaggatcaattgtcatcggtacacgtaaccgctcgttattttggtacaaccggatttcaaagaaagagccatctgcgattgcagctgttcctagagtctggataaactcaagccaatatggattgaatgtaaatcgacctaggttcttgaagtccatcagtgatgtcaggtcatctttactcaggcacaacaacccattaaagaatgtgaagcggtgcggtggaatttggtcagtatgccaatcatcgatatctggatgctggatataaggtagacccatatctcgcattaagagaaattgatgatctaatgttccacgtaaagatgtagtcttccgatcaaccgcttgataattctgatatcgatactccggtcggaatactttaggaatagtacactggttcattaggattggatagttaacacgcatatgcgtaggtcgttcataacgacacagatagctaaaattaacagtgtatccaccagcattatcagacgacttttgtggcgtatctggagatgtactaaagtcaaaccaaccgaccacatcaacttgacgttcgtatatagaaagtgtaggatgtgtacttgctagggtagccatttcggtttgaggttggcaccaatgtttctccatccactcacggaaggttagatcggttggccagtttgacttctgcattgtatcatacagtcctttcatcaaacctaaaagagatggagggacattatagtgatacgttagagacattgtcatctcagcaccgccggctgaacaacgtatccgttgatcgtctaaccagcgttgagccagtaccacgttaggtgcctgatattcaatgtctatcctgaagtcaacaaaacgtcgaatcggtcgaatagtaatatcatgaacatcatcaacgaatagaggaaagttctcgttgttataaaccgcagttgaaagagtaaagttctcttcggctatttcttcatatgcaactgtaatacgttcttctgggtcaaagtgaacagcatcggctgcatcgcaacagttaccaaacataccgtcgttcataggaacggtatcgacacgtccaggtaggtaaactcgggtagcaccgggtaactgcatcattgtagcaatttgtcgaatagcatcgactgataccttccgcattacggtttcgtatacgtctggcaaggggataattgcatggggcatggtaaccacctcatggtttaagatcataagatccggcataaagccctgcctttttagggcagggcaatatgttgttacttacagagctttacgaacaacactaacaataccatctgccacgtcaagagcatgctgtgttacgaacttatacgcatccacatgcgcgtaagacactttcagcattgcactagccagatcatccagctcagcttgttcatcccaacccgatgcacgggaagtagtatcgaactcactggagccagtgctcaatgcacggttgcgtgtaacgtcgagattgataatgtcatcgatagctttagaaccaacggaatcagcaagcttatcagccagggcgacgtatgccttagccatcttaagcatgttcgctagatcagctttggtcacatcgaaactaacttggcgatcctctactttgaccttcttgaagacaggtaccagagtatatgccaaagcctcgatcttactatcgccaccgcgtgggcctttctcgtattcaatagcccaaccacccatgagagcgttagccatgttttccggatacttggcaggtttgatattcagagcagtcttaactagcggaccagtcttatcgtaaccaccttcagtaacagccttgttgatgacacctactacttcttgcagtgcacgttcagagtctttaacgcccttaacagcgatctcggaagtgacacgaagatcttttgcaatagcttgcacgaggttagtttctttggtggctatatcgctagaaatacctttaacggtttcacgcccgatattggacttaccaagtttagtcagagcaaggtcgacatctttgttaagtgcttgagaacgcttcttaactttagtaacgaggggaccttcccaccatttaatcaacttctcgttcagtgcacgcttcagaccggtaatacgactaaggaaaccgcggaaagactcaagactagcagcatagtacttatcgagatcttctttaccatattgctccatcgaaggaacggaaggagcatagtcaccaaatgctttcttgagttcatcaagtttaacttgactcaggataagagtttgaacactatagctttcttgagagagaccatatttcagaatctccatgaagccttctacagactccttctctttctgaagatcttcgattgtacgactggcatcaatcgcttcctcttcatcagcatcggcttcttcttcggcctcatcggcttcttttacggcttcggctacatcgtcttcagtgacatcagtgtcaacgtcctcgatatccagttcaccttcatcgaagttagcttcaccgtcatcatcgatttctccatcgggttcgtcttcttcgatctcttcgaggactggttcgtcttcagtgacatctgtagtctcatcggtagactcggattgatcttcgacttgttcatctacaacctccgcttctgtctcaacaggagtttcctcttcgttgacgatgtcttcttcaggagtttcttccacttccgccggtgtttcttcttcgacttcagtttcctcgactactggttcttcctctgctggaatttcttccacagtagattcttcagtttcagtcacttgttcttcaactggagtttcttcagctggaatatcatcagtggaatcttcagcgatttcttcgttgacttcttccgtttcagctacatcttcagaaacttcttcttcggtagtttccgcgatagactcttcgacttcgggtacggtgacttcgtcagcgccttcttcaacttcaggggtagaaacaccatccacctgatcatttgcttcggtttgagcttccggttctaactcaggtagttcttcatcaccaccctgagtttcaccaccttctacagtggccggctcagtgttgtcgagttcaggggcagcatcactgacatcagctacttcttcaatctctgcttccgaagtctcttctacttcttcaaccggggtttccggttcttcaccgatggtatcagcggtagcagtttcaccaccgtcatcgacagtagtttcggtatcaagagattcaacatcgttagtcagttcggtttcaccagcaccgccgctattagtgatatctacgttttgttcaccagtagtatcttcagcaggtacagtgttaccatttacatctgtctcgttggcttcgatggcctcagcatctgccgcggctgcttcaacagtttcctgttgggttgcttgaatctgttcggcctgttcagtgagttctttcacttcggcagcttgtgcttcttcagcttgagcagcagcggcctcagccgcagattcattggtagtagccataggttctggaataccagacggctcttcactggtttcaccagcaagaggttcttctaccgtttccagatcaccatcgggttttacttcttcagtgggggtagcttgcgcaagttcatcgcctgcttcaactacatcgctttccggttctgcggatgcttctacattagtagcatctacagtttcaacaggcttatcttcaacttcggtggagctctcagcgaagtcttcaagactggtgatatatttgtgaatgttcttcaacatgttgtttaccttctgtacagaatacgagtagcgttattcgtcctaaacgctactcatggacgaaacactgtttcagattattgaacgccaaggcctacttaatattggaacgacatacattaagaacagcgttaagattacgcccggcaagagccaagatacccaagtaaggattagcaagccaatcaatgtagcgctcaagtacttcaacaaactgacgtagaattgcttcatctgcgccctcaacttgatcattgacaatctgattacgaatacctttgacaatattcaacattgatcgaatacgttctttccgacgatgacggatactcataccacttgcacggttaaacatctcggccatcttctctacttggcgcaatacagtaatctgtacaggtccagagaaatgttgaaatttaattaaatctggaaggggtaaaggatcacgttcagagttatctagtttaacactgatacccaacattcgatctataccagttgcttctggcgatttgtcaagaactacgacctgataattacccatcaggtgaagagactcatgccgatatccacgatgactataaagtggattagaagaaaccattttaaccgggttggataacatgattgtttcaacgagtttatttaattcctcagcggttgtaatgcgctgtgggatatggaatgctgcacgaataagttcttcattattgtaatcaaagaactgtttcccaatttgctcaaggttctttaggtttgcaatcaatccctgtacttcattgatggctttataacgaacacaaagattttgaattcgagtagtcacatcaaaggtcggttcctttgaacggcgtgcagtagtacgtgttaacgtattaagttcttctactcgaagaaggatattgtcaaatgctagagataaagctagactaccatcgaacatatcttccataattcgatttagaaatgcaatgactttatcaagaatacctacaacggttcctttgaaatcttcacaaccgagatctagtagatgtgattctctttcaaacattggataattttcaaaaccaccaattagatcaagaatacgattagcagtaacttcatctttctcaagtagcgcactcagtgccgcaggggagtcatcgaatacgacgatttcctcgggtggattagattccacatctaggggaatattttctgtttccattgttaactcctgaacataagacgggactccgaagagccccgtctatgtcttagtctttagccggctctttatgcagcttagcttcttgaatataaacagaagcgtatgcaacaacagtacgggttacataccggatgatttcacgagaacgcgggttggattcacgaatcagttctagtgcagtctgagttacttttcgagcagcagctttagatgcatcgtcgagatcttcattgttaagctgatcttcgattttactaactgctttcttaagggcttcagcaccttctttgatcttaacgtgttcatcgcgagctgctttcagaatctcgatgatatcgcgaaggcgcttcgtattggtacgcagagtacttggactggatactttaacctcaaattccgccggtgcttctttggcagaagtggctggaccaataccgtaaacgataccgtctgcttgaagttcaacacgcatgttaccagggaagatatcgtagtttgcaccgtagatgtcatcaagaggagcggtagctttgtacaacttctccgacatctcttcgccatcacctttaactacgttataaccgctaataagtttagcaaggttctcgtagtatttcttaacagcggccgggtatacgtaagccgagaaatgagctagaccactgagaactttggtatcaccaagtttggatttaccattcgcaaagacaggcgccggattgttaagaacaaaggtcttacctgtaccggtccagagattaccaccagaagcaagaatctcttcgagttgagtgacaactttatctgctttggagataccgttcatcagattatcgataccaccaataatggcgtcaatgatcttctcgatgatttctttcagtttctcaaatgccttgttggcgtattctttaatatcttctacagaaatttctgcacgaagaatatcagaacgttcgccggcattatagttttcaagtcctgtggatacctgattagtaccaagaacacgttcagcttgtttaataccaactcgaaggaatgctgccgtctgctgagaaatctccccacgagcttgacgcagtagaccggaatacgcttcaagggcatgttgcgtttcaatcagttcatctgcacgttgttcaaggatttctttttcaacgtgagcatgcgatacagcatcgatttcaccaacagcttcagtaacgtcaactggaccttcgataggagcaaactcagcaggtacttcaaccggctcggtttctacaacagtatcggtaccaactgcaccaatttcgggtacaggtgtcggaacgggtaattcaacaggagcctcatcgaccacattggtcggtgcttcgatgacttctacttcttgtgtttccaaaggagcttctgcaacagcagcaacttctggagtaatcggttcttctttgaattcttctagagaaccgacgtatttatgaatggatcgtagcattacattttcctcggaggagaatcatcgcgcgatgatgattgttaataaccatagaattggttaagaggtcgcactgagctctaattcacacactttatttcgaatgttagtgatagcattaatacgtgcaacaattggaccatagttcggccgtaatttcggaataagatccattacaatactagacactcgatctagagcatcccgagatcttttccatactgtctcaccacgacgatcttccaatgcaataagatctttggttagacatttcatttgctcaagtaccttagcttcctctttaaagagttcaccaaggctatttgtaacgaccagattctgtttaagagtcttttggatttccaatcgactgcgcactggatgttcatatgtttctggcccgctggtcatatcctcatcatggatgaccattggtagaagagatacgtcacggaaatggataacatagttacccggtagaacaacatctttgagcggatgaataatactggcatgcttaccaatgaattccgagttcgcttcaaatgtcgtgatatcaccagtttctacatcgtaactcttaagggacttacatagccgattaatattatcgacaaggtacttcgggtaagtattaatgaagaacttcattacagtggtttcagctttgaaatcatccaggcagaactcagagcctgcaaaaagcttggaagctccattaacagtgatagttgtaccgttgtcatggaattccatactggctttcttattgctgctctgttgagctaacttaagaagctcttctgttttcttttcagttgagctgataccagagataacacgttgtgcgagtagtttagcttcatcgattatcttttcgatgagctcaaggatttttctacccacctcttttaaacgatcaactagtgactcttgtgaaatagttggatcagtaagaagtgcttcaattgatacacgttcttgtttaccaagaatacggtctatatgctcaagaccaatagccatgaacttacgagtttgtaaacttaggccatctcgacctgcatcagttaattgatcaagataagcttcaatagcgatatgggcttcaaacaaatctttgaattcttgttcatgatcattgacgatcatatccggaagttcttcctgaggactatcttttaattgcgggcgatttgctggattctgacgagtgtccattttgatttctcgttatgttaaacatagaatttggcatagcagtcataaagccctccatagggagggcatttatgttagtacttagttagctcgtgtttagcgatagctagtttcgcaaaaacagaggtaacaatctgacgttcaacttgagcaagaacatcgagagaacggatcttagtgattagacttgtgatggcaccaaatacagctgggtcatccagctcagtcactagttttgcaccgagggagtccgatagctgttgaagttcaccattgtgccgatttacagatgcatcatcggtcatgacagctagaacagtttcacattcctgagcaaatttagtgatagcacttgctggacggagatcaacctcaataggtccattcgagtcagtaccctgaataatcttaaagcctaggttttccatatcccacgaaagacggatactaccgggtaggaaatcttgaccgatagaggcttgaacaacttttgtcatttcactgtgggtgtgatctagaacactttcaatatattcagaagcatcgcctttaccaacattatctttggcaaatttcatcacggacattagtgctttgggaagacgatcgtagaggaatacagcgtaagccttttcagttgcgatggtgtcgtatgtgttctctccatcggcaacaatgttagtggtatcttcaatacgaatcttcttagattcttcgtcgatatcacctttacgctctttaatctcagcagctttcttcttaagatcttccgaaacattttctggaacagagccacgcatcttaccgccaggataagcagggaaggcacgagaagcagcaattagttgttgtgctgccttttgtgttttaactttaggaccagccagtttttggtaaatcgccttcgctcgttcaatcagcctagcaatgaactctacaatgcgcttaccaagctctttaacgcgctctttaacatcttccatggaaacagtagtggtttgtagtccatcgcgcatagtgcacgttttaaagccttccaggctaagtgcttctcgtttgatattgagccgcgcatcaatctgtttcatgccaattcgcatcattgcagcagattgtttagtgatacctttgtcaccagcttgtttaaggagttgagagtaagcttctagagattcagcgacaccttcgaggtcttcggattctacaacttcttgttcagctacatcgttttggaaatcagatacgtcttcaatctctacctggatatcttccgctggttcgatgattgtttcagcaggttctgtatttacagtacagggcatttcagtgtcaagcatgttagcctcgaaatagaattagtttacatagcataaagggagccgaagctccccatgctttaacgggtggaagcatccatccagttgattagaccgcggatgtaagtgaaatagaattcccactgaccaccgccttctttgaagaatgtggcttcgccatcatcagcgaattcagcaatcttactggcaagcttaacacaccatttctggtcttcacctttagtgtacgtagcaatgttacggataacatccgtgtacttaccggaaccttccatgtgcgctggaataaatcgaccaaatagaccgtactcattctcaacgttgaaagtatcccaccactctttgcccatagatgttttccaatagccagtgatataatcaatagctttaatgatctcatctgcggctgaggctacctgttctggagtcattgcaggaagagtaacgtctacgtaagaatgtgccataccactgttatatttaacaggtttgaacttattcttatcaaagcttggcatgccgtcgtacattttctgagtcttctcaggatggttacgatattccatcttgatcaggaagtcagtatatggcttaacggagttagcagctcgggtaaacacagctgcgttaccacgggccgcctggttaagttgaccaactgccttagcgattacttgtttgaagttatccccaagagaaggatctcctttgaacttaatatcgccttcaatgaaacgacgattcttcagccaattcggatcaccaaacgttttagagatcttgctcttaaccgcattgtactgctctggcttaagatcttctttacgcccatgaatcatagcgttgaagaagtgaccgatttcggtaaagaggccttcattagagaatacgaacggatcgtgagactccatgccagcaccttgcactttaaggttctcaaggcatgcttcaagatacatggctttaccagaagacgtataagtaacaagagcagttaccatctggagattcatctctttgatcatatctgctacagctgtaacgtaaagttgttgtagctcttgaacataacgttcatcaccaccagtacgtgcagctttaattgcttcttgtgacttagtacgagcagaatctacaattcgagaaatacggtcagacttacctgcattctgatagaacttctgaagtgacttcaaagctttctcgatatcagtacgagaaagagcatctagttcttcacctgcatgttcatcttcaccacgctcaagaataagggcatggccttctcgaatgattttaccaccacctggaagatctttctcaacgtgatcacggttctgactcagacgtgtttcaataacatttctgaactcgttcacaccatcactagtcgcttccatcttagcaagttgttgaccaaggaatacaacgttagactgcattgccatggcagcagatacagctagatcaataacagctacttctgcacttgtatcagtgccaacgaatttaccgccagcatagaagaacttagctttcgatactttaatcttttcgttttcaggaatcgcgttgcgcggtacatcactgatctgagaaagcagcttgtctactttagcttcagattgtttacgctttagatcaaagttcttaatgtattcgatcagcttggcgagaagttcttgaatctttttgtagactgccccaccgatctgcttcattcgtccagtgatagtctcatcatcaatatcgacagattccattgccgaacgaggagtagtatcgaatgcctcaagtcctgttgctttgaccttgagattaaaagtccgatcaatatgaacaagacctttatgaagtactgcggcagattgcttagatacacgaccagtcttaacgacatcgtgataagcttctagagcagtctgtgctgtatgcaactgatcgatactattcgccacttgaccgatgcgatcatgtgccaacatagtttcttcacacatacccacatcagaaggttccattacttcaacaggcttatcttcttcaacgggatgagctagaggttccccgtcaacgttttctgtcgagggtttctcttcttcctgggtctcgctttcctcaatctcttcgatggggttagctgctgcttcatgggcttctacctgttcatgtacggtgggttcaaccactgactcactctcggcttccgtttcagaagtagcttcttccatagtctcactaggagaggctggattaacgataggttcaggagtagcgttttcttcaactacttcttcaacttgttcagtttcacttacaacctgttccgtggactcattggtaccctcaggagtgattgcaggttcatcactattttctcggacaacttcagattctgctctctgtgtttcgatattaggtttctcaccagtaccatcccacagaggttcatgcgcatcgccaaaatcttcgtggccataaataccttgacgcgtgacccattcacctttaacgaatacccagtcaacaccgttaacgtgataaacagcaccttcttctggattttctggtagatctttggtagtggtcaaggcttttacagaagtatcaactgtatcaactggtacttcgcgagctacgccatcagcaatagcttcgtttgaggaggtggctttaccaccaccaagatgtttgttcagattgtgaatagtcatttcgattctctgacatgtgaatagataacatagcataaaggggaaccgtgtggttccccaatatgtcatcaacccaaacgcttctgttcttcttccgtaggtttgcgaagaggagcctgatacgccttaagttcaaggtcggctaccatagccaaacctgcaattaagcgaatcataccagcgagagtgttgttatagtcaatgatcatccgcatgacattattaaggatcattgttagatcgttaacgacattagatacggatggccgggcttcatctctttcctcagcgccaggttttttacgaccttgactttggcgaagttgtccagcttttactctaatcttttcagcggattgttcaagtttacgaagttgagcagagatcttttggtcatagcctttgcgcgattgtaagcgtttagctaatccaagtagtactcctaaacgctgacgaacagcgtttatattcgacacttcaactttgttatcttgctcatttaatggtttctgttctggtacagtgtaatacttaaaacggaagtcccgaatggagtttaccataaactgccaatctttaagttgctcagtcttagtttcactcggaccagagaaataaagagccttattaccctgagttaactcagaacggaacaaagtagcattgactctaaacctgtcgtcttggtcgacttcaatagcccccttcatccaacgtttcgcattgaatatttcaaaccgaatagtggagtcatctgtccactcttgatcaagggtaagattattgaatgttttgtcgatcgcagtgagataaggcatgaacaccttatcatagaaatcaatggtgttttgtgtttgttccagaacaggtcgaatatccaatggtttaaactcgccattgatattaaacttctttgcctttctcagttcaatctccgatttaaatggtttagttccatttaagttcgaagccatctcataaagcatagtgattcgttctacagtacgatctataccagccatcagtactttagcgtagccatataggtcactattcgctctctttatttctaacttagtacgttcccaaacctgcctgctcgaatcactaatgtcttctgtagagacaacgtcagtgagaccgaatttctcaacagcataagctaacatctcaggactggctgtgtcatagttagactggataaatgtatcgagtcgctctatggtttccatccccatcattaacttatcaagtttttcagcacaagcatcgaactcgttgaattcatcttcaatcgagacggacagatcgacgggtgttaccccgtcgactgcgttaggttgggaatggttaactgagtcaaccatggacccctccttacttattgattttttcaggtacactaccaaacaacatgttcattgtgtacatgagatcatcgaagccacctttcttcttgagccattcctgaagcatgtcgttctcgttcggagaaagattgtagcttaggaaaagttcagcgatatcccgacgatcttcgattagttgaacacccgctggcggttctgctgtaagtagcattggccatgcatggatattcactcgacgtttacctgtggcaataaaccgtacagtatcttgcaggaatgcgtaattgtgatcagcaatcatggcattattatcttgacggataaaccagttatagttacccgagaatttaataagagcgagatcaattacacgtttacggaattcccaatacacagcgcggcgaggaaagttggtatattcaaccataagttcaacaacacgcggatcaccttggcgcatagtgaaacgttgttgagctttagcttgaccgccagaatactcacgattagcatcgaaaggtttgactgcattagtaggcattgtcaactccttattgtacgccagcgcgttcttcgatcttattgatctcgtattcatacgcggagatacgacgctcgtaagcttcgatctgtttttgcagaacagggctggtcggttctttagccagaagtgcacgtagttcttccaaccgaagttgaagaccatagtactcttcttgtgccacgttatatcgctcagcctgcatctctgcaatcagcttaccgatgatcaagaagggattctgacgaggagagaaaccagccatacccagaggatcagttttggtaagtccaagattctgctgtgcaacttggaaagtcgattcgtcaactgtagcattagaagcagcattaagcttttgcttcagtgcttgaggttgaagagtcatcgccggatacagtgcagcgaactgttccatgttggtatcgatccaatcggattcagccgacgtccatgcagcgcgggtagccttcccatgtagggcagcttcttgggcaacaaggaacagcagatatttacgaccaaatcgaatatagaaagccagaccttcgatgaacttgagcatgttagctcgatcgaatgtcaggtttgtattagtgaattggatcgagaatagactacggatttctttacgaataacttcgaagttaccacgaatgttatcgagagaacccagcatcagatcgatagccggctggttaaaagtaataccacgacgaagaacgttttccattcgtttggcgaggttagacttcagcgggataccttggaaagcttcccgaacatcagaaacaatcggggcaagggtatcgtcatattcggtctggagttgatccagaacgttcagcagttgacggcgctccattacaggtgcaagctgctggacatagttaagaatactcattggtcatgtccttggttaaatgttggtttgcatctgtttgctgaacatcttaaagatttcagtgatgtcttgacctttagatttctcagccatcttcacttcatcgatgcggaagctagatgcaatatccacaccacggtgataaatagtaacacgctgccaacgttcatcaacaacgatcaacatgagtagatagctattatcgaagatcttacgacgggtattcggatcttctagtttaccgtaaagagcattggcagttgttttcatcgtggtagacgaaacgacagcaatgttagaagcatctgccatagaaacacggccagtctgaacagacttgctcaggttattacgacgacgatcagtgatctctttgtaaactccggacttatcggaaatcagagctgcaaagtgtgcatcaatcatatcctgtccaagaacgaagtcgcgccagaaacgaatctgtccagttttaaccaggaacagacgatggctccaagtatcacggccgccggcactaaagatatgagtaagagtctgcgacggaactgctgccggaatgagacggatgagtacaggcagtttagccttagcatcaccatcggtaatttcaacgttcagtagtttacccacagcgaggttttcggtttcgtatactttctgagtatcacccgaagacatccgtggtgcagcttctttcttttccctatcacccttcttacgatcatcgtcttttgattgctcatacgcttcttgagagtattcagcaatcagttcaggacggatcttttggttgaacgcttcgagggacgggaaaccgttcatgtaattttctttcgagaagacagcgccactaacatcagcaccaatagaacggtacgggttcaggctatcgaatactttgagagtatcgattttacctacaccaagaaccatattaacagcttgcagataatatccggcgaattggctaagtgctattttaaggatatcttgcatgtaaggttggtcgaccagaacgctatcaataatagcaagtggttcaactcgacatgggcgagtcaaatctgcaagggagttaatctccatgctatttttggtcgcattaaggactgtggtcataagacctttaaaagcttggctaccggcagcagcgcctgctgcgccagccatagcactagctacgattggtagtggcatcgttctcttccttcatttgttcacagagatttgaaaaatggcattaagtgattatctaacgcaaattacacaaaacattgggatgtcgccgcgtgatcgttccattgaagattcattcaaaggcctgaacatcacaggtcgtaacaatgcgatttcgttaaatacagaaaaccatggttatactttctttacccgtccattactgaacctggctgaagataactgcatggtggacaggcgactgtccatgatcctgaatcctaacccacagagtatcgagcgtatggttagggcatatttggatccgagagcacatagtgaaggtggcacagcatggtgcggtggagtagatcctcttaacccgtttatcccccttcttagtaacaacttgattagtcttactggttgggaagattttactattaatctcggtaccacaacacccggtgtttaccgtgacgtaatgtcctatgtggacgacgtgccatatcagtacaacacctacgatttacaggcgacattccgcaatattgctggagatcctataacatggatgttcaagatctggctagtctatatgggacttaatagagaaggtcgtatcctaccctatcccgatttattgatgcttaatgaatacgatgccaacacgcgtatctatcgcctggtaatggactccactaaaacatttgtaacccgtattgctgcatgtggtgctgctttaccaatgaatgctccaactggtcaaattattaactttactggtgatggagcagagacaccgttccaaactgcaagtgatcaactcaactttagtttccgttgcatgggaatgacaatttacgatcatatcttgatctatgagtttaatgatcttgttgaaacatttaacccgctgatgcgagataacaaccgtgggcgtttgacacaaaagttacgacagcatgaaaagaaatggtttaacttccaggcctacccgtacattaatagtgcgaatatggaattagaatggcacgtacctaagtctatctacgaccaaatggccggcggtaacctaacacgcggatacaatccaagttgaggaaattttaatgagtcagtttaaagaacggatgtatagtgctcgacgtaatccagcgttgatgcaaaccatcgctcttaatgaactggatacacaaatgaacggctctagtaatggagccgtcattgctgatattccagatgcatctatcccttttgtattctcgcttgagatcggttccatggaaaccgcgatggcaattggtgaaatggaggcattgggacgtcagctgtatccacgtctttcgctgggtagtgaagagctctataaacacatgtcagatgatgactatattggacgctttgcttctcctgctagaacaaccttcaatttcttgattgcctacgatgaagttattgctaaagcagtggccgtcggagatacaggtatcaagaaactagttataccgcgcttaacggaatttgatgcagctggtattaaattcacgatgcagtacccaattgaaattcgggttatgcgtcacggtggtattactatcgaatatgtcctcgataaaaagtcacctgtggaaaccctatcgacgaacattgtaccatggtctatgctcgtcattgatcgacgtaaggttatttctcttagcatcccggtctatcagttcgcagtaaagacacataccgaatctcttaacccatctagtcttttccaagagtcgtatacattcaccgatcagttcttctatgcgcgggcgtacatcagccgtactgaagatgataattgggtggaacttaaaacgactcactcggctttggtctatgacccaatggaactgaccgttgtgtttaaagttattggtaataaactccaagtgagtattccaactatctatacaaacacacgaatggcgcagggtgatatccgtatcgatatctatactacccaaggaaagatggatcgcgacctgggtgcttataaagcaaaccagtttaagttctatctgaactctattgatgacgatagctcgtatgtgtctccgttgacaacgtttaacctcattcaatctctggcccgtggtcgagtagaaggaggtgcgaattcggttgattttaacgtactccgtaatcaggttattaataatacactcggtgcaaaccaagtacctattactaacgttcaaattactgacgctgttaatcggcgtggttatacactcgtatccaatatcgataacattacgaatagacagttcctcgcttcaaggcgtctaggagctccgaggtcgcttgatgttatttctggtgctggtgtagccatgtcgcaacttaaagtcgatatggagtctttggcgggctctatacatgtagcggacaatggtgatcgattaacgatcaaacctagtatgctctacacgttcaataatggtcgtgttaacaccgttgctgatgctgagattgctcgtctaaaaggcagcaccgccgaacagattgcacgtgaggtgaacaatggccgttacgtgtattctccgttccataacgtactagatgcgtcgcgtgagaattttgaggttcgtccctactatttagacaatccaacaatcaccgaaaagatttttgttggtgagaacgacacagccaatttacaagctgctatcgatgtctttgatatagttaaaacggatgaaggttatcgaattacagttcgtttagaatctggcgagcagttcaagaaactagctgatgaacaagttgtacttcaaattggctatcagccagctggtgaagtacgctgggcttctgttaatggtaagttcattggtatcgaagacggtgagcgcgtatttacttttgatatcaaaactaaccatgacatcaattccaagaacgagctctacacgactaacatgtcgatgttctccgaggtgcaaaacaatttcgcgagtactctaaataacatgtttgatatcactatccttgttgttaatacgagtacacctggttatcaacctaaccagatcgatgaaatggttcaagcccacctattgccacaacaattcatggttgtcaaccgtgaacgtctagttacaacacttggttatgacatgaccaaaatgtggcgacgtagtcgtactgtacttggtgatgagtcttatcagcactgggaacatgatgtaatgtggttctatgaggaaaacgaatataaacgcgatgaagcaggtaacatcattgtaacgattaaacctgatggtactctcgattatgagatacttcatcgtaaaggtgatccggtattggatgcacaaggtaatcaggttcgcaagcaccagaaaggcgatgtaatgttagactcaaacggtaaacctattttggttgcaccgcgtaagcgtctacgtgaaattactttaatgatggttgatggactattctactttgccaatgaaaaatcggcacttgactacaaagtcgaaattccgatggaattcgttacatggcttgagaatgacatcagtatcctcgatgcacagttacttgaaatgtgtgagatgtatctctatccgactaccacttatggtgatactactgttaccgtacgtgaaggtcagaaagctaccatctccgtcgatcaagcattcactcttagtttctatctgaaaccagctgaatataccaatactacaattcgacctagccttatggctaacggtaagtctgtacttaatgaatacatcagtcgtaagactgtatcgatgtctgatacagttgctcaacttgaagcgacgtctggtgacggggtacaggcacttgaggtattcggtttgggtggcactaataactacgccattcttacagttgaagatgatgctgttcgcctcgcgattcgtaagaagcttgttgttcttgctaaccaagagttaactgtagaagacgacgttcaattcaacttccttaaacacgaagtactgaataactaaacgacataaagcccggcattgagccgggctttatgttgtcaaataccaagctcacgtttgatatcttcaaaacgcttaatcagtttatcccaggcgacattagctacgtcacttgcgacatgaacatagaaatcctcacgaacgatgtcgtgcgccttgatgaagaagttggcatatgttgcaccagctttgtactgataaagaggaatacggctgaataccttaaccatgtcattcagtgcttcaataccagcgttaacgttggcaataacagcctgaagtttaggaagtggtacaacagattcttctagatcaaatcgattcactttacgcagttcgtctgcacatttaccatagagctcatagatgaacttatatgtaattggctcacgctttaacatgcgtttagtatcttcaaagaaacgaataccaactcgtttgtgtttgatatagaagttaggatcgtcagactgactatccatgttcttcagcgtttctgccagagactgtagtcgtggtccaatatgagattcaaagccaagttctaaacgagagcggtccattacttgacgaagctgtcgaatttgctccagcagttgtgcaccaaatttttgtgcttcttgttggatatttcggattcgacgaagatcatcatctacaccaaaagccaacaggccgatatcggagcggggtagcttaggatcaagtagaaccacttcggcagcttcgtaatacttacgatcaagattacgattacccaaacggttcaaagcttgcatctctttccagttggattctaatttaacgattttttcgttaatagaaacgatcctaccttggatcacttcgtcattcatctcaactgacttaacccaacggattgtctttacaataaagtcaaccagtacatggaaccattctttaatggtagccataatagccgaaccaatagcttcattagaaacctttagattcaagctagtacgtgtgggcgtgaatagagcgttatagttttccagagatggtagtactggcacattcaaaccaatagcttccatggaactatggataccacgaagagctgtgatatcatgcgaactaacaccttcggcacggatagtagaacgtagatcgtctagcgtgctaatatactccaatgcagcatgtagcttttcttgcagatttggatcgagctgaactccacggacgggagctgcttcaagctcttcacctaactgtcgttgtccttcaataagaacgtcatcgtgttcatgcattttcattacctttagaatgctcgtaaagcttgtcacgtaagaggtacaattctaaacgaataatttcttcaattgcttttcgcctggctactacaactccacgcttagaatcaaatgctgctttattcgctacaattgcatcggtgacaatccgatggccattacgtaatttagtaatgcagactgtcaccaacatttcagggtcagagatgatcttctcttttacgattaatgactttgcgtatgcttttgtaatacgcgggtgaactaagtcatcatgggtatggtcgatcatgacgacccctccctgaattagccttctacttcaagctgacgcagaacactggctatagcattttgactcttagcgaaatcaaaacgactggcaagcatgttagcggtagcggtttcatcgattgtctgataatcttctgctgtaacggatttcattgcagcttcaatgatagctgggtcgctaacacagttaatcagttccaatcggatacggatgacttgtttaaagagttcacgagtcagattcaggtcgagagcaatattctcgttaacctgaccagctaccttcttcaacataggcatgtgtgcatcaatcaactcttcacaagaaagagatggatcaagctggacaaagaaaccaacagcgttagctacaaacatggcgcgagcttgacgatcattgttggtcggggatttaatttctttcaggatacgggcaatttcaaaaccagtacgcatttcggtctaccttgtttattgagttaagcggaaagcttgtaagaacaaatcattgttcagcaatgtctcaagattctcttcagtttgtttatactgagtttctttacgacgagctggacggaagaattctaggacggtatcgaacaaattacggttattagaaaagtctcgaataatgtcatcgatagctttaacatcatcactcatcgaagctttatctttaactgtatcagttctacgtagttgagcaataagatctcgacggactttcatgattcgttcacgtgggtcatcgtaacgtgcagagaaattgaattcatctacttcgctatttgtaagaataaccaacatgactaatggtgagaaccaaagcatggccaaggcatggataatcaacatgatgtacccagactcttggtactccattccgtagtatttatcgaacttatggaggcatgtcgctagatcacgaccataacccaaacgagaggcaaacatatctgccatctgctcttcacgtcgcattgctgtaacagggttattcatcaaatggtgtcgtggtgcctttttataagcagatagaatagcacggcgaacgttaccgatatcagagcggtcattaatgtaggcctggtattcttcttctttaaggttttccttcaaccatttatcggtgagaacctcaagcttgaatacgttgtttttcttaccttgtagaatttcaattccatctgtaagataatagttaagccatacgtagtcgcccatgtacataaagacgttaaaggtgtgtcctatttcgtgaacaagagcagcagttacttcacgaatggtgaaacctagtttctcactaatgaacccaagagagatatacatcttaaacttcagttcatcggcgagaccacctttaacacgaacgttcttaacatcgataatggtttcaagtttccgcggatcgttatagctgttctctgctcgaagccacttatgtgcattataccaagtaccgctatgacccaacgccatcatttctaggctaacgccggcgtctaatccggagtcaccactgacagtaaactcgtaattaataccggtttcaacttttaattcttttgcaaaatcagtaaacaaactaacgggaatgatcttgtcctttttatacgcttctctgataagagtaacgtatttttcagtgatcggtccaatgttggatttagctccaactactaacatctcttgagagatagtgtatcggttatacatgagagtggcctactcgtcagttttattaatcataaagtaaagctcgaatgagagattactctggtgattaatactacgtgatttaagttttaaaaaggaagctcaaaaatgagtgataatatttctttcagtaaagaagatgtaatcggtgtcgaggctaaacatattacatacgtcaccgataggaatcaccgtaagcatgacttacatgttgttaaagaagtcgtgcatcttaaagataaacgcaggattccacgactgaggtttattgaggattatgaacggccatggtggctggatcctgaagcaaataaaaaagaaagccagcgtacttatcatgagaagaaagactatgagtacgctagtaagcttattaaacgtaagtctacccagattaacatgccgcatgcgattgctaaagctctgggtgattacagcatgggacctaaccctaggcttcgtcaactgagtcgaagtccttacctgtatggtgcggacgttagttctgtatgctgcttgaagaacgattatcgaactgctgcacctgatctcatttctcgtaacacggtagcaggtggtgatattgagaccaacgtttacgaagatggaaaagacggacagattatctgtatgtccgtaagccataaagaaaacgtttatcttgcctatcttaaacattgggttagtgatcttaaagaccccgtgaaagaaacgttcgaggaactagaacgtattcctgaattggttgcacttcgtaatggccgtaatcttaaaatagaaatcgaagtggttgatcaaccagttcacattgtcattaactgtattaagcggctacacgaatggaaaccagacttcttctctttctggaacatcagcttcgacatgagtcgaatcttgaagaccctggaagatgcaggagttgatccggcacttgtatttagcgatccgtctgttcctaataattacaagtatttccatttccgccaagaccaggcgatgacaactaccgcttctggtgttactaaatctaagggacctgaagatcagtggcattggattacatgtcctgcctctttccaacccattgatgcgatgtctacgtatcgggtaactcgtcttgctaaaggtaaagagccttcgtatgctctcgactatattcttaagaaggagctaaacgttgatgaagaaacagagattcttggtgaagaagatctgattaaattcaagaagagtcttgataaacttctggtagaacgtcctggtagttatccgtatctgtttgttaactatagcggtaaagaggatgattggacaccggtagagcatttcacttggggtgaaactgtacacctaggtaaccatgttcgttacacaatgaactttggtaaacttaagtttgctgaaactgatcaccttggtggtatcgaatggcacattgagatgcagaagaaccacaaggttcgttatggtctttacaacatcattgactccattcgtctggaacaactggatgaaaagatcaacgaccttgctagttcgattactctgttctctaagtcttctgactataagaacttcagctctaacccgaagcgtctctgtgatgacatgcacttctggtatctgaaccgtcctgagccatgcgtaattggcactagctccgaccagatggttcacgagctagatcaatacgttgtaggtcatgatagctggattgttacactgccgtcctatatggctggtccaaatgggttgaagtgtgttaaggacttacctgattacaagactttgatctttagtcacgtagctgaccttgacatcgtttcgacttatccgaacgttagtcagattctcaatatcgctcgggaaacaactgtcatggaattctccatgatgaaagatatctccgaacatcatcgtcgagaagtaggtgtgaacttgacaggtggacgtgttaatgccattgagatctgtcagaaaatcatgaaggctccgaagctggatgagatgctgaagctttatttggataagaaggctaactccccaaagtgatatatcgatggaaacgtcgcggaggatacgaatgttcctccgttggcgataaaaggttctccgccttaaatgctgtaatgcccgatggccgaactattgagatgcactaccaatgcgatgttaaaggttatgatgttggtggtactaattggaagctcggtaaaggcaagcctccgttgagtcctataaactcatgggatgcatatttagctctatgggaaacatgggcaaaggcgagtcctgacctgatgaaagaacttcgtaaaggagctgaagcaaacgaaggatatctttctgatgtctttgcatcgactaatatctcacaagcacgcgctttagcagaactcttgaataaagggtattgacaacatattgccccaccattaggtggggctttatgccgttaagctttaccaatcaactctagaacaggacgccaacccatatgtgcacccgtattggtgggtacgttaatattcaactgggacatgttactataaccgataccggcatatgctgttttaccatcgactaagccagtttcctgaccccagctataactaccggctccttgtccacctaccccgagatcagcgttggttaagttttcccatgcctttgtaccggttacagttccatggacgttatacattagatcacgccattctcttcctggagcagcgttattggttatacctgtatcggtagcgccaatatacatcaatcgacactggtatacgttgtcaccgatagtgattcgtttacccctaccattcaatccagcacttgccagagaattccatgtcatgttgtttttgagtggtttttgtgggatataaagaatggtacttctgtgagagaacttaaaccagtccggtgcctcattaagaacagtcccctcgctcaaaccaactaaggtagctaacgcagatgctgtaattaattcactagatgggacacgaccaaagtaacctatatcgtcattaccggctataagtgattcagtaccaggtcctttcgatggaataatgtccgggtcaatccaaattagaattggacgccatccgtagttattcatatttgaaccagctacttctctacccacatagctgattgaattaaaaccacgatagaagcctttacctacgtcagtaccagtagtttggacttcacgtacccaattagccccaccggtactagctaaaccaaagtcacttgttgagaatgactcaaatgccgctgcaccagattgtctgggtattaccatcgaataaaccaaacggttatattcgccgccaccagttgcactggcaccagggttatcaatacccgtcataacacgacataggaacttatgtctaccgatctgtatttccttaccatcgatgagtccatggttctctataatcgatctagcagcgcctcgtctaaaaggtgttttcggtaaataaataagtctgttattctctttgtatttaaaccaagttgtttcactagtgtgtaatgtaccctctgtgaaaccaactagattagagaatgcttcaggttgtggtaggcctgctttaaacccaccgaaataactaaagtaatcactaccagcaattggaatttgtgatcctggtggaaatgtatcatcgtacttattaagaactgctaataatgattcgaacatatgtaatcctgttctttcttaaaacctataccattgccggcataaagccctccctgaagggagggcgttatgtttactgtacttgttggaagtactgaagcaggagaggttgacgcttagtcgggaagagggataccagactaggaacatcgtactgggtccgcgcttctttgttctcatcggcgaagatgaagaacagagtcaggatctgaatgtgcgattcttgtacaccaccttgaacactcaaaccatcagtgaaacggaatgcatggctatcatcgaacaggccaggagacttacggttttcggtgatgaatttccgaataatttccataccgttcttaaagccaactggatcttcgagattgataacataacgaataacgttatccagttgtttctgcgccatgacaccagtttgcggagtcagtggtttacccggagcacaaatttctttgtatttcttgagagtttcttcaatgtaagtttggttcacttcggtaagtccttcgtaggagagttggatacgaacagcttcgacatctactttcggagcagccgcagtcggaatagttccggtcaaatgggtagtctgagttgtctgtccggtttgagctttataagccaggatgacatcttcaggagcattgctcttactaaccaacatcaaacgttctttcagttcaacggccagtgcgggttcactggtagaaccctctgggcgaatctcaccaagagcccagctttcaagttcttgtgtggtccattgagttgctttacgtgcaaaacgagtgatgtcggatttccaagcacctttagaagttttgtcaggaacaataccactgacaaggaactctttacattgctgtggattccaggctagatcaagagtagcttcacggcgttgatgttcaacaatagcttccttcagaacattgtaacgaacatcttcaacaagctcgcctttgatatacagttcgagttcttctttagtccaacccgatacaggagtatcaacgagaggcttgacttcctcaactacttcaggttcagaaatagctgcggtagcttcttctcgaagcagatcgaccagagcgggggtaggttctggatcagccagctcttcttcggtttcaccttccggaggaagatcagtagtctcttcgagatcactttcttcttctcctttagggtcaccactgtcttcagcttcagattcaacatcggtatcgaatttatcaacaacttcaccgcaagtcagcatccgaccatcgtcatcatagaacgcatcacgatggagtgcagctagaacaggagctacgagtgctgctacttcgttgtcatcatgaccttcgaaagcagcttgtagttcttcaaaagaaaggggaccgtattcaaccggtgactcttggggagtttccggaataacaggagtaacaggttctaccggtttagctacggtaggaatagagaaaccacgatttcgatttttagccatggggatttcctagtttgtgaatagtcaaagaattaggggaattggtaagattcccctttgtcttaagaaagacgacggaccgggtcccatttaacagtcttcagagtagcactgtgcatcttcgacatgaagatactcaagaagcgtccacccacaccagctgccgcagcaggaataccgttggggttctcagcaagagctttacccgcacaagtagcacagatattcttatctcgtccaaggatacccttttcaatgtcacgtccagacttacacgtcattggaccacgtacatcgataatttgacccataagtccatcaatgttttcagaggtaataagaatggattctccatccttaaccatagtgtaaccaacgagttctttagcattaaacttatctactcgcgttggaacaccaatatgtgttttacagtctggttctataattcggactgtaccgaccattcgataaatagtcttggtggactcgccacccaatgcagtctgagcaccacggttataagaaccataacgaagagagttgttcatcacaggcatgtgatctgtatcaatgccttcttcaagtgacttagagataagttcaaccgacgtaccatccgagaacggagattcaccaccaaatagatagtgaactttcttacgaacaccaccgaatagcttagcatgttttgcatcatagaactcatacgactcatcgtcagatagatactcttcatccatcttaataagttcgttacctatttttgcaacaatagctgggtcagttaattgatctttatattgttccaaaagagctgcacgtactttatctctgtctgggtgagcagtcatcgatttacgtgtaacagaagtaacaaggctatctgcgtaagcgggaatagctagacaatgatccgcaaacattagatattgccaaacgtagatcttaccatccggtgctcgttcagtgacgttaccatcttcacggtcgtcaatcagtctatctagcagctcattctcaattttagcaggtgagaaatatcctgtctgaaatgggaagatatccccgaacggaaggactagacagaggtagttaacgaatacattgccatacgtagtacgtaacggttcagtacctttgtagttttctatttcacccggttgtaaaatgaattcatcacggaagtgtaaaggagctcgaccttcgatgtaatcgtcgatgaaaattttctcatcgccattcggcatgtagaaccacattcggccttcaccaaaatgtggcttataaggcatgttaggaatatcatcgttattataaacgatgttgaacagactgttcatccaagcacgttttttacatagaccagctttaattcctaaaaggaaataatcacgcagtttcatagagctttcccattttacgcttgatctcgtcgatcacccgttccatgatattacgttccatctcgttctctgtgtattcatcgatagaaactttaacagtgctatagatactatcgaggtgaagattagagaagaatgcaagacctaccatttcataagccgcatcttgagcgttcttattgtccaggctttcaagactattagaaaggagttctaaccagtcatgtccgactcgcataccagaattagacagttcgagaaccatactaaacttatctcgacctatggtattcatcaatcgattaagaacacggatacgggatacaggagcgatgtattcgtcgatgtgaccacgcgtcatcatagtgtcttgcaccatcgcttttaaagcatcgatgaaagaaacagatacttcattaattaaaggccacacttcgtcgaaagaaaggcgttcaaacataggtaccagatgagcaagaatttcctcattatcgaaatcgccttgtagaatcaactcaatctggtcaggaagaatataatttggcaaacctaaaatagtacggacaattgcaagccgttgctcttgtgtcgcctcatccgatactttaacttcgtgtgcagctagaacctgatcatgggccacacggataatatcgtcgatacggccaagcaacatcatagtgtctgcattgtcatcagcaatagagcaaacggtatgcagttcatcaagagctgccgagtaatccatttcctctagggaagctacgcattcaagcatgatttcttttcgttcttccatcactaggggagtgaggatactatctagcatttctttcattggaattatcctgtataaatgaatatctaacatacggttatgttgcaggtatgtcttcgtaatatgtgaaaagttacgtttcctgtaacatctatgttactacactattccattaggagcttcaatgagtaagtttagtgagctgccgtttaatttgatggatacaatacaccatccaaaaccaactcctgaagatgaaaaacggctctctgaagcccttgataaaatattcccccataatccaaaattggagcacaatcaaatgaccgcactgtccccgaaagaacaactggaccaagctgtagaagcttctgctgtagcagcacaacaactcattaaagaagatggctgggccattcttcgcgaattgtatcgcactacagctgctgctcttaatgctacttccattgttatcattccggcgctggagcgtcgtgaagaaattctgagtaaactcagtgatcctgaaggtttctctaaagatctgcaaaactgcatgtctgatattgaacagatgatcagtgctctggaagctcttagtattcttcacgtaaacaaaactggtacacctgatctggctgatctcgatcaaatcggtaagctgactttgggttacgcaaatctccaacataaagtagaaacagctgttcaaccactgctgatgggtctcattgctaagatgcaagaagctggtgttgatactgtttccttcgtgaaataaggtaatacaaaatgcaagagcttgatatggataaagaagacaattatcctgctgagggtaattgggaacagcaagctgatgcagaagtagaacaggggcccacgggtcccactctaccggacgcacctgcggaagaagtatcttcttcgcctgctgttgaactacctcctctggtaattgaccagaaaccagttaacttcactgagacacgttcttgttctagtgaagctattcctggtatgacctctttgatgagtttcattctagaaaaccccaagacctttaaccaggtattggaacgtcactcggcgctattgaatggaatgcaccaaggtgatctcactactactagcagtgaccgagattggttgatttctctagtagctggtatgaaccatactaaccttgaccccactcctatcggtgggacggaacgtgaaggttctgtatggcaacaaggtattactggtcatgataacggtaaccttattcgaccaggtcgcccttctcaaaagatcgatcgtaataaacgacacagtaaagaagaactgttggcatacctctccaagaaatctggtcttggtgcgacatacgaaacgtttatgcctcgttcgggtatctggcttcgcctgcgtgctccgacacttactgaagtagtcgcattgcaaacagaaatgcagcagatcaagctacggctgggaatgcaaaccaaaggtatgtcgttctctaacgctggttccgtaatgatgaacgcgatgactgacctggctctgtcttgtgttattgcatcaaacaagtccttcattactccaagtgacctggaacatgaactatcgatctttgatgaagctatcctgcatcatgccctagcttctacaatgtacattgatggattcaactacgacgttccatgtattgcagacccggacaactgtacggctcgtatcactgcaaaacttaacatgtcgtctatcgtttggtttgacaacactgtattcagtaatgatcagcgtaaatttatcgctaagaaatttgcacctgctacggatgaagacttcaaagcttaccgtgaaggtttcggtattggcggtaagaaagtattctggtttggtgatattggtgttcgtcttgctatcccgactatcgctcaacgtaagatggctgcttctcagtggtctcagacattgatcgaaatgtctcaaggtacatttaacgaaccgccacatggtgttcaacgttcagcgtacattgataaactgagtaaagctactatcgccatgcagtatgctcattgggtagatggtatctatgaaaaggacgacgatgtagaagacttcgaagatcaactgctttccgacgatcaggaaatcattagtgattatctggcgaacactctgagtgatccgcagtacgcggagcagttctttgataccgtacatgagtatactaactcttgtgtactggctgtggtagctcttccatcgcataactgcaaagaatgtaaaggtcctcagggccaagcattcaacgaacgtttcccgcaccttgtaccgctagacatgatggcaatatttttcacgttggcgggccagaaagccaagcacctggagtaatcaacgaggacccccggcatagtcgtctaacaattaatttggaggacgacaacgggcacgttacaatgaactctttcggtcgcaagactgttaatggtaagagtgcattcgatgaactcgtgcgaacgctagatgccgtaaggccagctattgccgaaatgttgaccaggaaggcctaccataaagactacggtattttcgatcatgattcaccagaggctgatcctttagatctggttagaatgcatcctaaggaaaacgtcgtagaaggtggacctgaaagaacttggatacggaagtttgtcaattacaagatcaatgacatttatggtttatctttactagagttctttgaactaccctttaatgattgtttgttcatgattgaacttgcagagtcgaaggctattcaaagtacatcgcaagctagacaaatcgagaaagatcttggattaaaataaaaaaaaataaagcatagctcctacccgaaggtaggagctttatgccgtcttacacttgtgcttcaatcatcatgaaaagaccacccaagaagagagtgatcagcgctacgatagcagctccccatatgagagcagtgcaaatcatattaatgcggtcgagcatgatgatatctttctttggtaaacgagttcgacgaacatcatcgttatcttttaccagttttgctacgaacagggacccagcgataatcgaaatagagatccaccagatcagcatgatggtttccatgattaactccttgttagttcatgagcgtccacggcggtaactggagaggggtatacacgctaaccagggccgtaatgatcattactagataaatcgcaaagctaattgcccaactgacgcagaggaacatgcagaggtacttccaattaggaagccacttgcatacacccattacgaacaaccacgatacagcatagccagtcatgatcaatagtccaggaaagctaagtgtcccgtaaataaacgctattgggttagtaaacatcaaatccatgttaactcctattttggaagcatgtcgaataaatgatatccactatagccggtgatagcaataataactacgccaaatagaaccatagagattctatctgaaaaggttttactgctagttaccaagccatagaaagtcattacacctccaaccgtaagagaagcgaagaaggtgagtatcagtacaatccatcccatggtatcaactcagaaagatgttataaaaggttgccatgatcaagtatacggcaagaaggattgctgccaaaggaccagatgcattgaaagctttagccagtttaatcggcaggtggttcgttttgacacccatgaccgcaagtccctgtttcaggaaaaagacgatgaacagagtgatgatagcgaaagcaaatacattggtgataatagccattacattgtcctttatgtgggtgtatattcacagttgtaatataggctttaaatgaacttaaatgcatatttgagattagctgctgcgaacatagcaacagtgaagaacccaaatccagcgattagataataacgatactctctccagtgtttaggtgtatcgtaggcatttggatcaactagtgcattaccgatacctaaaacacaggtacatgcagctagtacacctgttgaaatagccagtgcagcataaggtagatagatgtatgccacaacgggaattgctataacaattaccagaaggaggaacattaggttggggaaagggagagcagagggagatgttttcatttgtatttccttagatgtgggatgcagcgattacgaacatggtcagcgtaaagtaagctaataccaagtaacatttctttacgaacgtatggatcaatcgggtcaatgcaatctcagaatactctatagactgctttattaacttcggtttgatgttctgtccggctaaacgtaacaagtgtttatagtgcgccgttctgtactcctcacggagcttcagttccaatacatacatcacgacggttaatatcggtgaaacaataagtaggatcacaggtgacatttctattcctcttaacggtataaagcccacccgaaggtgggctgttattagtgcatggctatccgtctgagtaccattgaaagagttttaccggcgaaatgctcacttttattccgagcatatctcacgtggtgcggtatgttttcacacactaggtaggtcaacctaggtaccacatcttggaagtctttcagtttacggagacgacccagaatttgaatgttatctttcttggaatcggtagcttgtaacaatactacctcacgaagattagggatgtctacacctgtaccagatgacttaatagtggacaccgtaatgtcgttcttaagtaactgttcataactgcaacctgagacatgtccgttaaccacaaggtcagggaacttagtcttcagatatttaaccagtttttcaataaaggcgaccgttgcacaaaggaggagtagtttctgaccaggtaaccgatctttcacatacacgccctcagcaatacgaccgaccatcctgaaatagtcatccatccgtttaggatctttcatcattaccgtttcgtaacgcgcatggttatacgtattcttaaacggtgtaagataatccttcggtttgatctttggttcagtgtagagtagccccatgcagttgatgtagacatcgtagttgggcaggcgacacatggtctctgctggcaacatcttgtcaatcatcttcgtcacgtaggcgttccctgtgtagggagtagccgacaaatagatctgcttattaatgttagagtaaatatcgatacggaaggttagtcctggatcttcttgaatctcgtcgttaatttgcagtcctgcttgtattgcttcgtggaaccggggtggaggtacattgtatccgagctcatggagtcggttaccatacttctcaaagttatctagatatgcccggtaggtagtagaagagattacaataacgtcaatcccttcaagatcgttttcgacgccgcgatctattagtttttggagttctgcggaacccgagatggtaatgtatctctgggcaatgtccttgtaagtgttctgaagagcctcaatccaaataccaaaatacttgggaggaaccatcacaacacatcttacccccatcgaagccaaggacgctaggctcgtgagggttttccctttcccgtttgcaagtctacccgtgcagaatgtaaccaatcacgcaaaatatcttcacggatgatttcctgataatcccggagtacgtatttctcgtacatttcgtaaacagcagttgctgctttagggacagggatatcctcaatctcgactcgttctcttgggatacctttgttctccagataaccgatcaggtcttctagtgaatttcggtggatataagtctctgatagatcttcgaaacaaccatagtactttttcttgagttccatgatgattcgattaccagggattttcttaggttctttcaaagaaagcccttcaagaaacccctgcatcttagcgaacgtttcccgagtatacccagatagtcggacaccatgcgtatagcgctcagccttgagtatcggtagcataaaaaattaacgaggggaaagggagagccaaagccctccctacctcgacctccatcttagagcagcttacctcccatgaccgcaagatcgtagggatggtcattcctcagtgtgtagaggaaactgccaggattgttcaacggctcatgttgcttctcaaacgacatcgcaccagcaagagaacgggacatcatcagtttgttgtatttttcaaactgacccgtaatacccggcttaggcagacgataatcgcgttcagcgatagagcgcaccatcatagcataaaccagaacctcacagtgaacggcattcaaagagaacttctcattcaacagcgacacagtggctgccaaagcatcaactgggtctttgtagttcttaagataagtcttgctagtaaaacctaccttatctgagctcagtttagacccttcagtatcactaccagagtgcaggaatgactgaatacgcttcatcacttcgtacatgtttacgtgcttattaggcaacgtcaggaacggcagggcaaagtcaaacccggccatatcgatcacgatattatcacgagcgtcaagttcccaacgtacacgtttgatatgttgcagcatttcagtcgatagactagctcgacggttatacagcgacaccgtcaatacatcgccttcgtctactccatcaaccgtccgtaccaaaccaatacgggtcagttcagaagcactcggtgctggatatgcactaaggtcatcgatcatcagaatatcagccaggttctgggcttcgttacgaccgatcatcaagcggaaacctttacccgagagttctttcttcagataaagagtttcagccgcagatccagttcgcaggtacttagcttcgacgccaccaatctgatactgttctacagccgaggttgcatcagtgtgttttgtcgacaataccgcagaagtgattttgtcacccatggatacagccgatacctgaccaatgacagttccttttggaatagagaaacttagtcgcccataacaccgcgaacatacaccctgaggatccggatgcacacatcccaaaatagaacgcatcttaatctttttaccgataagatgtttctcatcccctttcagccagtccagttgacctgtctgttcgttcagatagtacttgccacgaagagctttcaacgtaccctgcattacagggaagtcgatcaagtgaccattacaatcaccagtgtgtaggttctgtacatactgagcaatcaactgagacttccggttgaaatactcggttacacgcagtagctctttgttatacaacagagctttggtacccgatcgggattcgatcatgttttcatacaaaccccaaataccatcaatgtaaccagtggtacacggctcactgaaaatatcagagttaatgtctgtcgggaaaccacgtggtccgtatgcctgaagcaattgctccattttctgcgtacccgagcgcaggccctcaatgatgctgttaccacggaactgtgtttcgtcgttgaatgcttctttgatcatcccgtaagaaatgttttcaatcccgtacgtagtaggttgtacatcttggttagcctttctaactgccgggtgattgtacacttccataatgtcaaagatcgacagggttgcaatgtaagcactcagtcgagtcgtggtttcattataaagccaattctttccttcaatagccagtttagccaaaacctctggatcgatctgttcaccactccatgcatgaataccccaaataactttgttcaggtatttcacaagagatttagaggtaacccgagtagatgccagatggtaatctttcagaaccggggcatcagggaaagctttcagtggataccagagcagaaccgacagcttggtgatccgatcttttgcatagagtttctctccgtcatcaaagatgatctcatgccattcacttggaatcgcccagagttcatcgtaactcatattgagaagatcacgtgctttatactgattcattatttacctcttggcgtgcagcccggttaaacaccgggcgcgtacttgaactgcaatccacggcattccaacaagtgcgacagaagtccaactggtcgggagttaccgaatgggattttggaacgatcaactgctttctcaatgttggacggtttatccgcagtgaggatagagttgatcacagcaatgtgtgcttcggggttattggtttgatccaacagttctaccgtgggtagtgcaccgaccgtacagttgtaagatcgagtctcagattcaccaaacgaacgaatagcgctttctcgaccaggtgtactggaccgatcggagttattcagtttcgatggtagaccaaactgttgagtcttcaccgatgctacggccgaccagtcttcaccgatcttttcgagcagcatcatgtatagcgggccaagcaacattgggtcttttgtcgttacttctttacctgtttgatctcgatatgtcaccggtgcatatgttggacagaagcgagaattaaggatttggttacttgctgtcggcaaatgtacggggtcatcaaccggggaatacaagtacgcaaaaccatctctcaatacatgcgatacatgttgaatcggattcgggtgatccttaaccattccatgcattgtcggagtaacgattgcatagaaatcaagcagctcattaaaggcatacttgataaagtcaggattgtttctgatatggtttacaacgtcgtcaagttcataggaaccatgacgctctagcccacattcaactcggagacgttgagccagatcgcgagatgctgcaccgaaaccatgttcatagatacgaccatagttagaacgacgcatagtcgagccgccaaagataacaacatctgcaacgttaccattcacgtcacgaggcatatctgctcgcttcatgatcttacaaacgacacctttgccgccatggaaatcagtggctttatatgcaccgcccggttctttaatcgattcataggtgatttcaacacgccattcatcaagttgatccagtcgatacatacgggtcagcttacgttgaccttcggcttgaggcagatagatcatcgcttctactacaagttgacgaaactcctcggtcatatggaggcgatctttacggcgggcagacagacctttatataccttgatgatctcacggtaatacgacgccagtgcgtcatagtacttccgcagttgtccatccataccactcggagtataagatggattttgacgatcatcccaatacactttgatgtctttaatgattgcgcccggatcaccaattacggcacggtcgaacgtacgatcgagagtgcgcaatgcacgtggagtcatttcagctggcgagagatcgtcatcaaggtctcgaacagcgaagataacaccatcatcacgaatacgttcaccgatatcagggaagagcttgatgtttttatcgtcaccgtacatattgaggaagaatgctttcttaccagctccgccagtagcggttgtataagtacgaggagccatcttctcccgaaggaactcatcgcagaatacgaaaccatcctcaatagtaccaggcatagaaccgaacatcacggtggcgttaacgcccatgcccagaagaccattttcttttacagttgtggattgtgcaataaccgtatctttggcaaacatctcgccaacggcaaggttattccatacatctttctgcttctcaagtttgaatccaaagtcctggtgaaagcttaggtactctggtacatggataacaccgattcgtttaaactcgtcgtaatactcctcatacacgatcgtagttacggggttatgtcgaatagatccacgacccacaccagtgggatacttacggataatattcagaacaacgcaatccgttgggaaacgaatatcgaaggtatgttcagcataacgcatttcgatacccgccattacccgacgtggctcgttcccttccactactggcgattgtccaatatgtgacagcaacatggcaccgcgtgccgcggaggttgttccgtaatatggatcaattgccgcgtgaccgagcaaacgcaggttaatttcacggatggcatttggtagactttgcatctataactcctgttgatcgttggtgcagaatgattatatagatgtgaaaattatttttttgtaggattcctctatggcatttacaattatggaacaaaccggtgacggtggagcatcaatgttttatgatccagctttccgtttaattgtcgaaacacatatcaacattctccgtaatatcaactcggttagagtagagattccgaatgagttgtactggcaatacgaaggaaacttttatgggtatttaacagagatcggtattgagcctgaactccattggatttatttgcgtgttaatggcatggaaaatccaaaccagtttgcagcagatgtccgtaaccctttagacaaagtgtacaacaatatcttgatcaagccatctaacaacgagatcggtgcattacaacagttctacactagtcgaaaattttaaagcaatagcaggggaccctaaggccccctgctttatgccatcttacaccaatccaagaccattggtttgacgcatgccagccacagcctgcatgtacgggttagccggttgaccattacccatcatcatcatgccctgttgttggccacccatccacgcgggaatgggtgcgttcgcttggataccctggggctgcatgttacccatttgcataggttgcatcatcccacccatgccattcatctgcatcatgccattgcctggcatcatcatgccgttattcatcggcatcatcattcccatttgctgctgcatcatctgcggttggggattctgtgcggccatgaattcgctcatggagacagtatctttttctacaggtttgctaacaactgcggcgggacgagtcagctgaggagtactggcttgtggagcagtaacgctcggtgcttgttgctgggtttgtacagcttcggcagtttccggagtatcctcatcacgaccaccgaggttgccattcagcggagggataaggttatagatcttcgggaactcgtcgatcagatccagatcaaacacaggaataagattgacggggatttgcagtgggatcgcgtaccggttaatcagctgattgagcatcacgattactttgtgatacgctgtcagaagactggtgtaataaggtgcaacacggctggtagtaccaaaggcatactcttccggattgtcaccaaacggaacgatcagtttgaacagcgcagtgagaaccttacgttgtttcttcgccatcttgataccaagaacatcatcagtttcagcctgaagatcttccaggatcgggaagcgaatgatcgccatacggtttactttcttaccatcgaaagtaccgccattcttcaagtaaactgcaaccagtcggttcttcttagtagcagcaggcatcagtttctcgaacagaccgacagttgctttatccgcatctgccagtttcttcaggaagtcagttgcatccggcggcaggtccttgtgggacgacttgtccgctgcgatggtcagaagttgttcggccattttgtggacgacgaaactaatgtgtgcttttgctgcgcgttgcagatactgaatcaccggggaagtaccccggcgactcaatgcttcactcagcgggtggaacggctggaagtcttcaccgaatcccttgcgaaggaacttatcggttgggattacaagacgtttaccgtctacggtcgaaggagaagcagtacctaccggattacggaggctgatataaccttcttcatcgaactcgcaggcgaacgaggggagtacagacttatacgagtccaagatcaacgacattgcttgctccttggttaatagcgttaggcatcatgatgggtgcagctaccggatgttggtaaccgacagactgaagagcctgatgttgagtcggattgggaattacttcttgtaccagccacagcatatcaccagacaggttagtcgggtgttgctcgttacgggtaatcatcggggagaacagactatccgtaaaggtcggtgcaatgaaacgagtcagtgactgaccaccgatggcaatatcgatgatcgagtcaccagccaagtccgaatgcatcgagatacggaacggcagctggttaccacgggtgatgttgttcaggatatcgatagccaggcggcgttcgaattccagaatgtattgacgcatgtccaggttatcaatgatagccttagagttctgcggatggaactcgaacgaatagttattcggaccagtgccattagttacagcaaacgagcaagtgcggaggaaggtatccatcatgatcgacggaatggtctgtgccaacagacttgcaccaatggaggtatagtctgcaccgctccaaacttcggagtcttctgcctgagaaatacgacggattgaacggccatcgttcatggagaactgagtaacctgttgggtgccgcattcagggaagagccgcttgagatcacggaaagtgatatagccattctccatatacccggcatgatctttaagaacagccaagaaggtgttagtatggatctgctggttcctgcactgggcagcagcttcaccaaacattacatctttatcaggagccccgaacagatcatctccttggttctccattgcattctctttgacagcatgttggtatgcgccaagagtattcgacagataacgagttggagaggtatctcgacgttggctatacttgtatgctcctccttcaccaaccatcgtgcgatggtcgatggaccgattgatcattccgtcaaacaaaccagagctttgcagtttctgtgccacatgcgctgtttgaccaatactaaagatatcttcaggacggatcaggtgagcagttgcacgagagaacattccattcattccacccatcatgtcaacaggagaaacgatctggttggaacctacgatcgacgcaacgtgttggggaccatgaatggtttgttgaatagcttgagcaatgatagtttcggagttgaagtagatacgcatgtcatccggcagataattctgagatgcgtcagcgtggtcactatagccaaagaagatacgttgagtcagcgttcccgcaatgaatggatgttgctcattcactttcatcaagaagcggaaccggcgagaacgccagccatgtgcaataccgacactaccttctaccgatgcttggggagtgataaccgaagaagctacttcttgtacagcacttacccgaaggttcatgccaccatttgtagcttgttccagttgacgagctacttcttggttagcattaatcgagaaaggtcgaatgtgctgttcttgataggtgccggtttccaccagaacaaagttctgtacggacagcttcgagttgacagctgcaccagcggaaatgcccatgttgattccgtgcatgtaatttacctcttgaattttactggttgatctgagcgaggtgtagaaccacttcggtgatcgtgtgcttgatatttggaggtggaatcagaatgttgttctgagcaatctgaccagaaagcttgaacagctcaggtggaccatgatagatccaagtagaggagcggatggactggttacagttattcactgcaatacccgccatgttatctggcttaggaatctctcccgattgggggaccttagcgagtttcatatgcggatagagttcatcgagctgtgccttatacttctgagcaattctcgaaccacttcgggtattactaagctgattagtcgatccatgttcaccgtgataaacaggttcgacttgtaggaacacagctacatcaaggtaaccccaatgccacagtagagcctgggtagttgccaacagtgtattgactggcagtttggagatatgatagaaagcacgcgccgggaaagcttttgccattacccattgtgccagtagtacttggtgaggacggatctcaaagttcgcgacctgactcacgcaactaatacattttctcagtttctccatgtcgatagtaggatctaccgtttgtgccagtagctcataatccatcgcatcgatgttgtatgcctcaatgtcacctgggctaactcgacctttcgtcttgtgtgcctcaataaacgaagttttatcttcgtcgtcaccaccgccgccttctggacgcttttcattaacgcgatcagttggactacgctcggcaggattgagattgctacgtacgtaacggaacgtgttagctacgatagagtgggacattggatcgttcagaggaacgattgtcagtcggcgaaccagaaccttcgaacgaagatgtactggaatttcaactgaactcataccacgccaaaggctacccaaagtagtcggttcatcttcaacgcagaatttgacgtacccttccagtttgtcaaatgcagcatctacatcttcacccacttcatctttttcaagtagcggccagttagcaatttcacaacggctaatcaaaccaacaacttcgttttctttgtggagttcttgatccgtaccagaatcaatgtattctccccaaatcggaaccatcggtcgaagaccaagtgccacagtagcgaggttgatgtagtcatgttgaagataagtctgctcacgcttggtgtagcgcgattcatcagtgatcgttttctggatctctggtggaatatgcagattaccaatagtcaacagccaacgacggagtttgttcattggcagagctgagtacagttcatggatgtaatggatcagcgtactggagatgtgcgctggttcgaagtccatcttgaacagatcgttgattttgacatagctgttccagatacgatcttgatcagcctcatcgcagctttctaggtaatcattaaattccttgaaaacacgagttggatcattgagttttactttgctataagcccttgtactccacttgatttcgtttcctttatggctagtggttacttccacaaagccgttgccttgtaccccagtaacgtcgatgcgcatttatacctctttagttctggtgatgcacagttgtaatatagatctgagatattttttaatgtcaggaaatagagggcatacagcatctctcggtgtttaccaaagagatgctgtagatttatttagaagtcaggaatggaatcgtcaaagccattgtcctggaaaccaccggaggacggacgattgtaaccttgaggagcaccaccgctattaccaccacggttgccgccattatagccaccttgacgttgaccaccgccgccaccgttaccaaagttagctgggttggctacgttcttagcgttctggtcaaaactgcttaccatcatctggtaaatgattgcagtggccggttccaggaaaccggtagcgtaagcttcggacatctctttcggagagatgggagaaccatcaccattcaggatggtgtgatatttcgacggaccgaagaagaaccggatacgcgggcgctgttgctgagaagagataagagcaatgtaaatacgaccagagttctgttcgcggccgattaccagtgtggtgatcggaatgatcttatcgatctttttaccgccaacaaagtcatcttggtgaacaaacttacgttcttgaggaacatctttaccatcgacaagatcccgtgcatacttcattgcagctgcaaaagtagccaggtcagttttgaattcaatcttaccgttattcagatcaccttgaacgttagtacgtacggtcaggcgaggtacgttaccaaagacaccgaaacgcaggttaggacgtttctgagaaccttctaccggatcagcatgtagccaagtggacattacagagaacggagagagggcagggccttgggattgttgagacatgatgtgttagctccaattggattaattttttacacttcgcgaaagtgtttctacgtactatatcgatgaagagtattctttctaatcagcgtaatagcgcgtaacattctttaagttctttactgccatgagttgtaatgtcatgatagattttgtcttgtgtagttacgggcgaccaacgtctcgaagcagctaactgtttcagttgggccttaatagcttttggttgtgcatcgaaaacaacgctatcgccaaacacttgtagagtgaatttagtgaatgggatgggcgtatcctcttttatgccgttaagcttggtgtaccacaagttgtacggttttattttcccagtgtgggattccaacaaaagaagacgatcgaaatattgtttccacaatagctcatgtggaaaatgggtaaccaaagcgatcgtaccttgggtccttactggagctttatcgatctccatcacttctattcctgcatctttcatttgatgcagaagttcaattgccgcgtaacgttcgtatacttcatatgccatttgttttggcgttttggcttctttataaatagccttggggtattcccacttgaccgcgtctttagatgcgatataccaacgcaccttgactttcgatccatgttgccccagtgcaaccggaattgtctgtatttcctgcattaggattgtaacagcatcagctggattaatgccatggactttatccgtagctacagctgaattaagattacgggccaatgttcgaagattgacccatatctcttttaccgatttaacgtcaatcggatgcttaggttgattcgggtgaattcctaagaatccctcaaaggcaagagaagtaccgatactaactggaagctgtccgacatctctttcaatgagttccatatttaattcctaacgaactgtgccaacctttcaagacaacggacttgtatggtctgatcatcagtgacttttgaaatctcttctttaagaagatcactaattgtctctggtgtaatagcgataaacttagacatgtcaaattcttttagacttgtcgctacactattctttttcttagtagctttttccaccaagacagaccattcgtagttaggatactcaactcgaaatgtttcgatatcgccgttagctacgtccattgggtcacaacgcagtcgtatagcagaatacttgggtagttctgctaaggtttcttttactttattaagaagttgtttagtatcataaccgtgaacttctaaagtaacatacttcttagcattcttgttctttataaatgtcgccgtgaaattaccatcctcacgaacgataaaatgaaacaaccctttatcgatctcatcgccatgacagattcgatcgaaagaaccagctgcgtaaattctatcattaatagtcatgttgtggacatgaccaattaagatctgatgttttactaaagctaagtattcttcttcatcgtgagttggttcttctacaatggaaggtagctgataactaaatgcaccatgcataatagcaaagtcaaccttctctatgcccagtgaagccatctgttcttttacctgcgataaagtaacagctgttgatggatgccatttatctgggacataaagaaaatgtgcatcgagcttctcaatatactcaattgacagtgtcttagagtaatggagatcgactggaatatttacgtttactttttgctctacaaagaactgggtttgttccctatcatggctaggtgtaccttcaactattctgagcatcacgttatttgcagcgcagcgcatcatgaacgttgttgcccaacggtttatctgatgtacagattcatcaccgtagttaagctgtcggtcgaataggtcaccagtaataatgaccatatcgagttcctttaacatcttatctgtaataactttatctaagtttaacagaatatgagaggtaggagttgtccgatgacctaggtgaatatcacctaggcttatatatcgaaatgtaccggggaactttgttttatcagtcttcataatcgtcgtcaaatgagcttgtatcagcctgttgacgtacactaccattagaccctttaacgggaacacccccggcgagggtgtacaatggattcccactttcatcttcgaaagtgcggttgtacatcgccaggatgttagctaaaggaatgagaacacttttgtccacggttgtagtaatagatacactacttaagaattccgtgatatacggttcaagatcttgcagagaccgttcacgttcaatagcaatgtaatctactacatgtgaaatagatgcagttgtagcatcggctgcccatgaggtagctggcctgggatacaaagctggtacagtaaaaagaatcttcggctctgcttcattagaagctacacgcagaggatttgtcaattctagtacgtatttccgataacgggttaagttatcagtatcccatggtcttactagtaggggtaagacctctttcacaaacctgtcttccaggataatgggcaactgcatctcgtcgtttgcgatgattgtattcagacaatcatcgattccacgcgttacatgacgtgcgcggatttcttcagctgtatcagtttgatactggctcattcaattctccttgtactttttcaagtgcatctttagaagcaaggatattaatgacgattgcattctgaccttcaaacagttcatcatgttgcttcaggtattgaacgaatggttcggttccatggttttggatttgatcgggggtattaatagatgcgaaatcaataccaccatcttctcgtttggttgcaattacactattctcgtgtgccgttacgttaacaccatcaacaacttcaatagtaaaaccataacgacgtgtggatacttcttgagtcatatgctcaagactttcacgaaggctattattcaacccaccaaagaaactagagagaatcttaatgacacggagttcatgtagatcttccgattgggtcagtgcttccaaaatttgtttaatagccttttcagaaacatgaagcctttcgctcagccgttctaccgtgcgattaagatgttccactcgttgaatgagtgcatctgtttcattaaggtcaggagcagatttaacatctgattccccatcgaccagtacctgtgcttcttccatttgagaatcaagattcgacatatatttacccgttgttgatattagcaatattcacaatgtgtgaattttggaattgaaccagtttacccactgtatactctttagtaccatcagtgactatacctgtaaactgaatggagaatgcatccggattatctggactcgctggaacaatactaaccaaagcctgagctgattcaccaaacacggttcgtagtttatttgttagtacatcacgaagctgaatttccagattaaggatatcgttagcatattccttcagtagatattgaagcgaagtattttgtgtcctatgtaacgttgacatggacctatttgttgtaaggaaagtagagatgatgtagtctgctttggattccattgaggtaatccaaccatcagtacctagtgttgggagagagactgtcatggcaactccaaaaaaaataataggaaagtatgcggagtcctaagactccgctaactacatcattggactcaatcggactccacgaaaaggaagtctaagaaaggatgtccgaatggcaactcaatcctttttcgggtatagccgccaccgatagcgttgattgcttcccaaatacgaccatcatgaatttccacgaaatgtactttatcattagggtcattggaaatctgtaattgaatcgtatctgggaatccagggggacccatgacaattatttcatttttgtcaattacttcgacgccatcacgttcaatacaacaataccatttattaccgtcgcgatgtatcttaaccatcttatcggggttattggcacagtaagttactacattcatacgccctttttgagcttgtattttttgagcgtaactatcgagaatagggcgacgtgctttattaggatcggccttaaacgacaccggttcgatcatactaaattccttatatcctcgttataaaggagtcccctaagggactccgtttatgttgttaacccaacaagttccctacaggactggttggatccatttcgttttcatctagagcaacattcacaagattccatgaacggagaatatcaaccttctcgtagagagaaagctctttatcaccttctgggatttcttcgtagaactgcttgactacggtgtggtcatcattgacaaccagtacttcgtccatcacacgacgataatcgtaatggcgttcgccaacacgatcaccatgatggtttacatacgaatcagcataaccttcaaccatgttgttcagatacataccacgcaggcgttcttgtgccatgatgtatcgttgcatgatcggatttgcggtttgcaattgctctaacgtgtacagtccatgaatgttgttagacatccaactgttatccgttttagcaacaatgttccgcatcgcctgtaccgctgtgctggtactgatcatctggtaaagattttgtgcttgatcgaagaacgaagttgccatcgaactcaggttactacgaagtgtctgagaacgttcacccaaccagttcgtggtattttgatccagatggccaccagcgacgatgtccatcagatcgacgccgtatgcctgttgtaacatggattactcctcttggatcgttaagctgctttcgccaaccattcttccaaggacggaagatagtcctcgtgagcatagttgatgatggtctctactaccggaccttgtagttccaagttacccgagatctcgtgcggatcatcaggactcagtacccaagtatgcggagcgattcgttcagttgcatcagccagatagttatcgggcatcaacgtcaaattcaactgatcgccgtcgaaatcggccgttatgttcagataagttcgtaaagcttatcccgtctctcaatagtagacagctgcatgtcgccatgcagaccagactatatcatcaccttcaccctaagtggtcaggtgcctcccatttcgagccacttggccctactctactcggttcactttcgtgcctttcgatagtcgttgaacgttccttacatttctgtaaggcttcgctgctgattgtctcagagagagttcccagcaattagagaggttattcgacatggatttctccatgaaggaactatgtagttaaactttacccaagctttctttacaacacaactgctttatttaaagacagttctattatttccggattgggtataagttaaccctcttataaaagagcaactcttaactacttttattcggagctttaagacagaggaccgacatgctgattgagttatcgcgaatgtcattcttgataacggtgatgaagaactgttgagtcgaaccacgttgcagagtcgggttgcggtggaatacacaaggaagacccttatacttcgattccgcgatgatctctttgaacagttgatcgatgacttcgttgtacttcagaacgttctcgtaaatgaacgagttcgcttggcgagtcgtcatacggaatttgcgtttgagcttgttgatcagatgatacttcaacagctgacaaccgacaccccacggaatgtgaagttcatcgtaatcatgcggatcactgatagaagtaattactgcacgtgcagtcaggttaagacgaccacctagtacatgtcgacgaaccaaaccgggtttctgtgcaattcgttgtttgtcgtagttctcgtggaagatagctagaagcttcagtgcacgagctacacggttttgtacagtgattggtttcagcggaattgccgaactaccgatactactaatagtcagtaccgcatcgattgctgcgccgatcggcttatcgatgtaaacacccgaggtcgtagactctacaacgaagcagagtttagttgggatcggaatgttcttcgggaacagatgttctttattctggttaacgaatgcagccatctcacctttgttggtattgatgatactgctatcgagcaagaactggaagatcgtatcgaagttctgaacgaagttgttcagtccacgcgggaactggcgagccagcaacttgtcaagtttccgttttgtttccttcgaactgatcgtatcgtaatcgtactgatactgggtgttggtcagatactccaggaagtcgaattctttcatcgacatataacctgaaagcataatccacaactcgggactcaccagacgatccaccccttccggtgcccgaatccacatcgatgggacgatgggtcggttgctcgtgcttactactggtgtaccgcagttatcgcagattaccccaagcttgtatgcttctgtgatatgctcacagtcacacgaagctgagttctcgatcgcatctgcatcctgataatgggagaacagataacgttggaattcctccttttgttcagcattgctggtattaaagtcattagcgaatactactttacctctttggttagcgagcatctcgtcatgattgacaacctgagcatatagacccatacctacttcctattatgtctcgacaaaaaaaggagatagaagcggctcccgaaggagccgccttatctactatcgatggaccaccaacggagcctggcacgatcctagcatcgtctacaaagcttaacctccgctcttctctgtagcactttgacactaggaccttttaccatccatcgttgtttgatcacacgttacccaagagtaactcctttcggttaagtgatcactcacggcccgtgtagcgagaggtcgacctagactttacgtccactagtcgattacttcgcggaacctactcctaaccgttatcaccgaagtgaaccagggtcgcagtatttgaatcgggatgccagccttctgacacccctatcaaccgggggagttgtttcttagtacagagtaccaaccgaacctaccatgttcatctggtagccgccaccaacgcccatgccgttgacaacctgtgcggtagaaccgacagcgaagtcttggatcatggtgttgccaacgaagcgctgagcaccgaagacctgtgcaacgttgtccattgctacagtcagaccagcagcagcaatcgccttatccagaccctcgatgaacttcgggttgaagataccacgatgtgcacgagtggtgtaggttacagcacccaggaacgcacggtcgtagttcttggattgcttgttacgcagttccggatggatgttcgggttgcattgagtaccgtaccaggacatccactcttgttggttgccctcagcagcgttcagtgcacccagtgcatccaggtcacgacggtcacgtttctcgtcgccatcccagtagtagcccttgttcacttcagtgccagtcgatgcaatgatcggctgagtgttgaagtcgaagaagcgctcgaagccaccaccaaccaggttctgtacagcgcgaatgatcgcggcagtagctttctgttggttcgggccacccatggcatccaggaagattacgtccagtgctgcgttgtcgcccatgcgatccagatcgatcaggaaggacgggttcggacgaaccatgctcagcatcagatcagcgaagttctgatcggtgaaggtatcggacttggtatcgatcttcttacccaggttggacagccaacccagagcaccgatgtcacccaggtctttaactttaccaacttgaggcaggaacttacgagcccaagcctggccagcggttacacggaaggcgttcgacagagcgaagaggtacagttccagagtgtttgccttgatccagttggcctgacgaatgtcggttaccaggatcgccggggagaacggcggcagcggttgggtctgttgaccgaacatctgggcttgcggagtgggggtgtactccagggttacttgtaccgacacctggttcagcatggtgtctgcttcgtagaactcgttctcttgctgaccttgtttcttggtacggttcaggctgatcacgatatcggacttgatcgggttaccgacgctgtccattaccggacgaccggagaagtccatcttggcagccagggtttcatcttggccgcgcagcattgcgatctggaacggagtctcgccagctttcttagccagaacgtcgtcacacaggttgacggaacggatcagaatgtctttcagcaggacttcgtctttcaaatcgaattcagccgggatcggcagcgggccagccgggtgtacttcagccttcggacgaccggtggtctgacgaacgaattcgcagatgcggttccagtactgaacggtgaatacgtcttgtacttcgacgtctacatcgaagcgatcgtggctcatgccgttctgaatggtaacctgacgcggaggcagggtgattgccgggttcggcatgatcagcggacgaactacgatgataccgttaccaccagcagcgtgcttgacgatcagcagcgcggagtagccaacacggttggcatcacggtcgaaacgcagaatctggaaatcgttttccaggtcttgatggtcgatggcatctttgccaacgcgggtcattacttgcagcgcttcgctcgcacgggcgtcgccgccatcagtacgaccggaacgtttgaacatgttcggcaggccggaaataccgccttgcagagcttgaggtgcagcttgttgcatacgaggagcttcctgttgtgcgcgcggagcagcttgagccggagcgttgttggcttgagcttgagtgttttgagtttcggtatcacgaatcatgatttgttcctatgtttgtaacgtttcttgatcaagaatgagatccaacagtgtattggattcaaaactgttatatagatctcagattttttttaatgcaatatagaccggaggacccgctataaaagcaaggtcatttgaggacattcagtcttcacatactgtattacatatttgtttccttaagattcaaacttcagtatgcagtgatctggggcatagctcaaatagcaggtcaggacctcacggtcatttcctgtattaaataactagccccagtatttcttttcttatttctcgtcagacaagaggtcttcaagatcatccaagtggtctttcaacttactgtagatttccttcgcactcttaatgttcacaactttactgagttgatcagcgtattgcgcaatcgccgaagaatactctttcatgtgagtgagcatcgtgtcatcaaaacgattgtcatcttcaataaaggaagaatgcaaattgcgaagaccttgaatggccgtcactggatcgatggtgttgtttttaacacaatcccgaacatgcgccttgacgatagagaatacccagtctcgttccttcttatctttgatagaagagaaaacaatagtcagcggagaacggaaatactcaccccggcgaatactatctgccgaaagtgccgcaatcttcatcgattttacattgcctccttccttattaattttatttgcggtttcactaatacgctgagcctcttcaacaagaagttgtgcaatagaaggaccagaaaattcacgatggatagcagcacgcgcttcttcctctggggaaagtttaccactcgtgaaagcagtagagatccgatcaagtgtatgcgtattctcttctacatgtttgtcattatcgttattatcactctctgcatagtagagatcagtgagacctgggttttgcaggtatgacgaacttttcactgtttcatgttcgaacccagtattgatccgattaccaccacggaaaatagaaggcacggaacgaaggcgagtttcagcaatgaaatcatcaccgagttggttcgttttctgggagggcgcgtaactaatcggacctttcgaagtatactgaccaacgatgtacgggttatcgtgtttgatttcctttttctccattcgaccagtagagatcaaccaatcttcaaacagcatcccattcatctggccggcttcacagcaacgtttatagaagttaatatatttcccataaacgatagctcgttcatcgagagctttgctataattggaattaaggaagttcagtacttccccaacagttgggatcttgtccgaaggcaggtttcgaatatccagatcaatagctactttaactgccagttctttaacgaacttgccgttgtacccaatgaaatccatgcgatgttctgtaggtataacgctggcgatgaagtcagtaatggcttcggcaagattaatgtcaatattcttgtctttggattgcatctcactattctccactttgtcaataagttcgtcgtatttaccggactgagccaacatgataccttcgcgttgtctctcgtaataccagtcttcaaaaagaataccagtattacttttctgatatgtttctttaaatatactgaaattttcagacatcgctttaacgcgatcagaaacagtattaaggaactgaatacggatgtgattattaataacgtccgtgggtgcatgaaaatccggaagggttttcaaaatctcatcgaacatggctttaacaaatttcgggttatgtatcacgaaaagatccgtgttaattcgacccatcgtttcctcgaagaaacgtctgagcgaattattgacaacagcaagtttataagaagacgtgctgttcaatgctttatttatcattacaatttccttttctttgattagggtgaatatatcaaaactatgatatagatttgaaataatttctaatggacgaaaaccatgtacatgctattccgggacgccccagcgcggcgcttagggcaagcagttgacccaaagatcgtctatctccgtaggacgtatcgggaactgatcaatgatgtaaaaacgtattaccgtcgagcccccaaagcggttggctcggctaatattttcgccaacatgattcaacattttatcatcgactggaagattgatgatgccgcttgggcaaagaaggttgaagatcaggctaaaggtttatcacgcgtatttggtcttacctcagctattaatagagggaagattcatgagaaggggattacactaggtcccaactgtgaagaagtcgctatagccagttatgagaagttcgagaaggagggtctcggaaagcgctggagagatctgactccagttaaatatctttatcatacccggacagacgtgaatcttccaatgatgaataatactacagctggtaaaggttacggtgttatcacagttaacattccaatgctgttagttcaatatcgctattggttacgttggcaacaacaacgtggtgtagaacaactagagaatgcctatcgcttcgttgggagtatcgtcctccccaacatggtagagagctatttagatgttgcttacttcaataggttatctcgacaagcacagggtatcaaatgtttgaatttccctgtatctcatcctttctatctaaccgatatgactccacgggttgataagctcgtagagaatgtaaactttgagaactctattaaaggcatagagctggaaggtctagcttggattactcctgctattgttaagactaatcttttcgaagttatggagattcctcgggaacctatcacgtatcaaaacgaatgggcttacactttagcacgtctaccgtacattaagtatctagtaaccatgcttaagaagaacccaggttacgaccgttcccagatgaacgaagtattaatcgatctgattgacgctaccaacgaccaagtcttcaaaaccgctggtaataccgaaatggttaaagcgctacgtcgtgatgtagctatcctaattgaagaaatgaaaaaaacataataaacagcccctacccgaaggtaggggctttatgtcgttatttgaattgttccaagagtttatcgtagaactcttgattcttcttcttagttgcctcagcgcgaagaccgatcagttctttcttcagtacattagccttgaggaactgataaccagaataccaattgatatctttagatggaacgtcttcacactcagcatatacatccgacaacaaacgaatgtaacgctgattacgaatactgttctttacagtttcggcttttatgttagggtacttagcgatcagcttatcccatacatctttctttatcgaaatagagatgtgttgtgggtcgatctgccgtctaactgatacagctagtgcagccataccagtcacaacgaagtcattagaagataaattgtaatgactcttaaccctgagtagtggaccatgaacttttgggttatggatcatattaacctcgacataaagcccagcttaagctgggcgtttaagttaaacctgttcaccgtcctgtacagagacttcctcaacaggtttcaggggtttactatcagcacgctcttggaacttatccaggagacgtttctgatactcagggatagcctcgccggaaacagtttcaacgaaagaactcaaggtatggttcttgaggatctcacgtttaataccatcttgggtctgagtttgaatctgactcagcttagccaaaatagatccacccatcaaagctttcaccataccggacttacagttggtgatatgcttggaacgcttggcacctttctttttcttacggcgggtgcgcatgcgggattcgatcgaatcgatttcggtcggctcagcttcaacagtttccattttgctcaggtgttgttccagaaggtcagtagacatttcagattcagtatcagtagattccaacatgatgttgttatgtcctagttcacgaagtttattgtacatgtagagacggctattcgttttgggaatgtcgtccaatacaggagaggaaatgatttggagttcgcccggtttgaaacccttggtgaaaacgtcgtttatactcaaccattcaggaggagtaacgataccatcgaactttggcatttcattacattcggtatcgtaggtgggtatctttttcataagtacctcatgtcgtgtaccaggtagttcaccgtttttgctgatcaggttattgtactgggtccatagtctttggctttgcgaagttgtcgatcttgtaccatgcaatacccagctacgacgaaccagggtcataccagcccaaagagtttctagttgatccttagagagttcttcatgttctttcatgaagttagcgataagatcatctaattcttggagttcatccggtagatatcctgcaagtgtataacccgagtaagaatctgtaatcagtttgccttccggagcgaatgcctgacgtagagcaacatcaaaatggcagtacatgttgtaatccaacagtaatgcttgttccatataggggtagtctaagccaagtgtacagatctttgcgaaacggctagctccaggttgagcaatctcaccacatagattaccatccagtacattgtaagtaccgaaaggaaaagatacaacttctttattttgcgttggattggaattatacatcatattttctcatctgtggatttacgacataaaggagtcccgaaggactcctctggtttaaagttttccgatgtaatcaataatgatcggtcccttgaactcaataccactacggactatgcggtcgttacatggttgcttggctgtaacgataaccacatctttattaaacgtgaatttacgcatacgttcatagatcattttcaattcaggatcgctcattattcacctcttaatagaaatcggaaatcaaacgagtgttacctttatcgatcaggaagatacccaaagattcaaagatcagatagaagacacccatcgtgttggagatgatcgtacgaacatccgctacacgtgtgatctcatctgggataccacggttttctacaacagacattggaacatggaagttggtaataccagtcttcttattttccatagcccagcgttttagacgcatggccaagcctttatcttcgatggattcaacccattcgttaaaacgggttctgttgtccaccgttacagaaatctttacgaaactataaggtggttcttcaatctcaccaaaggatggactgcatacttctttccagaaagtatgtttggcataagtggcattatcttcagatttgtatgcatctattttcttacacttaccagtggtaagatattcagctttaccagaacgtacagatgcgataatgtctctttccagatctgctacttctttcaacattgctggtagatctaaaggtgtttcagctttaatggatttaataatatcatccatcattcgcttagcggtcttgttaatcttcggtggaactttagaatctcgaaggccgacacctttaacttccatacgtgctttagcaaacataacaccctcttgtgcatcttgagacgcgtaatagtgttttgaacgtgtggtcagggaaagtaccgcgaagtaatattcgttcttcatagcgagcaggcggagcttctctttcgatacgcccatgttagccgattgaatcgctagaatgtgtgctacaacacacgacaccaagaataccaacgcaaacactagacgcttggcttcgtcagtgaaagtgatcttaccaaagaactcttctacccaatactgcatcgtgaacatggtcgagtctgtatcggaaataacagctgcacgacgataagcagttgggaaagcatgaatgctggaaggaacgttcttggtcagcaatagtgcatcaataagacgcttgtatttccacagcgtatcagagatgttcttacctgttgcatagatcttgtcgaatacttcaggagactctttactcagcttgtcgtagttacgacctttaaccaagtcaaagcagatgaagttagccaacagttggaggtcaccatcgtaagtgttgtaaacttctttggtaaccttttgttcatcggtacctactttagcaagctcagtcaggaaaccgcgaatcaaagttttgttatgtttgtaagtatgatacagatcacctacgtacataacagcagcacgttgtagtggtgtgaagccagtaaccaacatccgaatctgttcggtgtagtcacggttctgccaatagtgcgcagtcgaatacagaaccatctcaaccacttcttccggagtcggatagtgcatgttgaaatgttcgatgcaatctttcagcttcttcatgtcggtgttgttagcaatcgacagaagattagccttggtgatttccggactataatagtgacggttaccggtgatgaacttctcgttgttagcgttagcatacgaggttgctgtacggcaggtcgatgtcaaactggagtgagtcgacttgtaatacagaattgttgcagctgatacggttgctccactataggagttattgttaattttgaagttctcttgttcgcctttacgaacctgggcaagttctgctgcttcaggagtaccttcaccttccagccgcatttgttctttctttacacgtttacggttagcaacaccttcagcaatatactgcgagtgtgtagactgtcgctgtgattctgggagatacacagtcatactcggcgacagcaaaagattctgtttttctacgcgtccaagaaaacccataaaagtggtttctttaagactacggtcaccatgggggtttttatcaaccaccagggtttttggattattcaaggcaaattgaccttgaggacgagattgttcttttacaaactccagacaggtttcaaaatcatctcccgtcattgccgagatataaagagcctgatcattgaggtatccttcaatgatgttcaagtcacgggcatattcatcgaccgggagaatgaacgggttaggcatactgcactggttcatatttcctctcttaaaatttgatctttcaagagatggctacgctaaaacggaaaaaaattaggacacccaatggatgtccaaagattgagcggtagcacatcaaattactttcacatattgatgtgccacaaggtaaaagttcgcgacgacatatatgccctccgagtggagggcactatgtttattccaagacaactgaatctggaacttcgttattcatcttgcaagcttcgatgattcgttccaaacgtcgttgatcgatattctggaatactaaggtagctttctgaccgttgttgacgaccacgcttccttcacgaatccatggaataccaatatactggtgctgcccgccttcaaattcaacgcgtacataactgtactgcgatggatcgtttggtgtacccgctgggagagtcggatacacgttttggtgagcggcgattaaatcgaaacccaggatacgtacaagatttgcgtctaggaatgcggccagtgttacattcttaaagttgtttccgtattgtgcagacggataaacttcaaaactgattttctggccaattgctacgtcacgaatggatggcatgattgactccgttgaactgattgttaagcactcataggtttgcgcgaaaccacgaatgcaaacgatccattcatatcaatcggccacattgacagaacgtctaataacgggttattcagtgtaaactctttaaagactttatacatctcaaccacgttgatatcatcgtcgtctaacagatcgtccgtagcgccggctgattcgagaatatgtatcccgaaattgttcattacttctcgttgaaaatagaacagaacgcgcttacggatttgatcaaccggcaacttaatatctttacctacagttgcagctaattcgtcttccagggaatcatctacttcctttttatcccgctcgtccatccaacgatcctgatagaaccgcaatccgaatctctctgcatactgagctcctgcaattgtaccagctatgacaagatcatgtatcatcgttcaatcccaacccgatttgttctttagttacgctaaggggtgaattaattgtacgcaaatatgactcacgatcctctggcggcagcattgcaagctgtagctcctgttcacgttcaagacaagcttgttcgcgatacggattgtcattaggattgtaaggttcacgtacatgtggaccatcggccggatcatctgtgtatggagcgtcaggattgtcaccgaccagaacataatagctgtcgtactgaccaacagcaaagttctctatcttatcgattaaacaaccattattttccaaatcagcgatcgctggttgaagacattctccgagcattcccgttgtctctgcaaacttagcttcaagataaagcatagttgtagagtcattaataagatcattcttaatgctcgggaaatattcttctacgtagtgtacaaaacctacgttttccttagctggggcagttaggatatattcgacgtgtttgttaacacagtcttgcatgagtgcaataacagaatcttcttctgctacatgatcgtcttcgttttttggtacatgtgtctgtaacatcttgttccggacaacatctgtcatctgaacaatctgacgatcaatcactttagagttgatcatgatcccgcaagtacggggaccagcagattcttggatatgtgttggggtgatgtactgggtgcgattagctactgccataatatcgacagtgccatccggattgaagatgtcgggtatcgctcgatgcatttcttggacattcatttaggggcctccatggagatcaccattattgagagtttgtatttgtcataacctactatgttcacagtagaaattatctctgattttgactggaacgaacgtagggtagataccatatcgtccttataggcatttacacagacatccatcaattctcgaaaacggaggcgccaatcgacagcttcaccatcgtcgttaattgtctttatgatgtcctgaccatcaaaatcttcactaataagagataaataagaatcctccagatagagctcataatagccatcccagctcggtaggtttaagtgcccgacgtactgccgaacacagtcggcaaagtaagccagcacacgcttaactagaagcgcgttttcttcctttaccaactggtcggttaaagtcttcgattcgaaaaccagtaacgatcgcatgctgttgccacttactcccatagtactctagcagaaatctagcagctgttcctttaaacattatcgggaatatactaacaattcctcgtggtaatgctttcagaaatatgatcgcgtgctctagaaacaactcctgatatcgttccgctagtttaccattataactaaaatttggtatggtaacatcctttggtattacctctggattttcatttaacgccttagatacgctaagtacccaagttataacgtcatcccatactcctcctggaccgtagcccttgaactctttcttcttgtagatcactcgatgtaatctttcaagctcgttgtaattagggaagaatattcccaggtccattgagaagactagggacgcgggtggcgataacatacactgcatctccataagttcttaagtaacgaagttcaatggtgtcggttggaaggtatgatattatctcttttatttgtcgtcggattgtcctaacgatacatttaccaatatctgaatccataaaaacttcagtgataattgcatcgtcatcgagatcagttccgtgacctatatcagcctcagccatcaatatagctaatgagttgatatcggataccgtgaagccaaccaaatctgcccatgcttctatttgccaactacgaggtccataaagaacatccatggatagcctcacgaatatcgtctcacgcaacgtaataccccacgattaagtagactgtatctgatttctcgtctaagtaaacttttctatttgcgtagtcaagatggatacaatctgggataagatatcccagtgccttaaccctattcatgacgaactcaatgagtatcttgtcatgagtgtctttgggtttagatttatttgactctttcttgtatccgcagattaaaagaactgatttctcaaagagctcaatatgttcttcattatcaaagtcaagctgccagcaaatagatgtggcaattagatcgacaagaccttctcgtccgatattacgcattacatcgtaatatttatcatcgaccataccgatgaaatccgacgccttgaatgttatcaataattgttctttcacatttatctctccggcataaagcctcctttcggaggccctatgttagttattttccaaataccaacgttctgcaatagcccgttgttctgggggaagataatcgttacgaaggaacgatgcaacaagctccatcatttctttctccgtacgactgatccctttcatttcgtatatggcgagaatgtgactagaactgtattcaagcgtgtatttcttatcccgtttaacatacgacgagaagtaactcaggccgaaagccgtgataactttacgcacgtaattttgtttgaattcctccatgttagcaataccaacaagtgcgaacaaatcatcgttcacttgaggacaaatgggatcaagggttatcattggatacatagttgtcagtgtatctaagaacactgctgccatggccctgttgggattattcaggaaatcaattactttctgaactcgttcaggtgtacgatgtttacccatcattgcaattgcacgggtcaacgtatttggatctcgcattacggctccaaatgtacgcatgaattcaccatgtagatacgacactagagaagtgcagttcaatgcaatctcggcatggctgtcatcattatgctgatcggtcaggcgatagtattcctggattctatgatcttcaccttcagcaagcccaataaggttaccaatgcagactggtttccattcggtataggtgcgtcgatcaatgtggtgttccaattgattatcgatttcaatcgtaacgccttcccagataacatcactagcaaagatcttataaacctccagttgtttttcatctaatgtgcctggaggtgaattaaatagggcacctgctttatgtacctcgtagtcaatctctgtttcgaatgcacttcgactagtcaagatttctttgactgtaaggaacaccagttgaatcgcggtgttacgagtcgggcgcggtagacccagatgcggattgcttttggtaaagtgttcgagatatgtatacaggacatctacctgtgggttaatctcaagcactacaaaccgtttggacgacattgcattgctccatttattaattgataggtattgctaagtagataacagaaccaatacgtctgtaaccaacatgcatcccggaagcttccactggaagattgagagtgtcgtaaagtaatgaacgcgcctcattatgaaatgccatccattccagttcggcctgcgtgttacgatatggtgcgtaacccattacaaaacaacattgaaacgaatttattgcgttctggatgaaatcatctattaactgttccttagcttttaccaggagtcctgagaagtcagtagtatccatgtcaaccgattcaattgctttagatttaactaaagccatgaagggtggttgagtaatggcctttatgactccagccaactcgaaggcatgaagttgaacttgtctttgaggaatcatagttagtattccggaaatcactcagagctatgatatagatttgaaatcttttaaaatcgtcacagaacccccgttgtatatgataccccacctgggtattatctccatgggtgttcgttcgctggcgagcttcctaggggcgtttaaacatgaatgctattcaatatgcacttcgagatttacctttccgaattccccgtcagattctagagtctgttttcattggacaagaagctgcatctaatgcagctatttgcggtgaagtcatttctcttgaaactagaattcgagaggcggtattagaaccacgtgtctttgcagacatgaacttgatcggtggaactaaaacttatattccactggactttcctgttaagtctgaatatgtcgatccgtacactgttatttactatatcccggatgaatacacccaacagcgtcccatcgtccaggtatttagtattcacttcggtatcctaggttatcagaactctggatatgcaatgcactataatgaatcgactattggtgctgaatcacgtaaagtattagactctgcgcgaagactacctgttgcacagactgcatacattaacttgattaaccataacactgtaatggttagatttatttacttgccttcacatgctgcgtatttatcgtgtcgcttgggcaatgatgacgagttacttaatattcgtcctcaggctatccctgtattctctaaactagttgaatatgctgttaaagcctactgctataatgaactttacatcaatatgggtgaagctcagttatccggcggtcaagagcttggtgtattccgtgacaaagtttacgaatggtctgaagcgaacgatctctatgatgagcaactgaagaagtggcggaaggtatcccggaacttcaatgaccctgaaggtaaccgacaccatatccgtactatcatggcggcgccgtaagggcgtaggtgtttatatgttcgagtctttactcgctacattagtcagaactaatcttggatggcaaggaatccctgtacagggtcctaacatgcctgttactagggtaggtgcacctgcaaccctactcaatggtaaagtatatattgctggtggcggcacgcaaggtggaacaaatggtgtatccacttcgacgttaatgacgtatgatcttgccactggtgtgtatgatcaaaacttcagtactgttccgtcgtctgtatatttctctggtatcgttaacgatggaacatatctgtaccacctcggcggcgctacatttccaggtaatgctgttaatagcacttttgttaggattgatccattaacaaaagaaaaactggttttgaaatccccacctgtggctcgttacgatttccacatgttctatgagtcgggctttatttatacttacggtggcacgccgtcaaacgacgtgttaatgaaatataatatcgctaccgacacttgggaaactgtaacccaaccaacacttcgcccgccagctagaacatcgtctgctagtgtttatctaaatggtaaattctatttaatcggtggcgttagcaatcgtaatgatttctgggaatatactttatccacaaatacgtgggtacagctaagtaatttcccaattactacttgggttggtagtggcttcaccatggatggtcggatattcctgatgcctggtgcacccttaatcaataacaacgcgaataaaaatatctacgaatatttacccgatgaaaataaatgggtattgttcaagaatatagctaatatcgtattcaattcgagtattgtatccgatggaaaacggttgtattgtttcggtggttctggtaacagttcagtcaacgctgctagtaataccatgtattatctaaaataaaaaaaaataagcatagcccctacccgaaggtaggggctttatgccattatgacaaacgctccaagcattccagaacgtcatcaggatcacatttcatgcaaaccaaatcaggtttcgatgccgatgcttcagcaacaagctctagattactatcattaatgatgaccttatcttcctgaacgaagacatcccaatccccataagtccaacggccctgaggattagtttcgacaacacgtttggcttcagcttggatcttatcaaagaaagcttgcataatcaatctccttacacgttattaagaatagacaggatcattgctttcggagtaacgccaacaccggcacaataacgacggaaagattcgcatggctgtgtagctttacgttcaactacattcaagttaaagcacatgttaccacgtgcatcaagaatggttacaaatttactattgctggttactcggtaatcacgaccgagaacctttacggttttgtacgcatggctattcatgtcgtgatacctctaaggtttattatcacgtttgtaatatagcctttaaattggtttgaatgtaaaaaagaaaaacaaaataaacccaccccgaagggtgggcctgtatctaaatgtttactaaaagagctttatccaacagaaagataacccagaaagaaaataagtatgcttcaacagcagcaggcttatatttctgttttacatcttccattaagttgaatacatgtatcgaatatagtttacctataatagcaattatcgctacaagcgtaacaatacccgcaccaatccacatgctatcaacattcttattaaggaagccaaccgtcacgcttgccatgaatacaacaaccgtggttatcaaccaattagctaactgattaacacgtagctccagttcaggatgacggttattgttatcgtctctatatttctttttatctatcgcaatgatagtaaaggaaataccaagaccgatgaagaaagacaaaaatatcgcaaacagacttatcattttatctcaccaataacgtctaaggaatacatcgagatcttgtacagcacgatgatccttagctcgtactttagggtctctcgattctatcttctcaagggcttcaaacgtttctttcaggtgaaggggatggagaacttggacctcgtaactattaacaagttgtccttgttgctcctttgtcattttgcgcaaacgggtgaaatcatagaagacaatgaacttaccttgatcgtcttctgtctcttcgttaccagcttcaatccagcgattgtattgagcaggtgtcagaaagatatcaatggtattcacttctttacgcagattgtaaataaccattgcactgagatgacctagggccatttcttcaggtgggcacttattggtagtagcccaagttttcatgatctcgatgatgtgttcacgttgcgacatgctaagtactctataatgattacatatcagtagttttggagtgtctttccaatacaaaactgtgccgtactgatccactgacggacttcaccttgcgtggacgagagttcaatttcatcacccgtcaaagtggcagtgagatattcctttgtatgtccgcgactacgactagaaaaggtaattacattacccttctttttgacagcaagacgagtatagctatcaccagctacgcaggtttcatcgagttcaagttcgatccattctcggatcatttctttgagttgctcatttggactttgcattaactttctccatcgcttcaattgctagcatgataccagcacgggtagggataggttcttcagtagagtaatcaaacgtcacggtcttttctgaaagattgacctctacgggccattgacgccatctggcggcagtgtgacggatccacagtatatctttgtcgataggagaactgtagaactctaggttattatgcacgctatcattccacgcttgacgtggaagtttagacacccgatctacgactgtcttttcaaacgatcgatgaacgataaattggagagtgttataaattaactcatgggcactatcctgatcttcagcccaaagacagttgatacgatcaagccgtttcgagagaggatcaagttcaaatacaacatcgggacacaaccgcttatttggatccgtcccttgcatcaggatagaatttttatttggcgcataccacaattgaacatggcgtttggtattagggtcgatacatgcagaacgctgacggccgagaagtctccagatctggatcagggtagctatatcgttaaacatttctatctcccatggacataagctctcccatctaagggagagcatttatgccactttttctttacatgtttcggttaatgttacaccccatccgggatgactctttctgttaaataacaatggcttactacgtataaacggagcatcctctgtaaaaacggtgaatgtacaatgaccggggttgtcatcaatcttgaaatagaaattttcttttaggtcatctactttagtaatgttcaatggaattaacattccacccccatgaacataccaacgtttgtaaatccttttagcaagcctatcctcgaccattggattagactggaaccgagctatcctcaaacgcattccattgacttcagaccacgcatcaactttgtcgtaacatgtgactccattcttgtcatatacaaacacaaagccttcaagaacgccgactaaggtgacggcatggtgtaacatcgctgtgtaattggagagttcgaggttaagctcagctgccattagctcatcgagctttttcgctgctgtcttagccatcattcctccttagaggtttaatcaggtttcattattgattccttactgttgttaattgatacaaaagattggacggttattaaggcttcatataaccttgataacgttctatagctcgttcacctacggctttacgatgttcatgcatttcaacagcatcgcgcctggcatacgtagcccaaatgcgggcactgtccattatatccctttgataaaggtcagttccactcagagcttgaataaactcatcgtccggtagatcttcctgtttgtagaaagtatcctctgcttggatataataaaacagtacttggagtgcagcccttgtctcggagtcagagagcaaagctttcaatgcactgcgcattgtgttattacagacgtcgcagttaatagcgagttcaccaatggtaatacggtcattctgtgccacagttcgcatcaatacttcagtgcaatcaacggccagtttgataagacgttcaggtgtaagctttatcatttcttctccttacaaacaaagataatcttcgttgttcgatttgtattgatgacatggagttcactgttatcgccacggtggtaactgatattccaattattccgggtatacaaagaactgtgttgatcgatgatggctctacacacctcaatggaagacacagaaacttcttcttctttaactacaggtaattcgccaatagctccggtagagacaatggtagctaagatccaactcatgaaacctccagacggaataaaaggggagccgaagctccccttttatttagaggacgaaaccatcatcagaacggttgtcatcgatatcaacgatcgcagctcgttgggtgtaacgaacttgctgacgatgatgttcctgtttttgatccaggagagacttaatccgctcttggataccaaccgagttgataacgaagtgcagttgctcagacagagcgtcttcgtcgtcaggggatgcgatacctacagtccgaacaaacggattaccataagctacttctttggaagcatctgtgtacagggatgcgacagaaatcatctcagggacagaagctgcttcttgacgagaagtatggatatgcagttcacacagttgcggttgaatgtaactatgcttactagtgaagcgtgcccagtgatccagatccagtacatcaagacgttcatgtttctgattagacaggtaaatcagagcatggacagcaaataccgcatctttgtcgatttcggaatacggaacgccgttcacgttttcgatcggacagatgttgatcggggtgttggttgcagcagcgataccttccagagtcttcatggtatcgatatcgttttgcagaacctcagtggattcaataccactgacaacgaccggaattacagtttcaccagctttagccagagccgatacaatcagcggaccaagaacagaaccagaaccaccgcccatagaaaacaggacgatattgaaatcgccagctggatatcgttcaaggaaaggtgcaatctgatggcgaaccttaggcatgatgaatgcacggttcttacctgccccacgagtaccctcggtcaaaaagacacgatcgatatcatgactagaacttacgttcttatcgcaggtgtcaatgtataccagatccggatgccattgaaggtttacaccaatattcagaccagcaccaccacagcagtatacacgagtttttactttagtcatttccacgtttcctcttgattaaccttcttgaattgtaactagcgtgtcgcgttcttgttcattgagcacagtcttgctgttcatcccaaaatgaatactaccaaacgctccattgtcacacatattaaccgtaactccggtatttgttagctaagaactagctcttggtctttgaacgaattgagatagactttaacctgaacatcgactccaagatagtaacctaccatcaaggttaccgtacagttatcgtgaaccatggtgttaacaatggatacactatccagattagcaaaattcctgattgtcggcgttatccgataaatcttcggaattgactcgaagtcaaactcgtgtcgttcactaaccttcagtgtattcagatccaagaacgtgattgtctttggacgacagtattcatcaacttcgacatgtttaatcgcagatgacgtattctcaggaactagaagctgatatactcgatcattactgtagaaagtaatacgaccgatttcctgtttgatccactcactgggtttataataactaaccgaatgaacaccggtatcgaagctccaagaactttggacatcgaagaatttatatccttcagcaatcatcagttcaataagcttctgataatgttctcccaattgatgaactgtattacgttgaccaattacactgaagaacgaacctagattctgtttagtgatttcaatatttgtctcactaggtttgtaagtcagttcgaagtcttcctgtgttacgttccattccgatactttcagaaagatatcgttggtaactgggttaactgcaccaaaggtgatttcatctacgttttcaataaccaggaagttcttgaagatatctttgatggctggaagtgcttcgccaatagatttcatttcgattcctctttaggaaggaccaagaaagtaaacccgttaccacttgcatggataaccagttccaatttgccaccgttgtcgatagcatgttgcatcaggcggttgtaattgatagcgctcatttgtacttcctcaggttagaatttcagaaatgggtaccacacgaataatcagggtcgttggagattgatactctttactaaccgttgccattatcactgacggataagaacagagaatcgtcttaggggagaccatgtcgactttgaacttaatgtacatctgtttgatcaactcatggacatcttcgtcgttgttaaccaagaacaaagaatcagggatcaatgttttcattttcggttttttccagttttacgagttaatattcaactaggtaatatagatttgaaataatttttactactgggtggatggggctttgtagccccacgacaccctcttccaagttttgcgacatagtcgtttttgtttccctaccccgtactaaagaataaggaaattatatatgggaccccccca

SEQ ID NO: 6 - protein, 259 aa, Artificial Sequence
  synthetic_Endolysin LNT102
MGTVLKRGDRGSAVEDLQMKLNVAGYNLSADGIFGGDTEKAVRDVQAGAGLVVDGKVGPKTLYAIAKSATVPAKWEAIPFPTANKSRSAAMPTLNAVGAMTGVDSRLLATFASIESAFDYTVKAKTSSATGWFQFLDATWDDMIKAYGSKYGIPKDPTRALRKDPRANALMGAEFIKGNAAVLRPVINREPSDTDLYLAHFLGAGGAKKFLSADQKTLGEVLFPKPAKANPSIFSNKGVPRTLAEIYKLFEDKVSKHRA

SEQ ID NO: 7 - DNA, 777 bp, Artificial Sequence
  synthetic_Endolysin LNT102 coding gene
atgggtactgtactcaaacgtggcgaccgcggctctgctgtggaagatctacaaatgaaacttaacgtcgcaggatacaacctgagcgctgacggaatcttcggtggagatacagagaaagctgttcgtgatgtgcaagctggcgcgggcttggtggttgacggaaaagttggacctaaaactctatatgcgattgccaaatccgctactgttcctgctaaatgggaagctatccctttcccaacagctaataaatctcggtcggctgcaatgcccactctgaatgcggttggagcaatgactggtgtggattctcggttactcgctacattcgcttccattgagtctgcttttgattacactgtcaaagcaaaaacatcttcggctactggttggttccagttccttgatgctacatgggatgacatgatcaaagcatatggttccaaatacgggatacctaaagatcccactagggcactccgtaaagacccacgtgcaaatgcattaatgggtgcagaattcattaaaggaaatgcagctgtattacgtccagtaatcaatcgcgaaccgagtgatacagacttgtatttggcacatttccttggtgctggcggcgctaagaaattcctatccgcagatcagaaaactctcggtgaagttctattcccgaaacctgctaaagcaaacccgtcgatctttagcaataaaggtgtaccacgtacccttgcagagatctacaagctgttcgaagataaagtttcgaaacatcgggca

SEQ ID NO: 8 - protein, 37 aa, Artificial Sequence
  synthetic_Cecropin A
KWKLFKKIEKVGQNIRDGIIKAGPAVAVVGQATQIAK

SEQ ID NO: 9 - DNA, 111 bp, Artificial Sequence
  synthetic_Cecropin A coding gene
aaatggaaactgtttaaaaaaattgaaaaagtgggccagaacattcgcgatggcattattaaagcgggcccggcggtggcggtggtgggccaggcgacccagattgcgaaa

SEQ ID NO: 10 - protein, 303 aa, Artificial Sequence
  synthetic_Endolysin LNT103
MKWKLFKKIEKVGQNIRDGIIKAGPAVAVVGQATQIAKGSGSGSMGTVLKRGDRGSAVEDLQMKLNVAGYNLSADGIFGGDTEKAVRDVQAGAGLVVDGKVGPKTLYAIAKSATVPAKWEAIPFPTANKSRSAAMPTLNAVGAMTGVDSRLLATFASIESAFDYTVKAKTSSATGWFQFLDATWDDMIKAYGSKYGIPKDPTRALRKDPRANALMGAEFIKGNAAVLRPVINREPSDTDLYLAHFLGAGGAKKFLSADQKTLGEVLFPKPAKANPSIFSNKGVPRTLAEIYKLFEDKVSKHRA

SEQ ID NO: 11 - DNA, 912 bp, Artificial Sequence
  synthetic_Endolysin LNT103 coding gene
atgaaatggaaactgtttaaaaaaattgaaaaagtgggccagaacattcgcgatggcattattaaagcgggcccggcggtggcggtggtgggccaggcgacccagattgcgaaaggcagcggctcgggtagtatgggtactgtactcaaacgtggcgaccgcggctctgctgtggaagatctacaaatgaaacttaacgtcgcaggatacaacctgagcgctgacggaatcttcggtggagatacagagaaagctgttcgtgatgtgcaagctggcgcgggcttggtggttgacggaaaagttggacctaaaactctatatgcgattgccaaatccgctactgttcctgctaaatgggaagctatccctttcccaacagctaataaatctcggtcggctgcaatgcccactctgaatgcggttggagcaatgactggtgtggattctcggttactcgctacattcgcttccattgagtctgcttttgattacactgtcaaagcaaaaacatcttcggctactggttggttccagttccttgatgctacatgggatgacatgatcaaagcatatggttccaaatacgggatacctaaagatcccactagggcactccgtaaagacccacgtgcaaatgcattaatgggtgcagaattcattaaaggaaatgcagctgtattacgtccagtaatcaatcgcgaaccgagtgatacagacttgtatttggcacatttccttggtgctggcggcgctaagaaattcctatccgcagatcagaaaactctcggtgaagttctattcccgaaacctgctaaagcaaacccgtcgatctttagcaataaaggtgtaccacgtacccttgcagagatctacaagctgttcgaagataaagtttcgaaacatcgggcatag

SEQ ID NO: 12 - protein, 6 aa, Artificial Sequence
  synthetic_linker
GSGSGS

SEQ ID NO: 13 - protein, 303 aa, Artificial Sequence
  synthetic_Fusion Polypeptide CecA-LNT101
MKWKLFKKIEKVGQNIRDGIIKAGPAVAVVGQATQIAKGSGSGSMGTVLKRGDRGSAVEDLQMKLRVAGYAVSADGIFGGDTEKAVRDFQASKALVVDGKVGPATLAELAKSATVPAKWEAIPFPTANKSRSAAMPTLNAVGAMTGTDSRLLATFASIESAFDYTVKASTSSATGWFQFLDATWDDMIKAHGSKYGIPKDPTRALRKDPRANALMGAEFLKGNAAVLRPVINREPSDTDLYLAHFLGAGGAKKFLSADQKTLGEVLFPKPAKANPSIFSNKGVPRTLAEIYKLFEDKVSKHRA

SEQ ID NO: 14 - DNA, 912 bp, Artificial Sequence
  synthetic_Fusion Polypeptide CecA-LNT101 coding gene
atgaaatggaaactgtttaaaaaaattgaaaaagtgggccagaacattcgcgatggcattattaaagcgggcccggcggtggcggtggtgggccaggcgacccagattgcgaaaggcagcggctcgggtagtatgggtactgtactcaaacgtggcgaccgcggctctgctgtggaagatctacaaatgaaacttcgagtcgcaggatacgcagttagcgctgacggaatcttcggtggagatacagagaaagctgttcgtgatttccaagcttctaaagctttggtggttgacggaaaagttggacctgctactctagctgaactagccaaatccgctactgttcctgctaaatgggaagctatccctttcccaacagctaataaatctcggtcggctgcaatgcccactctgaatgcggttggagcaatgactggtaccgattctcggttactcgctacattcgcttccattgagtctgcttttgattacactgtcaaagcatccacatcttcggctactggttggttccagttccttgatgctacatgggatgacatgatcaaagcacatggttccaaatacgggatacctaaagatcccactagggcactccgtaaagacccacgtgcaaatgcattaatgggtgcagaattccttaaaggaaatgcagctgtattacgtccagtaatcaatcgcgaaccgagtgatacagacttgtatttggcacatttccttggtgctggcggcgctaagaaattcctatccgcagatcagaaaactctcggtgaagttctattcccgaaacctgctaaagcaaacccgtcgatctttagcaataaaggtgtaccacgtacccttgcagagatctacaagctgttcgaagataaagtttcgaaacatcgggcatag

SEQ ID NO: 15 - protein, 313 aa, Artificial Sequence
  synthetic_Fusion Polypeptide LNT103 with MAS, His tag, and extra sequence
MASKWKLFKKIEKVGQNIRDGIIKAGPAVAVVGQATQIAKGSGSGSMGTVLKRGDRGSAVEDLQMKLNVAGYNLSADGIFGGDTEKAVRDVQAGAGLVVDGKVGPKTLYAIAKSATVPAKWEAIPFPTANKSRSAAMPTLNAVGAMTGVDSRLLATFASIESAFDYTVKAKTSSATGWFQFLDATWDDMIKAYGSKYGIPKDPTRALRKDPRANALMGAEFIKGNAAVLRPVINREPSDTDLYLAHFLGAGGAKKFLSADQKTLGEVLFPKPAKANPSIFSNKGVPRTLAEIYKLFEDKVSKHRALEHHHHHH

SEQ ID NO: 16 - protein, 313 aa, Artificial Sequence
  synthetic_Fusion Polypeptide CecA-LNT101 with MAS, His tag, and extra sequence
MASKWKLFKKIEKVGQNIRDGIIKAGPAVAVVGQATQIAKGSGSGSMGTVLKRGDRGSAVEDLQMKLRVAGYAVSADGIFGGDTEKAVRDFQASKALVVDGKVGPATLAELAKSATVPAKWEAIPFPTANKSRSAAMPTLNAVGAMTGTDSRLLATFASIESAFDYTVKASTSSATGWFQFLDATWDDMIKAHGSKYGIPKDPTRALRKDPRANALMGAEFLKGNAAVLRPVINREPSDTDLYLAHFLGAGGAKKFLSADQKTLGEVLFPKPAKANPSIFSNKGVPRTLAEIYKLFEDKVSKHRALEHHHHHH